European Patent Specification EP 3 911 147 B1, published July 16, 2025. Title: TOMATO PLANT RESISTANT TO TOMATO BROWN RUGOSE FRUIT VIRUS. Applicant: ENZA ZADEN BEHEER B.V. The sequence listing filed with the application follows.

SEQUENCE LISTING (116 sequences)

SEQ ID NO: 1 - DNA, 133515 bp, Solanum habrochaites
  TBRFV resistance locus
tctgtggtttgatgctttcaaatcacagcaatcctctgtataattatggtttatattttaggggttttcagtttacaaagtcattttatccttccaatcaccaaaagtattatcttggctctagtgactagtaacaagttagttttgtgttatgtggaaatttacaacagatcaccttcatactgaggagggagatgatcattttgtcgtggctcggcccgtctgtcttttagccaaatgctgcgggagagagtgggattataacagtaagtattttgtgttttaatactgcttctatcagctaatgtttcatagaaatgacagtgtgaatgaaattgcaaattttgtgtggtaaatagtttcaggctccaatctagtgatcattttttctgggtaatcagttaacaagatctctttaagcattcaaatttatgtatggtaggtaagtgcacatcatgttaggaccgaaaataagcgggtgtaaatgcggaagctagcaaagcaaacctcgaaagatcacgagtaagaagataacgagaaatataccaaaagacacaaagatttaacgtggttcggtcaattgacctacgtccacaaaggagatgagcaatccactataaatatgagagtacaaaatatagagagaaacaacctcaaccaattcactcggaatacatgggaggttcacacaagtgataacgtatcaagcttgtgacccacaaattctccctctaaccaaaactctcaaaactctttaagactacattgtgaatgctgattaagttagaaggaacatgtctctatttatagagtcctaaactttttcatactagaaaaaagattagtcaattcaaaaccttttcctaaaaggaaaacctatttatggtaagaaatcagggcaaataaaacccaacacatcatggtttgaaccgtactacataagaaaagttctagtatttaaattgagaaggatagaggggaggggcctatccttaaatctgttaaagttttacgtactagcccaactatttgtgcgcgtgaagaaaagatgtgacagctccactatagatttcagcactaccatttagtttgttacaacattttgctgaaattgagttaggatcttcttgagtcgcagagtaatatcttccatgcgaattctctcttcaggcaaatcatttgtacattcaagagctaattccatgattgatttgaagcatctatctttagaagtaaaattttcttcgttcagtgaaaatagattaatgtccactacatccaccaatcggtctggtaatgattggcatatccatcttttcaaggtgaagtctccaacgaatagatcatccacagggctctttcttgtaaaagtctccattaacaatataccaaagctataaacatctcccgaagttgatactttgccttcagacccatactctacaaaaaaaataaatcacgccatcattaatgaaaataattaacaacatttaaaatcctcaagtgaacttgataataacatttacctggtgccatgtagccgatagtacccaaagtcttggtatgtgctattagcgtctcagatgtaagaagtttggatatcccaaaatcactcacttttgccaccatatcttcatccaaaagtatgttacttggtttcaaatcacaatggacgactacaaacaaatgtcctccatgtaaatactccacagcagaagccacatcaatcatcacctttagtctttgagttatatccaaaactttgtcagtagagtgaagccaacattcgaggttttcattaggcatgtactctagcaccaacactttataatcgaaatttgcacaactacttatcaccttaacaaggtttctgtgtcgaatgctacctaaaacttgacattccacctcgaaacttctaaatgcaagttgcagttctgtattgaatacctttatcgccacaaccattccatctgctagtgtccctttatacaccaaaccaaggctcccccttccaatcaagtttgcttcatcaaagttgtttgtcccttgagaaatatcatagtacgaaatcctcttatgtacctgaccaaatgtatcaactagaggaagttccgtactcctttttcggcatttcagaaaccaaatgataaaaatggttgtgactacaattcctgaggaaactgatgcaagaacagaagttaggactctgttctttctttttctttcaagacttgtcactctgcattgcatcacatggaagcgtgatgatccacataatgcagggttacccatgaatgattcagctgtaaaatttacgaatggccctccatctggaatttcacccatgagcccattgaacgagacattgaaatgcatgagatgttcaagattcctcaaggacttggggatcatgcctgatagattgttgctagatagatccaaatattccaacgaaaccaaatcttcaaatacttcaggtatggaaccatctaacatattctttgacaatgaaaggctaaccaagctttgtagttggccaatcgtgctaggaatctgaccagagaactgattaccatgtaaatgtaatatccgcaaactccttaaattccccatttctactgcaagagacccattcagcaaattggaggccaaagtgagaattgaaatatctttgttcctccaaaaagttgatggaatatgggaaattagtgcattggaatctaagtagagttctcttaaagatgaaagatttccaaaacaatttggtaattcaccagtaagttgatttttccccaagataatttggtacaagttttccatgttacacaagctagttggtataattccatctaaattgtttttctctaggctaaatcttttcaacttcctcaagttccccaaatctggaggaatagatcctataagtttattgtctcccaagcttaaccactccaggttcctaaagttactgatgttaggtggtatttttcctgtgataccattttgaagggcaatgaaatattcaagggaaaaggaccagtttcctgaacctaaagatgttggaagacttccattaaattggttacctcctatttgaacggttttcatatacttgcaattagataatgaagtcaggaaacttaactcgcctgtagattgatcattcgtcaattggtttatttgcaagttgatgaattgtagctgttgtagctttccaagattcataggtacaggtccactaaacagattgcggccaaaatcaagctggataagcatggtggaattcacaatggaggtaggaatcagcccggtgaactggttatccccaaggtaaaggccttcaaggtttggaagagtatggcctatgtttgagggaagtgttcctgaaagctcatttgctacaaatgaaatcttttttagtccagaaatgttgtacaaacgccttggaacttcacccgataatctgtttggaccaagatacacttctttcaaatttacaagatgttcaaactcctgaggaattccaccatataaactgttgtcacctaggtctatcatctctagatttgacaaatttccaattgatggtggaagaattcccaccaaattgttccgtcgtagacttaatcttcgaattgctgataggttatcgatttcacttggtatatgtcctgtaaaatatatgtcgaattgtgtggttactacactgaaatgtccaatactgtataacagctttatagtcactaagttactataaataacagaaactgttagttgtatgccttttaaatagttcagcaatcctcacaaactgttttgatgtccttttgaagatgggactaaatggatcaacatggataattaggattcatatagcagacacaaactagaattgagccaatgtagtagttactgttgttgtttgaaaatgaagaacaaagagctataccaacattttttgctactaccctttgaaatgcaaatactaatttcttataaatgagttgaagagcaagtttttaaatatcaaagatctctagtgctacaaggtgagaagtccagcaataaagttaggtggattcagttaaaccagaacattataaatacctgttatgttattccatccaagaaatagatgttgaagttttgtcaagttccacatgtctctaggcaagtttcctgtaataggatattacgataagttatatgtacctctcacggcctatgattgtttaactaaaaaattgttgcaatctttgttgtcaatatgaaccaaaagtagcagagaaagaagttggttccgtttttttttacctgtgaagtggttatatgacaaggacaaatatattagctctttgcatttgtctaaattgcttggtagttggccagagagttgatttcttgctatttgtaatccctccagccgcggaagattatggcaaatgtcattcggcaaagtcccagatagtgcattataaatcaaattgatgaccttcaaagaagagacattgaagatagacgaaggaacagatccaaagagatcattttcagaaagatccaacaactcgagccttctcagtaatccaagactttctggaatttgacctgtgagattattcattgacaaggacaagtgcttcagcctcctcaaatagccgagttcatcagggatttcaccgttgatgctgttgttgccaatgtccaagaaactaagaaaggagaggttcccaatatctgtcgcgattgaacctcttagtctgagaccattgaggtctagtgatgtcactctttgatgccttttactgcaagatatgcctatccaattgcaaacgtgagtcccctttgtccagtttttcgacaacattccatttggatctgaagttatatgagctttgaaagctaaaagagcagcctcatcagttgaaatgttcgatgcattagtattcgagaggtacgttaacaaaactagcaatcctataatcatagccacggaaaccgttttgtgcaacttctcttgcagctatttgtgggggaaatttataagtgcctgattttttatttttcaagtgacattaatatatatttctataattaaaggcaataaagaatcatgtattagcactggaatatatagaatctagagttcaatgtcaatgatcaacatatatacgtaatatgttttgagacatttttttttaaattgaatgttgctgaacttgactgcaattcattgctgaagggaaatcattggttgtgggattctgtagtgatagtaaaataatttacttggatttataagccttgtatattcattattcaagaatattaaagactaaaatcatgatataatgtcatcattcgaatgtatatagcctccgctgaatagatgtttgacaaaagaacgtgaagtgttacggtcaaattagtgaatctaacgtgtaatgttggatttacgtgaattcaatagcttttattcctatcttttatatatattaagtaatttattaaaaatctaaaattatcgtatattactatcttgcagtctgtgtgagaatactattttgataatcgtcaaataattatctataaatttcaaatcttgaatcacacttatttaataggaggaaatggtaaaaaggaagtgaggttgacaagatctcaagactctttcttaattttgatgaaatgttgtaaaaacttgaattagtagattgcatggcatcactatacacgtgtcagtctagtgtttagagaaatttaatcaaagaatataagttataatatatattatccatgagaatcttgagaaagattttctgtatctgtctgatgaaatagaaattggagtttcccaattctatattacttggcttattctaacttctagtgcagaatctgcagatggtcaatattctttgaatatataatagcaaatttgattattagtttcatttttaaactattgatagttttaaaaatatttattatttaactaattaaatttaaatatatcctcgatcttgcaatatgagagaaatacatctctaaattctttccttttcaacatttctttcgtttttctaattaaaagcctcatacttatacaagagtttgaaaccacttgatatgtcacgtgacaaaaaagaattgtatctaagtttggctactcatgtagagaagtatttttaaagcggtcaatatctcaaaagagaaacaaataaattatgtatctacaaattataaaaaaaggagtctacctttattgggaaagtcatatgcaattcatgtatgctttcctaattggggatacaaagtcaatcttgttaaacccctaaactattacaatcattttaagaattatatatatatgtactatttgagtgttgacaaaagccttaaattatcataaaactcatattaaaatatctcttagagtaatatgacatgtcatgtgaatattatgtttgacaaactcaatttcaaagagttcaaagtggttatacacgtaggttttagaaaaattctaaactcactgttttgtgactttcatacctaaaattgttaggtgtttatataaccacccctgaattataccatgaaattattgtgccaggtggcctaatttgaaatttaatagggctgaattaagatttttgaagtcaattaaagaaaatatttttttaatttatcctgaataagcttgctatttgaggggtttgagaaatatcggtagggcggtacatgggctaataaaattgattaaaaatataatatgatattaaatttaaaattaaagagaatccaaactcaaaacaattaggttaatatttctatttagctatttatctttgttatcttgaaaaaaacttaataaatattataaagataattttatttgtggatttgattaacaagtagtaacattaacatcatgtaatattgttttgtggatatttttcgataatattttttaaattataatttataatttaatttaataattataaaaaaataaaaaaaaagtgggccacggcaagttctgtagctctcacgtacttatgggttggaccgacccattttctgacccatacaaaaaatgagctagcctagcttaacccataaaatatcaaaacatgtatggattagcccaggatgagatatgttagcccatattgacagctctattcccacatcaacaaggtatttaatatgtcaacttgaaaagaaaagatattccaaaattaatctgcttatactctatcaattccatatctcacttagtgaaatttcgcagaatatatcgttgaatatattgttgttgtcgttgtcctctcccatcattctaaatttaaagaacatgcaatgtaagaggtaatttagaaaacttagttcggccgtagaagaaggatcatctgtaaatttattcctctgcaagttgatgctctgttggaaatttattactacaagatagattggttaatttgaccgtaaaacagttgacattcttttgtcaaggatctattctggggaggttatagatatacatttgaataatgacattgtcaagtaaattatttaactgtcaatacagaattccacaaccaatggtttatttccctttagcaatgaattgcagtcaagttcagctagcaatatacgattaaaagttgtttcaaatcattggtattaattagataagtattgactcaattacaagtatacacacagtatatatagaatggcgtttgaaaacgaaaacataggcacaaatagcagctaaagaagttgaacaaatccaaatggttgcgaagactattattatagcatgcctagttttgttagcatgcctctcagttactaatgcatcaaacattacaactgatgaggcttctcttttagctttcaaagctcatataacttcagatcccaatgaaatgttgtcgaaaaactggacaaaaggaactcacatttgcaattggataggcatatcttgcagtaaaaagcatcaaagagtgacatcattagtcctcaaaggtttaaataaatgcaccaaacttgaagttctgtccttgtcttataacaaattcactggtaattaactaacttgtaaacttttcatttactaatttcttcttgaattaatcatcatttttgtgtgtgtctgtcattttataattgataggaaatttaccaagagacatgtggaacatgtcaaaggttcaagaactgtttattggatggaataactttacaggtacgtgattcttgtatgtattaaatcttgaatactcttcacgaagttcctaatttcactagatatagtcaatttgtgcattgtctagtaacaaacaaagattaatatatgttgtggagaacattttcgaaagacactctatgtctgatctttagcatgataaccatgtacttattttcaaaatgaatttgcaggaaatataccaaatgaaatgaacctaccatctatttgcaggaaagttaacaaagcttgagcatctcaactatctgaaagtctcttacaatgagttatcaggtgaaataccagatggagggccttttggtaattttcacagctgaatcattcatcggcaacgaagagttatgtggaccgcctagattccaagtcaaggtgtgtgaaatccagaacaacgtgacaagaagaaacaggaagaaaacagtactaaaatttgttcttggaccagttgcagctggaggtttagtcataggggttttaggcatgatatggttgttgaattatcggagacgtaacaaccaacttattcctttaactgattggtatgatcagttatcacacaaaaggttttcttactatgaacttgttcgagggactaacaactttgacgaatcaaatttgattggaaagggaagccttggtatggtttataaggggacatttacaaatgggaccatagctgctgtaaaggttttcaatgcacaactgcaagatgcattcaagaggtttgatttggagtgtaaggttttgcgtaacactcgaaataggaatcttgttaaggtgataagtagttgtgcaaatcttgattttaaggcattggtgtttgagtacatgcctaatggagatcttgattattggctttactcacacaacaatttcttggatttaaacaagaggctgaaaattatgtttgatgtggcttgtgtcgtagagtatctacaccaaggccattcacttgtagtggtccattgcgacttgaacatacttttggatgaagacatggttgccagagtaagtgattttggtatatccaaactcttgaccgcgtatgatccagtggcattgacaaagactttaggcaccattggctacacggcagcaggtactgatcaaacttttatttactaattactttcttcaacttgtattcgatatgcatatatgatgtatttcattttaatggcagagtagggatagtgtcaactatgggggatgtttacagctacggcattttattgatggaaaccttcacaagaaagaaaccagtagatgatgagtttgttggagaccttacattgaagagatgggtcgcggaatcatatcctcatagagtcattgttatgaaataaaaacgaatacacgctgaacgtcacttatgagtcatttatctaatatgatccattaacaattgattaatgtaacgcaaggaagaagaaaacaatttgcattgttatgaatgaatgtgtttgtactacaatatatacagtactgacaagtccagcaaactttctaaccaacttattctaaccaactctactcattattaatttagctcacttaatcaagaaattaaacttaacaactaactaccattactcattcaactgatcacggaacatcaacacattttgttgatttctttcacacacaccctctgcttcgaaaacccctctttttaacatgtaagcgacaatatcttttttttaggagagtgttcaacattgagcataaaaataataaaatagagaacaaaaaagatgagtataaaataaataataatataagatcgattttaccgattgtcaattttgtgtatggactaaagaaataacagcttcacatatctaatattaaatgtaatactgaatttcacatatggtcagaggtgaatccacctgcacccgatatattcttttttaaaaaaattatatgtatatatatagattgttgataagacggtaatatatttaattgtgcactcttataacgaacaaatgatttgacttgtccattggaaaaacgaaaagtgtcacataaattgagacatggggagtaacatttctttcttaaatttttcgtgtgaagtcaaactaattcatataaaatgagacggaaggagtactgtttaatattaattgcatatggtagtaaatttgatagacatggtcccgtgggagtgtgtgttatttccattgaataattgagtttgtaattgttacaagtccattctaatttccaacaccttacttcatttcaaaaatatactctatggctgaagctttccttcaaattatgttagagaatctgacttgtttcatccaagggaacttggattgattcttggttttaaggatgagttcaaaaagcttcaaagcacgtttactacaatccaagctgtggtacaagatgctcagttgaagcaattgaaggacaaggcaattgaaaattggttgcagaaactcaatggtgctgcatatgaagctgatgacatcttggacgaatgtaaaactgaggcaccaattatacagaagaagaataaatatgggtgttatcatccaaacgttatcactttccgtcacaagattgggaaacggatgaaaaagattatggagaaactagatgcaattgcagcggaacgaattaagtttcatttggatgaaaggactatagagagacaagttgctatacgccaaacaggtaaatatttttctaaataacagctttatatcatcaaattcatgtgtgttttggggattttgtctaagtagataagtggttcaaaatctattatctaaatctgtttggtgaagtctttaacatatatataaatccatagcttactcatatgccccaaagtctaaatgacaggataaagccagagttgttttagattttataaattaacaaagataataatgtaaattcaaaatagtgcatttgttttatatttgaaatatgtctgctgcttctgatcaagctgatcattgtcttttgcaaaattcttctttgttttttttgctgactcttaccgatcttggaccaggttttgttttaaatgaaccacaagtttatggaagagacaaagataaggatgagatagtgaaaatcctgataaacaatgcccaaacactttcagtcctcccaatacttggtatggggggactaggaaagacgacccttgcccaaatggtcttcaatgatcagagagtaattgagcatttccatcccaaaatatggatttgtgtctcggaagatttaatgaaaagaggttgataaaggaaattgtagaatctattgaagaaaagtcacttggtgacatggacttggctccacttcaaaagaagcttcgggacttgttgaatggaaaaagatacttgcttgtcttggatgatgtttggaatgaagatcaagataagtgggctaagttaagacaagtcttgaaggttggagcaagtggtgcttctgttctaaccactactcgtcttgaaaaggttggatcaattatggcaacattgcaaccatatgaattgtcaaacttttctcaagaagattgttggttgttgttcatgcaacgtgcatttgggcactaagaagaaataaatcttaatcttgtggctatcggaaaggtgattgtgagaaaatgtggtggtgtgcctctagcagctaaaactcttggaggtattttgcgcttcaagagagaagaaagacagtgggaacatgtgagagatagtgagatttggaaattgcctcaagaagaaagttctattctgcctgccctgagacttagttaccatcaccttccacttgatttgagacaatgcttttcatattgtgcagtattcccaaaggataccaaaatggaaaaggaaaatctaatctctctgtggatggcacatggttttcttttatcaaaaggaaacttggagctagaggatgtaggtaatgaagtatggaatgaattatacttgaggtcttttttccaagagattgaagttaaatatgatcgaacttatttcaagatgcatgatctcattcatgatttggcaacatctctattttcagcaagcacatcaagcagcaatatccgagaaataaatgtagaaggttacctacatatgatgtcgattggtttcgcaaaagtggtgtcttcttactctcctcctcacttgcaaaagtttgtctcattgagggttcttaatctaagttccatgggacttaagcagttaccgtcctccattggagatctagtacatttaagatacttgaacctctctctcaataacatgcgtactcttccaaagcagttatgcaagcttcaaaatctgcagactcttaatgtagagtattgctggtcactttgttgtttgccaaaagaaacaagtaaacttggtagtctccgaaatctcttacttgatggttgcgatggattggattctatgccaccaaggataggatctttgacatgccttaagactctaagtttctttgttattggcgagagaaaagattctctacttggtgaattacgaaacctgaatttgtatgggtcagttgaaatcacgcatcttgagagagtgaagaatgatagggatgcaaaagaagccaatttatctgcaaaagaaaatctgcattctttaagcatgagatggaaaaaaccacatagatatgaatcagaagaagttgaagtgcttgaatccctcaaaccacaccctaatttgacttctttactaatcactggcttcagaggattccgtcttccaaagtggatgaatcactcagttttgaaaaatgttgtctctattgcaattagaggttgtgaaaactgctcatgcttaccaccgtttggtgatctgccttgtcttgaaagtctagagttaggagatgggtctgcggaactgaagtatgttgaagattctggattccctacaagaagaaggtttccatctctgagaaaacttattatagtcaattttgataatctgaaaggattgttgaaagaggcaggagaagagcaattccccgtgcttgaagagatgacaattagctggtgtcctgtgcttgttattccgaccctttcttctgtcaagaaattggtagtttatcggaacatgtcagatgcaataggtttgaggtccatatataatcttagggctcttacttccctcaacattagccataacttgacagctacttcgctcccagaagagatgttcaaaagccttgcaaatctcaaatacttggaaatctctttcatcttcaatctcaaagagctgccaaacagcctggctagtctcaatgctttgaagcatctgaaaattgaatattgtgacgcactcgagagtctccccgaggaaggggtgaaaggtttaacttcactcacagaattatccataacaaattgtaagaggctaaaatgtttaccggagggattgcagcacctaacaaatttatcagttagggaatgtccaacactggccaagcggtgtgagaagggaataggacaagactggtacaaaattgctcacattcctcatctgcttattactaatgagatgtaattttctgatttttcttttggaaacaaatcaactatttgtaaccaattcgtattggacttttgagccctgcatttgttcgaatacgcctttcaacctgtatatcagtgtataacaaatgtatacaatatgtatactgctgctcaaatctgcagatttgattttccagcaacacatttgctgattcttccgacctgtaaattaatttccagcagctcatttttttgtgttcaacctgtacgccagttgtgagggtctaagacttgaggaggaggtttgagcctttacggctcagcgaggaagtgcagggatacgggcgaaatccgttaggactcatggcgaatgcacgtgaaacggatcaaaaggaaacataaagaaaaacagtcaacgatgaaaacaattctgcatttatacgcataactaaggcaatgtaaatcaaattgaagaatgggcagccaagataaatgaaagcaaataaagccacaatgcatgttttaaaatactataaccctgccatgctgcatagacacacatttatattcaagattcaagtcataacaaaatataatttgaaagtttaaagctctggatatcagcttactacagttcaatcttcttacttaaaaaagatgctaaaaaaaaacaaaattcaactcttccaggcaactaacaatatcaaacctacaaactaacatatgagcaaaaaaaaatcattgaaataaaggcatacaaatactaaaatgacaaccactagttcatgaaaaacaaaatggagcaggcaataaataataaacaagataatagataaatatgtcttttaattttattttattttatatttgtatccttcaaatttgaatgtacacataatttgatattttaacttgtatataattgaacaagtacatagttaagtcatatgtagcataaatatatatatatatatatatatatatgaaacaccacctatgacacaatttccatgaagcatgtacacttttatttgttcatttcaatactgagtttaagtattttactttgtttcatattatagttgaacaccataaatataaaataatatcaaatttaaaaaatatatttatgtattatgctttaaaaaatattttttaaaaatctagtaattgccccaccataaaagagatgcccattatacgccgaaagaatgtttaaaatcaaaagcaactgttagttattggattgaaaaataaaaccaaatactccaattgagagacatggcggccccatggtggaataattattacaacacaccttccataattaaagtttgaccttacacctagagacaatcaaattttggatttgggtcttattttactagttaacatttcagataatcacttaattttaaataatttatttcgatagtcattcaactttgaattattctgttagaaagtcattcaattctattttaaagtcaaaagtcactaatatttgagttgttggtttaaaaggtcattcaactctctttataattcaaaagtaacataattattttttgtttcacttaaaagacatccgatcaacttaaatattttttcataaaatcttatttttatgttaaactattctttttaaaaataataagatatttattttagaaaaagggaaaatatgttaaaaagttagttattccaaaaaagaagaaagaagttggaattgaaaagaaataatataaaaaccgcagcacagtgccttttttcttattactttttatttaaaagatagttataaagaaatattatacttcaacaaaatttaataaaataattaaaagcagcttataattttattttatttttgtattcagtcaaatttaataaaaaatttcattttaaaataattgtctgactttctaagtaaaattagttgagtaatttttaggttataaaacaaaattgagtgactttcgaagttaactcaaatctgagtgactttctaagtgaattattcgaagttgagtgaatattaactccttatacaagttcgaggaagatattgaaaaagattgtacatatggggttcgtaagctccttcatgtcagcttataaaaggcttcacacaagtatatatagcgggtaaaattttattttgtgagaggtagaaatgttactcggcagacaatacttgtatgacatgcttaaagcttcatttttttctctttcacctatttctatcttcttcttctctctttttttctccgtgcttcataaaattttattttatttttcatcaaaaacttgatacttaatatattttattgaatgaaaattgatttaataattttatttttcaaatgttaaaatcaagacaaatcaattaagttgatttttttcattactttattttttttccttgcgatttgttttttgtggacttctcgaaaatatataataatataaaattatcctctgaaaaaattatgcattacgaagaatttaatcattactaagaaatttgataaaaaattcccaatgattttactatattcttacaaaaattaaagatttaaggctgatatattaaagatgtcttgttaatattttatttaaataaaataatcaattaaattacgagttattttgaacatgaaaaaacactttcaattttatctaaataaaaatataaattaaattacaaagtaaaaagaataattattataaagagaaacacatgagtactcacaaagagaacaaaaaaaatatttataataatttttttagcttcagagaaggttatacgtataatcaaaattattacggatcatttattaataaaataataaaataaaaattctcctaaaaaattaatgtatgatctttttataagcaaacacaaaaattatttaattacactatattaaatttctttaatctcactaaaaaactattttttctcgtttcatttactttaagttttccttaaataaataatataaaaataaaatagttaaacattgtggctaattttttttaaaaaaaacacaaaagactacaaaggagaacaagagaatgagaaacaaaagtttacgggaaaagagtctgatataccccttaactttgtcatttggagctaatatatccctcgttataaaagtggctcatatatgcccttaccgttatacaaacggctcatatatacccctgtcgttataaaatgactcacatatacccttaatttgtggaagttaaaaattagttttaaatttatatttaatacttctaatttttaaaaaaaattatttagaggtatatatgattcttctatcaaagttcaaggtatattttaatttttttttcatacataaactatttttgacttcttttattataattatttgagtttcttattcttattttatttttttttctttcattccttagtttaaagagagagaaaaattaaactattttttttgtatgtattgtaatttaatttcgtattcaaagaaaaaaatttagtcatctacaataagttttacaagaatattagtgaaaaaataaataaatttgattatcaaaataataattataaattagtcattgaaaaaaaaagtcaaaaaaaaatgtttttgagaattaaatttattcatatgagattatattttatagaaaaaataataaaaatttagattaaaattatattttttcatttccgttagattaaagggatatctcgagccatttgtttacaagtagggtatatatatgctactttcatgttaggtatatcagctctaaataacaaaattgatgggtatatcagacccttttctcaagtttaaattaatgtgaaaaagttttaagtgtgggtcccatgttgtacatttaaaattctcatacaacagacaaaaggttagcttttcacaaaataaaatttttcccatgtgaaactcaaaataaaataattgcgtacagacatatttatgcaacacaacattaatttatttatttacccattcaataagtaaaggaataattataaagctttgtgctcttacttttagctgttcatatttcattccaacatcgatcttatagatttattgctaattcacaacaattccagcaatctacatggctgaagctttccttcaaattttgttgaaaaatttgacttctttcatacaagaggaacttggattgttttttggttttaagaacgagtttgaaaatcttaaaagcacgtttactacgatccaagctgtgcttgaagatgctcaggagaagcaactgaaggacaagccactagaaaattggttgcagaaactcaatattgctgcatatgaagttgatgacatcttggatgaatgtcaaactgaggcagcaagactcaaagagactaaatatgggagttatcatccaaaggctatcgctttccgttacaagattgggaaaaggatgaaagagataatggagagactagatgcaattgctgcagaacgaagcaagtttcatttggaaaaaaggactacagagagagaagctgctagacgagaaacaggtgctcatctttaattagtttatattcatttttttgcgattatcaagttcatgtgtgtttatggacccaagggacttttttctaatctaatgtttgtctcaagtctaaacagatttgtaattctaccacttatttatttagtgaagttcttaaacatatatacatggtgtaagccagctcagataaatccatagtcagttgtttcggactgaacttaacttggatgtcaatttttcaaagtcaatcatgttttcaactcctccccctgattctcatctctttgtagtgcaaaaatcttctctctgtttttcgctaaacatattctcgtgtgaacatatattgcttgaaacaggttttgttttaactgaaccagaaccttatggaagagacaaagaagaagatgagatagtgaaaatcctgataaacaatgcccaacaactttcggtcctcccaatacttggtatgggggggctaggaaaatcgactcttgcccagatggtcttcaatgatcagagagtaactgaccatttccatcccaaaatatggatttgtgtctcagaagattttgatgagaagaagttgataaaggcaattgttgaatctatcgaaggaaacccacttggtgaccacatggatttggctccacttcaaaagaagcttcaggacatgttgaatggaaagagatactttctcgttttggatgatgtttggaatgaaaatcaagaaaagtgggataagataaaagcagtcttagaggttggagcacgaggtgcttctgttctaaccaccactcgtcttaaaaggttggatcaattatgggaactttgcaaccatatgaattgtcaaatctgtctcaagaagattgttggttgttgttcatgaaacgtgcatttgagaaccaagaaaaaaataaatcctaaccttgtggctatcggaaaggagattgtcaaaaaaagtggtggtgtgcctctagccgccaagactcttggaggtcttttgcgcttcgtggatcaagaaagagaatgggaacatgtgagagataatgagatttggaatctgcctcaagatgaaagttctattctgcctgccctgagacttagttatcatcatcttccagttgatttgacacaaagttttgcatattgtgcagtattcccaaaggacacggtaatggaaaaaggaaatctaatctctctctggatggcacacggttttcttttatcgaaaggaaacttggagctagaggatgtaggtaatcaagtatggaatgaattatatttaaggtcttttttccaagagattgaagttaaagatggtaaaacttatttcaagatgcatgatctcatccatgatttggcaacatctctattttcggcaagagcatcaagcaacaatatccgtgaaataaatgtaaaacggaacccacatatgatgtcgattggttttgcaaaagtggtgtcttcttactctccttctcacttgcaaaagtttgtgtcgttgagggtgcttaatctaagtgaattaagacttaagcatttaccgtcttccattggagatctagtacatttaagatacttgaacctctaccgcaataacatgcgtagtcttccaaagcagttatgcaagcttcaaaatctacagactcttgatctacagtattgcgccttactttcgtgtttgccaaatcaaacaagtcaacttagcagtgtcagaaatcttttacttcatggttgctataaattgaattctatgccaccaaggataggatctttgacatgccttaacactcttggttgctttgctgtgggaaggaagaaaagttgtcaacttggtgaattacgaaacttgaatctctatggctcaattcaaatcacacatcttgagagactgaagaatgatagggatgtaaaagaagccaatttatctgcaaaagaaaatctgcattctttaagcatgacttggaaaggaccacatagatatgaattagaagaagttgaagtgcttgaagccctcaaaccacactccaatgtgacttgcttaacaatccatggcttcagaggaatccgtttcccagagtggatgaatcactcagttttgaaaaatgttgtctctattgatatccggggttgcgaaaactgctcgtgcttaccaccctttggtgagctgccttgtctaaaaagtcttaagttacaggacgggtctgcggaaatggagcatgttgattctggattccctacaagaaggaggtttccatctctgagaaatcttattatagtcaattttgataatctgaaaggattgctgaaagaggcaggagaagagcaattccccgtgcttgaagagatggatatttggtggttccctgtgtttgttattccgaccctttcttctgtcaagaaattgttagttcattggaacatgtcagatgcaataggtttgagttccatatcaaatctcagggctcttacttcactccacattagaactaacttcatagctacttcgctcccagaagagatgttcaaaagccttgcaaatctcaaatacttgaaaatctctttcttctacaatctcaaagagctgccaaacagcctggctagtctcaatgctttgaagcatctggagatgaattgttgtcccaaactggagagtctccccgaggaaggggtgaaaggtttaacttcactcacacagttatccattacatactgtgagatgctaaaatgtttaccagagggattgcagcaactcacaaatttatcaattaagaattgtccaacactggccaagaggtgtgagaagggaataggacaagactggtacaaaattgctcacattcctcatctgcttattactaatgagatgtaattttctgattttcttttggaaacaaatcaactatttgtaaaatctatttgtattatacttgatttttcttggttatgtaacaataaatatttgaaaattttcatataaaaatagttacatttctatatgtataattcgccagaataatacatatatatgtataatatacaattatttaaccgatatacatatataattcacctctctcccactctctgtcctctctcactcgcctctctcctccctctctcaatttcgctttccatatatacaaatacaattatctaaaagatatatatatatatatgcaattcatctctctcccactctttgcttcacttgacaactatgacatttaacattggacaagcacaaattgacacttaaaaactggttacagaaactcaacgctgctgcgtataaagttgatgacttattgaatgaatgagaatacgaggcagcaagactaaagcagtctcgactaggacggtatcatccaaaggctatcaatacaaactcagttgtttagaccacgaaaagactgtgaattcaatacaggagtagttaacgattactctaattctatgtcacagaaagtaatttcataagcgagaaaatcctctagcatttttccatttctctttatggcgtgcaaatatcgttatctattttctgctgtctcctagctaattatcttgaatgtacgtaacactctctatttatttccaagagattgaactaaaatctggtaaaacttatgatctctgttttcagcaaacacatcaagcagcaatatctgcgaaattaaacacatatgatgatgtcttcttactcaccgagttattagttatgctaaaatgtttacccgagggattgcagcacctaacaaatctcacaatttttttttattagtgaaagcatagttatcaaaataaaaacaaaaaatgagcaatatttatacaacagacaaaaaaaagaatgatttttcatattctttgcttatgttaccgattcataacccatataaaaacaaatttcaatcacccattaaaccaaaaatgattaaacaaaaaaaatcttctagatatctaactaatgaataataacatattcagtgtagtcccacaagtggaatctgggttaactatccaactaatcatagatcaaaattgcagtgaaaggtattttattagaccacttccaatctcaactatttcaacacaaaacttatattcaatctttgatggataatagaccatctatttttaattcccttttctcaccaacaaattgaaatgtcagtgatgtttctgagcaacaaaaagtactttaagatgatattctaaatgtgcacaatttcatgctccaacaatcgaccaattagattaaaaaatatactcattgagtatttcttctgtcacatggtcaataccatagaaaatgaaaaatataatcacaatttaacaacataactattgagatggaatatgtttcatctagttaaaaaaaatttacttgagaatgttgtttgtgagcattacactaatagacgtcagatgattttcggatggtggtcaaatgacacttgttactggttcaagcagagtaatgggatgtgaaattgcccttcaatcgtagaaaatggaatatataaagcaaagttacacaatttaatcgtactcttgaaacttatctctctataatccatgtttgctataaacaataatattgtcttacacatattcaacaattacatatcctatttaaactaatatacgaaatatattcaataaaaagtgcatgcagacgatttttctacaataaagactccaggtttagagtgtttagcgactcctgataaagacaatgagattatagtaaacaggagaaacagagcagctcttcataaataaagaggaggaaaaaatctaccgattgatgcacgtaaaagagtaaatgtgagactaatgacaataacctgttgttggagagatttatatagatgagtatttgaaaagtttacgatcaaatgaacttgagcgtcagaaaagttgtcgcttgagcagtaactgttatagtgatcaatgaggcattttttggagaattaaattaggtctcaaactatgagcaaatttaatttataataaattaatacttattaaaactgtagggttaaaacggtaaatcaagtttatgattaaactcttcccacttataataatataagattaaaaataatcataaaatagaatggtgcattggtatcaaacaagaaatatgtgaaactaattaagagaatatagtctctaagggtatgaatatatcgatgaatgcttgattgaaaaataataataaatgtatataagtctttaatgaaataacaaaggcacgagataaatttattagaaatataaatctacatattctaggtattacaaaaaagatcctaaaatatgtagcaaacaaatgacttattcttctataaagcacgtaaccatcgaagtttaatgttaatacgataagattgccttgagaatgcatttacttgtgataagtccacgggtctacgtataagtatagtttattgtattcttataaaataatagtaaaaataatagtctctttttatttcaaatttaatttttaataaacagaaaataaattaataaaataagacaaaaaacaataataatattatagacatgtttatgatgagtacgtataatttgaaggggaaaactacaaattcaaactcaagagaaaataataaaggtttggaataaaatatctaagatacggaaagattaaaatgtgttctctaactaaaatcttcatcttcatgaataattaacatgaaaatagaggatccaccaaaaattaaataggagaaggaaagagacttattagaaaaatgatgaattataaaatctaaaagcctatatgtgaaaataagagaacaagaatattgcataaaaaaaaattatagctacgaaaaatactatgtgtgattttaaagataaaatctattttattgttacatgtatcatatttattgttgaaatttcaccttttaaaaaatgaaaaacaagctaagaaaaaaaaagtaaaaagaggaaaatgaacaaataaaagattaatagagaaaagggaaaaataccaatgaatatcctgattgaaactgcattatataaatcttcggatcaatccatttaccttgaatttcaagaacactgcaaattcgatcataaattaatctaaaaagaggcatgtttatgataaaaggggggaaaacagtgttagaagaaaacaataaagaaatagtgttagaagtttgaaatcttcatgtttcaaaaaagaacaaattaatcttcaatgtcaagtaaaatctcaagatctctagtaaagaaaatttatttttatactacaaacaaattaatggcattttaaacatataaagaaatatgaggatcaacatattatagattaactacaagttttcatgtccttaaaagataacttatcaaccacaaacaaaagtaaattgaagggcaagagatgaagaagtcttcagtttgttaacttaattggtgtttctatcttccatgtcttttgaaatgtgtatgaagatgaaatgtttcaagtacttgaagatgaaatatagtttcttacttggatgcttaacaatgttattacttcaaaaagaacctgaaaaaaatcattattcacttggttgcttaactattctattacttcaaaagatttattactttcaattggcttttcacttaccctattcatggtgattaatatgtaagtttcatgcaatgtcttttcaattatcctaattattgtaattgaaatgtgaatttatttttcagataattaaaatattatgttttttttcatataataatgttcaagaataaattggtaattcaactttaagctaaagggcttcccacttataataatatgatatgatatgatgattattagatgtaattttctgatttttcttttggaaacaaatcaactatttgtaacatctatttgtattatacttgatttttcttgggtctgtaaaaataaatatttgaattttttcatattaagattcataattagtcttatagcttaactgtaagaaagaaattacaaattaaatttgacaaataattaagctacttaaataacttaattgttcaatataaaattttaaggattgcctaaacttagaaaaaaaaaacaattaaatttagttatatggttgcaatgtgtaatcaaatagtaataaatatgtggctgtttgtacagctacaatatgacatgagataattaaaatatatgtgtctttaagctctcctctttttgtttgttttgaggaaaatctgttgtattttgatgtgtataattggttaattatacactcttttagaaacaaatagtgttgaatctacaataacatgtgaatacatagatttgataaaatataaaatcgtaaatagattagaccatcttttttattgacagaggtgaaagacaaagcaaccccacaagaaaagataggtatgaaactagctagcagttttatgaacaattaatataaaatataaaacactttttattttactcaacaattaatttataagctatttttattttaaaacacttaaaataagttaattcgaacatgtactataaatcaaaacaaataaggaaaaaaaggaaaagctaaaggtgtgtttggtatgaaggaaaatgttttcctaaaaaataaatagattttggatttattttctcatgtttgattggtaagtagaaaatattttcctgtgtttgatttatgaatgaaattaatttttggggggtgggggtgggtgggggctggtaggggtggatagggggctggccgggtggaggagggtaggagtttaaaaataaaaatttgaagttgaaaatattttaaaaagcaaaattaatttttggggagggtgaggtttaggggctggtcggtggtgggtggacgggggtcaaggatcgagtgaaaaaataaattttaaaattgaaaatatttttattaatattgatattttcctaaatttttgaagggaagtcattttccttaatttttaggaaaatgagttgatttgaaaaatattttctaaaacttttattccaaccaaacatgaaaaaattgaaaaatattttccagaaaatgtttttcttcataccaaacacactcaaaaagagactcttttaatcaagtattattgctaaaaaaaaaagagacaaagaataataatttaccccataaatttcgcaaatcaatctataaaagattgagggtgagatattgataagataaaacaatcaaaataatagataaatatgtcttttagtttaatttaattttatatttatattccttaatttagaatggacacataatttgatatcttaacttgtatataattaaacaagtatgtatatatatatatatatatatatatatatatatatatatatatatatatatatatatatataacaccacctatgacacaatttccatgaaggatgtgcacgtttattttattgattctatacaagtttaagtatacgcttattcatactatagttgaataatataaatataaaataatatcaaatttaaaagatatatttatatattatcttaaacaaatatgttttaaaaaaaaataaaatctagtaactaccccaccataaaagtgatgcccttatacgccgaaagaacgtttaaaatcaaaagcaactgttagtgttattggattgaaaaataaaaccgaatactccaattaagagacatggcggccccatggtggaataattattacaacacaccttccataattaaagtttgaccttatacctaatgacaatcaaattttgagttcggatcctatttcatgagttaatatctcatataatcacttaattttaaataattcatttagtatgttattcaagtttaaattgttcacttaaaaagtcattcaactctattttataagtaaaaaatcactaatatttgagttgttcatttagaaagtcattcaactctctttataattcaaaagtaactcaattatttttgtttcacttaaaaagtcacccgatcccaacttaaatatttttttttcataaaatcttatttttatgttaaactattcttttaaaaaaaaaataagatatttattttagaaaaggggaaaacatgttaaaaagttagttattccaaaaaagaagaaagaagttggaattgaaaagaaataatataaaaaaaaaacgcaggacagtgcctttttttcttattactttttatttaaaagataggtataaagaaatattatacttcaacaaaatataataaataattaaaataagcagcttataattttattttatttttgtattcagccaaatttaattaaaaaatcatttaaaaataattgaatgacttcttaagtaaaattagttgagtaatttttaagttataaaataaaattgagtgactttcaaagtgaactcaaagctgagtaactttctaagtgaactattcgaaattgagtgaacatctgagatattaacaccttattttatacgtgaaacaatttaaactatattacaaaagttggaggaagatattgaagaaagattgtacatatgttcgtaagctcctttatgtcagcttataaaaggcttaacacaagtatatatagcgggtaaaattttattttgtgagaggtacaaatgttacttagcagacaatatttgtatgacattctctcagcttttgccaagtggagtttgggtctcacttacagaaaatgtgcttaaagcttcatttttttctctttcacctatttctatcttcttcttctctctttttttctccgttcttcataaattttattttattttctgtcaacaaacatcgatacttaatatattttattgaatgaaaattgatttaataatttttatttttcaaatgttaaaatcaagacaaatcaattaagtcgatttttcattactttttttttccttgcgatttgttttttgtggacttctcgaaaatatataataatataaaattatcctctgaaaaaattatgcattacgaagaatttaatcattactaagaaatatgataaattatttccttacaaaaaaattaaagatttaaggctgatatattaaagatgtcttgttaatatctgatttaaataaaataatcaattaaattacgagttattttgaacataaaaaaacactttcagtattatctaaataaaaatataagttaaactacaaagtaaaaaaaaataattattataaagagaaacacatgagtactcacaaagagaacaaaaaaaatatttataatgatttttttagctttagataaggttatacatataaccaaaattattacggaccatttgttaatgaaataataaaatataaagattctcctaataaattaatgtatgatcttttttaaacaaacacaaaaattagttaattacactatatttaatttctttaatctcactaaaaaaactattttttctcatcacatttactttaaattttccttaaataaataatataaaaataaaatagttaaacattgtggctaatttttttttttttttacaaaaaaacacaaaagactacaaaggagaacaagagaatgagaaacgaaagtttaaagggaaaaaagtctgatatacttctcaactttttcatttggagctgatatatttctcgttataaaagtgactcatatatgcccttatcgttatacaaacgactcatatatctgagtcatttgtttacaagtaaggtatcactttcttaaaaaagcaatgatatcatctctaaaacgacaaagattgaggggtatatcgatcctttttcaaagtttaaatgaatgagaaaaagttttaagtgtgggtcccatgttgtacatttaaaattctcataaactgacagaaggttagcttttcacaaagtaaaatttttcccatgtgaaactcaaaataaaataattgcgtacagacatgtttatgcaacacaacattaatttatttatttacccattcaataagtgaaggaataattataatgctttgtgctcttacttttagctgttcatatttcattccaacatcgatcttatagatttattgttaattcacaacacttccagcaatctacatggctgatgctttccttcaaattttgttgacttctttcatacaagaggaacttggattgaaaatctaaaaagcacgtttactacgatccaagctgtgcttgaagatgctcaggagaagcaactgaaggacaagccaatagaaaattggttgcacaaactcaatgttgctgcatatgaagttgatgacatcttagatgaatgtcaaactggaatttttaaccaaattaagtcattatataaaataatttaccaaagtaaaatatttttctaaaagtttacaaaactaatataaacgtatttcatggtaacgttttagggtatattttattttttaaaaactaatgactttaggttgatatcgttctttgtaagtaacgttttactcctaaaacgttattttcaataacattttactcttaaaacgttactcatagtaacgttttactcctaaaacgttattttcaataacattttactcctaaaacgttactatgagtaacgttttaggagtaaaacgttactgtgagtaacgtatatcaatctgacgccatcaacttttaaaaaataaaatatatcctaaaacgttactgtggaatacgtttatactagttttgtaaaattttagaaaaacatattattttggtgaatgactttatataatgacttagtttggttaaaacctcgtcaaactgaggcagcaagactcaatcagactaaatatgggagttatcatcctaaggctatcactttccgttacaagattgggaaaaggatgaaagagataatgaagaaactagatgcaattgctgcagaacgaagcaagtttcatttggaaaaaaggactacagagagagaagcttctagacgagaaacaggtgctcatcttaaatatattagtattaattacaacaatttaattagtttatattcatttttttgctattatcaagttcatgtgtgtttatggacccaagggacttttttctaatctaatgtttgtctcaagtctaaacagatttgtaattctaccacttatttatttactgaagttcttaaacatatatacatggtgtaagccagctcagataaatccatagtcagttgtttcggactgaatttaacttggatgtcaatttttcaaagtcaatcatgttttcaactcctccccctgattctcatctctttgtagtgcaaaaatcttctctctgtttttcgctaaacatattctcgtgtgaacatatattgcttgaaacaggttttgttttaactgaaccagaaccttatggaagagacaaagaggaagatgagatagtgaaaatcttgataaacaatgcccaacaactttcggtcctcccaatacttggtatgggagggctaggaaattcgacgcttgcccagatggtcttcaataatcagagagtaactgaccatttcaatcccaaaatatggatttgtgtctcagaagattttgatgagaagaagttgataaaggcaattgttgaatctatcgaaggaaagtcagttggtgaaaacatggatttggctccacttcaaaagaaggcattgtgtcgatttgagataatacgagaaaaatatacatgcgaaaaacaagacaacagatttcgtggttcaccaataaattggctcgtccacgggaagagggcgggttttattatggaggcaaaaaccaattctgagaatagggtttgccatagcgtctatatatagtgtaaactaagcccctaacaggcttgggcccaaaatataaattgaatgataattaagggcccaattcaaggcattcaacaaatctccaccttgacttgaattctccaagcagattcttgggcgcactatgatagtgccaggcctcccccctcttcctcgggttgcccttgagtataattacttgacacgatgttgagcaagtcaaacgagtgttgaaacttgctcacgtggagccaagctttgtgaacatatcagcgggattatcaacagttctactttcttcaccttgattctcttctcacttctcgggaaaatgatacctccgtcaatatgcttggttctctcatgatggacttgatccttggctagacaaattgcgctcaaaagctgtcaatacacacgtgctttgagtcatgatcgagaccaagatcactaaccagcccctttcaaccaaatcccttcttttgcagcctctgtcaaggccatgtactccgcttccgtagtagacaaagtcccatgtaggttgcaaagttgccttcaatgacgcggatcctcaagggtaaacacttgagtcatccgatcttcttgtgtcaacatctccaaagatagtctgaatcagaatagccaataaccaagcactgagtatcacctccataaatgggaccagcgtcggatgtacctctaaggcaccgaaaaattctcttctgactgccaatgttctctccacgttgtcccatgaatgctcactacactaatttgcatgtactaaatctggccttatacagaccatagcatacatcaaacttcctcagcactggcataagggactcgtgacatatactccttctcttcttctgactgtggagccgaacatggcgagtgggatggataaaggcgtggggtatcaatgggcttagatgaagacatgccaaacctagccaagaccttgaatgtaaccttctctgtgacaagaaaagtttccttctctctctgtctctaatgatctccatccctaaaatcttcggctcccggatccttcatctcaaactcagactaagtaaacccttgacttctgagatgtcatacttcttctttgcagctatcaatatatcatctacataaagcactagatagatgaatgaatcatccttgagcctattgtagtagacacaacaatcatatgagctccgagtatagcccaacttcaccatatagctgtcaaaccttttataccacatccttggagactgcttaagtccatataaggacttcttcaacttcaggacgtgattttccttctggaacttggaaaccatcctttgagtcatgtatatctcttcctccaactctccatgtagaaacgctgtcttcacatcaagttattcaagctccattctgatgtgtaactatcgctagtaacactcggatggaagtatgtctgaccactggtgagaagatctcattgtagtccactccctctctttggttgaaacctctggcaacaaccctggctttatacttgactccttctgctggtgatatcccttccttcttcttgaaaacccatttgcaagtaataatctttctccccgaaggctgtatgaccagatcccatgtctgattcttgtgtagggactccatctcatctcccatagcggcaaaccatttttcagaatcagaacttaaaatggcttctttgtaagtagacggctcagatgtatctacctcttcagcaacctgcagtgcataacccaccatgtcctcaaaaccatacctcgtaggtggccgaactccaaccctccttggccgatcttgagctaaactctgatggatatctgatggcatagattctggaatatcagtttctgtctgtggctcttgatcctcctcttcaggttctttcaaatcgctctcgttctgaatgacttgaaactccacctgtttatcaagactcccagtttctgacgtagttgtaggcttcacaatggttctaagcagagaactttcatcaaagacaacgttcctgctcataataaccctcttttctggagccggattacgaaacctttcactccatctcatgccccaaatactcctttttggctcttggtttctaacttaccttcactgacgtgatagtaagccgtacaaccaaaagctttcagatttgaataatcggcagcttttcgaccacatctccataggtgttttgcactgtggctgtatgtggtcccttgattatcagtagcaaagctgtactaaccgcttcttgagaatcttctatccccagcattgaaagcatgcaccttgctctctccagaagtgtttgattcatccgctcggctacaccgttctcttgtggtgtatttctaagcacatgcgatgtcgggcaatccttcatccttacgaattgatcaaattcagaccaacagaattccagcccattatcagttcgcaacctcttgatcttcttccctgtttgattttccatcaaaattttccactccttgaacttctggaaagcttcacttttatgcttcatcatgtacacccaagtcatccttgagtagtcatcaatcatggacacaaaaaatgggcgacctcccaaagactcaacacggcatggaccccaacaatcagaatggatataatcaagtgtgccttttgttctttgaatggcctttggaaacttgttgcgatgtagttttccaaagacacaatgttcacaaaactctaggctcttaaccttatgaccagcaagaagatcctctttttgatgaatttgcatccctctttcacccatatgaccaagtctattgccataacttagtcatatccttctggtgaaattctgacgatgcaacatgggctgaacctgtaaccggaaccttgtagaaaatataaaagtaccacatgacacctttcaagaatcaatttgaacctttccagaccccaagactccatcttttcccgaccatttgaatcccttgctgtcaaaagactgagagatatcagattttcgtcatcaatggaacgtgctgaccctcgttcaatgtgccaaaactaaatcgtcgtgtccttatcttgatcagcctgtcccaaccaccttgcggtgaaactgttggccatcgagatcttgcctcaaatctaccactcataagtcgtgaaccactctccctaggacagatgtgataggatgccccagaatcgagaacccacatatctgaatgatgagtgtgctcatcgtcaactagggcaatatcttcttgaattggtgtcttcttgactagcaacagcagagaccactgattgttttcgattgcttcttcttcttggacaatcaaatttcaatgtcccttctccttgcagtaattacaaacatcatccctttgcaccttcgacatcggcttatttttctttccgccgttttccttccctttccgctcttggtcagcaggcccggaaggtataatgtcgtacttgtgccgttagccttatgccgtaattccctgctatgaagggccgatctgacttcttccagtgacacagtatctttcccaacaatgaacgattgaacaaaattctcaaacgacattgggagagatactaacaatcaggcgacatcttcatcctcgatcttcacatcgatattcgcaattctaataacaaagtattcaattgctctaagtgttccctgagttgtaccttgaccattcgtaaaccgaataggcgttgtttgaagcagcttgttggttagagattttgtcatgtacaaactctccgacttcaaccgagaccagacggtctcttcatccgagacctctgcgtgatgacgtcatccgcgagacacaaagatgatcgtcagtgcgcctttcctccggaatctccatctcgggagtaacgacggcgttcttgtctttcgacaacggcgcccgtaaaaccttgttgtttcaacaaagcccgcatcttgatcgccataaaccaaactggctattcctccaccgtgaatttgtcgattttcacgttcaaagcgtacatctcaattctcaagaacacccgattaaccgagaggctcgataccaatttgttgtgcggaatttgagataatacgagaaaatataaacgcgaaaaacaagacaacagatttacgtggttcaccaataaattggctacgtccacgggaagagggaacattttattatggaaggcaaaaaccgtaattacgaatagggtttgccataagcgtctatatataactaaactaagcccttaatgcttgggccaaaatatagaattgacagataattaagggcccaattcaaggcattcaatgaagcttcaagatatgttgaatggaaagagatactttctcgttttggatgatgtttggaatgaaaatcaagaaaagtgggataagataaaagcagtcttagaggttggagcacgaggtgcttctgttctaaccaccactcgtcttaaaagggttggatcaattatggacactttgcaaccatatgaattgtcaaatctgtctcaagaagattgttggttgttgtgcatttgagaaccaagaaaaaataaatcctaaccttatggctatcggaaaggagattgtcaaaaaaagtggtggtgtgcctctagccgccaagactcttggaggtcttttgcgcttcgtggatcaagaaagagaatgggaacatgtgagagataatgagatttggaatctgcctcaagatgaaagttctattctgcctgtcctgagacatagttatcatcatcttccagttaatttaacacaaagttttgcatattgtgcagtattcccaaaggacaaggtaatggaaaaaggaaatttaatatctctctggatggcacacggttttcttttatcgaaaggaaacttggagctggaggatgtaggtaatcaagtatggaatgaattatacttgaggtcttttttccaagagattgaagttaaagatggtaaaacttatttcaagatgcatgatctcatccatgatttggcaacatctctattttcggcaagagcatcaagcagcaatatccgagaaataaacgtagaaggttacccacatatgatgtcgattggtttcggaaaagtggtgtcttcttactctccttctcacttgcaaaagtttgtgtcgttgagggtgcttaatctaagtgaattaagacttaagcgtttaccatctttggagatctagtacatttaagatacctggatttgtcttacaatagtaaaatgcgcagtcttccaaagcagttatgcaagcttcaaaatctgcagactcttgatctaaagtattgctggtcactatgttgtttgccaaaagaaacaagtaaacttggtagtctccgaaatcttttacttgatgattgcgatggattgaattctatgccagcaagattaggatctttgacatgccttaagactctaagtagatttgcagtggggaggagaaaaagttgtcaacttggtgaattctgaaacctgaatctgtatgggtcaattgaaatcacgcatcttgagagagtgaagaatgatagggatgcaaaagaagccaatttatctgcaaaagaaaatctgcattctttaagcatgagttggaatatcaacgaaccgcgtagatatgaatcagaagaagttgaagtgcttgaagccctcaaaccacactccaatgtgacttgtttaacaatcaaaggcttcagaggaatccgtctcccagagtggatgaatcactcagttttgaaaaatgttgtctctattacaattggaggttgtgaaaacttctcatgcttaccactgtttggtggtctgccttgtctagaaagtctagagttatggaatgggtctgcggaattggagtatgttgaagattctggattccctacaagaagaaggtttccatctctgagaaaacttattatagtgaattttgataatctgaaaggattgctgaaagaggcaggagaagagcaattccccgtgcttgaagagatgaaaattagctgttgtcctgtttttgttattcagaccctttcttctgtgaagaaattgaatgcttattggcacaagtcagatgcaacaggtttgagttccatatcaaatcttagggctcttacttccctcaacattagccataactccacagctactttgctcccagaagagatgttcaaaagccttgcaactctcaaatacttgaaaatctcttacttcgataatctcaaagatctgccaaacagcctggctagtctcaatgctttgaagcatctggagattaattgttgttatgtactagagagtctccccgaggaaggggtgaaaggtttaacttcactcacacagttatccattgcatactgtgagatgctaaaatgtttatcagagggattgcagcaactcacaaatttatcaattacgaattgtccaacactggccaagcgatgtgagaagggaataggacaagactgatacaaaattgctcacattcctcatctgctgattacatagtgtcatactaaattaaatgattcttatagcaatattattggttcaaccaacaaaactaaatctctaattatattacttaattgcttttagtttgctacaattatcactcatgactaacattatgtatcaattacgtggtttgtcttcaattttgtataattagtcatgtttttatatgtataattcgctagaataatacagatatatgtataatatacaattatttaactgatatacatatataattcacctctcttccactctctgtcctctctcacttgcctctgtcctctgccaatcgacgagatgagcctacgaaagatttcaagttcagactatgatgactgacatcctcacttacgcaacgaaatggagttgatggagtagccagtgcccttgagtcattctcttcggtatcgccttctctcatcgttaatggcgccgcaaggcactcgactagcaagttagaccttagttagggcgaaagatttcttggatggttcatttcagtctgaagtcgggtcaagtcatggaattgatgtgaagttctctcaatttcgctttccatatatacaaatatatatgtataacatacaattatctaaatgatatatatatatatatatatatatatatatataagcaatttatctctctcccactctttgtttcacctgacaactatgacaactatgtttgttagggctggaaggtctaacttcactcaccgagttatttgttgaacatatgctaaaatgtttacccgaggaattgcaccacctaacaaacctcacaattttttttttataagtgaaagcatagttaaactctcaaatgtagatgataattaagctcttgaagattattgctgaattaagtgaattcgtcaagctatatttgtaaaattcttatggccaaacaagtaatattgcaacaaattgtagaaggattattatactcttaacactaactaaaagattcttccaattctcaaagcaatttatattcctttccaaccaaagaggttttccaaatttgctttctagcaaaaaacaattttctgcacgataggaatagatctcatatatactccctccgtttcattttatgtgaagtagtttaactgagtacggaatacaaaaataaaagaaagacatttaaaatttatggtctaaaatgaagggaaaaaggtcgatatctcctcaactttgtcattttagaaatgatataccttgttatgaaagtggctcatatatacccctacttgtaaacaaatggctcacatatacctttttcctctaacgggaaatgaaaaataataattttcaatctaaattttttattttttttctaaaaaatataagtccatatgagtaaatttaattctcgtcaaacaatttttttttttttactttttttttgtttcaatgactaatttataattattagtttgataatcaaatttatttatgtttcactaatattcttgtaaaacttattgtagatgaaaaaaaaaaaatttgaatacgaaattaaattacaataaacacaaaaaaatagtttatttttttttttctttaaactaaggaatgatagaaaaaaataaaataagaataagaaactcaaataattataataaaagaagttaaaaataatttatgtatgaaaaaaaaattaaatatactttgaacttttattgaagaatcatatataccactaaataatttttttaaaattttttaagtaataaatataaatttaaaactaattatttaaaattttgttaaatgaagggtatatttgaacaattttgtaacggcaggggtatatgtgagccgtttgtataacggtaagggtatatacgagccacttttataacgagagtatatcagattcaaatgacaaagttgaggggtatatcaaacccttttcccctaaaatgaataataaaaaattgtgtgagtataaatcatttcattaagagtaaatggacaatttaaaattaaattgttacttaatatagtaacgtatcttttttgtttttgagtctgctttaaaaagaaaataaaccatataaattggaacatagggagtatctacttacaaagtaaaagttgtgtgtagaagattttggcatacaaatcaaatcatatatcatatcatatatcatcatatcatatatcacatcatatcatatattagtaaaagcatgaataaaaaaagttgaaagttgaattacggttttattccttctattaattaacttgttataaaatatttaaatatttgattttacaagtttaattaaaatgttaaatgacttttagacttcctacgattaatttctaattaaatatctaatttattaatatttatcatttataatctatatgtatataataattataattttttaaaataaaagtctaattataattttaatgactttttagacttcctaacactaattcctaattaaatatctaatttattaatatttttatcatctataatgttataataagcatctttagaaggtttctctgaaatactctttaaaagaatgcttggactatgccatcctaaggttgaaaccagtaggcaaaagaaggtcgttatggggagtaaacaaagttgaggcgctgttagggtaaccaattaaagaagaaagctgtagtagtgactaggcgagatgattattaaatcattattattacataataagtaagtataatttattaagaggtcggaaggaataaaacttttagcaaaaatgaataagatgactacctacctaattgatgatgatgatgaatataagatattattactttatatattaaaaaatcttaatactgatcaagttagcagtctcaaaaatctttttttacttcatggttgccataaattgaattctatgccaccaagtataggatctttgacatgccttaagactctaggtcactttgttgtgggaaggaagaaaggttctcaacttgatgaactacgaaacctaaatctctatggatcaatttcaatcacacaactagagagagtaaagaatgatagggatgcaaaagaagccaatttatctgcaaaagctaatctgcattctttaagcatgagttggaatatcaacgaaccgcgtagatatgaatcagaagaagttgaagtgcttgaagccctcaaaccacactccaatgtgacttgtttaacaatcaaaggcttcagaggaatccgtctcccagagtggatgaatcactcagttttgaaaaatgttgtctctattacaattggaggttgtgaaaacttctcatgcttaccactgtttggtggtctgccttgtctagaaagtctagagttatggaatgggtctgcggaattggagtatgttgaagattctggattccctacaagaagaaggtttccatctctgagaaaacttattatagtgaattttgataatctgaaaggattgctgaaagaggcaggagaagagcaattccccgtgcttgaagagatgaaaattagctgttgtcctgtttttgttattcagaccctttcttctgtgaagaaattgaatgcttattggcacaagtcagatgcaacaggtttgagttccatatcaaatcttagggctcttacttccctcaacattagccataactccacagctactttgctcccagaagagatgttcaaaagccttgcaaatctcaaatacttggaaatctctttcttcgataatctcaaagagctgccaaacagcctggctagtctcaatgctttgaagcatctgaagattagttgttgtcccaaactggagactctccccgaggaaggggtgaaaggtttaacttcactcacactgttatccattacatactgtgagatgctaaaatgtttaccagtgggactgcagacactcacaaatttatcaattaagaaatgtccaacactggccaagcgatgtgagaagggaataggacaagactggtacaaaattgctcacattcctcatctgctgattactgattagatgtaattttctgatttttcttttggaaacaaatcaactatttgtaacatctatttgtatgatacttgatttttcttggttatgtaacaataaatatttgaaatttttcatattaaagattcagaatgagttttatagctaactctatattttcacagtttaataacgtaaaaatgtgatatttatatcaaattattacttatgttgtcatttatcaacatgttggagatgattttgacagtttattaaagaatttctaagtttttattgtttgcacaagtaacaagccataaattaagtttcgagataaaagtgatttgtgtatcatggcttaattagtcggaatttcaagtttttttctcaagttatatatatgacaatttgtaaaaaatagatagtattgattttgatttaattcaagcatttttaaaaatataaacattataatatgggagatacacacgctaaacgcgtacccagaaactagtatataaagaatcatgaccgaaaaataaaatgaagttctgtcaacaactatctcgacatctttgctgatatatatatatatctaactagtgtacttattcggacttgacatggtataaaaagatattaaatatatttttaaataattaataaatgatataataaaaagaaagaaatacaaattcagttatgattctgataaaagggaaactaattttctgatttttcttttggaaacaaatcaactatttgtattatacttgttaatgttgcaattattagtgaacagttgtattttggattatcacttacagcagatgtctaaaatgtgaataagataatacttagaataatttatgcaatatacttttgtttaaatacaagaaatttaaataaagattgctaaagattattattttgaatgaaagattttgattttgttactttgtcgcctatgtaacatagtactgttgcaaacatatacatatgtgttcatttttccccttgtgtttcattttattttctacaactcataaatactaaaaagaaaacgttaggaatgagttttaactagatttaaattttaacaaaaacaacgtgattatatttcactaaattgacttaaatatatttatacttaaaaaaaaattattaatttataatattaatgggaccatatatttatataaaaattttctataaatatattatcttatatctcctctaaattcatttcacgagaattaaaaccatcctaacggatgacgttgccaaaaagaatagaaattttctttgaaagcgtgttaagttttttttaaaaaaaagtaatggtctcactttgtatatatgaagaaaaaaaaaacccacccctttcttcttcttcttcaaacccccacccccgctttttcaaaacccaccagccccctttacctgcttgtcttttcttcctcatattcccgacgtcaccctatccccaacccaccccatcctctttctcatttttcgaactctacattcaaagcacataaataaaaagaatcacatttaagattcatataatttttttactctttacttttgagatttgatttttcttaaaaagttatgatttttttgaaaataaagaatagggcataaaagaagatgaggttttgtcaaccaatctataatgttaatggctgggaatggtgattgaagcaatggatagagaaagatttttttttaaaaaaaaaagagaagaaaaatcactacaatcagtaaccgcaattgcagtaggcttacatcatggagtatcccaatgagtctcttcactgttcaatcggccatcggtaaccgcattacaatgggctttgggtcacccacccaatttcttataaatagaaagagacatgagatttatgattgcacctagatcacatagtgatttggcaaagtgtaataatacgaatggtacatgaaatagtgaaagcgccaggatcttccttcttctgcacaagagttcttgtgacaatagcactacaatgctgcattcagttatcatcctcaaaacttaccgatctcttctttgtaactatatccttcatgaacttggcataaccggaccatttgctccaaagcttctatcaaagggacattgatggaaagttgcttcaacatagtgataaaatgttggtatttaccattctcactattcttcaccaatctaaaagtggtggtggtctaggaatggggaccactttctagggtatctttgcttttttcgccgctttgtccaccaattcaccactagtttccaccacctcttcatcttttctcatctcatcttctaccacagacgacataggtgaatcaatagtttgcatacctcctcaagtagtgactgtcatgcaatgtccatcatttttaggatttgaatggaattactatgaaaagtgacagttgtcgcgggttctgatagtgaacaattggaccatttataattcaagatgcttaatcgagaccgcatgtgcatccacctttttcccgatattagccaaatcacctctcaatttcttggcgtgctcatcactagcatcaaaccttctcatcatctttagcaacatatcttcaacttgcgccgtactacctccaccatctcaaggagcaactttctgattttgaggtggaacatagggcacacttcaatcatttctattaccatagttaccccggttgaagttgttatctcggttgtagtttcttctcgaacttactggccctcttgttgtaattcccattctgcattttcaatttaaaattgttgataaaaaagacaaaaacataaaaattgatatgaaagagctttggttaagtaacaatctaattatcatagtgtcatattcaattcaatgattcttatagcaatattgttggttcaacagtttaactttactcgctgagttttctatttatgatgttaaaatgtttaccgaagggttattatacttgtttttaatgttgtaactattaggggtagattatcactttatgaatgaatattttggcacattggaaaaacaccaaatatagcgcgcaaaagctaaacaaggaaattttcatatattggatatagtctttgtcatttccaaaggtctccaacatagagatagtaattgagagaaaacttctattgctattaaatagaatctgcaattaaaaaaaaaataaattattattatattttatattataagtgggaagatgcttagtctaaaggtggattaagaaaacgccttcaacttttttaattatcattattatattatattataaataataattaattatttttctataagtgtgaaactattaaagttgaataaccttttaattctacaagaactcaccattaagttgaatgactttttaactcttcaagaaatcactaataagtctttttacacgtcgtcttataatgataatattgtacatttgaatttggtttagagagcataaatcccttattatactatgtgttttcaagcatttctttacatttagattttttttattttttgctataattcaagttatattcttaaattgatatttaagtgtttgatttctcacatgaaaatatacagttaaaattttgttttatgaactcatgatgtaattttttctcaggtataattttaatgtgattcttttgcagacaattgactaaaatttttagtagaaattgcaccaatacaaataaggtatgcggcatgtctctccaacaattttacattttttgcatgattattttttaataaatttgatatacatacgattattgtatttttaactagattttaataacttaatgcatgtttttttttataatagagcctccttgataactttacaattacttattgaaatttatttttcttcaatctcctagcttccgagataaaatgggtaactaatatttctccctcaacaacatggagcaaaaaaaatcgagaaaatctatgaagaagacatattctaacaaatggagtaatttaatttaatttaaaggagtacttaatagtcaaatatgaatagtaaagtaagagaaaaaaaaataaaaaaattagaatatgacaagtatgaaagacaaccatgaacaaattattggagttttttgttcatgctacaaagaacaataaagttactatgtcatttgaatgtaatatgtagacaacatatatacttgttacaagtatatatggtaattcaaattttggtacaaattgagcaggtgtgttatgtgtgtattgttcctttcttagaaaagtaacaaactaatatattgtagatttcgacctaataacataaaaatgtaaattatttatcacattaaattttgttgtccaaatttgacaagttattggaatatctaattatttgacatttacattttacaataaagaagtcatttttataggttgattgtccatttatttcgtttatatttttttcgttaaatcatttttgaaaattttcaaactgtgattttaatatatttttttagtttaatgtaattttaatataactcctacaatatataatatttttgtgggactgacatgcaaaacacgtgtcttggactagtctttcacataaagacagacaactaagaagattgtatcgcggataaacgctactggaatagccctattatgaagagtgtttgtcaaacagccaaatgactgtagttttttcttttccagaaatatgactgaaggactatatcttggatcgatcagagtgcatgaatcactcagttttggaaaataaagttttgcttgataaacacaaatttatctattcacaccacaagcaatggtaagtcatcataaaaaaaaagagagagagagaaatttgttgttagatcgagaaagattttgataattgacgaatagacgaacaaatgaaagaaacaggttgcatgtacatgttcctttcaaaccaaatccgactgggattgtcaaccatgcgaattagaagttataaagtaatggaagggttgctttttcgacccgaacgaagagtgcaaaaggtttcctttcataaagaaatcctaagcaaagtgggaagtgtaaacgaagtaggtagcataagcgagtaggaagtataacgacgtgaataaatttcaaatctgaatggagtagatgatcagatatgtaaaacaagtacaagatgaaaaaggttttgaagagtccaaagtttataaatagggcaatattttctttggagaaaattgtgcacttaaacagagagttacaagcaaaatacaatcaaatagagggagtttatatttgagtgaattctgattacgaactgcagccaacacaagaaaacaagaattgaagaactcattcattggcttatgttttatagttcttaagtcaagtttttttgtattgagtttttatcgagttgtatatttaaccctttctaaatccagtgaagtataaactggagtagaaatagagtctttaagttaaagacttggaaacataaaccttgggggattttgttggagtctaggaattagaatcagttctagtattgcaagagttggaatccgaattcataacttgaagtgggatcgacgatctagttggttgttggtagggccgactcaacaagattgagggcctaaagtcaaaccttaaagagggctccaatatttttttaattctttttaaaaaaaaaaaaaaaaaaactaataatcatgtatatattatttaaaatctattttctagcttttctagatgtgaagtcattaattactattttctaatggatttgttttaataattctttttcaattgataatatagctaatacattcaatctcattgttgatattacatatataagattttatcaatttaaattttaaaaaattctttcggccgaaacaatagttctggattgttaactttattcgttaagcaatatatgcattaggattagaatcaagtctttttattagattgcgtatttccattaaatcattatcttctacttgtattatttctcttaataataataactaaagcgagcatgtatacttactatgaatatcaacaacaacaaaagttcaagaaaaattacaaaataagttagtataataaaacttggcttgcgaatttgataaattgatataacaatactgaaatagtgtttcatttcttcaatataatgactgtttgtttaaacaagacactcaaaaacaaattttattttttttaacatgtaagcgacaataacttttttttaggagagtgttcaacattgagcataaaagtaataaaatagagaataaaaaagatgagtataagataaataataatataagatcgattttacctattgtcaattttgtgtatcgactaaagaaataacagcttcacatatgaatttgtattttaggctgctgtaagtactaaaagatagttattcaaccagtagaagagatgaaggtggggggcagctgttggcaatcaataagggcatattgagccaatttttttcttctctgaaaaactttggcagagaaattaaggctaacgaaaagtctttgtgcagttgtttcccaaaactttgtgaattgtatttcaaaaaatacattatttaatactccaacaactttgtgattccactctagactaccatcacatatctaatattaattataatagtgaatttcacatatggccagaggcgaacccacctgcacccaatatatttttaaaaaaaattcatatgtagattgttgataagacgctataatatatttaattgtgcactcttataatgaacaaatgatttgacttgttcattgaaaaaacaaaaagtgtcacataaattgagacatgaaaaataatatttcttttttaaatttttcgtgtgaagtcaaactaattcatatataaagcgaaagcggaaggagtactgtttaatattaattgcatatggtagtaaatttgatagacatggtcccgtggggtgtgtgttatttccattgaataattgagtttgtaattgttacaagtccattctaatttccaacaccttacttcatttcaaaaatatagattcattgcttactcaccacatactcgatggctgaagctttccttcaaattctgttagaaaatttaacatctttcatacaaggggaacttggattgttttttggttttaaggacgaatttgaaaatctgaaaagctcgtttactacgatccaagctgtgcttgaagatgctcaggagaagcaactgaaggacaagccactagaaaattggttgcagaaactcaatgttgctgcatatgaagttgatgacatcttggatgaatatcaaactgaggcagcaagactcaatcagactaaatatgggagttatcatccaaaggctatcgctttccgctacaagattgggaaaaggatgaaagagataatgaagaaactagatgcaattgctgcagaacgaagcaagtttcatttggaaaaaaggactacagagagagaagctgctagacgacaaacaggtgctcatcttaaatatattagtcttagttacaacaatttaattagtttatattcattttttggcgattatcaagttcatctgtgtttatggactgaacttaacttggatgtcaatttttcaaagtcaatcatgttttcaactcccccctgattcttatctctttgtagtgcaaaaatcttctctctgtttttcgctaaacatattctcgtgtgaacatatgttgcttgaaacaggttttgttttaactgaaccagaactttatggaagagacaaagaggaagatgagatagtgaaaatcctgataaacaatgcccaacaactttcggtcctcccaatacttggtatgggggggctaggaaaatcgacgcttgcccagatggtcttcaatgatcagagagtaactgaccatttccatcccaaaacgtggatttgtgtctcagaaggttttgatgagaagaagttgataaaggcaattgttgaatctatcgaagaaaacccacttggtgacgacatggatttggctccacttcaaaagaagcttcaggataggttgaatggaaagagatactttctcgttttggatgatgtttggaatgaaaatcaagaaaagtgggataagataaaagcagtcttagaggttggagcacgaggtgcttctgttctaaccaccactcgtcttaaaagggttggatcaattatgggaactttgcaaccatatgaattgtcaaatctgtctcaagaagattgttggttgttgttcatgaaacgtgcatttgagaaccaagaaaaaataaatcctaaccttgtggctatcggaaaggagattgtcaaaaaaagtggtggtgtgcctctagccgccaaaactcttggaggtcttttgcgcttcgtggatcaagaaagagaatgggaacatgtgagagataatgagatttggaatctgcctcaagatgaaagttttattctgcctgccctgagacttagttatcatcatcttccagttgatttaacacaaagttttgcatattgtgcagtattcccaaaggatacggtaatggaaaaaggaaatctaatctgtctctggatggcacacggttttcttttatcgaaaggaaacttagagctggaggatgtaggtaatcaagtatggaatgaattatacttgaggtcttttttccaagagattgaagttaaagatggtaaaacttatttcaagatgcatgatctcatccatgatttggcaacatctctatttttggcaagagcatcaagcagcaatatccgagaaataaacgtagaaggttacccacatatgatgtcgattggtttcgcaaaagtggtgtcttcttactctccttctcacttgcaaaagtttgtgtcgttgagggtgcttaatctaagtgaattaagacttaagcgtttaccatcttccattggagatctagtacatttaagatacttgaacctctctcgcaataacatgcgtagtcttccaaagcagttatgcaagcttcaaaatctacagactcttgatctacagtattgctggtcactttgttgtttgccaaatcaaacaagtcaagttagcagtctcagaaatcttttacttcatggttgccataaattgaattctatgccaccaaggataggatctttgacatgccttaagactcttggttgctttgctgtgggaaggaagaaaagttgtcaacttggtgaattacgaaacctgaatctgtatggctcaattcaaatcacacatcttgagagagtgaagaatgatagggatgtaaaagaagccaatttatctgcaaaagaaaatctgcattctttaatcatggaatgggacgacgatgaacgtccacatagatatgaatcagaagaagttgaagtgcttgaagctctcaaaccacactccaatgtgacttgtttaaaaatctatagattcagaggaatccgtctcccagagtggatgaatcactcagttttgaaaaatgttgtctctattagaattggaggttgtgaaaactgctcatgcttaccaccgtttggtgatttgccttgtctagaaagtctagagttatggagtgggtctgcggaagtggagtatgttgaacattctggattcccaacaagaagaaggtttccatctctgagaaaacttattatagacaattttgataatctgaaaggattgctgaaagaggcaggagaagagcaattccccgtgcttgaagagttgacaattagttgttgtcctgtgtttgttattccgaccctttcttctgtcaagaaattggtagtttatgggaacatgtcagatgcaacagtttttaggtccatatataatcttagggctcttacttccctcaacattagccttaactccatagctacttcgctcccagaagagatgttcaaaagccttgcaaatctcaaatacttggcaatctctttcttcgacaatctcaaagagctgccaaacagcctggctagtctcaatgctttgaagcatctgaaaattgaatcttgttatgcactcgagagtctccccgaggaagcggtgaaaggtttaacttcactcacacagttatccatagaatactgtgagatgctaaaatgtttaccggaggaattgcagcaactcacaaatttatcaattacgaattgtccaacactggccaagcgatgtgagaagggaataggacaagactggtacaaaattgctcacattcctcatctgctgattacatagtgtcatactaaattaaataattcttatagcaatattattggttcaaccaacaaaactaaatctctagttatattatttacttgctcatcatagctatagtttgctataatcatcactcgcgattaacattatgcatcaattacgcgggctgacttcgattttgtataattagtcacgtttttatgtgtataattcgccagaatatacggatatatgtataatatataattatttaaccgatatacatatataattcacctctctcccactctatgtcatctctcactcgcctctctcctccctctcttaattttgcttttcatatatacaaatacatatgtgtaatatacaattatctaaacgatatatatatatgcaattcatctctctcccgctcttttgcttcacctgacaactatgacatttaactttggatatgcacatttaaaaactggttacagaaactcaatgttgctgcgtataaagttgatgacttattggatgaacgtgaatacgaggcagcaagactaaagcagtctcgattaggacgttatcatccaaaggctatcaaatacgaactcagttgtttagaccacaaaaagactgtgaattcaatacaggagtagttaacgatttagaagagatctactcttaacgctaactaaaagattattccaattctcaaagaaaatttatattcctttccaaccaaagaggttttccaaatttgctttctagtaatttttttttttttctgcacgataggaatagatctcatatactccctccgtcccattttatgtgaagtagtttaactcgtacggaatacaaaaatgaaagaaagacatttaaaatttatggtctaaatgaataataaaaaatcgtgtgactataaatcatttcattaagagaaaatagacaatttaaaattaaattgttacttagtatagtaacgtgtctttttttttttaaactgtctaaaaaagaaaataaattatataaattggaacatagggagtatctacttacaaagtaaaagttatgtgtagaagattttggcatacaaatcatatcatatatcatcatatcatatatcacatcatatcatcatatattattataagcatgaagttcaaaacttaaaagttgaattaccattttagccttatactaaattaaaatattataaaataattaattaattaaatattaaatatgcttaaattgttaattaagttgattcacttattgttaaaataaataggagaatgaatagttgtaaaaataattaattataaagttattacaaaaacttattagagaaacgtttcatttctctatcgatcgattttaggtgtaattttgtcataatgtgtattaataccacacctccactatctcatcattaatatccacaccttcataatcttccacactctcaagaagttgatggcataattatgagacttttgattttactcaatgatgtcctataaattgcggtatttgacacaacaatctatacactttgaagatatttaggtacagtttggaagaaattaaaaaaaatgtctatatttctattgtttttatcctttagtatatatttaaatcactttttaaactgctcataacaccgattcattaattttccttatcttcatttgttgtttataggaaggaaatgtgtacaaattgttagatcttctaatggagtttacaacgagagaagggatgttcaagtcttccggaggttgaaatcaattttaatttcaagtattatattcatgcttttagatgtttatatatatatatatatatatatatatatatatatatatatatatatattcaaatgagtcaacatagactaatatgagacttaaaggtcggaaaattggagtatcacaattagtagtaaaacaaagtaagaaatctcaattagatatattttattattttttaagaaataatacactcatgggtataagtgtgaagctccaaaatgcaaaaagttgaattactattgtatccctataatagttaattatttttaaatattagttcatatgatattattaaattatacttctttgaaattaataacataataaaaaccaaattcatctttgaagtgcaaatttatcgtccttcattattgataatttgaatgcactaaaaactatttaatatcccggaaggtggaagagtgaaagtattcataattaatttctagataaaattttactagataaaaaagtatacatgcattggaattaataatttaaaaataaagaaataatgatttagccttttaagttacctacttttattatgctctttaaaccattgttattattttttaaaaaaaaaactcatattaaggtgttagcttgattagtctaaagatatcaaaatgtcatttcttggatcacttaatttgtaacgtttttatcttctattagcgtgattctccattttcctatattatatattatactttctcatgtaatcatgttatctatatttatttttttatataagtttgttatgctcaatgttttatttatctttatttgaactcatctaaattgttgaatatttcaactactaataaattttttaaatttgactttttttttatgaaaatacaattaagaaatgacgctaatatttcatagtgatgatgcagtaagtgaagcaacacagattgaactgtttcaagtggtatcaattttcaggtaataaatcattgttccttatatgcaattaattatttttgtgtaagttgatatgttcttaataaaattttggtttgatttttaaataaaaattattttatagaagttgagacggtacacttaattggattatccaaaaaaagaatcttttacacaaggacaagaagaaagacttctagctttatcactgcattcatgacaatcaatggaatatcctacaagacaaaaagttgatgtgattctgtacaagtgaatccaactcactaacaaaaaaattaaagaaagaaaaaaatgaacatgaagagaataaaaatgaagatgaagagaatcaatggtgtcttataagttgatgaaccactgtaacttcattattttttaaatttacgaggaaatgaattattgacgaaatttatgaaatgtacatatatacctttgggtcggtaacaaatgtgattgaaagtagtattttttcatgcataatagctaattcttgatatatatattgtttaaatttattatttgtactacaaacattgtatgatatattttaggataagcgtaacgcatgcgacgtggaaactagtatattagtaaaagcatgaataaaaaagttgaaagttgaattacgattttattccttctataattaacttgttataaaatatttaaatatttgattgtacaagtttaattaaaatgttaaatgacttttagacttcataagattaatttataattaaatatctattttattaatatttatcatttataatctatatgtatataataattatatttttttttaaataaaagtctaattaaaatattaatgacttttagacttcctaacactaatttctaattaaatatctaatttattaatatttttatcatctattatctctctctatataataattttacaaaaattaacaaaaaaagtctctacgtaaatttttatacttttttttttattctcataaatttttcctaaataacaaaatttaataatttgaaggatgcaaatctgcaaaatggagacacacacatttgataatgtcctcttaattatcattaaagaatgactctaactagcttcacaaatttaaattcattgatacttaattactcggagaaaagtagatgaagactcttaattttgatagtatatggaaggagtcaataaagtttcgtagatttatgcaataattttgtacttattttttcatctacatatacatagtcttatgagaatgatgtctacattgtattttttcttaaatctgtttcttttgtcttttatccccaattagacttcttaatttaattttatacaaatgttttattgtcataagtctttatacttattttgtaattgtagcattttattgttcattacaatttgcatatatatatttccatgaaatattagtaattctatcatatctataaaaattcacatgaaatacacgtgcaaagcacgtgttcagaaactagttaggaaaacaacacaaatatacatctgaactatcgtaaatgatatacagataccatcatcatacttttgggacattggtgtccatgtcgtcaaaaaaatagagcaaatatattaatggacatcacgtgtcagaatcatatcaattgatccaacatttattaaatgtttgatcgaagaatagattgtgtcacatgtccctatttagtcatctgttaaaatgaatgacatatgggttgggccgaccattttctgacccacacaaaaaatgggctagcccggtttaacccgtaaaatatcaaaacatgtatggattagcccggataaggtgtgttagccatattgacagctttatccccacatcaagaaggtatttatatgtcaacttgaaaagaaaaaattttccaaatatgatctgcttatactctatcaattccatatctcacttagtgaaatttcactgaatatattgttgttgttggtgtcctctcccatcattataaatttaaagaacatgcaatgtaagacgtaatttagaaaacttggttcgcccgtagaagaaggatcatctgtaaatttattcctctgcaagttgatgctttgaatctgttggtacatttcctctaaacatgttagattggattgaatcttaagtcatcatgtgttactatctgaaagaccaatatttaaatttattgctcacaagtaaaaattagaactaaaaatatacaaacatgaagttcaacatatattataacttaattcataaaagaaaaattatttgcatgcataatatttgtttattcatttcttagtgtacatattttaactttatcagcgtagtaatttggtttgatttgtttgtttgttataatgtaattacaagtgtacttagcttgtttgattacacaagtgtaatcatataattatactgaattttaaagataaaagttaattatttgaaacaaaaaaattatattaggcaaataagagcctttataaatgatattcaattgaatatttaagatatatagtgtcttttaaaaaatatgttatttaataaacatatgttcttaattaatattataaaaaaagcaaatgatttatatatttcaatgtagtatttttaaagtaaattaatcataaaaattaaaaatgcatgaacatcatgaaatgcttgtttcacaaaaaaattaatattataaatataatgtcataaaatcatagaaaaataattgacaaaagaactaatttatcaagtctaacttaaaaagaataggttgcaatggaatatcaagtcaatactcctaaaacaaatgaaattgaaaatataatataagttctaaatttaaaataaaaaatttaacataatacttttatgtcaaatttcaacataatatgattaaaagaaaaggaaaatttaagtccgtaactttgttcaacaataaattctactttaattcaaaaattagaatactaacaaaattatactaataatttttttagatattatgaagaattgcatgaaatcacatgaagtaaaagttaaaaataagaaggaaatgaaatataaataataaaggaaaactttcatatatagccacttaaaaataattaattactctccatagctatagtttgataattacaatttgtagctacatgttatgtggaggagagagaggcgagcgtcacttggagagagaggcgagagagagagggggaaaagagtgggagaaaggtgaattgtatatgtatattggctagataattgtatattatacatatgtaattgtatatatggcaagagagattgagagagggaggagagaggcgagtgagactgtgagagagagagagaggcgagcgagatcaagagagggaggagagaggtgagcgagagagggcagagagtgagagggatgtgaattgtatatgtatataattttatataactgtatattatacatatacatttgtataaatggcaagcgagattgggagagggatgagagagacgagcgagagagggcagagagtgggagagaggtgaattgtatatgtatataggctaaaaaattgtatattatacatatttatttgtatatcctggcaaattatacatatataaacatgataattatacaaacatgaagtcaacccacgtaattaatgtataatgttagtcgcgagtggtaattataacaaactatagttatgatgcataattaaaataatataagtttgtttattcgcataatttttccttttttaaattcctccttctattcaacttgcattttttgtcaaatataatcatcgttaaaaattatttgatgttgaattaacaaacatccatctttattatatcacatgttgtgacatgcaccaaaacgataaaaacgacaccttcaaaatgattttttttaaaataagcctagttaattgatgtttaacatataaataatcaactaataaggttaaaggcttacacatacaaactaaaaattagatcaaatgcactaaaaataaataatatgaggaaaatctgttttagggattatagtgtcccccaacgaccaagtcttatttttaatggagcatcattgattggtctattgacaaagaaaatttggaaattaatgattttgttttatcctctggaaatttattatgttatcacaactatttgttaatttgaactgcataaaagtttttgttcgaacttcatatatgaaaattctaaacaagaattggaaacttgaaatgaatccaacatttaaatcaatagataattattgattgaatttcttaatacgtatatatacaaaagatctgaataaaagctattgaatacattacatgttatattggttaatttgaccgtaaaacagttgacattcttttgtcaagcatctattctggggaggttatatatatatacatttgaataatgacgttatactatagcctaaaactacataaaaaatgtcaagtaaattatttaactgtcaatacagaattccacaaccaatagtttatttccctttagcaatgaattgcagtcaagttcagctagcaatatacaattaaaagatgtttcaaatcattggtattaattagataagtattgactcaattacaagtatacacacagtatatatagatggcgtttgaaaacgaaaacataggcacaaatagcagctaaagaagttgaacaaatcaaaatggttgcgaagactattattatagcatgcctagttttgttaacatgcctctcagttactaatgcatcgaacattacaactgatgaggcacaaatgactatatctagtgaaattaacatgcagatgaataggcatatcttgcagtaaaaagcatcaaagagtgacatcattagtcctcaatagctttggatttagaggttcaatcgcgacagatattgggaatctctccttccttaactttttggacattggaaacaacagtttccatggccaaatacctgatgaaatagggcgtttgaggcgtttaaaatacatgtatttgcagatgaataatctcgctggtcaaatcccagaaagccttggatttctcacaaggcttcaagttcttcatctttctgaaaatcgtctatttggaaatgttccagcttccattttcagcgtgtcttctttaaaggacattgatttgtctcagaattacgagttaactgggagtttaccaaatgagatatgcactaatcttccagtgttggaatatatatccctgcaagataatcaatttgtaggtgaacttcctaaaggtttaaataaatgctccaaacttgaagttctgtccttgtcttataacaaattcactggtaattaactaacttgtaaacttttcatttactaatttcttcttgaattaatcatcatttttgtgtgtgtctgtgattttataattgataggaaacttaccaagagacatgtggaacatgtcaaaggttcaagaactttttattggatggaataacttaacaggtacgtgattctgtatgtattaaatcttgaatactcttcacgaagttcctaatttcactagatatagccaatttgtgcattgtctagtaataaacaaagattaatatattttgtggagaacattttcgaaagacactctatgtatgatctttagcatgataaccatatacttattttcaaaatgaatttgcaggaaatataccaaatgaaatgaacctaccatctatttgcaggaaagttaacaaagcttgagcatcttgttgggttatgggtctttttcccttcctatttggataactaaaagcccaatttggaccaatccatttttgcctataagcccattcttatgaggcaaatataaactgattttagggtctgattttcagaacatatagagagttcttcagcagccaaaaagagagaaagagagattttcgcaggcaaaattcagatctaatagacaacttcaaattgcgattcccgcttcttttcttatccgattgagttgatttttggacagcatattgtcttcatctcaatctttgattagaaactgacagagttggatttggtggcctgcgactttcagttttgcttttgtcgtgagcgaagctgcaaaattggtgattttgctcctttaattttctagatttggtgcaatcttattttgttgttgctcgttgtttggcacttgttttgtggccaattttggagaacaatattgtaactcttggtgattatagtggagcttttggtccgtggtttttactcttcacatgaagggttttcaacgtaaatcttggtgtcttatgtgattggtttcacattgtcttgttatatttgtttggttgaattggaatcgccttactatcatattgcttgtggttgtttgtcttctcttggttcaaatcgaaaaagggaaagtatagacttggatattcttccgttatctgtcgtcagcattcttggtagtgtcttgtctttcccaacaaagtggtatcagagcattgggtattgttgattgtcgttttgaatgatggagacaaatatgagcaaaatggtgtttttaaatggtagtaactatcatatttggaaaggcaagatgaaagatcttctatttgtcaagaagatgcatttacctgtgtttgtttctaataagcctaagtctttgaatgatgaagaatgggaatttgagcatcatgcaggtttggctatattatacaatgggttgaagataatgttattagaaatcagtattgtgaatgagacatgccaaaagtttgtggacaagtcgagacactttatgcttcaagattgtgtaacaactgctcctattgaacaattaatgaatatcgtataaagagggcactcctatttctgatcatattaatgattttagggggttcttgaccggctgtccgaaatgggtgtaaagtttgatgatgagatacagggactttggcttcttaataccgccagatcttgggaaactcttcagtttctttgaccaatctgctcccaaagggtgttgtaaccatcggaatatactaaaagtagtgtcttgaatgaagaaataagaagaagatctgacctcatcttcagacttctacactccgatgtttttccactgaagatagggggagaaacaagtcggtaggaggaatgatagaggtaaaagtgtatgtcaaagtctaagtctaacacaagaatattacatgtgactattgccacaagaatgggcatatcatgaaatattgttacaagcctgagagatatgagacaacaaaaaagagaaggcgataatgaaaatcgtgttgttgttgttgctaatgatcttctttctttttttcttgatgcaaatgccattaatcttgttcgtgatgagtctagctggtttgtggattcgggtgctacttctcatgtcatgccaaagaaggaattctatttcttatactccggggtaattttgaaacgttgaaatgggcaataatcatgaagttgaagttattggcattgggacagtttgtttggaaaataacaatggttcaaaactagttctcaataatgtcaagcatactccggatgttcgcttgaatttgatttacgtaggatatcttgatgatgaggttatgttaaacacatttggtgttggctagtggaagcttactagaggtttgatggttgtggcccgtggtgacaagttgtctaactttgtatgtatttggggctccgtttcgagagactcaagaatttggtagagaatgatacttatcgaagttatggcatgtaaaatttgagtcatatgagcgagaagaggattgatagtttggctaagaaaaatttgctttctggagtgaaacaagcaaagttgaagaaatgtgttcattgcttagccggtaaacataaagagtttcttttgaaatcatccgccttcaagaaagcttgatttgcttggagttggtacattcccgattttgtggtccttttaaggtaagatcccatagtggtgcaattttactttgtgactttttattgatgatcattctcgcaaactcggggtatttcctttgaagtccaaggatcaagtacttgatgtgttcaagagttttcaggccttggttgaaagacaaacaggaagacattgaaatgcatccgctcgaataatggtggtgagtatattggtcctttttgatagatattgaagagagcggggtattaggcacgaaaactcctccaaaactcgcggttaaatggtttagcaaggaggatgggcagaactctagttgagaggcttagatgtatgctctcggatgctaatttgccattcctttaggcggaagcacttaatctgccgcttatgttatcgatttatctcctttgttgctttagatagatggtgatgtcacagcggagtttgggtggtaagaatgtttcttatgatcatcttagagtctttgggtgtaaagcctttgtacatgtttctaaggatgaaaggtcaaagttggatgttaaaactaggcgaggtatcttcattggttatagtcaagatgaatttggctatcgtttctatgatctgttgagaagaaacttgttagaagccatgatgttgagttctttgaagaccaaacaattgaagattttgacaaaagtgacaaggctgattttcgagtagtgagagcttagttgatgttgatccggttcctttgactattgccgaagaaaatcttcttaatgaagaaaatcaagttgataatgaagatggtgatcatgttctaatgaccggcatgatgttgtttatgctcccaagaagatgatgtggttgtccaacaaccaattatagatgctccggagagttctctcgcacgatctagtagagaattccttcatctcgtgattctcctaatgagtatgtacttgacttacggggagaacccagagtcttgatgaggccatggaaagtgaagaaaaagaaaggtggtttgatgctatggaagatgagattaaatccttgcatgataatcatacctttgatttgttgttacctaaactgaaaaactttttgaaaaaaggtgggttttttcgggtgaaacatgaagatggtaatccggttccaccagacaaagctagattagttgtcaagggatttaatcagaaaagggagttgattttgatgaaatattctctccgattgtgaagatatcatccattcggtgtggttctaggtcagctgcaagtctagatttagaggttgagcaaatggatgttaaaaaccgctttcctccatggtgacttagactaagaaatttatatggagcaaccggaaggttttgaagtcaaggtaaaagagaattatgtttgcaaattaaagaagagcttgtatggtttgaaacaagctcccgtgcaaaggggtacagtgaagtttggttttttatgagtcaaaggggcttcaagaagacttcttaaccattgtgttttgtgcaaagttctctgatggtgacttttattgttgcggttgctttatgttgatgacacgcttgttgtcgggtcataatacttgcagtaggatcaagttgaagcaaggagtcgaggcaagtctttttgcatgaaagacttagaccaaagaaggcagattcttggcatgcagattgcccgtgatagaaaaagccaagaaattggtattatcacaagagaaagtacatttttaaagtacttcaagcagattcaaagatggacaaagctaaggttgtcaagacaccttagctatgccttcaaattgaaagcatggaaatgctgtcctttctagcgatgatggaaaggaagatatgaagaaagttccttatgcttcaaattggtagtttgatgtatgcgatggtttgtacaagaccgatattgctcacgctgttgagttgttaagcgggtttctttctaatccaggaagagaacattggaatctttgtgaagtgggttatgagatatctcatggcacttctagtccgagtttgtttttggcagggaagcctatttttttgatttatcttgattaggacatggttggtgatgttgatactcgcaagtctacttggtgcttggttacttttaggggagtattgtcttggcaatctagattgcaaaatgtgttactctatctctactatggaaggcttattcttttcgtgaagcttgtaaagaattgctttggatgaagagattattaagaacttggtttgtgctcaaagaggtatgtactttattgtgaccggtcaaagtgctatacatcttggcaagaattctacgttccatggtcggttaaacacattgatgtgagataccatttgattcgagatgtattggattctaagttgcttgagcttgaaaaagattcatacaaatgacaatggttccgatatgatgactaaagctttgccaagaggaagtttgaagattgttgcatggtcgtggggacgggcggtcctccacatagtcgtgagggagaattgttgggttatgggtcttttttccttctatgtggataaataaaagcccaatttggaccaacctatttttgcctataagcccattcttatgaggcaaatataaactgattttagggtctgattttcagaacatatagagagttcttcagcagccaaaaagagagaaagagagattttcgcaggcaaaattcaaatctaatagccaacttcaaattgcgattcccgcttcgtttcttatccgattgagttgatttttggacagcatattgtattcatctcaatatttgattaggaactgacagagttggatttggtggcctgcagcttcagttttattgtgaggaattagctgcaaaattggtgattttgctcctttaattttctagatttggtgcaatcttattttgttttgttgctcattgtttggcacttgttttggccaattttggagaacaatattgtaactcttggtgattatagtggagcttttggtcccgtggttttactcttcacatcgaagggttttccacgtaaatcgtggtgtcttgtgtgattggtttcatattgtctcgttatatttgtttggttgaattacctgctgccttagtatcatattgcttgtggttgtttgtcttctcttggttcaaatcgaaaaagggaaagtatagacttgggtattcttccgctgttatcctgtcaggcattcttggtagtgccttgtctttcccaacacatctcaactatctgaatgtctcttacaatgagttatcaggtgaaataccagatggagggccttttggtaattttcacagctgaatcattcatcggcaatgaagagttatgtggaccgcctagattccaagtcaagatttgtgaaatccgaacaacgtgacaagaagaaacaggaaaaaacaagactaaaatttgttcttggaccagtgcagctggaggtttagtcatggggttttaggcatgatatggttgttgaattatcggagacgtaacaaccaacttattcctttaactgattagtatgatcggttatcacacaaaaagttttcttactatgaacttgtttgagggactaacaactttgactttaatcaaatttgattggaaagggaagccttggtatggtttataaggggacatttacaaatgggactatagccaactgtaaaggttttcaatgctggcgcaagatgcattcaagaggtttgatttggagtgtaaggttttgcgtaacaccgaaataggaatcttgttgggtgataagtagttgttcaaatcttgattttaaggcattggtgtttgagtacatgcctaatggagatcttaattattggctttactcacacaacaatttcttggatttaaacaaaatttgaaaattatgtttgatgtggctttgtgtcagagagtatctacaccaaggccattcaaaacatagtggtccatcatgacttgaacatacttttggatgaagacatggttgccgagtaagtgattttggtatattcaaactcttgaccgccagatgatccaaagggcattgacaaagactttaggcaccattatcctggcactgtgcccgatcaaatttttatttactaattactttcttcaacttgtattcgatatgcatatatgatgtatttcattttaatggtagagtacgggtcagaagggatagtgtcaactatgggggatgtttacagctacggcattttatttatggaaaccttcataagaaagaaatgatagatgatgagtttgttggagaccttacattgaagagatgggtcatggaatcatatcctcatagagtcattgttatgaaataaaaacgaatacaagttgaacgtcaattatgagtcatttatctaatatgatccattaacaattgattaatgtaacgcaggaagaagaaaacaatttgcattgttatgaatgaatgtgtttgtactacaatatatacaaagatcgacaagtctagcaaactttctaaccaacttattctaaccaactctactcattattcatttagctcacttaatcaagaaattagacctaacaactaactaccattaactcattcaactgattgttgggttataggtctttttcccttcctatgtggataaataaaagcccaatttggaccaacccatttttgcccataggcccattcttatgaggcaaatataagcctatttagggtcttattttcagacaaaacagatcagtttttcagcagccaaaaagagagaaagagagattttcgcaggcaaaaatttagatctaatagctaacttcaaattgcgattttcacttcgtttcttatccgattgagctgatttttggacagcatattgtcttcatctaaatatttgactaggaactgacagagttggatttggtggcctgtagcttcagttttgctgtcgtgaacagtagctgcgaaattggtgattttgctccctttaattctctagatttggtgcaatcttattttgttgttgctcattgtttggcacttgttttgtggccaattttggagaacaatattgtaactctttggtgattatagtggagctgttggtccgtggtttttactcttcacatcaagagttttccacgaaatcttggtgtctttgtgattggtttcacattgtcttgttatatttgtttggttaaattacttgccgccttactatcatattgcttgtggttgtttgtcttctcttggttcaaatcgaaaagagaagtatagacttggatattcttcatttgttatcccgtcgagcatcatttgttattgccttgtcttttcccaacaaagtggtatgtcaggagcattggttattgttgattgtcgttttgaatgatggaggcaaatatgagcaaaatggtgtgtttaaatggtagtaactatcatatttggaaaggcaagatgaaagatctttatttgtcgaagatgaatttacatgtttgcttctaataagcctaagtctttgaatgatgaagaattggaatttgagcatcctgggtttcggctatattagacaatgggttgaagataatgttagaaatcatattgtgaatgaaacacatgccaaagtttgtgggacaagctcgagacactttatcttgaagacggcaacaaacaagttgttctattgaaacaattaatgaatatcggtataaagagggcactctatttctacgatcatattaatgattttcagggtgttcttgaccagcctgtccggaatgggtgtaaagtttgatgatgagatcacaggggactttggcttcttaatactcatccggactcttgggaaacttcttctagtttctttgactaattgctcccggtggtgttgtaaccatggaatatactaagagtggtgtcttgaatgaagaaaatgagaagaagatcttgcctcatcttcttaaacttcactccgatgttttggttcttgaagatggggagaaacaagtcagtagatcgaatgatagaggtaaaagtagaagcaagtcaaagtctaaatacaagaatattacttgtgactattgccacaagaatgggcatatcatgaaatattgttacaagcacaagagatatgagacaacaaaacaagagaaggcgataatgaaaatcgtggttgctgttgttgctaatgatgatcttcttttttcttgtgatgcaaatgccattaatcttgttcatgatgagtctatttggtttgtggattcggtgctacttctcatgtcacgccaaagaaggaattattttcttcttatactccgggtaattttgaaacgttgaaaatgggcaataatcatgaagttgaagttattggcattgggacgttttgtttggaaagtaacaatggttcaaaactagttctcaataatgtcaagcacacccaaatgttcgcttgaatttgatttccgtgggatatcttgacgatgagggttatgttaatacacttggtgttggcggtggaagctcactagaggtttgatggttgtggcccgtggtgacaagttgtctaacttgtatgtatttaggggctccatatccggagactccaagaatttggtggagaatgatacttcatcgagttatggcatgaaggtcgagtcatagagaaggggattgatagtttggctaagaaaaattttctttctggattgaaacaagcaaagttgaagaaatgtgttcattgcttagcgggtaaatagaaaagagtttttttttagtcatccgccttcaagaaagcttgatttctttggagttggtacattccgattttgtgtggtcctttaaggtaagatctcatggtggtgcactttactttgtgacttttattgatgatcattctcgcaaactctaggtatttcctttgaagtccaatgatcaagtacttgatgtgttcaagagttttcgtgccttggtttaaagacaagcagtggaagacattgaaatgcatccattaagataatggtggtgagtatattggtccttttgatagatatttgcagagcggggtattaggcatgaaaaacctccaaagactccctcggttaaatggtttagaagcagaggatgagcgagaactctagttgagagggttagatgtatgcttttagatgttgtcgtcgattccttttgggcggaagcacttaacatcgctgcttatgttatcaatttatctccgttgctttagatggtgatgtcctcgatgtagtttggatcgtaagaatgtttttacatcatcttgtagtctttgggtgtaaagcctttgtacatgttcctaaggatgaaaggtcaaagttggatgttaaaactaggcaaagatatcttcattggatatggtcaagatgaatttggctatcgctttctatgatcccgttgagaagaaaacttgttagaagtcgtggatgttatgttcttttgaagaccaaacaattgaagattttgacaaactgacaaggctgattttgagagtagtgagagcttagttgatgttgatccggttcctttgactatcaacttgggaagaaaattttcataatgatgaaaatcaagttgataatgaagatggtgatcatgttcagtaatgacctatgacgatgacgctttttgatgctcgatgcagaagatgacgggttgtccaacaaccaattatagattctccgagagttctctcagacgcatctagtagagagagatttcttcatctcgttattctcccaatgagtatgtactcttggtgacggggagaacccgagagtcttatgaagccatggaaagtgaagaaaaagaaaggtggtttgatgctatggaagatgagattaaatccttgcatgataatcatacctttgatttggttaagttacctaaaagcgtaaaaagctttgaaaaaaaagggttttttttgttgaaacatgaagatggtaatcaagttccacggtataaaagtagttgtcaagggatttaatcggaaaagggagttgattttgatgagatattctctccgggttgtgaagatgtcatccattcgtgtggttctaggcttggtacgcaagtctagatttaagttgagcaaatggatgttaaaccgcttcccatggtgacttagatgaagaaatttatatggagcaaccggaaggttttgaagtcaagggtaaagagaattatgtttgcaaattgaagaagagcttgtacgggtttggaaacaagctcccaaagcaaattggtacagaagttttggttctttatgctggggaaaggcttcaagaagacttcttcagaccattgtgtttttgtgcaaaagttctctgatggtgactttattattgtgttgcttttatgttgatgacatgcttgttgttgggtcataatacttgcggggattcagaagttgaagcaagagttgagtaagtctttctttatgaaagacttaggaccaaagaagacagattcttggcatgcagattgtccgtgtgatagaaaggctaaaaattggtattatcacaagagaagtacattcagaaagtacttccacagtattcaagatggacaaagctaaaggttgtcagtgacacacttttagctatgcacttcaaattgagcactagcttaggtgtccttctagtgacagatgagaaggaagatatgaagaaagttcttatgcctagctgggttggtagtttgatgtcacgatggttttgtacaagaccggatgttgctccatatttggggttattaaccgttttcttttctaatcgggaagagagaacattggaatctttgtagtgggttatgagatatctttgtggcacttctagtaaagtttgtgttttagtgcagaagcctattctttgtggttatccggattcggacatggctggtgatgttgatactacgcaagtctacttgatgcttaattcttttttgtggggagctgtgtcttggcaatctaggttgcaaaatgtgttgctctatctactctctgctggaggcttattctttatcgttgaagcttgtaaaattactttggatgaaagattaacacgggaacttggttgtgctcaagagaggtatgtgctttattgtggtcaaaagtgctatacatcttggcaagaattccacgttcaatagtcggtctaaacacgttgatgtgagataccattggattcgagatgtgttggattctaagttgcttgagcttgaaaagattcatacaaatgacaatggttacgatatgatgactaaagctttgccaagagggaagtttcaagattgttgcatggtgcttgggatggcgggcctccacatagtcgtgaggggggagaattgttgggttataggtcttttttccttcctatgtgataataaaaagcccaatttgaccaacccatttttgctcatagcccattcttatgaggcaaatataagccttatttaggatcttatttcggaaaatgacagttagttttttggtgagccaaaatagagaaagagagattttcgcaggcaaaaattcagatctaataaccaactttaaattgtgattcccgcttcgtttcttatccgattgagctgatttttggtcagaatattgtcttcatctcaatctttgactaggaaccgacagagttggatttggtggttcggtaacttcagttttctttgcgaatgagcgatggctaaattggtgattttgctcctttaattctctagatttggtgcaatctttttgttgttgtcgttgtttgacacttgttttgtggccaattttggagaacaatattgtaactcttggtgattactggtgggagcttttggtcctgtggttttttactcttcacatcgggccgattttccgtaaatcttgatgtcttgtgtgattggtttcacattgtcttgttatatttgtttggttgaattcttgctgccttactatcatattgcttgtggttgtttcttctcttggttcaaatcaaaaggaagtatacttgggtattcttccatcgttatcctgtcgaggcattcttatttgtgccttgtctttcctaacactgatcacggaacatcaacacattttgttgatttctttcacacacacctcctcaaaaaaccctcttttttaacatgtaagcgacaatatcttttttaggagagtgttcaacattgagcataaaaataataaaatagagaacaaaaaaagatgagtataaaataataaataataatataagatcgattttaccgattgtcaattttgtgtatgaactaaagaaataacagcttcacatatgaatttgtattttaggctgctgtaagtactaaaaatagttattcaaccagtagaagagatgaaggtgggggccagctgttggcaatcaataagggaaagaaaagacaaggaatattgagccaattttttttcttctgtggaaaactttggcagagaaattaaggctaacgaaaagtctttgtgcaatgaccccatgggcatgtgcagttgtttcccacaactttgtgaattatattccaaaaaatacaaattcattatttaatactccaacaactttttgattccactctagactaccatcacatatctaatattaaatgtaatactgaatttcacatatggtcagaggcgaatccatcagcacctgatatattctttttttaaaaaaattatatctatatatacagattgttgataagacggtaatatatttaattgtgcactcttataacgaacaaatgatttgacttgtccattggaaaaacaaaaagtgtcacataaattgagacatggcgaataatatttctttcctaaatttttcgtgtgaagtcaaattaattcatataaaattagacgaaaggagtaatgtttaatagtaattgcatatggtagtaaatttgatagacgtggtcccgtgggagtgtgtgttatttccattgaataattgagtttgtaattgttacaagtccattctaatttccaacaccttacttcatttcaaaaatatactctatggctgaagctttccttcaaattatgttagagaatctgacttgtttcatccaaggggaacttggattgattcttggttttaaggatgagttcgaaaagcttcaaagcacgtttactacaatccaagctgtggtacaagatgctcagttgaagcaattgaaggacaaggcaattgaaaattggttgcagaaactcaatggtgctgcatatgaagctgatgacatcttggacgaatgtaaaactgaggcaccaattatacagaagaagaataaatatgggtgttatcatccaaacgttatcactttccgtcgcaagattgggaaaaggatgaaaaagattatggagaaactagatgcaattgcagcggaacgaattaagtttcatttggatgaaaggactatagagagacaagttgctacacgccaaacaggtaaatatttttctaaataacagctttatatcatcaaattcatgtgtgttttggggattttgtctaagtagataagtggttcaaaatctattatctaaatctgtttggtgaagtctttaacatatatataaatccatagcttactcatatgccccaaagtctaaatgacaggataaagccagagttgttttagatcttataaattaacaatgataataatgtgaattcaaaatagtgcatttgttttatatttgaaatatgtctgctgcttctgatcaagctgatcattgtcttttgcaaaattcttctttgttttttttgctgactcttaccgatcttggaccaggttttgttttaaatgaaccacaagtttatggaagagacaaagataaggatgagatagtgaaaatcctgataaacaatgcccaaacactttcagtcctcccaatacttggtatggggggactaggaaagacgacccttgcccaaatggtcttcaatgatcagagagtaattgaacatttccatcccaaaatatggatttgtgtctcggaagattttaatgaaaagaggttgataaagaaaattgtagaatctattgaagaaaagtcacttggtgacatggacttggctccacttcaaaagaagcttcaggacttgctgaatggaaaaaaatatttgcttgtcttagatgatgtttggaatgaagatcaagataagtgggctaagttaagacaagtcttgaaggctggagcaagtggtgcttatgttctaaccactacccgtcttgaaaaggttggatcaatcatggggacattgcaaccatatgaattgtcaaatttgtctcaagaagattgttggttgttgttcatgcaatgtgcatttgggcaccaagaagaaatgaatcttaatctagtggctatcggaaaggtgattgtgaaaaaatgtggtggtgtgcctctagcagctaaaactcttggaggtattttgcgcttcaagagagaagaaagacagtgggaacatgtgagagatagtgagatttggaatttacctcaagatgaaagttctattctgcctgccctgagacttagttaccatcaccttccacttgatttgagacaatgcttttcatattgtgcagtattcccaaaggataccaaaatggaaaaggaaaatctaatctctctctggatggcacatggttttcttttatcaaaaggaaacttggagctagaggatgtaggtaatgaagtatggaatgaattatacttgaggtcttttttccaagagattgaagttcaatatgatcgaacttatttcaagatgcatgatctcattcatgatttggcaacatctctattttcagcaagcacatcaagcagcaatatccgagaaataaatgtagaaggttacctacatatgatgtcgattggttttataaaagtggtgtcttcttactctcctcctcacttgcaaaagtttgtctcattgagggttcttaatctaagttccatgggacttaagcagttaccgtcctccattggagatctagtacatttaagatacttgaacctctctctcaataacatgcgtactcttccaaagcagttatgcaagcttcaaaatctgcagactcttaatgtagagtattgctggtcactttgttgttttccaaaagaaacaagtaaacttggtagtctccgaaatctcttacttgatggttgcgatggattggattctatgccaccaaggataggatctttgacatgccttaagactctaagtttatttgttattattagagaaaagattctctacttggtgaattacttaaacctgaatctgtatgggtcaattgaaatcacgatcttgagagagtgaagaatgatagggatgcaaaagaagccaatttatctgcaaaaaagaaaatctgcattctttaagcatgagatgggaaggaccacatagatatgaatcagaagaagttgaagtgcttgaatccctcaaaccacactccaatgtgacttgtttaacaatcactggcttcagaggaatccgtctcccagagtggatgaatcactcagttttgaaaaatgttgtctctattgcaattagaggttgtgaaaactgctcatgcttaccaccgtttggtgatctgccttgtctagaaagtctagagttacggagtgggtctgcggaagtggagtatgttgaagattctggattcccaacaagaagaaggtttccatctatgagaaaacttactatagaaaattttgataatctgaaaggattgctgaaagaggcaggagaagagcaattccccgtgcttgaagagttgacaattagatgttgtcctgtgtttgttattccgaccctttcttctgtcaagaaattggtagttcatgggaacaagtcagatgcaatagttttgaggtccatatataatcttagggctcttacttccctcaacattagccataacttcacagctacttcgctcccagaagagatgttcaaaagccttgcaaatctcaaatacttggaaatcgctttcatctccaatctcaaagagctgccaaacagcctggctagtctcaatgctttgaagcatctgtttattaattgttgttttgcactagagagtctccccgaggaagcggtgaaaggtttaacttcactcacacagttatccataacatactgtaagaggctaaaatgtttaccagagggattgcagcaactaacaaatttatcagttaggtattgtccaacactggccaagcgatgtgagaagggaataggacaagactggtacaaaattgctcacattcctcatctgctgattactgattagatgtaattttctgatttttcttttggaaacaaatcaactatttataacatctatttgtattatacttgatttttcttgattatgtaacaataaatatttgaaatttttcatattaaagattcagaatgagttttacagctaactctatattctcacagtttaataacgtaaatatgatatttatatcaaattattacttatgttgtgatttgatttatcaacatgttggagatgattttgacagtttattaaagaatttctaagtttttattgtttgcacaagtaacaagccataaattaagtttcgagataaaagtaatttgtgtatcatggcttaattagtcggaatttcaagttttttctcaagttatatatatggcaatttgtaaaaaatagatagtattcattttgatttaattcaagtatttttaaaaatatatacaaataatatgggggatacacacgctaaacgcgtacccaaaaattagtatataaagaataatgacgaaaaaataaaatgaagttctatcaccaactatctctacatcttttgctgatatatatatatatatatatatatatatatatatatatatatatatatatatatatatatatatatatatatatatatatatatatatatatatatatatatatatatatatatatatatatatatatatatctaactagtgtacttattcggacttgacatggtataaaaagatattaaatatattttaaataattaataaatgatataataaaaagagaaatacaaaataagttatgattctgataaaaggaaacttacataaatgtgttataataaaaaaatatttaccatttatagctataattttttttttcactcgatcacttttaattaatttataatacaagtttaatatatattacaaagaacaatttattattcacatacaatacaagttttaatgatggattttatcacacattttaatacacttataatataatgttactattttttaccaaacaaacacaatatatttcaaaaacaattataattcaaatatattgcataaataattcacttttaataaatattacagatttatcacaatattgctataaatgataataaacaaaagtatcgctaaaatcagtaattattttttaacatatattaattcatgtaatttttcttattatctattcagaaaaattgcttaaaaaatctcatttgacattttcaatttaaaattgttgataaaaaagacaaaaacataaaaattgatatgaaagagctttggttaagtagcaatctaattacatagtggcatactaaattaaatgattcttatagcaatattattggttcaaccaacaaaactaaatctctagttatattacttaattgctcatcatagctatagtttgttataatcatcactcgcggttaacattatgcatcaattacgtgggctgacttcgattttgtataattagtcatgtttttatatgtactagattctgagaacatgccttgcacgtttgtcctttattattattaactttttatatactaaaaagttaagtaattaaaaagatgcttaaataaacaataatagtttaaccatttatcttttattcgctaaataataactaatataatatgaagaacattaaatagatgataatatctaccttagtaattggttcttaaaaagcatattaaaaatttaattctcaaagtgtttttacataaatagtggagaatgactcttcacattgagcttttaattttaaaaaattatgtgtatgagaaataattaacattcaataattaggtagaataatatcacattatcataaataaaataatatctctaagtcaaaagtagacattctagtttggaaaataattactactaactatttatgggtccagctccaatcaataatctatagatgggagtttgacaatttttcagctatagttaaaattttacatcaacaataaataacttattatcacagtagatagacgtttgatgcataaaagttataaatgctaaaagattttgtcaatgtagtacatatgcaaacttatgataaaaacacttggtatattacgaaacacacttgaagccattaccatgattaacatatcaattatttttatcattatatcacatatacgtcttctttttaaccttaaaagtattgtacacatgatttatgaagagaaaagaatagtactccttttttcatgtaacgacctgtttagtcgttttgagcagcagaatttatttctggaaaaactgtctgagtcaacggaacccacgacggaccgtcatgggcacgacggaccgtcgatggtgtctcattccaaaacacttagaattttgaaatttgggtctgaaatcgactctccaacttcgtgcttgagatggccggggcgaacaagtaagtggagccgcacggctgcaccgtcacaaatcttccatggggaagtgatccgaatgtgtggatttggcggggagatgccgtccacgatccacgacgggacgtcactgttgcgcgtaatcccggtgggtcggatttctgttaagtgatttaaggggcgttttggactattcctgctttaattataaagttagtgggttaatgttaataagtttaattacttgggggttaaaagaggtaaccttgagttaattagtgggttattattgacatctttatacttaattatattctaattagggtaaaagaaagagggtttgaataagaaacaatagaaagaacaatgagagggaaagagaaacgagaaagagagaaacgaacgaagaggaaaacacaagctttgggaaaattgctttcttgatcaaaattcttcggtggaggtaggttattgtttttatactattcgtagtaaactcttaatagcgaatgatatgtgttgggttgtattgtaaagtcttctatatgcttaattgtatgcttgtataaatgtgattatataattgtgataaaataagcaagataaagctattgaatcccaaatcttgaaaaccccttgttaatgatgatgccttggtataaaagaaggcttgatgaactaaagtaatgatattgatgatgtcttggtataaaagaaggcttgatgaactaaagtaatggggttgatgatgccttggtataaaagaaggattgatgaattaatagaatgagattagtggagcgggtgtcacgaaccgacacatagtattagggggaccgggtgtcacgaaccgacacgtagtattagggggaccgagtgtcacgaaccgacacatagaattaggggatcgggtgtcacgaaccgacacgtagaattaggggatcgggtgtcacgaacccacatgtataattggggatcgggtgtccgaaccgacacgtgggaattaggagatcggtgtcacgtgcggacaaatagtagtaggggcgggtgtcacataccaaaccaagaggaataaagataatgaatcttgaaagatgttaatatactcaatctaatgaacctaatcccaaataggtatggtattgaggcttgagtctcatgtgaacttggcggtgcttattaatgattatagtacttgttgttgttacacatattgagtattgtagttgatttatgatattatcagtatatcttttgttttctattttgagttggccgatgatacctacctcgatgcccgtgttttatcttgaccctacttgtatttgttttctttgttatttgtggagtgtagcaagcgtaccgtcgtcttcaactcattgccaactctgtgatcttcattacaccggattttagggtgagctaatgcttctagcttggactggatcttcttcctcatgtcttgatgccttgaagttccggcatggactagattttgtttattttagcttctttagaatactcttagtttagtaatttgatcatagatgttcttgtggtgatgacgggattttggggaatactagttgttgaattttagaagttattgaattggttttattaatgagtttaagtcttcatattacttctgttgatattatattgaaatgttggggtttagattggttggttcgctaacataggatggtaagtgtgggtgcgttggctcggttttgggtcgtgacaaacttggtatcgagcattaggttcgttggtctcatcacacaagagaaccagtctagtagagtcttaaggagcgtagggggggccttttacttttctttgagaggctataagactttaggaaattttcctttcttttctttttctttattacttggatccaattggtatctaggtgatacaaattggtaatcgaccatcttcactctatttttcgcaaatggttagaacaaaagcgacgactaacaacagcaccgatagcgcgggcggagcgaggtgcgtcccgggcgtgctggggagtacatggctgggaaggcggctgacagaggccgtggtgaaattaggtggggagacgtctacaggggacaaacaccgccccatagtactgggcggtgactcactccacccggtaggtggtaagagagggtgaggaaggaggcccggcaagtgcgaggagatgaggaactaccgctgacctacccggagatgataaatcaggttctgcttaccttagtaggttgctctgatcaaggtcaaacacctcgatgtttctgctgcttctctcgggttttggaaatacgacgggcaaaatctgtttcacgcatggatatgccattggaagcgaaactatttcctcgtttgactacggggcctatgatgacaagcggtgacaaagatgaaccaagaagggattgaaattgaaacctccgtcttcaagggtgctaaccgggatgcctacgattttccgtcgattgtcatgagttaccaagataaaatgggcatagtggaacgattcggtgttgagtttttggacttatcagtttcaaaggaacgccaaatgcgcggcggtcacatgttgagtgtcaaccaacggaggaaccacctatgacttggccattctctagcttatttatggaagtatatcccctgaccttgagggataggaggagatgagttttttggcttagagcaagtagaacgacggtcacttcatatgaaggctaagtttcgtgcattatctaggtatgtcactttgcgcccgggttcacaagaagcggattcaaaccgttttgtgaaaggggttgaggtcagttttcagcccttttgtagcggtggcaaaatgaaatccttccagaaagtggtagacttctgtgatagaggtggaggagtaaagtaggatgacttcaccatggcatcgacatcaaaaaggtttgaaaagggagaggtttaatggttcttacactacagggcgagagttcgaggattttcggtgggccgttgtctgctcaggaggctgtggtggggtccgctaccggaccgtgacatttctgcgggagtagggtcattccagacctcaatcattctcacaaatactatactgggctccagagaatgttatggatgtgggaggctggaccataatgggaagttatgacgaggtcccatgggccaggccagctaggtggggtggtggtaggagaggcagttgataaggaggccagtggccaggtaatgggtgagtcctgaaggcagccaggagtgaggacaagtgaactacaaccttaccacatggtgagggcagccgaggcagcaggcaaattagtaggggctacggctgtgcagcctcgcagtctggcggggacatcagatgttgttatcaccggtaatcttttggtttgtgattgcatggctacgtcattatcggatcctgatccacatttcatatgtatcttcctatttgttactggtgtaatttacattgtgaattgcttgacatgctatttgtgtttctactccgttggtgagtcatgatagttgaaaaggtatataggtcttgtccgtgacttttgtggggagcacactcatgtagatttggttattttagaaatggttgatttctgatgtaattacgggtatgacttgctttccaaattttgcaatcttagattgtaatgctaaaagcgtaacgttggccaagccagggacatccagattagtaatgggagtgtgactacacttccgctccagataaatatcatatcctttttcgtgctaagagaatggttagtaaagggtgtttagccttcttggcacctcagtgatgatactaagtaccttcgagtgagcctggggtttcggtagttcgtgagttttagacgtgttccctcgcaccttctccggtatgccaccgacgaggatattgacttttgcattgatttgggccgagtactcattcccatttcccccccttatagaatggctcaaacgagttaaggagttaaaagcccaacttcaaaaactgttaggggaagagctttattaggccgagtgcatccccttagggtgctttgtttttgtttgtgaagaagaagatgggagtcttcggatgtgcatagattactggcaactaaataaagtaactgttaagaacaggtaccctcttccctcgcattgatgacttgaccgatcgatttctaaggtgctatgtcttctctaagattgacttgagatggttatcatcaattgaaaatccaggcgtgagatatgccaaggcccttttcgaagacggtatgggcattatgaattcttggtaatgtcctttggactaacaaaatgcccctgctactttctgcgagcttgatgagcattttttaagccatatctatggatctctttagatcgtatttattgatgatatcttgatatactcaagagaaagaaggaacatgaggagcatttgagagttgtgttggaaatgttgaggagaaaaagctttatgccaaattctccaagtatgagttttggctagattgattgtccttcttgaggcaacgtagtttctaagggaggagtgatgtagatccttctaagatcaagtagttagaagaattgggtaagacctactaatatgtcgtaaataagaagctttgttggtttaaccattctaccgtcgatttgtcaagggattctcttccattgcttcccaattcgaacttaactaagcagaatgttccatttgtatggtcggatgaatgtgaggaaatctttcgtaaactcaagaccttgtttgacttcaccgcacctatccttacctttccaaagagagagggtaagaacttcattgtgtattgtgatgcatcatattctggttcgcaaaaaaaaaaaaaaaagtgctaatgcaagagaagaacgtaattgtgtatgcttcgaggcaattaaaggtgcatgaacgtaattatccaacccacgtatttggagttggtcatggatagtgtttgcattaaacaatggagacactatctatatggggggttaagtgaagtctatcacggatcatcgtagcctacagtatgtctttaccggaaagatttgaatttgagacggagggaggtggatggaactaatgcgaaggattatgatgtttaccatcttgtatcacccagaaaggctaatcttgtggcggtataggtagaaaaagcaggagcatggtagtttagctcacttgcaagcttctaggcgcccattggcctagagaggtgagactacggctaataactttatgagattggaagtaaaaaatgagaagggagtgattttttggcggtgtggaggcgtagatattcttttcttgacaagatcaaaggaaaaacagtttttaatgatgagaaattgatccgaattagggatatggtgttatgagggagagtctaaaaaagcaacaatcgatgaggaaggtgttttgagaatcaagggaagggtgatgtgtaccctgcgttgatgacttgatcaacactattatgagaggctcatagttcaaggtattttatacacctggtgcaaccaagatgtatcgtgacctaaagcaacacttttggtggagtagaatggtagcgacattgttgattttgttgccaaatgtccaaattgtcaacaagtaaagtatgaacaccggaggcaggaggaacactttcagagaatgcccattctgaatggaaatgggagaaattgcaatggatttcgtggttggtcttccaaagacaatgggtaaatgactctatttgggtgattgttgataggttaactaagtctgctcatttcattcgtcaaggtgacttacaatgctgagaaattagccaaactttacatccagtagattgttaggttcatggagttccactctccatcatatcggataaattaccagtttactttaagttttggagaacattgcatgcggaattaggtactaggttgaaccttagtgcgcatttcacccctcgagacgatggagatgatcggcgagcgattcaagtgttggaggatatgccgtgcatgtgtgatagaatttggtggccatgggatagcttcttacccttagcggagttttcatacaataatagctatcactcaagtattgacatggccccatttgaagcattgtatggtaggagatataggtctcccattgggtggtttgatgcatttgaggttagaccttgggggtcttgaccttttgaggttattagaggcggtgaaatctattcagaaaagcttttaagcggtaaagtaggcaaaaataatgtccggatcgaaggttagagacttaaggtttatggagggtgagcaagtcttctttgaaggttttcgccaaagaaaggggtgatgcggtttggtaaagaggtaagctaagcccaaggtatattggaccatttgaagtacttagcgaataggggaggtggcttatgaattagccttgcctcggggttgtcagagtgcatccggtatttcatgtgtctatgttgaaaagttaccatggggatggaaacacatcatcgttgggattgatctggctttgatgagaatttgtcccataagtatgagcctttgtgccattctagatagagaaattcgcaagttaagatcaagtgagattgcatccatcaaagttcaatggaagaatcgacccgattgaagaggccacttggggagaaggaagtcgatgtgcaaagaaagatacccacaacctacttacgtattcgtgtactcccgcttttttttttggcgtgatcgttcgaggacgaacgatgggtaaattggtatctattgtaacgactgcttagtcgcttttgagtattgattttatttccccgaaaaactgaagtcatcggaacccacgacggaccgtcacgggcacacgacggaccgagggtgtctcattccaaaacacttagaattctggaatttgggtaccgaatcgactctctcgaacttcgtaacgatggcgacggaccgtcgtgagcggcggaccgtcacacatcttccataggaattgagtctacgaacttctgtgtgacggcggcggagacggaccgtcgcagtacccgtcactgcaatcccgtaatcccagctggccggtcacattaagtgatttaaggggcgttttggactattccctttaattataaagttagtgggttaatgttaataagtctaattactgagggttaaaaagaggtaaccttgagttaatttgggttattattgacatctttatacttaattatattctaattagggtaaaagaaagagggtttgaataagaaacaatagaaaagagcgagaggaagagaatgagaaagagagaaaacaagcgagcgaaaaaacacaagatttgaaattgctttttgcttgatcaaaattcttgattggaggtaggttattgtttttatactattattagtaaactcttaatagcgaatgatatgtgttgggttgtattgtaaagtcttctatatgcttaattgtatgcttgtatgaatgtgattatataattgtgataaaataagcaagataaagctattgaatcccaaatcttgaaaaccccttgttaatgatgatgccttggtataaaagaaggcttgatgaactaaagtaatgagattgatgatgccttggtataaaaaaagggttgatgatgccttggtataaaagaaggattgatgaattaatagaatgagattagtggagcgggtgtcacgaaccgacacgtagtattagggggaccgggtgtcacgaaccgacacgtagtattagggggaccgggtgtcatgaaccgacacatagaattaggggatcgggtgtcacgaaccgacacgtgggaattggggggatcgggtgtcacgaaccggccacgtataattgggggatcgggtgtcaccgaaccgagccgcgtagaattaggggatcggagtgtcacgcatcgaccacatagtagtaggggagcgggtgtcgtcgcaccgacacaagaggaataaagataatgaatcttgaaagatgttaatatactcaatctaatgaacctaatcccaaatgagtatggtattgaggcttgagtccgcatgtgtgaacttggcggtacttattaatgattatagtacttgttgttgttacatgttgagtattgtagttgatttatgatattatctgatatatatactattttctattttgagttggccgatgatacctactcagtacccgtgttttgtactgacccctacttgtatttgttttctttgttatttgtggagtgtagcaaacgtaccgtcgtcttcaactcaaccgcaactctagccagtcttcattacaccggattttagggtgagctaatgcttctagcttggactggatcttcttcctcatgtcttgatgccttgaagttccggcatggactagattttgtttattttagcttcttagaatactcttagtttagtaatttgatcatagatgttcttgtggtgatgacttccagattttggggaatattagttgttgaattttagaagctattgaattggtttttattaatgagtttatgtcttccgcattacttctgttgatattatattgaaatgttaaggtttagattggttggttcgctcacataggagggtaagtgtgggtgccagtcgcggctcggttttgggtcgtgacatttcataacattactctttgaataattaatataaattgagcaatataaacttttcaaaatgacttattctagatatatgatcaatttgaggaatgaatgttccaacaaacatataatagactaataagatcaataaattatacatataaacgaaaagtttaaataaaaatacaacctcaaaatcacatatatactacatagaatatgattcattctttatctccaattaggtgggtcatttttattttagttcatatatatatgtgtgtgtgtgtgtgtgtgcgtgtgtgtgtgtgtgtggcgtcttggcgtcttggcgtgtcttggtgtgttaatgtgcgtgtgcgtgtgtgtgtgtgtgtatgaatttcatcagtaattaagatacatagtagaacatgaattgtatattactattttcttcatgtaggatacaaaatattctaataaaaaaatctaagaaagtacatcaacatatataaaaaggaaatatataatacttaggacggacaaaaggagcggataaaaacaaaaaataattactacacatacaaaatgatttgcaaagttcatttttgcatgataatctctcatcctcttcttgtcatatacatgaagatcatgctagataatttatagaagtagctatgatgacctttgaatagataattaatttgcattaaattagttcaatggttttagtccatatcaaatttgtttaatggaaaaaattttcaaatactcctgattttcacaatagagtaattaattattaatgtgaatttgatacatgcatcaatctaaatgagttatttatcaaaaataaaatgaaatagagtagactaaaaataataaaatagctaatgaattctaaaacttttaaataacaaaaattaaagaaagaaatagttctagtttataagaatagtggaacttcctcaataactaacaaaaacataaacaaatctatatcttttttattgcatatgttatgaacaattacattcatcaacaattatccatcaataattatacattagaataacaaagcatatgcatcaacaaaaagtaattgtgttgaacaatgtgtcaagtgtaattacatccaccaataattattcataaacaattatacatcggaataactaagtgtgcattaatataaagtgattttgaagataattttttggtatttatagttacaagtttggaattgtaaaagtcatttaaaaattaatgatatacataacgtttatgagaattagattgtttaaagttgagcatatgtaaagtttcttactaaaatctaaatgtgtcatattaagatgtatggtaattcaaaggacatttttgttctttaatgttaattgatattttgaatataatttatcatctttttgttatgaaatacttcatctcttgaactctattttagaataaaagacaaattaaacatttctttaattatttctacctagaaacataatggattaataccatataagtattatttaagtaatattttattaattatttctttaataatatttaaattagtaaaagggtagaatcataatcctattttaaagttaagatcttctcacttataataaaataataataatttacggactagccccgcttgtttacctatattagtcaatacatttttaaaaaaaagtataaatattattaataatattgttttatgtttaaaaattaaaaggagtatatactccttaaaatgagtaaaagaatctatgagattttttatccaaatactttttttttctagatagaataaatgaaataataagttctaaatttaatcaataaaaacataaagttgcagaatataaaaatatttagcaatactgtttttcttcttcaacgctacctcgtctttcgttattaggggtatttatttacaaacatgaaatcacaccatgattttattttcatacaagtagtaaatcatttataaattctaaaaaaacacattaaatataatgcatgctaattttttgtagatttaattatgagaaaaaactaattacatcaattattcaattctcttatccaataacctagagtgttcactacatgataatcaacttgttataacaaacataatctttaaaagaagatttgtacatcagacatgtaaatgaaaaattttcttttcttttttcactgccattattcaagaaaaagtagtcaatttaccttccttcaaccgaaaaattgaatgtaacaaataatgaactaagtaaaaatatgcaacattgaaatgaaaaataatacttaccaaacaacaaataaatgtccatgacgcctttaaccttcttgaagaatgcatcgaatgcactgaaatgattaaattctaattcagatactatattctccaagatttaccgtcaataaattaacaaaacaacatacatattttttctcacacaagtaggtttgttttacctcatgaacgttgagcagactatttgtccaaatgaaaaactctctagaattatttatcacctgtttgcgttgaaaacataaattttcgatgaaaagaataaaacaaaacatgtaatattagttctatctatatacatatatgcctaaaatttattgatcaaaagaaacatgaaaattttgaagaagaatttttgagataaatcaattcacatgctattgtcatgagaagacatcaaaataatgtattttgttggaaaaatcatgtatataattttatcaatggaactcttcaaattctttaacttaaaattaaataaaagatgttttgaaatgtttgaacttcatttgtttgaatgactatttatctttcattatatctttattactttaaagtttattatctaattatttattaaaaatacttttacattttaaaaaatagaaaaaatttaagtgaatggtaaaatggtaatttaactttgaggttaggagcttcccacttataataatatatgatgataattcgccagaataatacagatatatgtataatatacaattatttaaccgatatcatatctgattcctctcttccactctctctcctctctcacccgcctctctcctcccactctcaattttcctttccatatatacaaatacatatgtataatatacaattatctaaacgatatatatatatatatgcaattcatctctctctcactctttgcttcacttgacaactatgacacttaactttggatatgcacaaattgacatttaaaaactggttacagagaaacttaatgctgttgcgtataaagttgatgacttattggatgaacttgaatatgaggcagcaagactctgtttttcagcaaacacatcaagcagcaatatctgagaaattaaacacatatgatgatgtcttcttactcaccgagttattagttatgctaaaatgtttacccgagggattgcagcacctaacaaatctcacaattttttttgataagtgaaagcatagttaaactctcaaatgtagatgataattaagctcttgaagattatcgctgaattaagtgaattcgttattagtttcaaaatgtttagcctccttgggacctgacgaatgatttaaatttcaaacacaaggtcaagctatatttgtaaaattcttatggccaaacaagtcatactgcaacaaattgtaaaaggattattatactccaaaagtaaagatttagaagagatctactcttaacactaactaaaagattattccaattctcaaagcaaatttatattcctttccaaccaaagaggttttccaaatttgctttctagtaattttttttttctgcacgataggaatagatctcatatactccctccgttccatattatgtggtgtagtttaattcaatacggaatataaaaatgaaagaaagacttttaaaatttatagtctaaaatgaataataaaaaattgtatgactataaatcatttcattaagagtaaatgtacaatttaaaataaaattgttacttaatatagtaacgtgtctttttttttggaaactgcctaaaaaaaaaaaaatagtcatataaattgaacacagggagtatctacttacaaagtaaaagttgtgtgtagaagattttggcatataaatcatatcatatatcatcatatcatatattagtaaaagcatgaattaaaaaaagtcaaaaagttaaattacgattttatcccttctattaattaacttgttataaaatatttaaatatttgattgtacaagtttaattaaaatgttaaatgaattttaaacttcctaatattaatttctaattaaatatctaatttattaatatttatcatttataatccatatgtatataataattataattttttaataaaagtctaatcaaaatattaatgacttttagacttcctaacactaattcctaattaaatatctaatttattaatatttttatcatctataatctctctatatataataattttacaaaaattaataaaaagtctctacgtaaatttttatacttttcttattctcataacttttaccctaaataacaaaatttaataattttaagggtgcaaatcttcaaaatggagacacacacattgataatgtcctcttaattattattaaagaatgactctagcttcacaaatttaaattcattaatgcttaattacttagagaaaagtagatgaagactcttaattttgatagtatatggaaggattgtgtactaattttgtacttattttttcatctacatatacatagtcttataaaaatgatgtctacattgtattttttcttaatctgtttctttttgtctttttcccccaattagacttcttaatttagttttctacaaatgttttattgtcgtaagtctctttacttattttgtaattgtagcattttattattcattataatttgcatatatgtatttccatgaaatattagtaattctatcatatctataaaaattcacatgaaatacacgtgctcagaaactagtaaggaaaacaacacaaatatacatccgaactatcgtaaaaatgatatgcagataccatcctcatacttttgggacattgctgtccattacgtcaaaaaaatatagcatatatattaacggacatcacgtgtcataatcatatcaattgatccaacatttaataaatattcgatcgacgaatagattgtgtcacatgtccctatttagtcatatgttaaagtgaatgacatatatgctctagttttgaaactttcttgtaaaatttaagtatatgccctaaatttttaacaatattttgctacattttacgttttttccattcacgtattttcttatttactaaacaagtttctatcgtcctcagagtatttccttaattagcactaaatgttgtgatgtttttcttcaactaagtttcattgaaggattgagattaaacctatttcggtatccacgatctttgaatgaatcgccaaactctatctatgaatttaatagcaaaagctcagattttgttccaaattgagatataatatttctataaagaaatttaaattaatgatgtgatataatgataatgaattcagtttttacattagaaagactctatttttctctcttacttcacaacaatgcaagaattcttaaagacctaaaaatggggtaggggtgggggaagggggccaacaacaacaagattctaaattcttgaatatttttaactaaaaaattaattcttttcccaatggattcaaattgaaaaggaaaactacaactttgtgattatcgcgctttcaaaatgttgaatagattgtcttcaggtgtgagaagaatgagagtgagatggagaaccatacgaataaagaaattctcaagtacgattccaatggaaggaattgaactacctattttgatcggagataacaagtcattcgatagagagattttgaaactgcatatgtttcctaaatgaaagttatatattagctagatagggatatagatgggttgaattctcaaaatctaagaataattttggatatgtctaaagtgattggaaagtgaatatatttaggacaaattacatgattcgatatacttcactattatatatattatttttacatatacttttaaaacactagtttctggacacgtgcattgaacgtgtatctcaaatatatgaaatagatatttttgaaattgtaagacaattctaaaatatggttgtgatgtttagttatgtatgagagcaatttaataaaatatgtatgagacttttttaatttgtttcccatttggtgttccgctagctaattcaaattcatgtgtgacattccactttgaggatacttcctataaagtctttccatcatcaagaattgaattcaaaagattgaatttagaacgaacgaatatttatcaatcaatcaacttatttgatgaaaacatatatgaatttcagtttgcacatattataaaagggcaaacttcatatttcaagggtactacctataaggtctttccattatcaagaattgaattcaaaagattgaatttagaacgaacgaatatttatcaatcaaccaacatattcgatgaaatatatatgaatttcggtctgcacatattttaaaagggcaaacttcaaaatttatcgtatatgccccaaatttttaacaatattttgctagtttttagttttttccattcacgcattttcttatttactaaacaagttcctatcgtcctcagggtattttcttaattcagcactaaatgttgcgatgtttctcttcaacaaagttttcattgaaggactgagattaaacctatttgggtatccatgatctttgaatgaatcgccaaactccatctaagaatttaatagcaaaagctcagattttgttcaaaattgagatataacatttctatatagaaatttaaatcaatgatgtgatataatgataaatatgaattcagtttttacattagaaggattctttttttctctcttatttcacaacaatgctagaattcataaaaacctaaaaatgggaatattatcatattataattaaaagtaaaactctattttagaaatagtggactaaacatctaaactaataattcaatggcctacgttgatgtaagttacgttattttagcaaaattaagaagaaattccttcatttgagggtagaatcataaaaataaaaaatagaaaaatacatatgaaatatcttaccgcaatcatgtgccctctttgtatttttcattactattgtctctccccccaacttgatcaattactttttttaggaaaaataatccacgatgaatgtattcgtcaattttcactgattatgtgaacacaaattattaagttctctcttgaatgaaaacaaaaaaaaaagaaattatttaaagaatcaaaaaaaattaaacgtaaatccccttgcactatttagagaaattttctatgtgaagcatatttcacaattaattgcacatttctctgttctcttcttctcttcttgaataaaaagtcaatacctaaattcccatgataagagtatcaaagaaacatattactggattagggatgaatcatttatgaaattgtgaagtgattttagatactcacagaaaaaaaatcaccaagaatttataaggagtggatgattgtgatttatgatcgaaaaaagatgaaggttaaaattgttgtgactattaatacgaaatatgtcttctttaacaaataaaagtttatttaattttaaatgatacaaataatattgaagtatgtacatgatgaaaatcgtaagaagaaatacaagtatgattgatgaataagttgctataatttattcaccgattctttcttatgtagtacctcgagtttggttgaatttcgaacttgatcaatagttgcaaacaacacttgagatattttaagaagaagaaatataaaaatgtgaagaaacacttcaatttatagctaacaaattgtgttatgaatatgtgttaattgtgtctttttagtaaagctacaacccttcgaaaaaggcattgctcatgagaaagtcacaatactgagaaaaagttacaacttatcaaaaaagacacaatgctttcgaaaactcaaaaccttttgaaaaaatcacaacccttctgaaaagtcacaactcaccgaaaatgtcacaactgtcaatttcaacccttcaaaaagttacaattcatagcaaaaattcacaaaccgtttaatgaaaaaaaactatctatatttaatataatataagtaaataaaataaaaataaattaattgtgtatttttttttaattggggatattatagtaatttaacattcattttgggagttcatgctttttaggtagtgctagtttcgagcacgtgttttgcacgtgtgatccatgtgaattttatagatatgttagaatgactaaaaattaatggcaatatatatgtaaattgtaatgaaaaataaaatgtaacaattacaaatctagtataaagacttacggcaataaaacattcatagaaaactaaattaagaagtctatagagagaaaaaaagacaaaaagaaacagatttaagaaaaatacaatgtagacattattcttataagactgataaatatatagctgaaagaataagtataaaattagtacatataactctctgagttcttcaactcctttcatatcctatcaaaattcaagagtcttcttcatctactttaacaatagaataaaattaatagcctaataatcttggtaggggtttcatgagataaaaagttgaattttatagatagagtagaaggaatatcaaaagatatctttaagtttaagtttagatatttggaagttatgaatatgaaaagattagagttatgaatgttgagagtaaaaaagttgaataagtaattataaaataataataaataagtaaataatatgaaaaagaaaattaaaggtagcaaaccatgtagaaagaacaactaaagttcttatcacgtaattaattttaatttaaatttgttaagctagagtcattctttaataataatcaagaggacattatcaatgtgtgtctccattttgcagatttgcaccttttaaattactaaatttcgttatttatcataaagaataatactttatccacataaattatattattcatgagaggggttaaggaaagttatgagaagaggaaaagtatagcaatttaggtatagactttttaattttattttttttttataattattatatacatatagattatatgataattattaataaattagatatttaattaggaattaatcttagaaagtctaaaagtcattaagattttaattaaataaacaatcaaatatttaaatattttataacatttaatttatagaagagataaaaccgtaattcaactttcaactttttttgttcttgcttttagtaatactagcaattataacaaactcatcagcatcaactcgacctgtatatttcataatcaataatgtcttgtaaatattcatcgatgtgtcgaaacaaagccccccacgtataatacaatcatcttctaattaattgagctcaagcactttgatgaaaaatcgaatggcaggattccacaagtaaatatgcttgtttataccaatcagtataaaactatgactgttaggttgtggagcctgattaatatttgatgtattatttattctctgtaactaaatatactctgaattattaatatataccccaccgccgtggaagtttacccacgggggtgttaccacgaaatattggtttctctctttctagatctctctagatctctcatctctctcaaaagtttttgtgttcttcattcatcaagtgtgtgtggattcgatcctaacaacgacaagaacctaaaatcatacaagttgggggaaaagctcattatcatgacttagaggataggtgagttcttccacaatgagttgttggtttatttattgaaagcaagggttagagttctacgttgcattgacaattgctcctccttctcgacgttgatttgagagatgaataaaatttggacttgaaattcaagaatgtcatgatcgtgaaacacacttgaatcgtaatagagatttcacagataaaattgaaagaattatcataatggtttcattgggtagatacaccatcttgacaagtagtagattttctgggtaattttaattctcgtatttctgatatagacatatgctcacaaattgacgtgaaaccgcatgcgaaatttaggaacttatgcaggtgtttgggcgcagttttgactgtctattgttgttccctaattaaatatacaccttctctgtttcaactttccaacagttttgtgctaaagtatttgttgttgcatttatttattcaaacttaatttgttccaaaatatcatcagagtacaaactaaaggattcaacatgccttgagtacattttatactgtcaatggcaatgctacagcaattaagcaccagtacatgaagcaaccgtttattggttgagatttgagtgtcagtgtcattccttttccattctttgtttttggtagtaactatgatattgccattgtttataacttcaatgatctgctgatattgtggagcatgcaaaactaaaagctatcgagtaaaagtgatcataatgtgctagttcatataagaccatctaaaagctatcaattaaaacttatcgcagtgtgctaggaagttaagggtgtacatatatttgcaattggcagcaaaacagagcaaaagcaaagcattaagatcagaaaaagtagattaaccttaacaaatcgagctcgcctattgtcccctacagcaaagttaaacacctgcagtgtttaaaaaccacaaacaacatttaacaaaagtgaatgattaaaagtaaaaaaagaaaaaatcgagaaagataaaaaagaacagaagacggcataaactacaatatatgttttccatcacaggttattcatatcatcccccataaaactttctacttgagcactaccaagaaactattgaggatgtgggaccttgggatggttagtcaaaatgagcttctattatatccttctgtgtccttctattaaagctctcctcttcttgtttattttgtggagtcccaattttggcgtggccaattccatgatgccaaattggtaacaaatacttgaaagagtgatgactcaagagagatggtgaagaaagtagacatagttcaacgaattgaagtcatattcgagaacaatattatccagatagttcaatgaagtcatttattcaaaattcataagcaaatattaatgtggaaaagttctattcatttccaaattgaacaaaagaagcaaacaatagataaggtctccaacatggagataataattgagagtaaaaacttctattgctattaaatagaatctgcaattaaaaaaaaaattacatagatacaatatggaacttcaatatgtacaacttggaaaccctttcaatgcttgaggtctcagtttttaccacattcagatacaaaaatgtagtaacaatggcaattgtgcgcgattctaaaatggcaaaaaaataatgccaacttaactatggaaattatgtacagatataactaactataaaacttaaatcgtacagtggcatatcaacagagccttcttaggctctgctgctatcatcaaaaaaagcttttgactgattctggcagttcatggagtagtataagcttcggacgatttgaactgattcacacagcatgtaactgatttaaaaattcagttttactctatcagagtcaccaactcctttcttcccagaagaactagcagccgcttgttccttcaaagcttccttctccagtttcttcttttcagcatcagctgcttgttcattctcatcacgtgattttttaaacatcttcatgaacaccaccaaaatttgtgtcactgcatccagaaagtaaggaaatgaaaactgacaaagttcgtcacaaacattgtccggttaaagagttggtgaggaaaaatctgttgaagcaattctcacaccagttaaaacaagatctcaaggacaaacgcaattcgagaaatctagccgatggctatatgcactcaacaaaagctacaaaggccataaatgttgcatcccataatcttcacataaagatagacaactaaaaagcatcactgataaacgctactggaatatctatattaccaagactgtttgaacgactgtagttttttcttttccagatgactgataagtgataatacagcaagaaaataacgtatgtatctctaaccttgctcaaaggggcatcgagctggatcttcgccaaaatacagggatagggagtctgcactccttccctgcagatttacaggatagaaaaacaatcaataaacttggcatggcttatacatccaggaggctttaaaatatgacataatggatgcaagaaactcaccacttcaatataaagagtagtgagagacttgacttcagcctcagcagtatcaaggaaattctttaacacctgagaaggaatgcacgagtcacaaaccgcatatttcagatgtttataacaaaattatatgtacaccaaatcacagacatcgcaatcaagtttgactgcatcaccagactccactctaaaaccatgtccaacacaaaccaaattgggagttttcccagcgcaagcctttttcacttgaccttgttaagaacacaaatgtcatccatccattggggacacctatcactcttctaaaacagtggtacactgcttccttactttgttttctcaaactatctagaataaagctttttgatagtaaatagggatccttgtaatgtataatgaaggaaacctggggaaagaggaatccgcacaacgccgttcatttcatatctggcgtaagaaaatctcgagaatttgataatacatttaggggtcgtttggtagagcgtattaagaaaaatcatggatgcattagccttgtttattgctagtaccatgtttggtactcttttctaaactatgtacaactagtgttgcattagttatacactatcgtttattaaagtagattatgatatgaccttcaaagttaaaatttaaaactaaaaagaaacattatcttggaagtacaagtaactcatttggtttgtaggaataattcacatgttaccattctcttttctcaccttctgaaatcctgaagatattgtaccatcattgtcggatgcagtaagttcttgttcaactttctcaagacctttactcactgcttgcatttcttcagccaaagacttcagttgaatctaaccatataatatgatgtaaacaaacatttcagttcaccaaaataccagtagtactgcaaaggaagaccataataaatagcaagggtaccttagaagcagcttccaagtgaagaagatccttgtcaaaatcaagcaactctggcattttctcagcaaggagctgacaaaaaaacgaatttacacatttggcatcacattgagaagtgcaaacatatatatgccgaagagtaaagactaaggctggtcaagccagctatagttgatagctaaaggctatcaactaaagttcactgatggttgggcaaaagaacagcataaacgtagaatactgaaagtagaaaataaatacaaaaacatatagttttctacagaactcaaccttctatattacaggaacctcatgggtgcaccaaaaagcaataagggacaagaggctattccttaactgtgcaaattactctacactttcaaaagctctcctaattctcactctccacaaaacccacataagtgcaaaagcatacctttcacgccttgtgtctcctccttcatcttccgccatttcagttgagcaacattacttatacagtgacgggcatcacccaaatttaccaaacgaacaccacatttcccaccataaccgagaagttatcgcacaatctagaagacgattcgcgtcttcacctgacccccttacacataaaacaccgcccaacataagtagttctcctcttcattcttttatcatccatcaagatcacccctcttgttcctaaccaagtgaaaaaacctacctttctcagtaccttagggatccatatcaaaatatatggaaggctatctttcttctcattgatcaaaaatttgtccaaagaaaaggactttagcaaatttattcttaggcggccaaaatgaaacttagattacaatgaaaccttaacaaagacaagaattcaatgaaacctaaacaaagacaaggaccagacaatagagtctagctaaaaagaatctgggcttgctttttcaattcaaatctgtgagcgaggattcctctttctcttctccacaaaaatttgaagtggtttataacttacggagtatccgataatctcttgcaatcttgtataagcctgtgcagatgaaataacttgaacatttccaggagtcaatcgatttgcaccagtcgaccagtgggagcgataattttaagatataaacatcatataaccttccttttagcctattcccacttgagcgtacttcacagctgatacgctcataatacttgacgccccgaaataatgaacagggatagatatggagatacaatttaagaaaatgaaccttaggcacttcaatataagagaagagagaagtagaacaaaataaagaacaatgcaactggaaaaatgttgaaaataaagtgaacgatataagatggattagttttcagattttcatctttaagagctgctgactctcaaaaatctgctacaccgccttgccgccgccttcttgtttgagtgctcaacagaagcacctatacgcacttggactttccttagggtgatttaatagattttttgtgtattttatttccaattgtttcatttggcaagatactctaagcttgaaatttttaatttctatttagatagtcttgtatgcctaatttcatgtttgatcttctatttcattttagagtattggagttgatactggatctagctatcaccgacctactgtcgtactagcgtcaagtgcagcacttagccaataatccccaataataggggctacacttagacaaagtatgaatcaagaagttgtaagtgttagatgcatgtgtggcatttagctatgtttaacctcttttgctggagtaatctctcctttgtaaatgatatggatcaatcaacccaccaatagttctagtaattcctgaactactaagtgtactaccaagcattctaaagcctcatgcatcttccttgattgtgtagaacatgccatacttatgtggtgagccttgcttgtgcactatggctcccacttgtgcatcaccatgcctcgtgcatgctacatcatcagaccatgctcttgtgctaacactatcaccataccagcccagccatgcctccatgaaacagttcctaattttctttgcgttactactaagacaacgaatcgtttgatcttgaaattccttgcctcctctctgttagcctggtccatggctttgttgcacttgcgcatcatgccacacttatgtttgtgaaccgtgcttgtacactatggcttccactagtgcttcttcaccatgcctcatgcatgcttcatcttagtagcatcctcttgtgccaaaacaaccacgcctaccagccatgcctaacatggaactgttccccaatttctttaactttctaattaaaacttaaacaaagaatcatttggtttttgagtgttgaaaccttgaaagcgctcgcctcctctaaagtagcccccttcatggttttagatgggttatgacatagacctcaaatacacttggcactttttcaatccaatcatgagctactcaacaattattactgagccaaaactaatctgattcaacttacgcttaagtcacctccaactcttcccaattcagagctaattgatcaatactaattacataaaggtaaaaacagaaaggcatcataatgcagtaattctaccttgcacagataatgcatcaaggtcattttgttgtttctcgcacgagtgtcagaaagcttaagaagactgtccaacttgaaccctacagcagatcctgtaacgtaattacaaaacaaagatgttagtcacgatgcctccacccaacaactgattattttcttatagagatatagatcttagaaaactgtacctcgtgctgtaccctgattcagtgcattacccaatgttagaatggtctgcattatctgacgtaatttggcagattctttcacctacttgaccaggaaattcagttagagcctagttaaatcagaatgtgccaaatcaaacttcataaggtattaaaaatacctctctagtagcatcattgattgtactcaggttacttctcaagtccttcacctgaacaattcaacatattatagtcaacagaaaattaatggcagaatccatagacattagatcactaagaagtacaagagaaaatacctgattagagaaagtgatagtaaatgaaaacactcgtaacttggactcaactcgtgggaccttcatcagctccaggaaaaactgaaacgggtattacttatccggttaattacttataacttaaaggataggaaaacttgtacttccccacatatatggtcaaaatggagaagacctgctcacactttccaagcatccccttgtccccattatagttctggaaaatagaacataaccagtaagatcaaattgtgaaatcaagaataacaattaaatatcaaattgcaagtatagactgtcaagaaactaacataactaagttcacaaagagagggggaaatcaagcagaaacaagtatggatctacatacacaaaagactaagatatatgcctatgtttatacacatccacacccaccgggaaaggaagttcccaggaaaaggtatctgcatgattagacattgaaacagacacatgagcatgcacgcacagcatagatgcaagtacatactgtataagcatgaaaccgccaaatgggtcattgacttatgggcatcaacctacacagctacttgcaacaaatggcacatcaacaaaactataggctcctgctgttcctacgactcacttaactattcttacgttaagtacaattgcagaatgtgaaggttccgactcttgtttccaaatactatgggcaaaaaacttcaatatggagtattttctctaaacgggaaaagttaaaagaagaatcaaagcaaacttcagaacatacctctaatattacttgtgaactcaaaataaatgactagacacacattataagcatattattgtaacttaaactttgccatgataggcaagcacagtaggatgagaaagagattataccctcagtgtctccatttcttcttttgttgggcaaaattttatcagattttcaacctgatcaatgtccagagctgatgaatccaaagccaaaatagcattctgtatgacatgcatacaaatataatttgtaagaaatccgcggtaaattttcctttgtaaacagaaattttatttgcatttgcataatactggccgcgagttcaaatagcggaccccaacttgtctggaactgaggcgcaactgttgttataatattagtaaaaagaaatccatggcaaatatttcattcatttcaatgtacctccattaaaactcaaaataaggaaaaaagaacttccaaagaaaccatgcatgagcatcctaaagaaatgctcgtcagtcattacacttattgaacacatgcatgaatcagcatattgatactgtgcattatgaaacatgattttgaccaaaggccaaaggatagaatattttatacaatttctatcatgattcctttgaatttcaaaggaaaaatatccataagagttcaattttgaactcttcaagttcggtgaaattacatgatcttttcaacacaataaaattatcaaaaatataaaaaataagaaagtcttttggataaatagttctacagctacttccatagaaagctccttttctccttgtacaaaataaaggtttctttatccatttcattgaactccggctaaaaaatatttctaataacgatagtgtctgatcctacttgtgctcgtatcttgactaatttatagggtacttgacacctcctatcaacataggtatggggaactatgccctccaaaatgcaatcagatgaggaaaaccaccaagtcttagttttggtcgctactagaaaaaccacttggccacactctaaagtgctcattgaactccaccaatatgagaaaagcataactaacttgaaactgaattacaaggagaactgttataggttaatggctaacataaaaatagtcaaactaccaaactcctctgtgtatgacctaaatgttatgtgtagttaaccgatttatacgttcttcattcctttgttgagaaaaaatatagatagttaatcaatatattgtacttctattaagcagaaacgaagatacttcaatttagagttcagtacataatataatctttttgatctagtaaaaagattatagcatgaagagttcaatacatacaagatacaacaatcttttccttttttttgttgttgagaatggacttttagtcaaacccattaagctgattcaataattttgcagatctatttgattcatcagatacatacttctatagttttagcaaatgtacaaagggattaaaaaaaactaaaatactaaattgtaatcttttggaaaataaagtcaaacaacatatgcattcaattgcatatgtaatttgttacttgatttcaattgataaacacatcaggattcgttaattttaatggctgtttagtttgtgttactttttaaattattagcagctcaatttccaaatatctgattgtcctaaagcccaagtaaagatcacataatctaatagtttcatctgataaacaataatagattattatcaaaagacccacctgttggctagaagacataaattagtgcgcaatagataaaagtatcgaagctcatagtagaaacgagaagacacaaaaagaactcacaagcatatcaggcaggggaatcttgatttttgtaagcatgatttcacaattgtatgccctgcgcaaatcaatctggcaaaagcatatgttaagaaatcatcccggtcttttaacagttagaccaaaatgtaacacttccagtctttcactataaataatgggagttgtgtaaaataaacctcaatacctcaggaagaaaaagaagccaacaccaatagactgttcaccaactattccatagtgatctcatattatacagtgaaagctttgaaaactatcagtttctttctatagaagttttctatctctttcccaatttagcactaacagataaattaagaagcaagtgaactgcaattcattcatggtcaatggccatccccatgggacacagtgcccattatgagcacagcctccgcaactctttcattagatctagacatgtatcgcagcctaataaaattactctgttgcatgaatttacatctcaaagtattaacacaacttttaagaatttttcaaaggcaaccattatttttttatatgattgactccatccactaaaccctctgcctaagacgcccaagagaggtttccccctttatcccttcgttaatcaaacccccaaccttatggttggagatgaaggaccttaccctaggatatcactccagtcaaagataattgtcttaactttcatgaaacagaaatggtattacctacaggatggagaaaggaggacttttccacccaaagtttatgtaatcatccacatccaggctgaaaaaacataagttcttctctataagggcatgcttgtttcgaaacgtcacctatgttaaacccatttaagcctttctatttacttcttttcttccaccttgttagccacaagataccacaaaaagtgctctttaaaacctatctaatatttaattgttttgttaaactagtaaagaaaggagatacactcatcctacaacactcactttactacatgaaagacttgctagataatgcctactggagaataacagttgtagagactggaaacaagataaagcatatataacttgccaattgcactttttctggtttgttgatttttgaaccacgtcggcctccacctttgctagtgccatcagtagctgaagccaccgaaaacaaattctcaagctccgtaatatcaatttcaggtgctctgtcatgtacattaataaaatcttatcagaactacccataacagacagataacaaataaaagttgcagtacccaacacaaactaggttaagctcaaagggctcagaactactatatctgtaatctattaagcattcgaagttgaaaccatgagaatgatagtgcttatgacaacctgttaaggggtttcacgagacacgagaaatagcgaacaatttagctctgactattaacttgaaatgacacacaaagttctcattgtaatttttcatccccaaaaataaaatctttatacctggaagtattttccttgttttgcgtatcagcccataaactcccttgcatagcccgtgtaactttcgaccaatgtaagggcttcaatgaagcttttttcggaggaattgaagtacctcctgtacctcgcccttttcctagagcagttgaacctacagaggctcttacacgtccggtagatggaggtggtggcgctggcacactaaggccctttccaccaggcgggggaggtggagtgggtgtcaaaccccgcctagggggtggtggagcattaggagcctttggtgctggtggaggtgctggtggagtggaaccttgcctaggaactcccaaaggaggtggaggaggtgcaggtggccttgtagaattgtttgacggtggaggtggtggcggtggaggtgccaacggagtaggcctatttgatgaagaaggcggaggtggaggcggtggtggtggaggtgccaacggagttggcctatttgacgtagaggatggaggtggaggcggtggtggtggaggtgccaacagagttggcctatttgacgtagaggatggaggtggaggtggaggaggtggaggtggaggtgccaacgaagttggcctttttgacgtagaagatggaggtggaggtggaggcggtggaggtggaggtgccaacagagttggcctatttgaagtagaggacggaggtggaggtggaggtggaggtggagcgggaggtggagggcctttggaaagggctgaaggggtaagcgggggaggtggagaaggcggggaagttacacaaagcaagggtgaacacttcaatgacatgaaaggggaggggaggggtggaggaggagctgataaattacagttagatggaccccgaggaggaggaggtggaggtggaggtggaggcaaggcacttctagaagtagaaaacgtagggacagatggtggatgtggaggagcagaagagcataaaaggctctgattaggaagtggtggaggtggtggaggtggcggaggtcctctagaaaagctatcaggggaagttgaagaagtaggttgtcttggcggtgaatgttctctatggctaccaattgaaggtggtggtggtggtggtggtggaggtggaggtggaggtgatctattagaacttgcaagtggtggaagcggacgagtacgttggacagaagaagggacaccaattataggaggaggtggaggtggtggaggaggcggaggaggtaatgagacctccttgctaggagaaccaaacagagagggtggtgaagggggagatggagctgatgattgagtgacttttatactagaaatcacagaggcaggtgacggaggtggtgaaggtagcggagaagaagaggaagtccttgtatcgcaaatttgaactccctttaaacgttcaggagaaatggcagtatccaattgacagttactttcagaaagagactgaacaggaccaagatctgactttgaaagcttcatttgaccctcagaaatcttgggatcagaagttccatcagaagctgaatcctgttcatctaaaaagttgacatctgttgtattagcataactaatactactagctttctctgagtccagaaaatccaaactgtcggcaatgctcgatgcattattttcttcttcagaatcaaatggggatgaatacccactcatcctactttgcaaaattgacaaatctttcatatcattcagcaccgatagctgtttaaacaaccacaacgcagcatcatcaccagtatcaacccaatcagcaccactaaaaagttcttgtacccttgaaaaggcttcaataggaagtccaccagtctcctcaccattgagagctgcagtgggagcttttagtggagatatgctctcaacatcaccaaataaaacctgcaaagcagaaagtataagttagaggagaaatatgaagagcaaaggtgatccaataaaacaaaactaatcagacagtttgtaaataagtattcacctcagctcgaaagccttttggatagcgtgcctttgaatcccatagaatatccaggttatcgcagtttaacatcaaaatgttagagcgaataaaagcagtgttaaacacaatacggaacatcatgacttccctttcaggatccaggtctaagtggacacactccaaaactacatctccttgcaccaaacactgaatatcaatcttgatgacatcactgtccttctgcaaaacaataacaatcatgttgccacagagcagaattgaagaagacaacaaacaagatgcagtgatagcaatttttcacctggcgataatgtcgaaggcttctacctttcttcggcatggagtacaacatatgagttgacaatccatccttgctgagaaggttccttccaaaaatgcgcacaattggcctacaccctttttgattgtcaaatcttggaatggcacgaagaatgaggcaatccagagaaagagcttgttcaggaggaggccactcgggagatatatttcttcttgatatatattgcaggtaacgaagctgagaagggaatgggttcaaaggtgacaacaattgcgataaacctttaggtgcctcacgataaaccatctcgagagtttttctctctccgctttgtaactttctgaaaaccaagaaactggcgaaaatgaaggctagaaggggccaaccacctctctcacagtgtaacaaaattacattgttatgattttgaagagagagccaactctcacagatacatagaaaatgatgtatcaatgacaatggcagtacaggacagccttcatattgtcttgggtaatccattacagtcacatcatactcgcataaaatctcagcaaactggctccttttctcgccttctctgaaattgaaagcaagaaaggaggaatctggaaattcttcatgtagttcatttatgatttcgtgcaagtaaagctgataaattccctcaggcagtacttcagtcgaaaaacaagaatcaaaaactgcagatattcaacataagataaaaagatgttgagaaaactacaatgcacttccaatgttcaataaaaaacacattataaagtcaaagctagttcctttaccatatactctatcatcaagttccagcaacccatctgggggccttctatagaaaaatctactcaacagcgacataatactgagccaatatatcacctaaatttacctgacatcaaagaaattcaaacccattttcattcctttggtgtcccaatatcaaaagggtcagagaatcagctcgtacaaattcaagaaaatgtgaaattcataagaagaactcaaaattaatctcaaattcagaatacccacaaagctaaaaagggattgaactatatttcaggcgaaaaaattggaacttgacaccaaataaactacaacaagactgaaacacacacaaaactcacatggaaaatatttgcatataaaacaccaaaaaaggaaatctttgaactgaagcaaaccgacagaagccgttgaggaaggattcgagatgtgaggtgaagaaccgacagtgttgccagtaaagttttcacctgcgctttccgattttagtatgaatttttttttttttctgattacggatttgaactctttggagttcaaaattttgggaacgaaaaaaaaggggctgattttttattttaacatatggttgttttcaatttttgaaattacagaaccaacccaatacttgtatggataacttttagttagtgttttattttcgaaaactctacgatgaaggatcgatcggaaataatttttattttctactcataattaggaataagattataatgtgaaatattcaatgatgattaatgaatagtgttatatttaattgattattattgacttgaataataataaaaatataaattacaaatatatataaattaaatacgaatgagtataatataactttcttaaaacaattgagtgcgatggcttaatggtcaagatgaatatattgtactggatgatcatgtctttgaatccccatttatatcagggtcaaatacataaagagatttctaaacttgttgggtttttttcttcacgtactttaactacgtcatttttctattgaatcattgaaccatccaaaaatttattcctttaagaacattgttggtttattttgatcggctattctattgtaaatgcctttaattgggttcgaattgtaatgattttgattgaaggaatgaagacaacccgttttagtctcatttgttttttaacgtcttcaaatgacttaattaaaatacaattattctcgaacatttttactatcaattggactaatgatttctgaaacaacatatatatcctctatcaatccccctcacaaatctggtttcacatcagacaacagtgtttatttaaatggaacaaattataggggtttaatgattcaataggaaaatgacgtagttaaagtacctgaggagaaaaaacacaagtttagagatttgcttatgtatttgaccttaaatcagctatccaacatgcacttttgagctttctatgggtgcgctaatacttgtgtgtcaacttttttaaagatatatatgaataaatatatataacatgattttttttttgaaattaacaggtatacgtgcacctcatttatacatgttaggtctgtctctaaaatcagatctacaaagttacatcgggtatgtttttaatattattgtggttgtttgtaataaatattttaattagagttgttcaaaatcaaatcgaaattgataattcgaattggaaaaaaaagttattgatttatcagtattgggttattgatttagcgatttagttaagggtctgattttttttgttatcgggttatcagtttgaagttttttctcccgatagtaaattaaataattatatttataccattttatgtttgactcgaagtttgctttcctacttttatttttggttattcaatgtatctgcttttgagtaagatgtaacttgtgaactgatgtgcatagtttatttggtttgtcaccttgtttctaagtgatttttaatataaatttttgtgtcaaatcttaaccagttaaactgataaccaaatcgatagcgataaaaaatcgataagccaatatgttaatagttctataacgatttaacatctctacacactatcaaccaataagccaatcaataaactttaaaaccgaatcgaacagaccgatacgcagagctaattctaatgacaataatcgattgtggaatctatattaatgcatggctgcattgaactctaaattgaagtatcttcttttctgcttaaattacctccaaaaggtaccaatgataccaaaatttccaggcttggttgatgggccaaagtgaccatgtgatcgcctttattgggcttttagcccagttaaacttagggcccaatgacgcatattctatcagcaacaagaagtattgttggtgactagagaattttagaatgtaattaaactatttttggccaacaaaaaatataaatgatatacaatatttaatataaaactagaaaaagttaacattattcctcaatgagtatgattcgaaatgcatagacgaggctatatacaaaaatagaggaagattggatcgcctatttgaatctggtttggtgttagaaattcgtagataaatcgagttgaaaaaaacgttgtgacacgtgttttacgtatgagagccaaatgatatggactttgatcaacttttcaagatgtattttttcgtcatattgatattgagaaagattgcaatttatagtattgtcctcattgttttagaaaaccaaaagattttaagtttgaagtatagaattaatccaatcaaatttagttttgaaagtcaattaaagtgactctcaaaaacgcaaatcatgataatattttgaaataaattagggtgttttttttattgttctatctcatttgtttgaaatatagtatttagaaattacgcgaacattctaatcgttattcattgagtaatatacctgattataagacgattaatattgagattgtgagacaaaaggaagaaaatataaatttatagtactaaggacaagggcggacccacaaggtgtcaagtcgggtgctcgaaacacccattaaccgttattgaaatatgtatatctatgttaaaatcgatagctatttgtataaaattaacatagagcacccaatgaataaatcatatagttggcccaatggttctagaatgggtacttaagactcttttaatgttattgtaccaaggttcgaattccgccactgactaaggatcacgatggagtcatggagatcattatttggataatataacaagcaaatgcaacttaaattcaaatttcttttattcaattacaattaattaaattatgattaaatcattttataagtggagatcattatttggataatataacaagcaaatgcaacttaaattcaaatttcttttattcaattacaattaattaaattatgattaaaaaatcattttataagtaaaaatacttctataaaaggaaattttatccttaaaattcaaatattaaacttcaaattaacaacacatgcaaccttatacaaaacaaatcaactaggatacctcccccaataattaaattggtggtcaataaaattgtactccataattatgaattgtagttggcaataataaatatgcattgtattgtcctcatcgactagtcaatggaacatttatgaaaccaaaaaacatgaatcaatgttctctacttgcaccaaagtttttatgaatgagaaataatattagatttgtccgttaaggatttcaaatgttttaaatattgtacttggggtataaatgagcttttttttatcagtaaatttttatcgtatatctgatgattatagatctccattctcagaaacatcacttgaaaatagttgttactccatccgctcacccaattataacatcgatcttaataaaaatacataaaaatcatttagttcaaatggtttccctcactttatatttttatcatttttttctattaccaattaattagttttgttataaaatcgttgatggtcaacaattataactctatcttgattgtcatacgattgttaagatggagtttcagcgaggttaaaaattaactcgttggtataattatgcattatttaaattttatttgagatgattttatagattaatggtaattaatttagtcttgaggagtaaaataaaatcgttataggtttttgagtgttcctaacatcagaatggtgacatcattatgaagttataaagacatataatataatttaaactaggaaaaaagataaatatccttttgaattatcgtaaatagtatgtaaatgctctctgtcaattttttgggacactgatgctcctgtcgttcaaaaactagaaataatatatactctttacactaacggacacacacgtgtcataatcttattcaccaattctacatttattgacggagaagattgcgccatgtgtttctatttagtcttcctttagagttaacggcatataaactttagttttttttttacagcaggaacatcaatgtcccaaaaatatgacaaagaatatttccatatcatttacgatagtttgagatatattttccctttttccatttaaactaatatgcaaaatacgatcctgctcctctttatttctcttctctccattttccccaagtttccatttggattaatgacacatgtcatgggttaaaataaatggttaaaatttaatttttcaaagtaaacctctaaacatgatttagttaatatatatattatatatcaagtatcaaaatttttataatttcacaatcttagcaaacatattattttgtccatattatttatgtaaaaagttttcttcctataatttttttttttcgtaggatcttttttattttttattttatacaatattttaattgtaatcttttgttaaaggtatattggtccgtgattaataaattacctagagataatcaaatcattttgacaaactaattttaatttcataataagattaagaatacggtgataccaagacatacgatagattaattatagttttcatacttctattcagttgcttattcttctaattagataaaaaaaaatttatataaagggaaaaaaaagatcctacgtaaaaagaaataataggaagaaaactttttttacctatatttatggacaaaataatatgttcctaagattgtgagattataataattttgatgcttgatatataatatatttattaactaaatctgtcacgacccaaacgggtcgcgagtggcacccacatttactctcctatgtgagcgaaccaaccaatctaatcccaacatttcaaccataataaacagaaaataaagcgaaagacttaaaactcattaacgaaatcaattaataacttctaaaatttaatattcatcatccccaaaatctggaagtcatcaccacaagaacatctatcctcaaaatactaaatctaagaatgtctagaaaactaaaataataaacagctagtctatgccgaaacttcaaggcatcaagacacacgaaggaagatccgtcaagctgctaaagcgttagctcaccccgagatccgacgtgatgaagaccggctagagttacggttgagttgaagacgatgatacgtttgtgcgactccacaaataacaaagaaaacaattacaagtagggtcaagataaaaaacagtaatcgaaagtagtatcattgccaactcaaaatagaaagcaatatatttcagataatatcataaaatcaactaatattcttaacaggtgatagcaacaagtataaaactcatttataacaaaccaaccacatccatgaggactcaagcctccataccatactctttagggaaacaagttctttggattgactatattaacatatttcaagattcattatctttctatctccggtgtcggaacgtgacaccgatcctcatcatactatctggtgctctaacgtgacacccgatccatattctatcctgcgtgggaacgtggcaccgatcctcattctatctcggtgccgaatgtggcaccgatcctcattctatcccagtgccgaacgtgggcactccgatcctcattctatcacggtgcgggaacgtgacacccgatcctctattactatcccggtgctcaacgtgacacccgatcctctaatctcattactttagttcatcaagccttcttttataccaagacatcatcattaacaaagtaaaatttaggatttaagattcaacagcctcatcatgctagtttcatcacaattatatatataaactcatcatgctagtttcatcacagttatatatataaactcatcatgcatacacacaattaagcatatagaagagtttacaatactacccaaaacatatcattcgctattaagagtttactatgaaatagcataaaccataacctacctccaccgaagaatcgcgatcgacaagctatcttcccaaagctgcgttcttcctctctctctttgttctttctatttttcttattcaaacccccttttcttttaccctaattagcatataattaagtataaaagatgataaaataccccactacttgtttccaaggttatctcttttaacccccaagtaattgaattattaacattaaaccactaactttataattataagcaggaatagtccaaaacgtcccttaaaatatttaacagaaatccgacccattcggtcacgcgttttagacggcccgtcgtgctgcgacggtcaaatctctttgcttccgtacaaagttcgggagactcaattcattaaaaagtccagcggcggcccgttatgctcggagacggtcgccccgccacccgtcgtgacgttcgatcgatctcggtacccaaatttttaaattctaagtgttttagaacgagacccctcgacggtccggtcgtgcccatgacggtccatcgtgggatccgtcgactcaccagctttttccggaaataaaaatcacgctaaaaacgactaaacaggtcgttacaaaatcatggttaaaggtttactttgaaaaattaaatcttaactatttattttaacctataacatgtgtcattaatccaaatagaaacttgaaaaaaatgaagagaaagagaaatggagaggagccgaatcccgcaaagtagaaatatatttgacccctgctattaactattaaaacgttcttgtttcattttgaacttgcaaatatctgtggtacactacaaatttaagggttataatatctattaataaacctaattagtaagggctaatgagactttaaacacaataggcaaatgacaggtaagccctcagattttgattctcctatatcacacatgacgttgtcagaggtcaaaactgtcattatatgtccaaaatacgtgagtatgattttttagcagcaagaaaccaaaaaaaaaaaaagagatacagattttggcaatttatacctttttgaattgaaatgattacacacctttttcacattgtcagtttattttctttttggggtctaaaagttttggtttttgaaaaaaaaaatatccgttgatttaattttggagtaatttaagggggatgtttggttatgaaaatataaaaatattcattttatttaaaaaaaattaaagttgaagtttgaattgtgttgggttatattttttgtaaataatatgtataattggttatgtttttgggtgactaaaagtatttactttagaaaagaagatatttatgtcaagaaaataagtgttgcttaagagtagaaaaatattattttgacaaaaaaaatgcacttaaaaacactttgaagaaatgcaattaaacactaattgtcgtgtaagaggtctttaaaaattaattggtcaatgcattatgatcacaaaagtatttttaaaaaattaaacctttactaaaataaattaattttagaaattcgacctaacaagtcataaaaataaaataaacttttacttatttaatgtttgaaggccattaacaattgaattaatattgctttttcaataaagatttgattttaaccaacctcaattaataccaattaaagtttaattttgtaaattggattgaagttgcacaaatgagtatatttagttatgtactaacatcttccatattaattctcctaaatctttaggtacatatttttcttttccatatttttaacgattttactttctaagttttaaactttaacttttttaaattaattagttcaatcttcttcttcttcttttttttttggagggacataatttgatcgatctattaatcataaaacatgtctttttttttgtccaatattatatgaattttatgaaataaatttattttagaactttttaacgtattttgactttaagctttattcaatccgccttcactgacaaaaattccaaataaaaataaagtgctaaagtataatttatatactctctctgttttataaagaatggtctaatttgacttgatacgatatttctcctattttataaagaatgatctaatttgatttgatacgaaattaaatatacaacccttacatgccacgtggaaagttattgtcagaaaaaaaaaattattctttttgatatggactataaaaaaaaggtcattcctttttaaaacgagcagaataatatatatcccaaaactttattattgagaaagcatctaaaatttgatatggcaattgcatgaatgtggagtaaaattattctaatacaccagatatgatgccatgcagaaatgatgtggaaactatatatagcacaattcccaatgaaatttaatgtactgtctcataactatatagtataggctttcctctaactatacataaagttacccctaaaatataggctagctacccttctagctttcccccaaattctaaattagaacaaaaaaatatttctacatctttttacagtttttagtccctttcactctttggggttatttggaggtaaattatttatagtaatttagaattttatatgtataaattataaaaacttatatttgtggcatctttggaggtaaattattaatagtaatttagaattttatgcgtatgagttataaaaacttatatcattcatataaggtagaagatataataattaaattttatataataattatctgtattactaatatttgtataactttaatcaatcattctttaatgagcaattttcacatataacaaataaaaaaaatcatatttgtatgttataacaaagtttgcttaattaaggctccataaagaacatagaaacatataattcgctatacatatacggttgaagcaaattgtataaaacgaagtgtataaaacaagaaagagaaagacatcaagagaatcgtataaaaataaattgtattattataagtgtatagaacgattatatacaatttgaatttgtataaaatgagaaatagagaaagacaaaagagacttgacagggaatatacaattgaatcgaattgtataaaacgagaaaagagaaattagatacaatttgaaaattgtataaaacgagaaagagagaaagacaaaagaaactggtcagatgagtatttttattgtataattataagtgtataggacgaaaatatatgtacttgtatgtgtatatacaattttctcacgctttatacaaacataaacacaatttatacatttagcttctgtttgtataagtgagaaaggcgagggtggtgagcgagatttgggagagtggcgagcgagatctggaagaggagagagaggggaacaaaaatatatgtattatacaattttctctgctttaaacaattagaaataatttttatatacttgtgtttgtataaaaaataaggaagcgagtgagagattagaggaaagtggcgagcgagataattgggagagaggcgcctggcaatttttcgcaaatatttgcgatggagcacaattatatcaaactctaactacatttattttagattattagtttgctattatatataattttcttttttttaattgtttagtacttgaaagttgagtaagtgttctaacccaaaatgagttatatttatacactgatactcctatttaaagtttagtaatagtacttatgtagaccattgtataagtttttaactggccaacaatctatttcatacaatatatttggacttacaaacactatagaacttatctttaagtattaaagataattttttatcacataagcaggagcctctatttgatctatttcgctttaatataacgtgcaatatcctatttgattttcttatttactttaattatagactcgagatttgtaaaacttcttattttgaggataactagtgtatcaatatcactttcctatttaccttatgtgacgcgacacataacttccatttaatgtactttcttttagtcccgctcatccaaaaatatttaaactctttggtcggtctccaaatctcttatatatcattaattcaatagcatgactcatcaataaaatattatatcatctacacataacatacattgtgatacttccactcgaatatgtcatgttaattcatcgatcatcaaagcaaataaaaacaaattgagaactaattcctagtgcatcccatctcgattggtatcaaggtctttttctttaacagtccttacttagatcttgactccattatacatgcctttaattactctaatatatatcgtaattatatttctagactccaaacatcttcgtaaaacctctctcataatcaccatataaataaaagataactcaaacttgacctattaagagttgattggttgaaattccatgttaaagatctgaaaaaggccttatataaaaatggtcctttgtacagtctgttgattctgattccaaattgtttatgcctaaaacaaacatgatctaaatatttaattaaaaggtctctaattcaatcaagatccattttgtagtcaaaatatatactattttggtggaattttggacataagaattaatgaaaaatagtccattatatttttttcatagttaaacaacacactttatactacatgcctattttttgctagtaatttcgcctaagaattaaaattaaaagtgctaattaattaagacattaagctgtaaaaatatttaaatatgcaaaggctaatcattaatgcaaaaacaataggctccccaaccgcactttcatatataaatagcaagaaggaaataataagtaaaatggataaaaatatgataacgtctagatacacaaagactatcttatttgaaaaaattgtttatataatagcaacctattagtttaaattaaatgttataaccatagtttgatttaactgtaactcttattaaattcttgttgttcacatcccgttcaccactctcactcgtctctccactttatagaaacacaaatgtatacattgcgtttgtgtttgtataaagcaaaaaaaattgtatatacaaaaataatgcatatattttcgttcgatacacttatgattatgaaaatacaatttttccttgcccaatttcttttgtctttctatctttttcgttttataaacacaaattatacaattgattcttttgtatatgtataccgaaacatattatataattttttttttgtatataagtataacgaaatatccatagcaaacataaagtttgctataaagcgtaattaatgtaaactatagttataacttacaaatataatttttgtatttcttatatgtgaaagttgctcttttttttcaagtgtgtgaataaattaatacttaaagtatgtaatcacttttaattgggaaaatgcataagtatcccaacaacctatgtccgaaatcacagagacacacttatactatactaaggtcctattaccctatgaacttgttttataaataactttataccctttttcggccttgatgcgggagaggcatgagtgcaattcaatcttgtggtgtattcgtttgtagtgagtagggcctctttctcgttgatctgacactatcaaccacataacttaaaaaaattgtcagcacactttgggcccacaagagagtgtcacgtaggccgtaaagggatagaaagttatttataaaataagtttacatgggtaatatgaccttagtatattatgagtgtatctctaaaatttcggacatatgttgaaggggtacttaagcatttctcccttttaattatatgcattaacctctattagttataaaaaaaaaacttattttgagattgaagcatataatgaaatgcaataacacatattattcacatttttaaaacgttcaacataattatatatcgtggatcttgctttcgaaataactggaatcggcatgctagtccgaaattctcgtggaagcttcattagaggccacactcgtcggttaggatgacaacaagatccacttatggccgaggaactgggtgttcaagaagcactaagctggttgaaggacactttacggcaaacaacccagatagttatagagatggacaatctttttggttaaacaagagataaaaaaggtgcaaaaactactcttacttttatgttattattcatgattgtaaagcattcgtgtgtgactttacttctatttctttgtctttcgataaaagatgagcaaaccagtgtacccatcagttagctcaaattttgggttttatgactaatgctataaagcggataatagatctccatctttaattcaagatgtactcaattttaatttgatcaataattaattaaaatgtttgattaaaaaaaaaaagaatgttcatcatactaaacctactttgtaatgacatatataactaactattttgatgaataatcaaactactcaactttctttaaaggttttgaagaacaaaaatgtcatattggctatttacacttcatttagctaataagaaattgattttcctttcttataattttttttgtgtttttctttctcacctccattttttctgacttagagctcgttttgattgatttaaaagaatagtttttaaatcaaacttaaataattttaaattaaaaaataaaaagtagaaggagatctacttttaattttaaacttattttaagtcatttataatcttgtcaatcatataaagtcaaaattctgactcaaaaataagtttgattaactcttgagtcaattcaaacaccctcttagttttaattgacatctataacctctaattttaggtatgtacaaataaatacttaaatttatataaaaattaaacaaattaatatttgtgatatgtgacattgcataagacaattttatatcaacgtgatgtcctacctatattacgccacataaattacatatatattgatctttcaattttatatcgtttaaattatacatatataccctatcaaaaaagtattatgcttgttgaatagttctaacttgtaacatccactttcctctttccacttcaatcccaaaaacatttcttacaaatttgcaaaaaacaatgaaaaggacttaattagcaaaagagaccacaaaatgaaagggtcacatggggtgtgttaaaactcaagcctaaaaagactttgttttgtttttgaatagatatatcactcaaaaacccaaaaagcaaaccagtaaaaggtgaccccaaaaagcttccccacacacacactgaagacaactttccagtaatggcggcacatgaagaacaacaccaccatcatcaacaacaagaacaagagaaccccatttcctctttatccttaaaacccaacaataaacacttggagaagattttctcctcatatttgggtctaagtttcgctgtctttcttgggtctttaccaagaaatgcagtttctttggttgggagacttcagaaccgtaacaaggagctaacttttcagcttattgatacagaggagcagttaaagcagctacttttcaggagaaaagaggattcaaaggcaaatgcaagagttgtggaaatctttgcaagtcatagacatgcctggcagcaagaagagaagaggttgttacagcagatcgatgagtgtgatgaagaaattgctgagttaagagggagagctgagcagtttgagacaatggaaagtgagttgagggctaatattgaggacttgaaaagggagattagtgaaagagatgaaatgttgaactttatgagtagaaggggttgtgagatggagaatagtactagtggagatggtgggagtgatggtgttggagattgttatgctgaaatgggtttgaggtttgggaaagttgggatatctgaagggatggatttgggggtagggatggaagagtgttacttggctaatgggattcctaatgctgaacaaatgagtggtgtttatggacagagtaatgggtttaactcagaatacttgaattctgcttctaagttttgggctgaaaaagctagtccttggcaggtatgatccattcattatttctttttgggaacttttttgttctttatagttgttgttatttggggttttatagtgagtggtgtcataatgtggtaaaaataaacgcaaaagtcctttccaggatcttcatatgtaggaagaacttggactaaagtttgtcgctttaatgtttgtcttatatatggtttttcatggtgaaacttatgaataaagttgcttcttttatttaaccatgggattgtactttaagtactaccacctgatattctttcttttagtgtttatctgtttgttcatcttgaggctgtggaatttgtttttgtatgtgatatctgatgaaacaaatgatccagagcaattgaggatgaacgaaattaagtaataaaatgtttggcttatagggttcttggtgaagtacaggcctttatgatctttcttcacatacctgaaaatttcacaggaatatccacttctaattgtttctgataaagctgaaatgaaggtgtttctccaggagtagttcagcgccaaattcaaattgaattgtataatgattacattctgagatgcttattaatgaaatatgtagtttagtgtgtactcagtgacctcctacttgtcttgtgatttgtctttattgttgagactcttgtctctattatctaaaattttgaatggtttgatcttcttagtggctgctgaaagttcaaactacccaggatatggttttctgtttactgaaagataatactcacctcaactgttcatttttaccctatactggtgttatggaccactgcttgaaaaccaggtcaccgttttgtacttttcttctttcaccgttttcgtcctattagaggtttgcaattcttgcttcaagaatggtcccctttggctgaatactttgcatgaaggttggtttcctggttatgaaggaagctcaaaaaaatgtattcgggtaactctagaaatccgaaatccgtttaaaacggaccgttttgttggcatagaccactgtgcctctaaaataccaactaatgacatccaattatatatcccctttggtttgggaagttcaattctggttaaaatggatccgtatatcagcaaaggatgggctgttatcagtcaacatctagtccatctgttatatttctgtttaagattcatcaacctcaatggaaagatgtcctctccctttcttgttgcaagctgtatcttgtccttgtctgtctctgtatcttattttccaattacaatgttatctttggtaattcgttacacatccttgaaataaagcaaatgcctccatgaaacttgaactccccgcggcctctaatccaggcactaatctttcccgttcaaaaggatcactggaacattttcctatacttggtggatgtgtcaaagtttggactaggtagagatcacacattcaatttatggctgtgttttttgtcttttatcatttttgtctttttatattatatagaaaagaagatctggattttcttacccttggtacagtcacccttttcatttatttggaaccagagggaactggagcatttcactatgttgtcttcaactttaatagaaaggctaaagaaaacacacaaccttaaaaataaacctaaattgcctaactattagttgatctatgccttgtgagctggttaaggattagtcatatttacaatggttagagcaaaaagagaaataaacatctagatcacaatgcttatattctagtttcaagcttgaatggtaggagaaatgaggttcttttgactcttattcagcttcttccttctatgtgagatgtcctacctatcttagtaaaaccagcttggtatttaggatgctattgggtcttaagaaaatgtgttttcttcatgcaggatatgcagtatgattctggcgattcacttcaccatttaaagcattttgtagcaaggtaaacattctgtgattagttagacagatgcttagatgtttgcattttgatgttgaatcaactaactagggtgagcccttttgctttctcagacgggaggccccttggaagatagatggtgaatcaacaggagtctcctccaaactaaagttacttgagcaggagctactgaatttggaaaaaattgggaagactgatttatctaaggtaccatcatcaacgcggaagcaagtgaagagataccaagctctagctggcaagattgatgatttatgcagaagaatggtaattactgcatctctgcaagcttattggttataactttagtatatggatttcaaagcttgttacatgcatgcttaggtttctctaagaatggacaatagtcttgattacatctgctaactcaaatatttagatgttgggttatactcttagcttgcacgactaggccttacaattagctttttacctaacacaaacatacatctgataatgatctccctccctcttagcagcaggccagtgatccttgcgaatcaaacctgagtcctgagttccggacccaaagacagaccgagtttttgcttgaagcatttcgacttcagcagcgtgcatctgaaactgcacagaagctgatggtactacaaactgacagtggaaaaagttattacggggacgaatttgaagggcaagcccaactagccactaaacgatcctttgactccatccggaacaacttaaaagaaatccaacggaatttagagatatggcttgccagaattattggggatctggagggaatcctttctcgagatggtgcttctcgtgtaagggattattacatatctagatatccttttgttcaatagttatgtcttaacatgctcagtaaaatcatgattgaaaaaatgatgtataggtccttcctgttatgttaacaagatagctccagctgaatgaacaatatgaggttgataagtccatttatgcacataaatctgcttcacagaagcaaactattaatgctaactagtactttaaagagtgaagatttttgacagaattattgctggatgtcactgttcctgatctggatgcttgtcatttactagttttacttggtcccggtctttctggattaaaaagttgaaaggatggtgtggccctttgcaactggataaatgtcatgtctacacaaatctggcaaacattaaatatttgtggaccaagtttacagccccatttgatttgaaatcagattgattttaagttgatatttgttttgatttggattcttaagctgtattgattattcttaagcttagcaaatgagcaaatcatattttcatgaataagatatcaaaatattctaggaagttgaattaacaagttatatagcttcatgttactttttttataaataaatatttgtaattatatgttattataaactttcaaatatgttcaataaaccaaacaacagtaatactttcttttgataaaagttattcgcttggtacaaacaatttcttccgctagattttcttttttaaattttaaaattatgggtcttttcttgtaaaaattaggtttctttttctcacctaacctagtcgtggacatgagttcataagttgaataatctctaactaaaaggatagtcaaggatgtgccaccgtcgaacaagaaggatagttaaggacactctcaagcaaaggccagtagcatgtactctaaatttagtcaaagttccaatacaagctttttgagcgccactgtgactttgataggtggaaaaataattaaaatttatctttaatatataatactcccttcattttaccacaatacctattaattgatgtaatggcctgaggttataacttttaaccatctctgttctatttatgtcaagaagtgcaatcaggttttgaaccaagtagctaatcactcaatataaagaaaccaaattcaaacttttttaggggtttattatagaaggttcagacatacttatagcagtaattttttttcctagccaggaaaaggcatacacctgctgttacactaaaatcaaacaagccacataatccaattccaataacaatttaacaacatagatagatgagccttatgctgaagcagcaccttcttccagcaactgtttcaccttggtgatgtagtcgttcatggcttcatcggtggattttcctgtcatagatgcatgcagtgcaattagttgtgtttctcatacaaccaagagaaaggaagtcaatctgaacactgttgttagatcacataccttcaacagccttccatgcatcccactttgctctgtctctcatgttgaaaatgccaggacggcctgcccataagaaagggcgtaagaacaaagtgtagctagtttgagacagcatgtacatatgcataagacatttcaagcattatactcacttgtgttgacactgccaacggtggcttgcttgtaaagtccgtaaagaataagcttgttctcattggtggtactctcaggcaatgtcttagctttctcagcatgtgcttcaaattcctcctgaaacccaaatagttcagtaaaaaggtgtggtagctgaagttacaaagataaatttccaggtatactttcttagtgataaaataaggatgagaatccaacttaatagttgagatcgaaactatttgtgaattaagagggaactgaacttatggaaatctaaaatacaaattgagtgttccttcattgggtaaatgaaaagtttgcagttcaggatatcaaatatgtacgaattcattgatggactttagcacaagtgtacgcttagcctagcggtgaaaagggttcattctatttagccaacccgagttcaattctcgctttattttattttataacttgaatccgcttcgtgaaaatcctaggtccgccactggttagtgaaagagtatttgcaagaatgttagacaagaaaagcacaacaatacattcctcaacattgtaagagattctgctggccaacattttgctttgacaatgttaagacgcaaattttagacacatgtgttaatcatacaattctccaaccttttcctcttctagaaatgcttctatttacagatcacagtgaagcaccaaaaacatcctcagataatgtattatgacctcttcagtttgtttactggtttgccctgtttgttaccctacgattcaaccattaccactcagtagcctacatacttgtggtaacaggaatccttttagtgcgaggcgattggccaaccaacaatttttgtagtcacttaaaaataggtcagactaaattacatccactataggttatgaacagcagagaaatttcaaagacaggctgaacacaaagtgcacatttccttcaacttttccccttccccaataaaagaaatatggaagggtgatgataggtttttgaccaggaaacaaaaactagtcttggactaggcaatacaggataggaaagagaaagaagcgggcgctatctcatattcaatttttgctagactatttacacagaagttggccaatgtagcaccatataaatttgagaaagagccatttgttcactactaacattttgatggccctaactgcacatgaactaatagtaatctgattctaacatctcgttccctgggtttagtcatcgacttaagcttcaaagtatacaccatatatatagccaataatatcaacaatctcaaaaactaaaagaagaagacattcataagatgaaatcttcaaaacattgttgaaattatggactacttctgggccagagacaatatatatgccttttgataaggccaaaaatgacatacacaaatccggaccaaagtactactcatctgccattacattcgcactacttcttatcgaattcagtgcttacattgctataattaccataaatctttcaacaaggccaaaaatgtacagcataattgaattcattataagatctatttataagatggtatgccgccactcaaccacagtatgaactgctaaaaaaaaaataatcttaaacatcaattacaccaacagatcagatcaatccaatcaccgagccttcacactaaataataaccaaacaatcctcacgtaacacagcatccacaaaattacagcacaagctgcacaatcgacaaagaaaactaacagatccgcaaataccaattgcacaaacaacacaaaacccagaattgaaaacgaacattaatcacagaaaaatacttttcactgtcaaaaaagattaacactcgcttcaaacaagataaatacatactgaaaggcaaaaaaaaaacagaaatctaaaggggttttaaagaatttaccttcaacgccattgttgtggaaatctgatctggttagcttgataaaaacgagagaaaactggagatgtgattgtgatggagattgaagaagaagggtgggtatatatatatagtggagtatttagcataggaattaacgtaaaattcgattcgattatgataatctaaacaagttgcacttggatcacttactagtcatagtggacccaaaaattgagtatagattatggacctatactatgtgagctccacaac

SEQ ID NO: 2 - DNA, 15891 bp, Solanum habrochaites
  >Genomic fragment 2
tctgtggtttgatgctttcaaatcacagcaatcctctgtataattatggtttatattttaggggttttcagtttacaaagtcattttatccttccaatcaccaaaagtattatcttggctctagtgactagtaacaagttagttttgtgttatgtggaaatttacaacagatcaccttcatactgaggagggagatgatcattttgtcgtggctcggcccgtctgtcttttagccaaatgctgcgggagagagtgggattataacagtaagtattttgtgttttaatactgcttctatcagctaatgtttcatagaaatgacagtgtgaatgaaattgcaaattttgtgtggtaaatagtttcaggctccaatctagtgatcattttttctgggtaatcagttaacaagatctctttaagcattcaaatttatgtatggtaggtaagtgcacatcatgttaggaccgaaaataagcgggtgtaaatgcggaagctagcaaagcaaacctcgaaagatcacgagtaagaagataacgagaaatataccaaaagacacaaagatttaacgtggttcggtcaattgacctacgtccacaaaggagatgagcaatccactataaatatgagagtacaaaatatagagagaaacaacctcaaccaattcactcggaatacatgggaggttcacacaagtgataacgtatcaagcttgtgacccacaaattctccctctaaccaaaactctcaaaactctttaagactacattgtgaatgctgattaagttagaaggaacatgtctctatttatagagtcctaaactttttcatactagaaaaaagattagtcaattcaaaaccttttcctaaaaggaaaacctatttatggtaagaaatcagggcaaataaaacccaacacatcatggtttgaaccgtactacataagaaaagttctagtatttaaattgagaaggatagaggggaggggcctatccttaaatctgttaaagttttacgtactagcccaactatttgtgcgcgtgaagaaaagatgtgacagctccactatagatttcagcactaccatttagtttgttacaacattttgctgaaattgagttaggatcttcttgagtcgcagagtaatatcttccatgcgaattctctcttcaggcaaatcatttgtacattcaagagctaattccatgattgatttgaagcatctatctttagaagtaaaattttcttcgttcagtgaaaatagattaatgtccactacatccaccaatcggtctggtaatgattggcatatccatcttttcaaggtgaagtctccaacgaatagatcatccacagggctctttcttgtaaaagtctccattaacaatataccaaagctataaacatctcccgaagttgatactttgccttcagacccatactctacaaaaaaaataaatcacgccatcattaatgaaaataattaacaacatttaaaatcctcaagtgaacttgataataacatttacctggtgccatgtagccgatagtacccaaagtcttggtatgtgctattagcgtctcagatgtaagaagtttggatatcccaaaatcactcacttttgccaccatatcttcatccaaaagtatgttacttggtttcaaatcacaatggacgactacaaacaaatgtcctccatgtaaatactccacagcagaagccacatcaatcatcacctttagtctttgagttatatccaaaactttgtcagtagagtgaagccaacattcgaggttttcattaggcatgtactctagcaccaacactttataatcgaaatttgcacaactacttatcaccttaacaaggtttctgtgtcgaatgctacctaaaacttgacattccacctcgaaacttctaaatgcaagttgcagttctgtattgaatacctttatcgccacaaccattccatctgctagtgtccctttatacaccaaaccaaggctcccccttccaatcaagtttgcttcatcaaagttgtttgtcccttgagaaatatcatagtacgaaatcctcttatgtacctgaccaaatgtatcaactagaggaagttccgtactcctttttcggcatttcagaaaccaaatgataaaaatggttgtgactacaattcctgaggaaactgatgcaagaacagaagttaggactctgttctttctttttctttcaagacttgtcactctgcattgcatcacatggaagcgtgatgatccacataatgcagggttacccatgaatgattcagctgtaaaatttacgaatggccctccatctggaatttcacccatgagcccattgaacgagacattgaaatgcatgagatgttcaagattcctcaaggacttggggatcatgcctgatagattgttgctagatagatccaaatattccaacgaaaccaaatcttcaaatacttcaggtatggaaccatctaacatattctttgacaatgaaaggctaaccaagctttgtagttggccaatcgtgctaggaatctgaccagagaactgattaccatgtaaatgtaatatccgcaaactccttaaattccccatttctactgcaagagacccattcagcaaattggaggccaaagtgagaattgaaatatctttgttcctccaaaaagttgatggaatatgggaaattagtgcattggaatctaagtagagttctcttaaagatgaaagatttccaaaacaatttggtaattcaccagtaagttgatttttccccaagataatttggtacaagttttccatgttacacaagctagttggtataattccatctaaattgtttttctctaggctaaatcttttcaacttcctcaagttccccaaatctggaggaatagatcctataagtttattgtctcccaagcttaaccactccaggttcctaaagttactgatgttaggtggtatttttcctgtgataccattttgaagggcaatgaaatattcaagggaaaaggaccagtttcctgaacctaaagatgttggaagacttccattaaattggttacctcctatttgaacggttttcatatacttgcaattagataatgaagtcaggaaacttaactcgcctgtagattgatcattcgtcaattggtttatttgcaagttgatgaattgtagctgttgtagctttccaagattcataggtacaggtccactaaacagattgcggccaaaatcaagctggataagcatggtggaattcacaatggaggtaggaatcagcccggtgaactggttatccccaaggtaaaggccttcaaggtttggaagagtatggcctatgtttgagggaagtgttcctgaaagctcatttgctacaaatgaaatcttttttagtccagaaatgttgtacaaacgccttggaacttcacccgataatctgtttggaccaagatacacttctttcaaatttacaagatgttcaaactcctgaggaattccaccatataaactgttgtcacctaggtctatcatctctagatttgacaaatttccaattgatggtggaagaattcccaccaaattgttccgtcgtagacttaatcttcgaattgctgataggttatcgatttcacttggtatatgtcctgtaaaatatatgtcgaattgtgtggttactacactgaaatgtccaatactgtataacagctttatagtcactaagttactataaataacagaaactgttagttgtatgccttttaaatagttcagcaatcctcacaaactgttttgatgtccttttgaagatgggactaaatggatcaacatggataattaggattcatatagcagacacaaactagaattgagccaatgtagtagttactgttgttgtttgaaaatgaagaacaaagagctataccaacattttttgctactaccctttgaaatgcaaatactaatttcttataaatgagttgaagagcaagtttttaaatatcaaagatctctagtgctacaaggtgagaagtccagcaataaagttaggtggattcagttaaaccagaacattataaatacctgttatgttattccatccaagaaatagatgttgaagttttgtcaagttccacatgtctctaggcaagtttcctgtaataggatattacgataagttatatgtacctctcacggcctatgattgtttaactaaaaaattgttgcaatctttgttgtcaatatgaaccaaaagtagcagagaaagaagttggttccgtttttttttacctgtgaagtggttatatgacaaggacaaatatattagctctttgcatttgtctaaattgcttggtagttggccagagagttgatttcttgctatttgtaatccctccagccgcggaagattatggcaaatgtcattcggcaaagtcccagatagtgcattataaatcaaattgatgaccttcaaagaagagacattgaagatagacgaaggaacagatccaaagagatcattttcagaaagatccaacaactcgagccttctcagtaatccaagactttctggaatttgacctgtgagattattcattgacaaggacaagtgcttcagcctcctcaaatagccgagttcatcagggatttcaccgttgatgctgttgttgccaatgtccaagaaactaagaaaggagaggttcccaatatctgtcgcgattgaacctcttagtctgagaccattgaggtctagtgatgtcactctttgatgccttttactgcaagatatgcctatccaattgcaaacgtgagtcccctttgtccagtttttcgacaacattccatttggatctgaagttatatgagctttgaaagctaaaagagcagcctcatcagttgaaatgttcgatgcattagtattcgagaggtacgttaacaaaactagcaatcctataatcatagccacggaaaccgttttgtgcaacttctcttgcagctatttgtgggggaaatttataagtgcctgattttttatttttcaagtgacattaatatatatttctataattaaaggcaataaagaatcatgtattagcactggaatatatagaatctagagttcaatgtcaatgatcaacatatatacgtaatatgttttgagacatttttttttaaattgaatgttgctgaacttgactgcaattcattgctgaagggaaatcattggttgtgggattctgtagtgatagtaaaataatttacttggatttataagccttgtatattcattattcaagaatattaaagactaaaatcatgatataatgtcatcattcgaatgtatatagcctccgctgaatagatgtttgacaaaagaacgtgaagtgttacggtcaaattagtgaatctaacgtgtaatgttggatttacgtgaattcaatagcttttattcctatcttttatatatattaagtaatttattaaaaatctaaaattatcgtatattactatcttgcagtctgtgtgagaatactattttgataatcgtcaaataattatctataaatttcaaatcttgaatcacacttatttaataggaggaaatggtaaaaaggaagtgaggttgacaagatctcaagactctttcttaattttgatgaaatgttgtaaaaacttgaattagtagattgcatggcatcactatacacgtgtcagtctagtgtttagagaaatttaatcaaagaatataagttataatatatattatccatgagaatcttgagaaagattttctgtatctgtctgatgaaatagaaattggagtttcccaattctatattacttggcttattctaacttctagtgcagaatctgcagatggtcaatattctttgaatatataatagcaaatttgattattagtttcatttttaaactattgatagttttaaaaatatttattatttaactaattaaatttaaatatatcctcgatcttgcaatatgagagaaatacatctctaaattctttccttttcaacatttctttcgtttttctaattaaaagcctcatacttatacaagagtttgaaaccacttgatatgtcacgtgacaaaaaagaattgtatctaagtttggctactcatgtagagaagtatttttaaagcggtcaatatctcaaaagagaaacaaataaattatgtatctacaaattataaaaaaaggagtctacctttattgggaaagtcatatgcaattcatgtatgctttcctaattggggatacaaagtcaatcttgttaaacccctaaactattacaatcattttaagaattatatatatatgtactatttgagtgttgacaaaagccttaaattatcataaaactcatattaaaatatctcttagagtaatatgacatgtcatgtgaatattatgtttgacaaactcaatttcaaagagttcaaagtggttatacacgtaggttttagaaaaattctaaactcactgttttgtgactttcatacctaaaattgttaggtgtttatataaccacccctgaattataccatgaaattattgtgccaggtggcctaatttgaaatttaatagggctgaattaagatttttgaagtcaattaaagaaaatatttttttaatttatcctgaataagcttgctatttgaggggtttgagaaatatcggtagggcggtacatgggctaataaaattgattaaaaatataatatgatattaaatttaaaattaaagagaatccaaactcaaaacaattaggttaatatttctatttagctatttatctttgttatcttgaaaaaaacttaataaatattataaagataattttatttgtggatttgattaacaagtagtaacattaacatcatgtaatattgttttgtggatatttttcgataatattttttaaattataatttataatttaatttaataattataaaaaaataaaaaaaaagtgggccacggcaagttctgtagctctcacgtacttatgggttggaccgacccattttctgacccatacaaaaaatgagctagcctagcttaacccataaaatatcaaaacatgtatggattagcccaggatgagatatgttagcccatattgacagctctattcccacatcaacaaggtatttaatatgtcaacttgaaaagaaaagatattccaaaattaatctgcttatactctatcaattccatatctcacttagtgaaatttcgcagaatatatcgttgaatatattgttgttgtcgttgtcctctcccatcattctaaatttaaagaacatgcaatgtaagaggtaatttagaaaacttagttcggccgtagaagaaggatcatctgtaaatttattcctctgcaagttgatgctctgttggaaatttattactacaagatagattggttaatttgaccgtaaaacagttgacattcttttgtcaaggatctattctggggaggttatagatatacatttgaataatgacattgtcaagtaaattatttaactgtcaatacagaattccacaaccaatggtttatttccctttagcaatgaattgcagtcaagttcagctagcaatatacgattaaaagttgtttcaaatcattggtattaattagataagtattgactcaattacaagtatacacacagtatatatagaatggcgtttgaaaacgaaaacataggcacaaatagcagctaaagaagttgaacaaatccaaatggttgcgaagactattattatagcatgcctagttttgttagcatgcctctcagttactaatgcatcaaacattacaactgatgaggcttctcttttagctttcaaagctcatataacttcagatcccaatgaaatgttgtcgaaaaactggacaaaaggaactcacatttgcaattggataggcatatcttgcagtaaaaagcatcaaagagtgacatcattagtcctcaaaggtttaaataaatgcaccaaacttgaagttctgtccttgtcttataacaaattcactggtaattaactaacttgtaaacttttcatttactaatttcttcttgaattaatcatcatttttgtgtgtgtctgtcattttataattgataggaaatttaccaagagacatgtggaacatgtcaaaggttcaagaactgtttattggatggaataactttacaggtacgtgattcttgtatgtattaaatcttgaatactcttcacgaagttcctaatttcactagatatagtcaatttgtgcattgtctagtaacaaacaaagattaatatatgttgtggagaacattttcgaaagacactctatgtctgatctttagcatgataaccatgtacttattttcaaaatgaatttgcaggaaatataccaaatgaaatgaacctaccatctatttgcaggaaagttaacaaagcttgagcatctcaactatctgaaagtctcttacaatgagttatcaggtgaaataccagatggagggccttttggtaattttcacagctgaatcattcatcggcaacgaagagttatgtggaccgcctagattccaagtcaaggtgtgtgaaatccagaacaacgtgacaagaagaaacaggaagaaaacagtactaaaatttgttcttggaccagttgcagctggaggtttagtcataggggttttaggcatgatatggttgttgaattatcggagacgtaacaaccaacttattcctttaactgattggtatgatcagttatcacacaaaaggttttcttactatgaacttgttcgagggactaacaactttgacgaatcaaatttgattggaaagggaagccttggtatggtttataaggggacatttacaaatgggaccatagctgctgtaaaggttttcaatgcacaactgcaagatgcattcaagaggtttgatttggagtgtaaggttttgcgtaacactcgaaataggaatcttgttaaggtgataagtagttgtgcaaatcttgattttaaggcattggtgtttgagtacatgcctaatggagatcttgattattggctttactcacacaacaatttcttggatttaaacaagaggctgaaaattatgtttgatgtggcttgtgtcgtagagtatctacaccaaggccattcacttgtagtggtccattgcgacttgaacatacttttggatgaagacatggttgccagagtaagtgattttggtatatccaaactcttgaccgcgtatgatccagtggcattgacaaagactttaggcaccattggctacacggcagcaggtactgatcaaacttttatttactaattactttcttcaacttgtattcgatatgcatatatgatgtatttcattttaatggcagagtagggatagtgtcaactatgggggatgtttacagctacggcattttattgatggaaaccttcacaagaaagaaaccagtagatgatgagtttgttggagaccttacattgaagagatgggtcgcggaatcatatcctcatagagtcattgttatgaaataaaaacgaatacacgctgaacgtcacttatgagtcatttatctaatatgatccattaacaattgattaatgtaacgcaaggaagaagaaaacaatttgcattgttatgaatgaatgtgtttgtactacaatatatacagtactgacaagtccagcaaactttctaaccaacttattctaaccaactctactcattattaatttagctcacttaatcaagaaattaaacttaacaactaactaccattactcattcaactgatcacggaacatcaacacattttgttgatttctttcacacacaccctctgcttcgaaaacccctctttttaacatgtaagcgacaatatcttttttttaggagagtgttcaacattgagcataaaaataataaaatagagaacaaaaaagatgagtataaaataaataataatataagatcgattttaccgattgtcaattttgtgtatggactaaagaaataacagcttcacatatctaatattaaatgtaatactgaatttcacatatggtcagaggtgaatccacctgcacccgatatattcttttttaaaaaaattatatgtatatatatagattgttgataagacggtaatatatttaattgtgcactcttataacgaacaaatgatttgacttgtccattggaaaaacgaaaagtgtcacataaattgagacatggggagtaacatttctttcttaaatttttcgtgtgaagtcaaactaattcatataaaatgagacggaaggagtactgtttaatattaattgcatatggtagtaaatttgatagacatggtcccgtgggagtgtgtgttatttccattgaataattgagtttgtaattgttacaagtccattctaatttccaacaccttacttcatttcaaaaatatactctatggctgaagctttccttcaaattatgttagagaatctgacttgtttcatccaagggaacttggattgattcttggttttaaggatgagttcaaaaagcttcaaagcacgtttactacaatccaagctgtggtacaagatgctcagttgaagcaattgaaggacaaggcaattgaaaattggttgcagaaactcaatggtgctgcatatgaagctgatgacatcttggacgaatgtaaaactgaggcaccaattatacagaagaagaataaatatgggtgttatcatccaaacgttatcactttccgtcacaagattgggaaacggatgaaaaagattatggagaaactagatgcaattgcagcggaacgaattaagtttcatttggatgaaaggactatagagagacaagttgctatacgccaaacaggtaaatatttttctaaataacagctttatatcatcaaattcatgtgtgttttggggattttgtctaagtagataagtggttcaaaatctattatctaaatctgtttggtgaagtctttaacatatatataaatccatagcttactcatatgccccaaagtctaaatgacaggataaagccagagttgttttagattttataaattaacaaagataataatgtaaattcaaaatagtgcatttgttttatatttgaaatatgtctgctgcttctgatcaagctgatcattgtcttttgcaaaattcttctttgttttttttgctgactcttaccgatcttggaccaggttttgttttaaatgaaccacaagtttatggaagagacaaagataaggatgagatagtgaaaatcctgataaacaatgcccaaacactttcagtcctcccaatacttggtatggggggactaggaaagacgacccttgcccaaatggtcttcaatgatcagagagtaattgagcatttccatcccaaaatatggatttgtgtctcggaagatttaatgaaaagaggttgataaaggaaattgtagaatctattgaagaaaagtcacttggtgacatggacttggctccacttcaaaagaagcttcgggacttgttgaatggaaaaagatacttgcttgtcttggatgatgtttggaatgaagatcaagataagtgggctaagttaagacaagtcttgaaggttggagcaagtggtgcttctgttctaaccactactcgtcttgaaaaggttggatcaattatggcaacattgcaaccatatgaattgtcaaacttttctcaagaagattgttggttgttgttcatgcaacgtgcatttgggcactaagaagaaataaatcttaatcttgtggctatcggaaaggtgattgtgagaaaatgtggtggtgtgcctctagcagctaaaactcttggaggtattttgcgcttcaagagagaagaaagacagtgggaacatgtgagagatagtgagatttggaaattgcctcaagaagaaagttctattctgcctgccctgagacttagttaccatcaccttccacttgatttgagacaatgcttttcatattgtgcagtattcccaaaggataccaaaatggaaaaggaaaatctaatctctctgtggatggcacatggttttcttttatcaaaaggaaacttggagctagaggatgtaggtaatgaagtatggaatgaattatacttgaggtcttttttccaagagattgaagttaaatatgatcgaacttatttcaagatgcatgatctcattcatgatttggcaacatctctattttcagcaagcacatcaagcagcaatatccgagaaataaatgtagaaggttacctacatatgatgtcgattggtttcgcaaaagtggtgtcttcttactctcctcctcacttgcaaaagtttgtctcattgagggttcttaatctaagttccatgggacttaagcagttaccgtcctccattggagatctagtacatttaagatacttgaacctctctctcaataacatgcgtactcttccaaagcagttatgcaagcttcaaaatctgcagactcttaatgtagagtattgctggtcactttgttgtttgccaaaagaaacaagtaaacttggtagtctccgaaatctcttacttgatggttgcgatggattggattctatgccaccaaggataggatctttgacatgccttaagactctaagtttctttgttattggcgagagaaaagattctctacttggtgaattacgaaacctgaatttgtatgggtcagttgaaatcacgcatcttgagagagtgaagaatgatagggatgcaaaagaagccaatttatctgcaaaagaaaatctgcattctttaagcatgagatggaaaaaaccacatagatatgaatcagaagaagttgaagtgcttgaatccctcaaaccacaccctaatttgacttctttactaatcactggcttcagaggattccgtcttccaaagtggatgaatcactcagttttgaaaaatgttgtctctattgcaattagaggttgtgaaaactgctcatgcttaccaccgtttggtgatctgccttgtcttgaaagtctagagttaggagatgggtctgcggaactgaagtatgttgaagattctggattccctacaagaagaaggtttccatctctgagaaaacttattatagtcaattttgataatctgaaaggattgttgaaagaggcaggagaagagcaattccccgtgcttgaagagatgacaattagctggtgtcctgtgcttgttattccgaccctttcttctgtcaagaaattggtagtttatcggaacatgtcagatgcaataggtttgaggtccatatataatcttagggctcttacttccctcaacattagccataacttgacagctacttcgctcccagaagagatgttcaaaagccttgcaaatctcaaatacttggaaatctctttcatcttcaatctcaaagagctgccaaacagcctggctagtctcaatgctttgaagcatctgaaaattgaatattgtgacgcactcgagagtctccccgaggaaggggtgaaaggtttaacttcactcacagaattatccataacaaattgtaagaggctaaaatgtttaccggagggattgcagcacctaacaaatttatcagttagggaatgtccaacactggccaagcggtgtgagaagggaataggacaagactggtacaaaattgctcacattcctcatctgcttattactaatgagatgtaattttctgatttttcttttggaaacaaatcaactatttgtaaccaattcgtattggacttttgagccctgcatttgttcgaatacgcctttcaacctgtatatcagtgtataacaaatgtatacaatatgtatactgctgctcaaatctgcagatttgattttccagcaacacatttgctgattcttccgacctgtaaattaatttccagcagctcatttttttgtgttcaacctgtacgccagttgtgagggtctaagacttgaggaggaggtttgagcctttacggctcagcgaggaagtgcagggatacgggcgaaatccgttaggactcatggcgaatgcacgtgaaacggatcaaaaggaaacataaagaaaaacagtcaacgatgaaaacaattctgcatttatacgcataactaaggcaatgtaaatcaaattgaagaatgggcagccaagataaatgaaagcaaataaagccacaatgcatgttttaaaatactataaccctgccatgctgcatagacacacatttatattcaagattcaagtcataacaaaatataatttgaaagtttaaagctctggatatcagcttactacagttcaatcttcttacttaaaaaagatgctaaaaaaaaacaaaattcaactcttccaggcaactaacaatatcaaacctacaaactaacatatgagcaaaaaaaaatcattgaaataaaggcatacaaatactaaaatgacaaccactagttcatgaaaaacaaaatggagcaggcaataaataataaacaagataatagataaatatgtcttttaattttattttattttatatttgtatccttcaaatttgaatgtacacataatttgatattttaacttgtatataattgaacaagtacatagttaagtcatatgtagcataaatatatatatatatatatatatatatgaaacaccacctatgacacaatttccatgaagcatgtacacttttatttgttcatttcaatactgagtttaagtattttactttgtttcatattatagttgaacaccataaatataaaataatatcaaatttaaaaaatatatttatgtattatgctttaaaaaatattttttaaaaatctagtaattgccccaccataaaagagatgcccattatacgccgaaagaatgtttaaaatcaaaagcaactgttagttattggattgaaaaataaaaccaaatactccaattgagagacatggcggccccatggtggaataattattacaacacaccttccataattaaagtttgaccttacacctagagacaatcaaattttggatttgggtcttattttactagttaacatttcagataatcacttaattttaaataatttatttcgatagtcattcaactttgaattattctgttagaaagtcattcaattctattttaaagtcaaaagtcactaatatttgagttgttggtttaaaaggtcattcaactctctttataattcaaaagtaacataattattttttgtttcacttaaaagacatccgatcaacttaaatattttttcataaaatcttatttttatgttaaactattctttttaaaaataataagatatttattttagaaaaagggaaaatatgttaaaaagttagttattccaaaaaagaagaaagaagttggaattgaaaagaaataatataaaaaccgcagcacagtgccttttttcttattactttttatttaaaagatagttataaagaaatattatacttcaacaaaatttaataaaataattaaaagcagcttataattttattttatttttgtattcagtcaaatttaataaaaaatttcattttaaaataattgtctgactttctaagtaaaattagttgagtaatttttaggttataaaacaaaattgagtgactttcgaagttaactcaaatctgagtgactttctaagtgaattattcgaagttgagtgaatattaactccttatacaagttcgaggaagatattgaaaaagattgtacatatggggttc

SEQ ID NO: 3 - DNA, 85327 bp, Solanum habrochaites
  >genomic fragment 3
gtaagctccttcatgtcagcttataaaaggcttcacacaagtatatatagcgggtaaaattttattttgtgagaggtagaaatgttactcggcagacaatacttgtatgacatgcttaaagcttcatttttttctctttcacctatttctatcttcttcttctctctttttttctccgtgcttcataaaattttattttatttttcatcaaaaacttgatacttaatatattttattgaatgaaaattgatttaataattttatttttcaaatgttaaaatcaagacaaatcaattaagttgatttttttcattactttattttttttccttgcgatttgttttttgtggacttctcgaaaatatataataatataaaattatcctctgaaaaaattatgcattacgaagaatttaatcattactaagaaatttgataaaaaattcccaatgattttactatattcttacaaaaattaaagatttaaggctgatatattaaagatgtcttgttaatattttatttaaataaaataatcaattaaattacgagttattttgaacatgaaaaaacactttcaattttatctaaataaaaatataaattaaattacaaagtaaaaagaataattattataaagagaaacacatgagtactcacaaagagaacaaaaaaaatatttataataatttttttagcttcagagaaggttatacgtataatcaaaattattacggatcatttattaataaaataataaaataaaaattctcctaaaaaattaatgtatgatctttttataagcaaacacaaaaattatttaattacactatattaaatttctttaatctcactaaaaaactattttttctcgtttcatttactttaagttttccttaaataaataatataaaaataaaatagttaaacattgtggctaattttttttaaaaaaaacacaaaagactacaaaggagaacaagagaatgagaaacaaaagtttacgggaaaagagtctgatataccccttaactttgtcatttggagctaatatatccctcgttataaaagtggctcatatatgcccttaccgttatacaaacggctcatatatacccctgtcgttataaaatgactcacatatacccttaatttgtggaagttaaaaattagttttaaatttatatttaatacttctaatttttaaaaaaaattatttagaggtatatatgattcttctatcaaagttcaaggtatattttaatttttttttcatacataaactatttttgacttcttttattataattatttgagtttcttattcttattttatttttttttctttcattccttagtttaaagagagagaaaaattaaactattttttttgtatgtattgtaatttaatttcgtattcaaagaaaaaaatttagtcatctacaataagttttacaagaatattagtgaaaaaataaataaatttgattatcaaaataataattataaattagtcattgaaaaaaaaagtcaaaaaaaaatgtttttgagaattaaatttattcatatgagattatattttatagaaaaaataataaaaatttagattaaaattatattttttcatttccgttagattaaagggatatctcgagccatttgtttacaagtagggtatatatatgctactttcatgttaggtatatcagctctaaataacaaaattgatgggtatatcagacccttttctcaagtttaaattaatgtgaaaaagttttaagtgtgggtcccatgttgtacatttaaaattctcatacaacagacaaaaggttagcttttcacaaaataaaatttttcccatgtgaaactcaaaataaaataattgcgtacagacatatttatgcaacacaacattaatttatttatttacccattcaataagtaaaggaataattataaagctttgtgctcttacttttagctgttcatatttcattccaacatcgatcttatagatttattgctaattcacaacaattccagcaatctacatggctgaagctttccttcaaattttgttgaaaaatttgacttctttcatacaagaggaacttggattgttttttggttttaagaacgagtttgaaaatcttaaaagcacgtttactacgatccaagctgtgcttgaagatgctcaggagaagcaactgaaggacaagccactagaaaattggttgcagaaactcaatattgctgcatatgaagttgatgacatcttggatgaatgtcaaactgaggcagcaagactcaaagagactaaatatgggagttatcatccaaaggctatcgctttccgttacaagattgggaaaaggatgaaagagataatggagagactagatgcaattgctgcagaacgaagcaagtttcatttggaaaaaaggactacagagagagaagctgctagacgagaaacaggtgctcatctttaattagtttatattcatttttttgcgattatcaagttcatgtgtgtttatggacccaagggacttttttctaatctaatgtttgtctcaagtctaaacagatttgtaattctaccacttatttatttagtgaagttcttaaacatatatacatggtgtaagccagctcagataaatccatagtcagttgtttcggactgaacttaacttggatgtcaatttttcaaagtcaatcatgttttcaactcctccccctgattctcatctctttgtagtgcaaaaatcttctctctgtttttcgctaaacatattctcgtgtgaacatatattgcttgaaacaggttttgttttaactgaaccagaaccttatggaagagacaaagaagaagatgagatagtgaaaatcctgataaacaatgcccaacaactttcggtcctcccaatacttggtatgggggggctaggaaaatcgactcttgcccagatggtcttcaatgatcagagagtaactgaccatttccatcccaaaatatggatttgtgtctcagaagattttgatgagaagaagttgataaaggcaattgttgaatctatcgaaggaaacccacttggtgaccacatggatttggctccacttcaaaagaagcttcaggacatgttgaatggaaagagatactttctcgttttggatgatgtttggaatgaaaatcaagaaaagtgggataagataaaagcagtcttagaggttggagcacgaggtgcttctgttctaaccaccactcgtcttaaaaggttggatcaattatgggaactttgcaaccatatgaattgtcaaatctgtctcaagaagattgttggttgttgttcatgaaacgtgcatttgagaaccaagaaaaaaataaatcctaaccttgtggctatcggaaaggagattgtcaaaaaaagtggtggtgtgcctctagccgccaagactcttggaggtcttttgcgcttcgtggatcaagaaagagaatgggaacatgtgagagataatgagatttggaatctgcctcaagatgaaagttctattctgcctgccctgagacttagttatcatcatcttccagttgatttgacacaaagttttgcatattgtgcagtattcccaaaggacacggtaatggaaaaaggaaatctaatctctctctggatggcacacggttttcttttatcgaaaggaaacttggagctagaggatgtaggtaatcaagtatggaatgaattatatttaaggtcttttttccaagagattgaagttaaagatggtaaaacttatttcaagatgcatgatctcatccatgatttggcaacatctctattttcggcaagagcatcaagcaacaatatccgtgaaataaatgtaaaacggaacccacatatgatgtcgattggttttgcaaaagtggtgtcttcttactctccttctcacttgcaaaagtttgtgtcgttgagggtgcttaatctaagtgaattaagacttaagcatttaccgtcttccattggagatctagtacatttaagatacttgaacctctaccgcaataacatgcgtagtcttccaaagcagttatgcaagcttcaaaatctacagactcttgatctacagtattgcgccttactttcgtgtttgccaaatcaaacaagtcaacttagcagtgtcagaaatcttttacttcatggttgctataaattgaattctatgccaccaaggataggatctttgacatgccttaacactcttggttgctttgctgtgggaaggaagaaaagttgtcaacttggtgaattacgaaacttgaatctctatggctcaattcaaatcacacatcttgagagactgaagaatgatagggatgtaaaagaagccaatttatctgcaaaagaaaatctgcattctttaagcatgacttggaaaggaccacatagatatgaattagaagaagttgaagtgcttgaagccctcaaaccacactccaatgtgacttgcttaacaatccatggcttcagaggaatccgtttcccagagtggatgaatcactcagttttgaaaaatgttgtctctattgatatccggggttgcgaaaactgctcgtgcttaccaccctttggtgagctgccttgtctaaaaagtcttaagttacaggacgggtctgcggaaatggagcatgttgattctggattccctacaagaaggaggtttccatctctgagaaatcttattatagtcaattttgataatctgaaaggattgctgaaagaggcaggagaagagcaattccccgtgcttgaagagatggatatttggtggttccctgtgtttgttattccgaccctttcttctgtcaagaaattgttagttcattggaacatgtcagatgcaataggtttgagttccatatcaaatctcagggctcttacttcactccacattagaactaacttcatagctacttcgctcccagaagagatgttcaaaagccttgcaaatctcaaatacttgaaaatctctttcttctacaatctcaaagagctgccaaacagcctggctagtctcaatgctttgaagcatctggagatgaattgttgtcccaaactggagagtctccccgaggaaggggtgaaaggtttaacttcactcacacagttatccattacatactgtgagatgctaaaatgtttaccagagggattgcagcaactcacaaatttatcaattaagaattgtccaacactggccaagaggtgtgagaagggaataggacaagactggtacaaaattgctcacattcctcatctgcttattactaatgagatgtaattttctgattttcttttggaaacaaatcaactatttgtaaaatctatttgtattatacttgatttttcttggttatgtaacaataaatatttgaaaattttcatataaaaatagttacatttctatatgtataattcgccagaataatacatatatatgtataatatacaattatttaaccgatatacatatataattcacctctctcccactctctgtcctctctcactcgcctctctcctccctctctcaatttcgctttccatatatacaaatacaattatctaaaagatatatatatatatatgcaattcatctctctcccactctttgcttcacttgacaactatgacatttaacattggacaagcacaaattgacacttaaaaactggttacagaaactcaacgctgctgcgtataaagttgatgacttattgaatgaatgagaatacgaggcagcaagactaaagcagtctcgactaggacggtatcatccaaaggctatcaatacaaactcagttgtttagaccacgaaaagactgtgaattcaatacaggagtagttaacgattactctaattctatgtcacagaaagtaatttcataagcgagaaaatcctctagcatttttccatttctctttatggcgtgcaaatatcgttatctattttctgctgtctcctagctaattatcttgaatgtacgtaacactctctatttatttccaagagattgaactaaaatctggtaaaacttatgatctctgttttcagcaaacacatcaagcagcaatatctgcgaaattaaacacatatgatgatgtcttcttactcaccgagttattagttatgctaaaatgtttacccgagggattgcagcacctaacaaatctcacaatttttttttattagtgaaagcatagttatcaaaataaaaacaaaaaatgagcaatatttatacaacagacaaaaaaaagaatgatttttcatattctttgcttatgttaccgattcataacccatataaaaacaaatttcaatcacccattaaaccaaaaatgattaaacaaaaaaaatcttctagatatctaactaatgaataataacatattcagtgtagtcccacaagtggaatctgggttaactatccaactaatcatagatcaaaattgcagtgaaaggtattttattagaccacttccaatctcaactatttcaacacaaaacttatattcaatctttgatggataatagaccatctatttttaattcccttttctcaccaacaaattgaaatgtcagtgatgtttctgagcaacaaaaagtactttaagatgatattctaaatgtgcacaatttcatgctccaacaatcgaccaattagattaaaaaatatactcattgagtatttcttctgtcacatggtcaataccatagaaaatgaaaaatataatcacaatttaacaacataactattgagatggaatatgtttcatctagttaaaaaaaatttacttgagaatgttgtttgtgagcattacactaatagacgtcagatgattttcggatggtggtcaaatgacacttgttactggttcaagcagagtaatgggatgtgaaattgcccttcaatcgtagaaaatggaatatataaagcaaagttacacaatttaatcgtactcttgaaacttatctctctataatccatgtttgctataaacaataatattgtcttacacatattcaacaattacatatcctatttaaactaatatacgaaatatattcaataaaaagtgcatgcagacgatttttctacaataaagactccaggtttagagtgtttagcgactcctgataaagacaatgagattatagtaaacaggagaaacagagcagctcttcataaataaagaggaggaaaaaatctaccgattgatgcacgtaaaagagtaaatgtgagactaatgacaataacctgttgttggagagatttatatagatgagtatttgaaaagtttacgatcaaatgaacttgagcgtcagaaaagttgtcgcttgagcagtaactgttatagtgatcaatgaggcattttttggagaattaaattaggtctcaaactatgagcaaatttaatttataataaattaatacttattaaaactgtagggttaaaacggtaaatcaagtttatgattaaactcttcccacttataataatataagattaaaaataatcataaaatagaatggtgcattggtatcaaacaagaaatatgtgaaactaattaagagaatatagtctctaagggtatgaatatatcgatgaatgcttgattgaaaaataataataaatgtatataagtctttaatgaaataacaaaggcacgagataaatttattagaaatataaatctacatattctaggtattacaaaaaagatcctaaaatatgtagcaaacaaatgacttattcttctataaagcacgtaaccatcgaagtttaatgttaatacgataagattgccttgagaatgcatttacttgtgataagtccacgggtctacgtataagtatagtttattgtattcttataaaataatagtaaaaataatagtctctttttatttcaaatttaatttttaataaacagaaaataaattaataaaataagacaaaaaacaataataatattatagacatgtttatgatgagtacgtataatttgaaggggaaaactacaaattcaaactcaagagaaaataataaaggtttggaataaaatatctaagatacggaaagattaaaatgtgttctctaactaaaatcttcatcttcatgaataattaacatgaaaatagaggatccaccaaaaattaaataggagaaggaaagagacttattagaaaaatgatgaattataaaatctaaaagcctatatgtgaaaataagagaacaagaatattgcataaaaaaaaattatagctacgaaaaatactatgtgtgattttaaagataaaatctattttattgttacatgtatcatatttattgttgaaatttcaccttttaaaaaatgaaaaacaagctaagaaaaaaaaagtaaaaagaggaaaatgaacaaataaaagattaatagagaaaagggaaaaataccaatgaatatcctgattgaaactgcattatataaatcttcggatcaatccatttaccttgaatttcaagaacactgcaaattcgatcataaattaatctaaaaagaggcatgtttatgataaaaggggggaaaacagtgttagaagaaaacaataaagaaatagtgttagaagtttgaaatcttcatgtttcaaaaaagaacaaattaatcttcaatgtcaagtaaaatctcaagatctctagtaaagaaaatttatttttatactacaaacaaattaatggcattttaaacatataaagaaatatgaggatcaacatattatagattaactacaagttttcatgtccttaaaagataacttatcaaccacaaacaaaagtaaattgaagggcaagagatgaagaagtcttcagtttgttaacttaattggtgtttctatcttccatgtcttttgaaatgtgtatgaagatgaaatgtttcaagtacttgaagatgaaatatagtttcttacttggatgcttaacaatgttattacttcaaaaagaacctgaaaaaaatcattattcacttggttgcttaactattctattacttcaaaagatttattactttcaattggcttttcacttaccctattcatggtgattaatatgtaagtttcatgcaatgtcttttcaattatcctaattattgtaattgaaatgtgaatttatttttcagataattaaaatattatgttttttttcatataataatgttcaagaataaattggtaattcaactttaagctaaagggcttcccacttataataatatgatatgatatgatgattattagatgtaattttctgatttttcttttggaaacaaatcaactatttgtaacatctatttgtattatacttgatttttcttgggtctgtaaaaataaatatttgaattttttcatattaagattcataattagtcttatagcttaactgtaagaaagaaattacaaattaaatttgacaaataattaagctacttaaataacttaattgttcaatataaaattttaaggattgcctaaacttagaaaaaaaaaacaattaaatttagttatatggttgcaatgtgtaatcaaatagtaataaatatgtggctgtttgtacagctacaatatgacatgagataattaaaatatatgtgtctttaagctctcctctttttgtttgttttgaggaaaatctgttgtattttgatgtgtataattggttaattatacactcttttagaaacaaatagtgttgaatctacaataacatgtgaatacatagatttgataaaatataaaatcgtaaatagattagaccatcttttttattgacagaggtgaaagacaaagcaaccccacaagaaaagataggtatgaaactagctagcagttttatgaacaattaatataaaatataaaacactttttattttactcaacaattaatttataagctatttttattttaaaacacttaaaataagttaattcgaacatgtactataaatcaaaacaaataaggaaaaaaaggaaaagctaaaggtgtgtttggtatgaaggaaaatgttttcctaaaaaataaatagattttggatttattttctcatgtttgattggtaagtagaaaatattttcctgtgtttgatttatgaatgaaattaatttttggggggtgggggtgggtgggggctggtaggggtggatagggggctggccgggtggaggagggtaggagtttaaaaataaaaatttgaagttgaaaatattttaaaaagcaaaattaatttttggggagggtgaggtttaggggctggtcggtggtgggtggacgggggtcaaggatcgagtgaaaaaataaattttaaaattgaaaatatttttattaatattgatattttcctaaatttttgaagggaagtcattttccttaatttttaggaaaatgagttgatttgaaaaatattttctaaaacttttattccaaccaaacatgaaaaaattgaaaaatattttccagaaaatgtttttcttcataccaaacacactcaaaaagagactcttttaatcaagtattattgctaaaaaaaaaagagacaaagaataataatttaccccataaatttcgcaaatcaatctataaaagattgagggtgagatattgataagataaaacaatcaaaataatagataaatatgtcttttagtttaatttaattttatatttatattccttaatttagaatggacacataatttgatatcttaacttgtatataattaaacaagtatgtatatatatatatatatatatatatatatatatatatatatatatatatatatatatatataacaccacctatgacacaatttccatgaaggatgtgcacgtttattttattgattctatacaagtttaagtatacgcttattcatactatagttgaataatataaatataaaataatatcaaatttaaaagatatatttatatattatcttaaacaaatatgttttaaaaaaaaataaaatctagtaactaccccaccataaaagtgatgcccttatacgccgaaagaacgtttaaaatcaaaagcaactgttagtgttattggattgaaaaataaaaccgaatactccaattaagagacatggcggccccatggtggaataattattacaacacaccttccataattaaagtttgaccttatacctaatgacaatcaaattttgagttcggatcctatttcatgagttaatatctcatataatcacttaattttaaataattcatttagtatgttattcaagtttaaattgttcacttaaaaagtcattcaactctattttataagtaaaaaatcactaatatttgagttgttcatttagaaagtcattcaactctctttataattcaaaagtaactcaattatttttgtttcacttaaaaagtcacccgatcccaacttaaatatttttttttcataaaatcttatttttatgttaaactattcttttaaaaaaaaaataagatatttattttagaaaaggggaaaacatgttaaaaagttagttattccaaaaaagaagaaagaagttggaattgaaaagaaataatataaaaaaaaaacgcaggacagtgcctttttttcttattactttttatttaaaagataggtataaagaaatattatacttcaacaaaatataataaataattaaaataagcagcttataattttattttatttttgtattcagccaaatttaattaaaaaatcatttaaaaataattgaatgacttcttaagtaaaattagttgagtaatttttaagttataaaataaaattgagtgactttcaaagtgaactcaaagctgagtaactttctaagtgaactattcgaaattgagtgaacatctgagatattaacaccttattttatacgtgaaacaatttaaactatattacaaaagttggaggaagatattgaagaaagattgtacatatgttcgtaagctcctttatgtcagcttataaaaggcttaacacaagtatatatagcgggtaaaattttattttgtgagaggtacaaatgttacttagcagacaatatttgtatgacattctctcagcttttgccaagtggagtttgggtctcacttacagaaaatgtgcttaaagcttcatttttttctctttcacctatttctatcttcttcttctctctttttttctccgttcttcataaattttattttattttctgtcaacaaacatcgatacttaatatattttattgaatgaaaattgatttaataatttttatttttcaaatgttaaaatcaagacaaatcaattaagtcgatttttcattactttttttttccttgcgatttgttttttgtggacttctcgaaaatatataataatataaaattatcctctgaaaaaattatgcattacgaagaatttaatcattactaagaaatatgataaattatttccttacaaaaaaattaaagatttaaggctgatatattaaagatgtcttgttaatatctgatttaaataaaataatcaattaaattacgagttattttgaacataaaaaaacactttcagtattatctaaataaaaatataagttaaactacaaagtaaaaaaaaataattattataaagagaaacacatgagtactcacaaagagaacaaaaaaaatatttataatgatttttttagctttagataaggttatacatataaccaaaattattacggaccatttgttaatgaaataataaaatataaagattctcctaataaattaatgtatgatcttttttaaacaaacacaaaaattagttaattacactatatttaatttctttaatctcactaaaaaaactattttttctcatcacatttactttaaattttccttaaataaataatataaaaataaaatagttaaacattgtggctaatttttttttttttttacaaaaaaacacaaaagactacaaaggagaacaagagaatgagaaacgaaagtttaaagggaaaaaagtctgatatacttctcaactttttcatttggagctgatatatttctcgttataaaagtgactcatatatgcccttatcgttatacaaacgactcatatatctgagtcatttgtttacaagtaaggtatcactttcttaaaaaagcaatgatatcatctctaaaacgacaaagattgaggggtatatcgatcctttttcaaagtttaaatgaatgagaaaaagttttaagtgtgggtcccatgttgtacatttaaaattctcataaactgacagaaggttagcttttcacaaagtaaaatttttcccatgtgaaactcaaaataaaataattgcgtacagacatgtttatgcaacacaacattaatttatttatttacccattcaataagtgaaggaataattataatgctttgtgctcttacttttagctgttcatatttcattccaacatcgatcttatagatttattgttaattcacaacacttccagcaatctacatggctgatgctttccttcaaattttgttgacttctttcatacaagaggaacttggattgaaaatctaaaaagcacgtttactacgatccaagctgtgcttgaagatgctcaggagaagcaactgaaggacaagccaatagaaaattggttgcacaaactcaatgttgctgcatatgaagttgatgacatcttagatgaatgtcaaactggaatttttaaccaaattaagtcattatataaaataatttaccaaagtaaaatatttttctaaaagtttacaaaactaatataaacgtatttcatggtaacgttttagggtatattttattttttaaaaactaatgactttaggttgatatcgttctttgtaagtaacgttttactcctaaaacgttattttcaataacattttactcttaaaacgttactcatagtaacgttttactcctaaaacgttattttcaataacattttactcctaaaacgttactatgagtaacgttttaggagtaaaacgttactgtgagtaacgtatatcaatctgacgccatcaacttttaaaaaataaaatatatcctaaaacgttactgtggaatacgtttatactagttttgtaaaattttagaaaaacatattattttggtgaatgactttatataatgacttagtttggttaaaacctcgtcaaactgaggcagcaagactcaatcagactaaatatgggagttatcatcctaaggctatcactttccgttacaagattgggaaaaggatgaaagagataatgaagaaactagatgcaattgctgcagaacgaagcaagtttcatttggaaaaaaggactacagagagagaagcttctagacgagaaacaggtgctcatcttaaatatattagtattaattacaacaatttaattagtttatattcatttttttgctattatcaagttcatgtgtgtttatggacccaagggacttttttctaatctaatgtttgtctcaagtctaaacagatttgtaattctaccacttatttatttactgaagttcttaaacatatatacatggtgtaagccagctcagataaatccatagtcagttgtttcggactgaatttaacttggatgtcaatttttcaaagtcaatcatgttttcaactcctccccctgattctcatctctttgtagtgcaaaaatcttctctctgtttttcgctaaacatattctcgtgtgaacatatattgcttgaaacaggttttgttttaactgaaccagaaccttatggaagagacaaagaggaagatgagatagtgaaaatcttgataaacaatgcccaacaactttcggtcctcccaatacttggtatgggagggctaggaaattcgacgcttgcccagatggtcttcaataatcagagagtaactgaccatttcaatcccaaaatatggatttgtgtctcagaagattttgatgagaagaagttgataaaggcaattgttgaatctatcgaaggaaagtcagttggtgaaaacatggatttggctccacttcaaaagaaggcattgtgtcgatttgagataatacgagaaaaatatacatgcgaaaaacaagacaacagatttcgtggttcaccaataaattggctcgtccacgggaagagggcgggttttattatggaggcaaaaaccaattctgagaatagggtttgccatagcgtctatatatagtgtaaactaagcccctaacaggcttgggcccaaaatataaattgaatgataattaagggcccaattcaaggcattcaacaaatctccaccttgacttgaattctccaagcagattcttgggcgcactatgatagtgccaggcctcccccctcttcctcgggttgcccttgagtataattacttgacacgatgttgagcaagtcaaacgagtgttgaaacttgctcacgtggagccaagctttgtgaacatatcagcgggattatcaacagttctactttcttcaccttgattctcttctcacttctcgggaaaatgatacctccgtcaatatgcttggttctctcatgatggacttgatccttggctagacaaattgcgctcaaaagctgtcaatacacacgtgctttgagtcatgatcgagaccaagatcactaaccagcccctttcaaccaaatcccttcttttgcagcctctgtcaaggccatgtactccgcttccgtagtagacaaagtcccatgtaggttgcaaagttgccttcaatgacgcggatcctcaagggtaaacacttgagtcatccgatcttcttgtgtcaacatctccaaagatagtctgaatcagaatagccaataaccaagcactgagtatcacctccataaatgggaccagcgtcggatgtacctctaaggcaccgaaaaattctcttctgactgccaatgttctctccacgttgtcccatgaatgctcactacactaatttgcatgtactaaatctggccttatacagaccatagcatacatcaaacttcctcagcactggcataagggactcgtgacatatactccttctcttcttctgactgtggagccgaacatggcgagtgggatggataaaggcgtggggtatcaatgggcttagatgaagacatgccaaacctagccaagaccttgaatgtaaccttctctgtgacaagaaaagtttccttctctctctgtctctaatgatctccatccctaaaatcttcggctcccggatccttcatctcaaactcagactaagtaaacccttgacttctgagatgtcatacttcttctttgcagctatcaatatatcatctacataaagcactagatagatgaatgaatcatccttgagcctattgtagtagacacaacaatcatatgagctccgagtatagcccaacttcaccatatagctgtcaaaccttttataccacatccttggagactgcttaagtccatataaggacttcttcaacttcaggacgtgattttccttctggaacttggaaaccatcctttgagtcatgtatatctcttcctccaactctccatgtagaaacgctgtcttcacatcaagttattcaagctccattctgatgtgtaactatcgctagtaacactcggatggaagtatgtctgaccactggtgagaagatctcattgtagtccactccctctctttggttgaaacctctggcaacaaccctggctttatacttgactccttctgctggtgatatcccttccttcttcttgaaaacccatttgcaagtaataatctttctccccgaaggctgtatgaccagatcccatgtctgattcttgtgtagggactccatctcatctcccatagcggcaaaccatttttcagaatcagaacttaaaatggcttctttgtaagtagacggctcagatgtatctacctcttcagcaacctgcagtgcataacccaccatgtcctcaaaaccatacctcgtaggtggccgaactccaaccctccttggccgatcttgagctaaactctgatggatatctgatggcatagattctggaatatcagtttctgtctgtggctcttgatcctcctcttcaggttctttcaaatcgctctcgttctgaatgacttgaaactccacctgtttatcaagactcccagtttctgacgtagttgtaggcttcacaatggttctaagcagagaactttcatcaaagacaacgttcctgctcataataaccctcttttctggagccggattacgaaacctttcactccatctcatgccccaaatactcctttttggctcttggtttctaacttaccttcactgacgtgatagtaagccgtacaaccaaaagctttcagatttgaataatcggcagcttttcgaccacatctccataggtgttttgcactgtggctgtatgtggtcccttgattatcagtagcaaagctgtactaaccgcttcttgagaatcttctatccccagcattgaaagcatgcaccttgctctctccagaagtgtttgattcatccgctcggctacaccgttctcttgtggtgtatttctaagcacatgcgatgtcgggcaatccttcatccttacgaattgatcaaattcagaccaacagaattccagcccattatcagttcgcaacctcttgatcttcttccctgtttgattttccatcaaaattttccactccttgaacttctggaaagcttcacttttatgcttcatcatgtacacccaagtcatccttgagtagtcatcaatcatggacacaaaaaatgggcgacctcccaaagactcaacacggcatggaccccaacaatcagaatggatataatcaagtgtgccttttgttctttgaatggcctttggaaacttgttgcgatgtagttttccaaagacacaatgttcacaaaactctaggctcttaaccttatgaccagcaagaagatcctctttttgatgaatttgcatccctctttcacccatatgaccaagtctattgccataacttagtcatatccttctggtgaaattctgacgatgcaacatgggctgaacctgtaaccggaaccttgtagaaaatataaaagtaccacatgacacctttcaagaatcaatttgaacctttccagaccccaagactccatcttttcccgaccatttgaatcccttgctgtcaaaagactgagagatatcagattttcgtcatcaatggaacgtgctgaccctcgttcaatgtgccaaaactaaatcgtcgtgtccttatcttgatcagcctgtcccaaccaccttgcggtgaaactgttggccatcgagatcttgcctcaaatctaccactcataagtcgtgaaccactctccctaggacagatgtgataggatgccccagaatcgagaacccacatatctgaatgatgagtgtgctcatcgtcaactagggcaatatcttcttgaattggtgtcttcttgactagcaacagcagagaccactgattgttttcgattgcttcttcttcttggacaatcaaatttcaatgtcccttctccttgcagtaattacaaacatcatccctttgcaccttcgacatcggcttatttttctttccgccgttttccttccctttccgctcttggtcagcaggcccggaaggtataatgtcgtacttgtgccgttagccttatgccgtaattccctgctatgaagggccgatctgacttcttccagtgacacagtatctttcccaacaatgaacgattgaacaaaattctcaaacgacattgggagagatactaacaatcaggcgacatcttcatcctcgatcttcacatcgatattcgcaattctaataacaaagtattcaattgctctaagtgttccctgagttgtaccttgaccattcgtaaaccgaataggcgttgtttgaagcagcttgttggttagagattttgtcatgtacaaactctccgacttcaaccgagaccagacggtctcttcatccgagacctctgcgtgatgacgtcatccgcgagacacaaagatgatcgtcagtgcgcctttcctccggaatctccatctcgggagtaacgacggcgttcttgtctttcgacaacggcgcccgtaaaaccttgttgtttcaacaaagcccgcatcttgatcgccataaaccaaactggctattcctccaccgtgaatttgtcgattttcacgttcaaagcgtacatctcaattctcaagaacacccgattaaccgagaggctcgataccaatttgttgtgcggaatttgagataatacgagaaaatataaacgcgaaaaacaagacaacagatttacgtggttcaccaataaattggctacgtccacgggaagagggaacattttattatggaaggcaaaaaccgtaattacgaatagggtttgccataagcgtctatatataactaaactaagcccttaatgcttgggccaaaatatagaattgacagataattaagggcccaattcaaggcattcaatgaagcttcaagatatgttgaatggaaagagatactttctcgttttggatgatgtttggaatgaaaatcaagaaaagtgggataagataaaagcagtcttagaggttggagcacgaggtgcttctgttctaaccaccactcgtcttaaaagggttggatcaattatggacactttgcaaccatatgaattgtcaaatctgtctcaagaagattgttggttgttgtgcatttgagaaccaagaaaaaataaatcctaaccttatggctatcggaaaggagattgtcaaaaaaagtggtggtgtgcctctagccgccaagactcttggaggtcttttgcgcttcgtggatcaagaaagagaatgggaacatgtgagagataatgagatttggaatctgcctcaagatgaaagttctattctgcctgtcctgagacatagttatcatcatcttccagttaatttaacacaaagttttgcatattgtgcagtattcccaaaggacaaggtaatggaaaaaggaaatttaatatctctctggatggcacacggttttcttttatcgaaaggaaacttggagctggaggatgtaggtaatcaagtatggaatgaattatacttgaggtcttttttccaagagattgaagttaaagatggtaaaacttatttcaagatgcatgatctcatccatgatttggcaacatctctattttcggcaagagcatcaagcagcaatatccgagaaataaacgtagaaggttacccacatatgatgtcgattggtttcggaaaagtggtgtcttcttactctccttctcacttgcaaaagtttgtgtcgttgagggtgcttaatctaagtgaattaagacttaagcgtttaccatctttggagatctagtacatttaagatacctggatttgtcttacaatagtaaaatgcgcagtcttccaaagcagttatgcaagcttcaaaatctgcagactcttgatctaaagtattgctggtcactatgttgtttgccaaaagaaacaagtaaacttggtagtctccgaaatcttttacttgatgattgcgatggattgaattctatgccagcaagattaggatctttgacatgccttaagactctaagtagatttgcagtggggaggagaaaaagttgtcaacttggtgaattctgaaacctgaatctgtatgggtcaattgaaatcacgcatcttgagagagtgaagaatgatagggatgcaaaagaagccaatttatctgcaaaagaaaatctgcattctttaagcatgagttggaatatcaacgaaccgcgtagatatgaatcagaagaagttgaagtgcttgaagccctcaaaccacactccaatgtgacttgtttaacaatcaaaggcttcagaggaatccgtctcccagagtggatgaatcactcagttttgaaaaatgttgtctctattacaattggaggttgtgaaaacttctcatgcttaccactgtttggtggtctgccttgtctagaaagtctagagttatggaatgggtctgcggaattggagtatgttgaagattctggattccctacaagaagaaggtttccatctctgagaaaacttattatagtgaattttgataatctgaaaggattgctgaaagaggcaggagaagagcaattccccgtgcttgaagagatgaaaattagctgttgtcctgtttttgttattcagaccctttcttctgtgaagaaattgaatgcttattggcacaagtcagatgcaacaggtttgagttccatatcaaatcttagggctcttacttccctcaacattagccataactccacagctactttgctcccagaagagatgttcaaaagccttgcaactctcaaatacttgaaaatctcttacttcgataatctcaaagatctgccaaacagcctggctagtctcaatgctttgaagcatctggagattaattgttgttatgtactagagagtctccccgaggaaggggtgaaaggtttaacttcactcacacagttatccattgcatactgtgagatgctaaaatgtttatcagagggattgcagcaactcacaaatttatcaattacgaattgtccaacactggccaagcgatgtgagaagggaataggacaagactgatacaaaattgctcacattcctcatctgctgattacatagtgtcatactaaattaaatgattcttatagcaatattattggttcaaccaacaaaactaaatctctaattatattacttaattgcttttagtttgctacaattatcactcatgactaacattatgtatcaattacgtggtttgtcttcaattttgtataattagtcatgtttttatatgtataattcgctagaataatacagatatatgtataatatacaattatttaactgatatacatatataattcacctctcttccactctctgtcctctctcacttgcctctgtcctctgccaatcgacgagatgagcctacgaaagatttcaagttcagactatgatgactgacatcctcacttacgcaacgaaatggagttgatggagtagccagtgcccttgagtcattctcttcggtatcgccttctctcatcgttaatggcgccgcaaggcactcgactagcaagttagaccttagttagggcgaaagatttcttggatggttcatttcagtctgaagtcgggtcaagtcatggaattgatgtgaagttctctcaatttcgctttccatatatacaaatatatatgtataacatacaattatctaaatgatatatatatatatatatatatatatatatataagcaatttatctctctcccactctttgtttcacctgacaactatgacaactatgtttgttagggctggaaggtctaacttcactcaccgagttatttgttgaacatatgctaaaatgtttacccgaggaattgcaccacctaacaaacctcacaattttttttttataagtgaaagcatagttaaactctcaaatgtagatgataattaagctcttgaagattattgctgaattaagtgaattcgtcaagctatatttgtaaaattcttatggccaaacaagtaatattgcaacaaattgtagaaggattattatactcttaacactaactaaaagattcttccaattctcaaagcaatttatattcctttccaaccaaagaggttttccaaatttgctttctagcaaaaaacaattttctgcacgataggaatagatctcatatatactccctccgtttcattttatgtgaagtagtttaactgagtacggaatacaaaaataaaagaaagacatttaaaatttatggtctaaaatgaagggaaaaaggtcgatatctcctcaactttgtcattttagaaatgatataccttgttatgaaagtggctcatatatacccctacttgtaaacaaatggctcacatatacctttttcctctaacgggaaatgaaaaataataattttcaatctaaattttttattttttttctaaaaaatataagtccatatgagtaaatttaattctcgtcaaacaatttttttttttttactttttttttgtttcaatgactaatttataattattagtttgataatcaaatttatttatgtttcactaatattcttgtaaaacttattgtagatgaaaaaaaaaaaatttgaatacgaaattaaattacaataaacacaaaaaaatagtttatttttttttttctttaaactaaggaatgatagaaaaaaataaaataagaataagaaactcaaataattataataaaagaagttaaaaataatttatgtatgaaaaaaaaattaaatatactttgaacttttattgaagaatcatatataccactaaataatttttttaaaattttttaagtaataaatataaatttaaaactaattatttaaaattttgttaaatgaagggtatatttgaacaattttgtaacggcaggggtatatgtgagccgtttgtataacggtaagggtatatacgagccacttttataacgagagtatatcagattcaaatgacaaagttgaggggtatatcaaacccttttcccctaaaatgaataataaaaaattgtgtgagtataaatcatttcattaagagtaaatggacaatttaaaattaaattgttacttaatatagtaacgtatcttttttgtttttgagtctgctttaaaaagaaaataaaccatataaattggaacatagggagtatctacttacaaagtaaaagttgtgtgtagaagattttggcatacaaatcaaatcatatatcatatcatatatcatcatatcatatatcacatcatatcatatattagtaaaagcatgaataaaaaaagttgaaagttgaattacggttttattccttctattaattaacttgttataaaatatttaaatatttgattttacaagtttaattaaaatgttaaatgacttttagacttcctacgattaatttctaattaaatatctaatttattaatatttatcatttataatctatatgtatataataattataattttttaaaataaaagtctaattataattttaatgactttttagacttcctaacactaattcctaattaaatatctaatttattaatatttttatcatctataatgttataataagcatctttagaaggtttctctgaaatactctttaaaagaatgcttggactatgccatcctaaggttgaaaccagtaggcaaaagaaggtcgttatggggagtaaacaaagttgaggcgctgttagggtaaccaattaaagaagaaagctgtagtagtgactaggcgagatgattattaaatcattattattacataataagtaagtataatttattaagaggtcggaaggaataaaacttttagcaaaaatgaataagatgactacctacctaattgatgatgatgatgaatataagatattattactttatatattaaaaaatcttaatactgatcaagttagcagtctcaaaaatctttttttacttcatggttgccataaattgaattctatgccaccaagtataggatctttgacatgccttaagactctaggtcactttgttgtgggaaggaagaaaggttctcaacttgatgaactacgaaacctaaatctctatggatcaatttcaatcacacaactagagagagtaaagaatgatagggatgcaaaagaagccaatttatctgcaaaagctaatctgcattctttaagcatgagttggaatatcaacgaaccgcgtagatatgaatcagaagaagttgaagtgcttgaagccctcaaaccacactccaatgtgacttgtttaacaatcaaaggcttcagaggaatccgtctcccagagtggatgaatcactcagttttgaaaaatgttgtctctattacaattggaggttgtgaaaacttctcatgcttaccactgtttggtggtctgccttgtctagaaagtctagagttatggaatgggtctgcggaattggagtatgttgaagattctggattccctacaagaagaaggtttccatctctgagaaaacttattatagtgaattttgataatctgaaaggattgctgaaagaggcaggagaagagcaattccccgtgcttgaagagatgaaaattagctgttgtcctgtttttgttattcagaccctttcttctgtgaagaaattgaatgcttattggcacaagtcagatgcaacaggtttgagttccatatcaaatcttagggctcttacttccctcaacattagccataactccacagctactttgctcccagaagagatgttcaaaagccttgcaaatctcaaatacttggaaatctctttcttcgataatctcaaagagctgccaaacagcctggctagtctcaatgctttgaagcatctgaagattagttgttgtcccaaactggagactctccccgaggaaggggtgaaaggtttaacttcactcacactgttatccattacatactgtgagatgctaaaatgtttaccagtgggactgcagacactcacaaatttatcaattaagaaatgtccaacactggccaagcgatgtgagaagggaataggacaagactggtacaaaattgctcacattcctcatctgctgattactgattagatgtaattttctgatttttcttttggaaacaaatcaactatttgtaacatctatttgtatgatacttgatttttcttggttatgtaacaataaatatttgaaatttttcatattaaagattcagaatgagttttatagctaactctatattttcacagtttaataacgtaaaaatgtgatatttatatcaaattattacttatgttgtcatttatcaacatgttggagatgattttgacagtttattaaagaatttctaagtttttattgtttgcacaagtaacaagccataaattaagtttcgagataaaagtgatttgtgtatcatggcttaattagtcggaatttcaagtttttttctcaagttatatatatgacaatttgtaaaaaatagatagtattgattttgatttaattcaagcatttttaaaaatataaacattataatatgggagatacacacgctaaacgcgtacccagaaactagtatataaagaatcatgaccgaaaaataaaatgaagttctgtcaacaactatctcgacatctttgctgatatatatatatatctaactagtgtacttattcggacttgacatggtataaaaagatattaaatatatttttaaataattaataaatgatataataaaaagaaagaaatacaaattcagttatgattctgataaaagggaaactaattttctgatttttcttttggaaacaaatcaactatttgtattatacttgttaatgttgcaattattagtgaacagttgtattttggattatcacttacagcagatgtctaaaatgtgaataagataatacttagaataatttatgcaatatacttttgtttaaatacaagaaatttaaataaagattgctaaagattattattttgaatgaaagattttgattttgttactttgtcgcctatgtaacatagtactgttgcaaacatatacatatgtgttcatttttccccttgtgtttcattttattttctacaactcataaatactaaaaagaaaacgttaggaatgagttttaactagatttaaattttaacaaaaacaacgtgattatatttcactaaattgacttaaatatatttatacttaaaaaaaaattattaatttataatattaatgggaccatatatttatataaaaattttctataaatatattatcttatatctcctctaaattcatttcacgagaattaaaaccatcctaacggatgacgttgccaaaaagaatagaaattttctttgaaagcgtgttaagttttttttaaaaaaaagtaatggtctcactttgtatatatgaagaaaaaaaaaacccacccctttcttcttcttcttcaaacccccacccccgctttttcaaaacccaccagccccctttacctgcttgtcttttcttcctcatattcccgacgtcaccctatccccaacccaccccatcctctttctcatttttcgaactctacattcaaagcacataaataaaaagaatcacatttaagattcatataatttttttactctttacttttgagatttgatttttcttaaaaagttatgatttttttgaaaataaagaatagggcataaaagaagatgaggttttgtcaaccaatctataatgttaatggctgggaatggtgattgaagcaatggatagagaaagatttttttttaaaaaaaaaagagaagaaaaatcactacaatcagtaaccgcaattgcagtaggcttacatcatggagtatcccaatgagtctcttcactgttcaatcggccatcggtaaccgcattacaatgggctttgggtcacccacccaatttcttataaatagaaagagacatgagatttatgattgcacctagatcacatagtgatttggcaaagtgtaataatacgaatggtacatgaaatagtgaaagcgccaggatcttccttcttctgcacaagagttcttgtgacaatagcactacaatgctgcattcagttatcatcctcaaaacttaccgatctcttctttgtaactatatccttcatgaacttggcataaccggaccatttgctccaaagcttctatcaaagggacattgatggaaagttgcttcaacatagtgataaaatgttggtatttaccattctcactattcttcaccaatctaaaagtggtggtggtctaggaatggggaccactttctagggtatctttgcttttttcgccgctttgtccaccaattcaccactagtttccaccacctcttcatcttttctcatctcatcttctaccacagacgacataggtgaatcaatagtttgcatacctcctcaagtagtgactgtcatgcaatgtccatcatttttaggatttgaatggaattactatgaaaagtgacagttgtcgcgggttctgatagtgaacaattggaccatttataattcaagatgcttaatcgagaccgcatgtgcatccacctttttcccgatattagccaaatcacctctcaatttcttggcgtgctcatcactagcatcaaaccttctcatcatctttagcaacatatcttcaacttgcgccgtactacctccaccatctcaaggagcaactttctgattttgaggtggaacatagggcacacttcaatcatttctattaccatagttaccccggttgaagttgttatctcggttgtagtttcttctcgaacttactggccctcttgttgtaattcccattctgcattttcaatttaaaattgttgataaaaaagacaaaaacataaaaattgatatgaaagagctttggttaagtaacaatctaattatcatagtgtcatattcaattcaatgattcttatagcaatattgttggttcaacagtttaactttactcgctgagttttctatttatgatgttaaaatgtttaccgaagggttattatacttgtttttaatgttgtaactattaggggtagattatcactttatgaatgaatattttggcacattggaaaaacaccaaatatagcgcgcaaaagctaaacaaggaaattttcatatattggatatagtctttgtcatttccaaaggtctccaacatagagatagtaattgagagaaaacttctattgctattaaatagaatctgcaattaaaaaaaaaataaattattattatattttatattataagtgggaagatgcttagtctaaaggtggattaagaaaacgccttcaacttttttaattatcattattatattatattataaataataattaattatttttctataagtgtgaaactattaaagttgaataaccttttaattctacaagaactcaccattaagttgaatgactttttaactcttcaagaaatcactaataagtctttttacacgtcgtcttataatgataatattgtacatttgaatttggtttagagagcataaatcccttattatactatgtgttttcaagcatttctttacatttagattttttttattttttgctataattcaagttatattcttaaattgatatttaagtgtttgatttctcacatgaaaatatacagttaaaattttgttttatgaactcatgatgtaattttttctcaggtataattttaatgtgattcttttgcagacaattgactaaaatttttagtagaaattgcaccaatacaaataaggtatgcggcatgtctctccaacaattttacattttttgcatgattattttttaataaatttgatatacatacgattattgtatttttaactagattttaataacttaatgcatgtttttttttataatagagcctccttgataactttacaattacttattgaaatttatttttcttcaatctcctagcttccgagataaaatgggtaactaatatttctccctcaacaacatggagcaaaaaaaatcgagaaaatctatgaagaagacatattctaacaaatggagtaatttaatttaatttaaaggagtacttaatagtcaaatatgaatagtaaagtaagagaaaaaaaaataaaaaaattagaatatgacaagtatgaaagacaaccatgaacaaattattggagttttttgttcatgctacaaagaacaataaagttactatgtcatttgaatgtaatatgtagacaacatatatacttgttacaagtatatatggtaattcaaattttggtacaaattgagcaggtgtgttatgtgtgtattgttcctttcttagaaaagtaacaaactaatatattgtagatttcgacctaataacataaaaatgtaaattatttatcacattaaattttgttgtccaaatttgacaagttattggaatatctaattatttgacatttacattttacaataaagaagtcatttttataggttgattgtccatttatttcgtttatatttttttcgttaaatcatttttgaaaattttcaaactgtgattttaatatatttttttagtttaatgtaattttaatataactcctacaatatataatatttttgtgggactgacatgcaaaacacgtgtcttggactagtctttcacataaagacagacaactaagaagattgtatcgcggataaacgctactggaatagccctattatgaagagtgtttgtcaaacagccaaatgactgtagttttttcttttccagaaatatgactgaaggactatatcttggatcgatcagagtgcatgaatcactcagttttggaaaataaagttttgcttgataaacacaaatttatctattcacaccacaagcaatggtaagtcatcataaaaaaaaagagagagagagaaatttgttgttagatcgagaaagattttgataattgacgaatagacgaacaaatgaaagaaacaggttgcatgtacatgttcctttcaaaccaaatccgactgggattgtcaaccatgcgaattagaagttataaagtaatggaagggttgctttttcgacccgaacgaagagtgcaaaaggtttcctttcataaagaaatcctaagcaaagtgggaagtgtaaacgaagtaggtagcataagcgagtaggaagtataacgacgtgaataaatttcaaatctgaatggagtagatgatcagatatgtaaaacaagtacaagatgaaaaaggttttgaagagtccaaagtttataaatagggcaatattttctttggagaaaattgtgcacttaaacagagagttacaagcaaaatacaatcaaatagagggagtttatatttgagtgaattctgattacgaactgcagccaacacaagaaaacaagaattgaagaactcattcattggcttatgttttatagttcttaagtcaagtttttttgtattgagtttttatcgagttgtatatttaaccctttctaaatccagtgaagtataaactggagtagaaatagagtctttaagttaaagacttggaaacataaaccttgggggattttgttggagtctaggaattagaatcagttctagtattgcaagagttggaatccgaattcataacttgaagtgggatcgacgatctagttggttgttggtagggccgactcaacaagattgagggcctaaagtcaaaccttaaagagggctccaatatttttttaattctttttaaaaaaaaaaaaaaaaaaactaataatcatgtatatattatttaaaatctattttctagcttttctagatgtgaagtcattaattactattttctaatggatttgttttaataattctttttcaattgataatatagctaatacattcaatctcattgttgatattacatatataagattttatcaatttaaattttaaaaaattctttcggccgaaacaatagttctggattgttaactttattcgttaagcaatatatgcattaggattagaatcaagtctttttattagattgcgtatttccattaaatcattatcttctacttgtattatttctcttaataataataactaaagcgagcatgtatacttactatgaatatcaacaacaacaaaagttcaagaaaaattacaaaataagttagtataataaaacttggcttgcgaatttgataaattgatataacaatactgaaatagtgtttcatttcttcaatataatgactgtttgtttaaacaagacactcaaaaacaaattttattttttttaacatgtaagcgacaataacttttttttaggagagtgttcaacattgagcataaaagtaataaaatagagaataaaaaagatgagtataagataaataataatataagatcgattttacctattgtcaattttgtgtatcgactaaagaaataacagcttcacatatgaatttgtattttaggctgctgtaagtactaaaagatagttattcaaccagtagaagagatgaaggtggggggcagctgttggcaatcaataagggcatattgagccaatttttttcttctctgaaaaactttggcagagaaattaaggctaacgaaaagtctttgtgcagttgtttcccaaaactttgtgaattgtatttcaaaaaatacattatttaatactccaacaactttgtgattccactctagactaccatcacatatctaatattaattataatagtgaatttcacatatggccagaggcgaacccacctgcacccaatatatttttaaaaaaaattcatatgtagattgttgataagacgctataatatatttaattgtgcactcttataatgaacaaatgatttgacttgttcattgaaaaaacaaaaagtgtcacataaattgagacatgaaaaataatatttcttttttaaatttttcgtgtgaagtcaaactaattcatatataaagcgaaagcggaaggagtactgtttaatattaattgcatatggtagtaaatttgatagacatggtcccgtggggtgtgtgttatttccattgaataattgagtttgtaattgttacaagtccattctaatttccaacaccttacttcatttcaaaaatatagattcattgcttactcaccacatactcgatggctgaagctttccttcaaattctgttagaaaatttaacatctttcatacaaggggaacttggattgttttttggttttaaggacgaatttgaaaatctgaaaagctcgtttactacgatccaagctgtgcttgaagatgctcaggagaagcaactgaaggacaagccactagaaaattggttgcagaaactcaatgttgctgcatatgaagttgatgacatcttggatgaatatcaaactgaggcagcaagactcaatcagactaaatatgggagttatcatccaaaggctatcgctttccgctacaagattgggaaaaggatgaaagagataatgaagaaactagatgcaattgctgcagaacgaagcaagtttcatttggaaaaaaggactacagagagagaagctgctagacgacaaacaggtgctcatcttaaatatattagtcttagttacaacaatttaattagtttatattcattttttggcgattatcaagttcatctgtgtttatggactgaacttaacttggatgtcaatttttcaaagtcaatcatgttttcaactcccccctgattcttatctctttgtagtgcaaaaatcttctctctgtttttcgctaaacatattctcgtgtgaacatatgttgcttgaaacaggttttgttttaactgaaccagaactttatggaagagacaaagaggaagatgagatagtgaaaatcctgataaacaatgcccaacaactttcggtcctcccaatacttggtatgggggggctaggaaaatcgacgcttgcccagatggtcttcaatgatcagagagtaactgaccatttccatcccaaaacgtggatttgtgtctcagaaggttttgatgagaagaagttgataaaggcaattgttgaatctatcgaagaaaacccacttggtgacgacatggatttggctccacttcaaaagaagcttcaggataggttgaatggaaagagatactttctcgttttggatgatgtttggaatgaaaatcaagaaaagtgggataagataaaagcagtcttagaggttggagcacgaggtgcttctgttctaaccaccactcgtcttaaaagggttggatcaattatgggaactttgcaaccatatgaattgtcaaatctgtctcaagaagattgttggttgttgttcatgaaacgtgcatttgagaaccaagaaaaaataaatcctaaccttgtggctatcggaaaggagattgtcaaaaaaagtggtggtgtgcctctagccgccaaaactcttggaggtcttttgcgcttcgtggatcaagaaagagaatgggaacatgtgagagataatgagatttggaatctgcctcaagatgaaagttttattctgcctgccctgagacttagttatcatcatcttccagttgatttaacacaaagttttgcatattgtgcagtattcccaaaggatacggtaatggaaaaaggaaatctaatctgtctctggatggcacacggttttcttttatcgaaaggaaacttagagctggaggatgtaggtaatcaagtatggaatgaattatacttgaggtcttttttccaagagattgaagttaaagatggtaaaacttatttcaagatgcatgatctcatccatgatttggcaacatctctatttttggcaagagcatcaagcagcaatatccgagaaataaacgtagaaggttacccacatatgatgtcgattggtttcgcaaaagtggtgtcttcttactctccttctcacttgcaaaagtttgtgtcgttgagggtgcttaatctaagtgaattaagacttaagcgtttaccatcttccattggagatctagtacatttaagatacttgaacctctctcgcaataacatgcgtagtcttccaaagcagttatgcaagcttcaaaatctacagactcttgatctacagtattgctggtcactttgttgtttgccaaatcaaacaagtcaagttagcagtctcagaaatcttttacttcatggttgccataaattgaattctatgccaccaaggataggatctttgacatgccttaagactcttggttgctttgctgtgggaaggaagaaaagttgtcaacttggtgaattacgaaacctgaatctgtatggctcaattcaaatcacacatcttgagagagtgaagaatgatagggatgtaaaagaagccaatttatctgcaaaagaaaatctgcattctttaatcatggaatgggacgacgatgaacgtccacatagatatgaatcagaagaagttgaagtgcttgaagctctcaaaccacactccaatgtgacttgtttaaaaatctatagattcagaggaatccgtctcccagagtggatgaatcactcagttttgaaaaatgttgtctctattagaattggaggttgtgaaaactgctcatgcttaccaccgtttggtgatttgccttgtctagaaagtctagagttatggagtgggtctgcggaagtggagtatgttgaacattctggattcccaacaagaagaaggtttccatctctgagaaaacttattatagacaattttgataatctgaaaggattgctgaaagaggcaggagaagagcaattccccgtgcttgaagagttgacaattagttgttgtcctgtgtttgttattccgaccctttcttctgtcaagaaattggtagtttatgggaacatgtcagatgcaacagtttttaggtccatatataatcttagggctcttacttccctcaacattagccttaactccatagctacttcgctcccagaagagatgttcaaaagccttgcaaatctcaaatacttggcaatctctttcttcgacaatctcaaagagctgccaaacagcctggctagtctcaatgctttgaagcatctgaaaattgaatcttgttatgcactcgagagtctccccgaggaagcggtgaaaggtttaacttcactcacacagttatccatagaatactgtgagatgctaaaatgtttaccggaggaattgcagcaactcacaaatttatcaattacgaattgtccaacactggccaagcgatgtgagaagggaataggacaagactggtacaaaattgctcacattcctcatctgctgattacatagtgtcatactaaattaaataattcttatagcaatattattggttcaaccaacaaaactaaatctctagttatattatttacttgctcatcatagctatagtttgctataatcatcactcgcgattaacattatgcatcaattacgcgggctgacttcgattttgtataattagtcacgtttttatgtgtataattcgccagaatatacggatatatgtataatatataattatttaaccgatatacatatataattcacctctctcccactctatgtcatctctcactcgcctctctcctccctctcttaattttgcttttcatatatacaaatacatatgtgtaatatacaattatctaaacgatatatatatatgcaattcatctctctcccgctcttttgcttcacctgacaactatgacatttaactttggatatgcacatttaaaaactggttacagaaactcaatgttgctgcgtataaagttgatgacttattggatgaacgtgaatacgaggcagcaagactaaagcagtctcgattaggacgttatcatccaaaggctatcaaatacgaactcagttgtttagaccacaaaaagactgtgaattcaatacaggagtagttaacgatttagaagagatctactcttaacgctaactaaaagattattccaattctcaaagaaaatttatattcctttccaaccaaagaggttttccaaatttgctttctagtaatttttttttttttctgcacgataggaatagatctcatatactccctccgtcccattttatgtgaagtagtttaactcgtacggaatacaaaaatgaaagaaagacatttaaaatttatggtctaaatgaataataaaaaatcgtgtgactataaatcatttcattaagagaaaatagacaatttaaaattaaattgttacttagtatagtaacgtgtctttttttttttaaactgtctaaaaaagaaaataaattatataaattggaacatagggagtatctacttacaaagtaaaagttatgtgtagaagattttggcatacaaatcatatcatatatcatcatatcatatatcacatcatatcatcatatattattataagcatgaagttcaaaacttaaaagttgaattaccattttagccttatactaaattaaaatattataaaataattaattaattaaatattaaatatgcttaaattgttaattaagttgattcacttattgttaaaataaataggagaatgaatagttgtaaaaataattaattataaagttattacaaaaacttattagagaaacgtttcatttctctatcgatcgattttaggtgtaattttgtcataatgtgtattaataccacacctccactatctcatcattaatatccacaccttcataatcttccacactctcaagaagttgatggcataattatgagacttttgattttactcaatgatgtcctataaattgcggtatttgacacaacaatctatacactttgaagatatttaggtacagtttggaagaaattaaaaaaaatgtctatatttctattgtttttatcctttagtatatatttaaatcactttttaaactgctcataacaccgattcattaattttccttatcttcatttgttgtttataggaaggaaatgtgtacaaattgttagatcttctaatggagtttacaacgagagaagggatgttcaagtcttccggaggttgaaatcaattttaatttcaagtattatattcatgcttttagatgtttatatatatatatatatatatatatatatatatatatatatatatatattcaaatgagtcaacatagactaatatgagacttaaaggtcggaaaattggagtatcacaattagtagtaaaacaaagtaagaaatctcaattagatatattttattattttttaagaaataatacactcatgggtataagtgtgaagctccaaaatgcaaaaagttgaattactattgtatccctataatagttaattatttttaaatattagttcatatgatattattaaattatacttctttgaaattaataacataataaaaaccaaattcatctttgaagtgcaaatttatcgtccttcattattgataatttgaatgcactaaaaactatttaatatcccggaaggtggaagagtgaaagtattcataattaatttctagataaaattttactagataaaaaagtatacatgcattggaattaataatttaaaaataaagaaataatgatttagccttttaagttacctacttttattatgctctttaaaccattgttattattttttaaaaaaaaaactcatattaaggtgttagcttgattagtctaaagatatcaaaatgtcatttcttggatcacttaatttgtaacgtttttatcttctattagcgtgattctccattttcctatattatatattatactttctcatgtaatcatgttatctatatttatttttttatataagtttgttatgctcaatgttttatttatctttatttgaactcatctaaattgttgaatatttcaactactaataaattttttaaatttgactttttttttatgaaaatacaattaagaaatgacgctaatatttcatagtgatgatgcagtaagtgaagcaacacagattgaactgtttcaagtggtatcaattttcaggtaataaatcattgttccttatatgcaattaattatttttgtgtaagttgatatgttcttaataaaattttggtttgatttttaaataaaaattattttatagaagttgagacggtacacttaattggattatccaaaaaaagaatcttttacacaaggacaagaagaaagacttctagctttatcactgcattcatgacaatcaatggaatatcctacaagacaaaaagttgatgtgattctgtacaagtgaatccaactcactaacaaaaaaattaaagaaagaaaaaaatgaacatgaagagaataaaaatgaagatgaagagaatcaatggtgtcttataagttgatgaaccactgtaacttcattattttttaaatttacgaggaaatgaattattgacgaaatttatgaaatgtacatatatacctttgggtcggtaacaaatgtgattgaaagtagtattttttcatgcataatagctaattcttgatatatatattgtttaaatttattatttgtactacaaacattgtatgatatattttaggataagcgtaacgcatgcgacgtggaaactagtatattagtaaaagcatgaataaaaaagttgaaagttgaattacgattttattccttctataattaacttgttataaaatatttaaatatttgattgtacaagtttaattaaaatgttaaatgacttttagacttcataagattaatttataattaaatatctattttattaatatttatcatttataatctatatgtatataataattatatttttttttaaataaaagtctaattaaaatattaatgacttttagacttcctaacactaatttctaattaaatatctaatttattaatatttttatcatctattatctctctctatataataattttacaaaaattaacaaaaaaagtctctacgtaaatttttatacttttttttttattctcataaatttttcctaaataacaaaatttaataatttgaaggatgcaaatctgcaaaatggagacacacacatttgataatgtcctcttaattatcattaaagaatgactctaactagcttcacaaatttaaattcattgatacttaattactcggagaaaagtagatgaagactcttaattttgatagtatatggaaggagtcaataaagtttcgtagatttatgcaataattttgtacttattttttcatctacatatacatagtcttatgagaatgatgtctacattgtattttttcttaaatctgtttcttttgtcttttatccccaattagacttcttaatttaattttatacaaatgttttattgtcataagtctttatacttattttgtaattgtagcattttattgttcattacaatttgcatatatatatttccatgaaatattagtaattctatcatatctataaaaattcacatgaaatacacgtgcaaagcacgtgttcagaaactagttaggaaaacaacacaaatatacatctgaactatcgtaaatgatatacagataccatcatcatacttttgggacattggtgtccatgtcgtcaaaaaaatagagcaaatatattaatggacatcacgtgtcagaatcatatcaattgatccaacatttattaaatgtttgatcgaagaatagattgtgtcacatgtccctatttagtcatctgttaaaatgaatgacatatgggttgggccgaccattttctgacccacacaaaaaatgggctagcccggtttaacccgtaaaatatcaaaacatgtatggattagcccggataaggtgtgttagccatattgacagctttatccccacatcaagaaggtatttatatgtcaacttgaaaagaaaaaattttccaaatatgatctgcttatactctatcaattccatatctcacttagtgaaatttcactgaatatattgttgttgttggtgtcctctcccatcattataaatttaaagaacatgcaatgtaagacgtaatttagaaaacttggttcgcccgtagaagaaggatcatctgtaaatttattcctctgcaagttgatgctttgaatctgttggtacatttcctctaaacatgttagattggattgaatcttaagtcatcatgtgttactatctgaaagaccaatatttaaatttattgctcacaagtaaaaattagaactaaaaatatacaaacatgaagttcaacatatattataacttaattcataaaagaaaaattatttgcatgcataatatttgtttattcatttcttagtgtacatattttaactttatcagcgtagtaatttggtttgatttgtttgtttgttataatgtaattacaagtgtacttagcttgtttgattacacaagtgtaatcatataattatactgaattttaaagataaaagttaattatttgaaacaaaaaaattatattaggcaaataagagcctttataaatgatattcaattgaatatttaagatatatagtgtcttttaaaaaatatgttatttaataaacatatgttcttaattaatattataaaaaaagcaaatgatttatatatttcaatgtagtatttttaaagtaaattaatcataaaaattaaaaatgcatgaacatcatgaaatgcttgtttcacaaaaaaattaatattataaatataatgtcataaaatcatagaaaaataattgacaaaagaactaatttatcaagtctaacttaaaaagaataggttgcaatggaatatcaagtcaatactcctaaaacaaatgaaattgaaaatataatataagttctaaatttaaaataaaaaatttaacataatacttttatgtcaaatttcaacataatatgattaaaagaaaaggaaaatttaagtccgtaactttgttcaacaataaattctactttaattcaaaaattagaatactaacaaaattatactaataatttttttagatattatgaagaattgcatgaaatcacatgaagtaaaagttaaaaataagaaggaaatgaaatataaataataaaggaaaactttcatatatagccacttaaaaataattaattactctccatagctatagtttgataattacaatttgtagctacatgttatgtggaggagagagaggcgagcgtcacttggagagagaggcgagagagagagggggaaaagagtgggagaaaggtgaattgtatatgtatattggctagataattgtatattatacatatgtaattgtatatatggcaagagagattgagagagggaggagagaggcgagtgagactgtgagagagagagagaggcgagcgagatcaagagagggaggagagaggtgagcgagagagggcagagagtgagagggatgtgaattgtatatgtatataattttatataactgtatattatacatatacatttgtataaatggcaagcgagattgggagagggatgagagagacgagcgagagagggcagagagtgggagagaggtgaattgtatatgtatataggctaaaaaattgtatattatacatatttatttgtatatcctggcaaattatacatatataaacatgataattatacaaacatgaagtcaacccacgtaattaatgtataatgttagtcgcgagtggtaattataacaaactatagttatgatgcataattaaaataatataagtttgtttattcgcataatttttccttttttaaattcctccttctattcaacttgcattttttgtcaaatataatcatcgttaaaaattatttgatgttgaattaacaaacatccatctttattatatcacatgttgtgacatgcaccaaaacgataaaaacgacaccttcaaaatgattttttttaaaataagcctagttaattgatgtttaacatataaataatcaactaataaggttaaaggcttacacatacaaactaaaaattagatcaaatgcactaaaaataaataatatgaggaaaatctgttttagggattatagtgtcccccaacgaccaagtcttatttttaatggagcatcattgattggtctattgacaaagaaaatttggaaattaatgattttgttttatcctctggaaatttattatgttatcacaactatttgttaatttgaactgcataaaagtttttgttcgaacttcatatatgaaaattctaaacaagaattggaaacttgaaatgaatccaacatttaaatcaatagataattattgattgaatttcttaatacgtatatatacaaaagatctgaataaaagctattgaatacattacatgttatattggttaatttgaccgtaaaacagttgacattcttttgtcaagcatctattctggggaggttatatatatatacatttgaataatgacgttatactatagcctaaaactacataaaaaatgtcaagtaaattatttaactgtcaatacagaattccacaaccaatagtttatttccctttagcaatgaattgcagtcaagttcagctagcaatatacaattaaaagatgtttcaaatcattggtattaattagataagtattgactcaattacaagtatacacacagtatatatagatggcgtttgaaaacgaaaacataggcacaaatagcagctaaagaagttgaacaaatcaaaatggttgcgaagactattattatagcatgcctagttttgttaacatgcctctcagttactaatgcatcgaacattacaactgatgaggcacaaatgactatatctagtgaaattaacatgcagatgaataggcatatcttgcagtaaaaagcatcaaagagtgacatcattagtcctcaatagctttggatttagaggttcaatcgcgacagatattgggaatctctccttccttaactttttggacattggaaacaacagtttccatggccaaatacctgatgaaatagggcgtttgaggcgtttaaaatacatgtatttgcagatgaataatctcgctggtcaaatcccagaaagccttggatttctcacaaggcttcaagttcttcatctttctgaaaatcgtctatttggaaatgttccagcttccattttcagcgtgtcttctttaaaggacattgatttgtctcagaattacgagttaactgggagtttaccaaatgagatatgcactaatcttccagtgttggaatatatatccctgcaagataatcaatttgtaggtgaacttcctaaaggtttaaataaatgctccaaacttgaagttctgtccttgtcttataacaaattcactggtaattaactaacttgtaaacttttcatttactaatttcttcttgaattaatcatcatttttgtgtgtgtctgtgattttataattgataggaaacttaccaagagacatgtggaacatgtcaaaggttcaagaactttttattggatggaataacttaacaggtacgtgattctgtatgtattaaatcttgaatactcttcacgaagttcctaatttcactagatatagccaatttgtgcattgtctagtaataaacaaagattaatatattttgtggagaacattttcgaaagacactctatgtatgatctttagcatgataaccatatacttattttcaaaatgaatttgcaggaaatataccaaatgaaatgaacctaccatctatttgcaggaaagttaacaaagcttgagcatcttgttgggttatgggtctttttcccttcctatttggataactaaaagcccaatttggaccaatccatttttgcctataagcccattcttatgaggcaaatataaactgattttagggtctgattttcagaacatatagagagttcttcagcagccaaaaagagagaaagagagattttcgcaggcaaaattcagatctaatagacaacttcaaattgcgattcccgcttcttttcttatccgattgagttgatttttggacagcatattgtcttcatctcaatctttgattagaaactgacagagttggatttggtggcctgcgactttcagttttgcttttgtcgtgagcgaagctgcaaaattggtgattttgctcctttaattttctagatttggtgcaatcttattttgttgttgctcgttgtttggcacttgttttgtggccaattttggagaacaatattgtaactcttggtgattatagtggagcttttggtccgtggtttttactcttcacatgaagggttttcaacgtaaatcttggtgtcttatgtgattggtttcacattgtcttgttatatttgtttggttgaattggaatcgccttactatcatattgcttgtggttgtttgtcttctcttggttcaaatcgaaaaagggaaagtatagacttggatattcttccgttatctgtcgtcagcattcttggtagtgtcttgtctttcccaacaaagtggtatcagagcattgggtattgttgattgtcgttttgaatgatggagacaaatatgagcaaaatggtgtttttaaatggtagtaactatcatatttggaaaggcaagatgaaagatcttctatttgtcaagaagatgcatttacctgtgtttgtttctaataagcctaagtctttgaatgatgaagaatgggaatttgagcatcatgcaggtttggctatattatacaatgggttgaagataatgttattagaaatcagtattgtgaatgagacatgccaaaagtttgtggacaagtcgagacactttatgcttcaagattgtgtaacaactgctcctattgaacaattaatgaatatcgtataaagagggcactcctatttctgatcatattaatgattttagggggttcttgaccggctgtccgaaatgggtgtaaagtttgatgatgagatacagggactttggcttcttaataccgccagatcttgggaaactcttcagtttctttgaccaatctgctcccaaagggtgttgtaaccatcggaatatactaaaagtagtgtcttgaatgaagaaataagaagaagatctgacctcatcttcagacttctacactccgatgtttttccactgaagatagggggagaaacaagtcggtaggaggaatgatagaggtaaaagtgtatgtcaaagtctaagtctaacacaagaatattacatgtgactattgccacaagaatgggcatatcatgaaatattgttacaagcctgagagatatgagacaacaaaaaagagaaggcgataatgaaaatcgtgttgttgttgttgctaatgatcttctttctttttttcttgatgcaaatgccattaatcttgttcgtgatgagtctagctggtttgtggattcgggtgctacttctcatgtcatgccaaagaaggaattctatttcttatactccggggtaattttgaaacgttgaaatgggcaataatcatgaagttgaagttattggcattgggacagtttgtttggaaaataacaatggttcaaaactagttctcaataatgtcaagcatactccggatgttcgcttgaatttgatttacgtaggatatcttgatgatgaggttatgttaaacacatttggtgttggctagtggaagcttactagaggtttgatggttgtggcccgtggtgacaagttgtctaactttgtatgtatttggggctccgtttcgagagactcaagaatttggtagagaatgatacttatcgaagttatggcatgtaaaatttgagtcatatgagcgagaagaggattgatagtttggctaagaaaaatttgctttctggagtgaaacaagcaaagttgaagaaatgtgttcattgcttagccggtaaacataaagagtttcttttgaaatcatccgccttcaagaaagcttgatttgcttggagttggtacattcccgattttgtggtccttttaaggtaagatcccatagtggtgcaattttactttgtgactttttattgatgatcattctcgcaaactcggggtatttcctttgaagtccaaggatcaagtacttgatgtgttcaagagttttcaggccttggttgaaagacaaacaggaagacattgaaatgcatccgctcgaataatggtggtgagtatattggtcctttttgatagatattgaagagagcggggtattaggcacgaaaactcctccaaaactcgcggttaaatggtttagcaaggaggatgggcagaactctagttgagaggcttagatgtatgctctcggatgctaatttgccattcctttaggcggaagcacttaatctgccgcttatgttatcgatttatctcctttgttgctttagatagatggtgatgtcacagcggagtttgggtggtaagaatgtttcttatgatcatcttagagtctttgggtgtaaagcctttgtacatgtttctaaggatgaaaggtcaaagttggatgttaaaactaggcgaggtatcttcattggttatagtcaagatgaatttggctatcgtttctatgatctgttgagaagaaacttgttagaagccatgatgttgagttctttgaagaccaaacaattgaagattttgacaaaagtgacaaggctgattttcgagtagtgagagcttagttgatgttgatccggttcctttgactattgccgaagaaaatcttcttaatgaagaaaatcaagttgataatgaagatggtgatcatgttctaatgaccggcatgatgttgtttatgctcccaagaagatgatgtggttgtccaacaaccaattatagatgctccggagagttctctcgcacgatctagtagagaattccttcatctcgtgattctcctaatgagtatgtacttgacttacggggagaacccagagtcttgatgaggccatggaaagtgaagaaaaagaaaggtggtttgatgctatggaagatgagattaaatccttgcatgataatcatacctttgatttgttgttacctaaactgaaaaactttttgaaaaaaggtgggttttttcgggtgaaacatgaagatggtaatccggttccaccagacaaagctagattagttgtcaagggatttaatcagaaaagggagttgattttgatgaaatattctctccgattgtgaagatatcatccattcggtgtggttctaggtcagctgcaagtctagatttagaggttgagcaaatggatgttaaaaaccgctttcctccatggtgacttagactaagaaatttatatggagcaaccggaaggttttgaagtcaaggtaaaagagaattatgtttgcaaattaaagaagagcttgtatggtttgaaacaagctcccgtgcaaaggggtacagtgaagtttggttttttatgagtcaaaggggcttcaagaagacttcttaaccattgtgttttgtgcaaagttctctgatggtgacttttattgttgcggttgctttatgttgatgacacgcttgttgtcgggtcataatacttgcagtaggatcaagttgaagcaaggagtcgaggcaagtctttttgcatgaaagacttagaccaaagaaggcagattcttggcatgcagattgcccgtgatagaaaaagccaagaaattggtattatcacaagagaaagtacatttttaaagtacttcaagcagattcaaagatggacaaagctaaggttgtcaagacaccttagctatgccttcaaattgaaagcatggaaatgctgtcctttctagcgatgatggaaaggaagatatgaagaaagttccttatgcttcaaattggtagtttgatgtatgcgatggtttgtacaagaccgatattgctcacgctgttgagttgttaagcgggtttctttctaatccaggaagagaacattggaatctttgtgaagtgggttatgagatatctcatggcacttctagtccgagtttgtttttggcagggaagcctatttttttgatttatcttgattaggacatggttggtgatgttgatactcgcaagtctacttggtgcttggttacttttaggggagtattgtcttggcaatctagattgcaaaatgtgttactctatctctactatggaaggcttattcttttcgtgaagcttgtaaagaattgctttggatgaagagattattaagaacttggtttgtgctcaaagaggtatgtactttattgtgaccggtcaaagtgctatacatcttggcaagaattctacgttccatggtcggttaaacacattgatgtgagataccatttgattcgagatgtattggattctaagttgcttgagcttgaaaaagattcatacaaatgacaatggttccgatatgatgactaaagctttgccaagaggaagtttgaagattgttgcatggtcgtggggacgggcggtcctccacatagtcgtgagggagaattgttgggttatgggtcttttttccttctatgtggataaataaaagcccaatttggaccaacctatttttgcctataagcccattcttatgaggcaaatataaactgattttagggtctgattttcagaacatatagagagttcttcagcagccaaaaagagagaaagagagattttcgcaggcaaaattcaaatctaatagccaacttcaaattgcgattcccgcttcgtttcttatccgattgagttgatttttggacagcatattgtattcatctcaatatttgattaggaactgacagagttggatttggtggcctgcagcttcagttttattgtgaggaattagctgcaaaattggtgattttgctcctttaattttctagatttggtgcaatcttattttgttttgttgctcattgtttggcacttgttttggccaattttggagaacaatattgtaactcttggtgattatagtggagcttttggtcccgtggttttactcttcacatcgaagggttttccacgtaaatcgtggtgtcttgtgtgattggtttcatattgtctcgttatatttgtttggttgaattacctgctgccttagtatcatattgcttgtggttgtttgtcttctcttggttcaaatcgaaaaagggaaagtatagacttgggtattcttccgctgttatcctgtcaggcattcttggtagtgccttgtctttcccaacacatctcaactatctgaatgtctcttacaatgagttatcaggtgaaataccagatggagggccttttggtaattttcacagctgaatcattcatcggcaatgaagagttatgtggaccgcctagattccaagtcaagatttgtgaaatccgaacaacgtgacaagaagaaacaggaaaaaacaagactaaaatttgttcttggaccagtgcagctggaggtttagtcatggggttttaggcatgatatggttgttgaattatcggagacgtaacaaccaacttattcctttaactgattagtatgatcggttatcacacaaaaagttttcttactatgaacttgtttgagggactaacaactttgactttaatcaaatttgattggaaagggaagccttggtatggtttataaggggacatttacaaatgggactatagccaactgtaaaggttttcaatgctggcgcaagatgcattcaagaggtttgatttggagtgtaaggttttgcgtaacaccgaaataggaatcttgttgggtgataagtagttgttcaaatcttgattttaaggcattggtgtttgagtacatgcctaatggagatcttaattattggctttactcacacaacaatttcttggatttaaacaaaatttgaaaattatgtttgatgtggctttgtgtcagagagtatctacaccaaggccattcaaaacatagtggtccatcatgacttgaacatacttttggatgaagacatggttgccgagtaagtgattttggtatattcaaactcttgaccgccagatgatccaaagggcattgacaaagactttaggcaccattatcctggcactgtgcccgatcaaatttttatttactaattactttcttcaacttgtattcgatatgcatatatgatgtatttcattttaatggtagagtacgggtcagaagggatagtgtcaactatgggggatgtttacagctacggcattttatttatggaaaccttcataagaaagaaatgatagatgatgagtttgttggagaccttacattgaagagatgggtcatggaatcatatcctcatagagtcattgttatgaaataaaaacgaatacaagttgaacgtcaattatgagtcatttatctaatatgatccattaacaattgattaatgtaacgcaggaagaagaaaacaatttgcattgttatgaatgaatgtgtttgtactacaatatatacaaagatcgacaagtctagcaaactttctaaccaacttattctaaccaactctactcattattcatttagctcacttaatcaagaaattagacctaacaactaactaccattaactcattcaactgattgttgggttataggtctttttcccttcctatgtggataaataaaagcccaatttggaccaacccatttttgcccataggcccattcttatgaggcaaatataagcctatttagggtcttattttcagacaaaacagatcagtttttcagcagccaaaaagagagaaagagagattttcgcaggcaaaaatttagatctaatagctaacttcaaattgcgattttcacttcgtttcttatccgattgagctgatttttggacagcatattgtcttcatctaaatatttgactaggaactgacagagttggatttggtggcctgtagcttcagttttgctgtcgtgaacagtagctgcgaaattggtgattttgctccctttaattctctagatttggtgcaatcttattttgttgttgctcattgtttggcacttgttttgtggccaattttggagaacaatattgtaactctttggtgattatagtggagctgttggtccgtggtttttactcttcacatcaagagttttccacgaaatcttggtgtctttgtgattggtttcacattgtcttgttatatttgtttggttaaattacttgccgccttactatcatattgcttgtggttgtttgtcttctcttggttcaaatcgaaaagagaagtatagacttggatattcttcatttgttatcccgtcgagcatcatttgttattgccttgtcttttcccaacaaagtggtatgtcaggagcattggttattgttgattgtcgttttgaatgatggaggcaaatatgagcaaaatggtgtgtttaaatggtagtaactatcatatttggaaaggcaagatgaaagatctttatttgtcgaagatgaatttacatgtttgcttctaataagcctaagtctttgaatgatgaagaattggaatttgagcatcctgggtttcggctatattagacaatgggttgaagataatgttagaaatcatattgtgaatgaaacacatgccaaagtttgtgggacaagctcgagacactttatcttgaagacggcaacaaacaagttgttctattgaaacaattaatgaatatcggtataaagagggcactctatttctacgatcatattaatgattttcagggtgttcttgaccagcctgtccggaatgggtgtaaagtttgatgatgagatcacaggggactttggcttcttaatactcatccggactcttgggaaacttcttctagtttctttgactaattgctcccggtggtgttgtaaccatggaatatactaagagtggtgtcttgaatgaagaaaatgagaagaagatcttgcctcatcttcttaaacttcactccgatgttttggttcttgaagatggggagaaacaagtcagtagatcgaatgatagaggtaaaagtagaagcaagtcaaagtctaaatacaagaatattacttgtgactattgccacaagaatgggcatatcatgaaatattgttacaagcacaagagatatgagacaacaaaacaagagaaggcgataatgaaaatcgtggttgctgttgttgctaatgatgatcttcttttttcttgtgatgcaaatgccattaatcttgttcatgatgagtctatttggtttgtggattcggtgctacttctcatgtcacgccaaagaaggaattattttcttcttatactccgggtaattttgaaacgttgaaaatgggcaataatcatgaagttgaagttattggcattgggacgttttgtttggaaagtaacaatggttcaaaactagttctcaataatgtcaagcacacccaaatgttcgcttgaatttgatttccgtgggatatcttgacgatgagggttatgttaatacacttggtgttggcggtggaagctcactagaggtttgatggttgtggcccgtggtgacaagttgtctaacttgtatgtatttaggggctccatatccggagactccaagaatttggtggagaatgatacttcatcgagttatggcatgaaggtcgagtcatagagaaggggattgatagtttggctaagaaaaattttctttctggattgaaacaagcaaagttgaagaaatgtgttcattgcttagcgggtaaatagaaaagagtttttttttagtcatccgccttcaagaaagcttgatttctttggagttggtacattccgattttgtgtggtcctttaaggtaagatctcatggtggtgcactttactttgtgacttttattgatgatcattctcgcaaactctaggtatttcctttgaagtccaatgatcaagtacttgatgtgttcaagagttttcgtgccttggtttaaagacaagcagtggaagacattgaaatgcatccattaagataatggtggtgagtatattggtccttttgatagatatttgcagagcggggtattaggcatgaaaaacctccaaagactccctcggttaaatggtttagaagcagaggatgagcgagaactctagttgagagggttagatgtatgcttttagatgttgtcgtcgattccttttgggcggaagcacttaacatcgctgcttatgttatcaatttatctccgttgctttagatggtgatgtcctcgatgtagtttggatcgtaagaatgtttttacatcatcttgtagtctttgggtgtaaagcctttgtacatgttcctaaggatgaaaggtcaaagttggatgttaaaactaggcaaagatatcttcattggatatggtcaagatgaatttggctatcgctttctatgatcccgttgagaagaaaacttgttagaagtcgtggatgttatgttcttttgaagaccaaacaattgaagattttgacaaactgacaaggctgattttgagagtagtgagagcttagttgatgttgatccggttcctttgactatcaacttgggaagaaaattttcataatgatgaaaatcaagttgataatgaagatggtgatcatgttcagtaatgacctatgacgatgacgctttttgatgctcgatgcagaagatgacgggttgtccaacaaccaattatagattctccgagagttctctcagacgcatctagtagagagagatttcttcatctcgttattctcccaatgagtatgtactcttggtgacggggagaacccgagagtcttatgaagccatggaaagtgaagaaaaagaaaggtggtttgatgctatggaagatgagattaaatccttgcatgataatcatacctttgatttggttaagttacctaaaagcgtaaaaagctttgaaaaaaaagggttttttttgttgaaacatgaagatggtaatcaagttccacggtataaaagtagttgtcaagggatttaatcggaaaagggagttgattttgatgagatattctctccgggttgtgaagatgtcatccattcgtgtggttctaggcttggtacgcaagtctagatttaagttgagcaaatggatgttaaaccgcttcccatggtgacttagatgaagaaatttatatggagcaaccggaaggttttgaagtcaagggtaaagagaattatgtttgcaaattgaagaagagcttgtacgggtttggaaacaagctcccaaagcaaattggtacagaagttttggttctttatgctggggaaaggcttcaagaagacttcttcagaccattgtgtttttgtgcaaaagttctctgatggtgactttattattgtgttgcttttatgttgatgacatgcttgttgttgggtcataatacttgcggggattcagaagttgaagcaagagttgagtaagtctttctttatgaaagacttaggaccaaagaagacagattcttggcatgcagattgtccgtgtgatagaaaggctaaaaattggtattatcacaagagaagtacattcagaaagtacttccacagtattcaagatggacaaagctaaaggttgtcagtgacacacttttagctatgcacttcaaattgagcactagcttaggtgtccttctagtgacagatgagaaggaagatatgaagaaagttcttatgcctagctgggttggtagtttgatgtcacgatggttttgtacaagaccggatgttgctccatatttggggttattaaccgttttcttttctaatcgggaagagagaacattggaatctttgtagtgggttatgagatatctttgtggcacttctagtaaagtttgtgttttagtgcagaagcctattctttgtggttatccggattcggacatggctggtgatgttgatactacgcaagtctacttgatgcttaattcttttttgtggggagctgtgtcttggcaatctaggttgcaaaatgtgttgctctatctactctctgctggaggcttattctttatcgttgaagcttgtaaaattactttggatgaaagattaacacgggaacttggttgtgctcaagagaggtatgtgctttattgtggtcaaaagtgctatacatcttggcaagaattccacgttcaatagtcggtctaaacacgttgatgtgagataccattggattcgagatgtgttggattctaagttgcttgagcttgaaaagattcatacaaatgacaatggttacgatatgatgactaaagctttgccaagagggaagtttcaagattgttgcatggtgcttgggatggcgggcctccacatagtcgtgaggggggagaattgttgggttataggtcttttttccttcctatgtgataataaaaagcccaatttgaccaacccatttttgctcatagcccattcttatgaggcaaatataagccttatttaggatcttatttcggaaaatgacagttagttttttggtgagccaaaatagagaaagagagattttcgcaggcaaaaattcagatctaataaccaactttaaattgtgattcccgcttcgtttcttatccgattgagctgatttttggtcagaatattgtcttcatctcaatctttgactaggaaccgacagagttggatttggtggttcggtaacttcagttttctttgcgaatgagcgatggctaaattggtgattttgctcctttaattctctagatttggtgcaatctttttgttgttgtcgttgtttgacacttgttttgtggccaattttggagaacaatattgtaactcttggtgattactggtgggagcttttggtcctgtggttttttactcttcacatcgggccgattttccgtaaatcttgatgtcttgtgtgattggtttcacattgtcttgttatatttgtttggttgaattcttgctgccttactatcatattgcttgtggttgtttcttctcttggttcaaatcaaaaggaagtatacttgggtattcttccatcgttatcctgtcgaggcattcttatttgtgccttgtctttcctaacactgatcacggaacatcaacacattttgttgatttctttcacacacacctcctcaaaaaaccctcttttttaacatgtaagcgacaatatcttttttaggagagtgttcaacattgagcataaaaataataaaatagagaacaaaaaaagatgagtataaaataataaataataatataagatcgattttaccgattgtcaattttgtgtatgaactaaagaaataacagcttcacatatgaatttgtattttaggctgctgtaagtactaaaaatagttattcaaccagtagaagagatgaaggtgggggccagctgttggcaatcaataagggaaagaaaagacaaggaatattgagccaattttttttcttctgtggaaaactttggcagagaaattaaggctaacgaaaagtctttgtgcaatgaccccatgggcatgtgcagttgtttcccacaactttgtgaattatattccaaaaaatacaaattcattatttaatactccaacaactttttgattccactctagactaccatcacatatctaatattaaatgtaatactgaatttcacatatggtcagaggcgaatccatcagcacctgatatattctttttttaaaaaaattatatctatatatacagattgttgataagacggtaatatatttaattgtgcactcttataacgaacaaatgatttgacttgtccattggaaaaacaaaaagtgtcacataaattgagacatggcgaataatatttctttcctaaatttttcgtgtgaagtcaaattaattcatataaaattagacgaaaggagtaatgtttaatagtaattgcatatggtagtaaatttgatagacgtggtcccgtgggagtgtgtgttatttccattgaataattgagtttgtaattgttacaagtccattctaatttccaacaccttacttcatttcaaaaatatactctatggctgaagctttccttcaaattatgttagagaatctgacttgtttcatccaaggggaacttggattgattcttggttttaaggatgagttcgaaaagcttcaaagcacgtttactacaatccaagctgtggtacaagatgctcagttgaagcaattgaaggacaaggcaattgaaaattggttgcagaaactcaatggtgctgcatatgaagctgatgacatcttggacgaatgtaaaactgaggcaccaattatacagaagaagaataaatatgggtgttatcatccaaacgttatcactttccgtcgcaagattgggaaaaggatgaaaaagattatggagaaactagatgcaattgcagcggaacgaattaagtttcatttggatgaaaggactatagagagacaagttgctacacgccaaacaggtaaatatttttctaaataacagctttatatcatcaaattcatgtgtgttttggggattttgtctaagtagataagtggttcaaaatctattatctaaatctgtttggtgaagtctttaacatatatataaatccatagcttactcatatgccccaaagtctaaatgacaggataaagccagagttgttttagatcttataaattaacaatgataataatgtgaattcaaaatagtgcatttgttttatatttgaaatatgtctgctgcttctgatcaagctgatcattgtcttttgcaaaattcttctttgttttttttgctgactcttaccgatcttggaccaggttttgttttaaatgaaccacaagtttatggaagagacaaagataaggatgagatagtgaaaatcctgataaacaatgcccaaacactttcagtcctcccaatacttggtatggggggactaggaaagacgacccttgcccaaatggtcttcaatgatcagagagtaattgaacatttccatcccaaaatatggatttgtgtctcggaagattttaatgaaaagaggttgataaagaaaattgtagaatctattgaagaaaagtcacttggtgacatggacttggctccacttcaaaagaagcttcaggacttgctgaatggaaaaaaatatttgcttgtcttagatgatgtttggaatgaagatcaagataagtgggctaagttaagacaagtcttgaaggctggagcaagtggtgcttatgttctaaccactacccgtcttgaaaaggttggatcaatcatggggacattgcaaccatatgaattgtcaaatttgtctcaagaagattgttggttgttgttcatgcaatgtgcatttgggcaccaagaagaaatgaatcttaatctagtggctatcggaaaggtgattgtgaaaaaatgtggtggtgtgcctctagcagctaaaactcttggaggtattttgcgcttcaagagagaagaaagacagtgggaacatgtgagagatagtgagatttggaatttacctcaagatgaaagttctattctgcctgccctgagacttagttaccatcaccttccacttgatttgagacaatgcttttcatattgtgcagtattcccaaaggataccaaaatggaaaaggaaaatctaatctctctctggatggcacatggttttcttttatcaaaaggaaacttggagctagaggatgtaggtaatgaagtatggaatgaattatacttgaggtcttttttccaagagattgaagttcaatatgatcgaacttatttcaagatgcatgatctcattcatgatttggcaacatctctattttcagcaagcacatcaagcagcaatatccgagaaataaatgtagaaggttacctacatatgatgtcgattggttttataaaagtggtgtcttcttactctcctcctcacttgcaaaagtttgtctcattgagggttcttaatctaagttccatgggacttaagcagttaccgtcctccattggagatctagtacatttaagatacttgaacctctctctcaataacatgcgtactcttccaaagcagttatgcaagcttcaaaatctgcagactcttaatgtagagtattgctggtcactttgttgttttccaaaagaaacaagtaaacttggtagtctccgaaatctcttacttgatggttgcgatggattggattctatgccaccaaggataggatctttgacatgccttaagactctaagtttatttgttattattagagaaaagattctctacttggtgaattacttaaacctgaatctgtatgggtcaattgaaatcacgatcttgagagagtgaagaatgatagggatgcaaaagaagccaatttatctgcaaaaaagaaaatctgcattctttaagcatgagatgggaaggaccacatagatatgaatcagaagaagttgaagtgcttgaatccctcaaaccacactccaatgtgacttgtttaacaatcactggcttcagaggaatccgtctcccagagtggatgaatcactcagttttgaaaaatgttgtctctattgcaattagaggttgtgaaaactgctcatgcttaccaccgtttggtgatctgccttgtctagaaagtctagagttacggagtgggtctgcggaagtggagtatgttgaagattctggattcccaacaagaagaaggtttccatctatgagaaaacttactatagaaaattttgataatctgaaaggattgctgaaagaggcaggagaagagcaattccccgtgcttgaagagttgacaattagatgttgtcctgtgtttgttattccgaccctttcttctgtcaagaaattggtagttcatgggaacaagtcagatgcaatagttttgaggtccatatataatcttagggctcttacttccctcaacattagccataacttcacagctacttcgctcccagaagagatgttcaaaagccttgcaaatctcaaatacttggaaatcgctttcatctccaatctcaaagagctgccaaacagcctggctagtctcaatgctttgaagcatctgtttattaattgttgttttgcactagagagtctccccgaggaagcggtgaaaggtttaacttcactcacacagttatccataacatactgtaagaggctaaaatgtttaccagagggattgcagcaactaacaaatttatcagttaggtattgtccaacactggccaagcgatgtgagaagggaataggacaagactggtacaaaattgctcacattcctcatctgctgattactgattagatgtaattttctgatttttcttttggaaacaaatcaactatttataacatctatttgtattatacttgatttttcttgattatgtaacaataaatatttgaaatttttcatattaaagattcagaatgagttttacagctaactctatattctcacagtttaataacgtaaatatgatatttatatcaaattattacttatgttgtgatttgatttatcaacatgttggagatgattttgacagtttattaaagaatttctaagtttttattgtttgcacaagtaacaagccataaattaagtttcgagataaaagtaatttgtgtatcatggcttaattagtcggaatttcaagttttttctcaagttatatatatggcaatttgtaaaaaatagatagtattcattttgatttaattcaagtatttttaaaaatatatacaaataatatgggggatacacacgctaaacgcgtacccaaaaattagtatataaagaataatgacgaaaaaataaaatgaagttctatcaccaactatctctacatcttttgctgatatatatatatatatatatatatatatatatatatatatatatatatatatatatatatatatatatatatatatatatatatatatatatatatatatatatatatatatatatatatatatatatatatctaactagtgtacttattcggacttgacatggtataaaaagatattaaatatattttaaataattaataaatgatataataaaaagagaaatacaaaataagttatgattctgataaaaggaaacttacataaatgtgttataataaaaaaatatttaccatttatagctataattttttttttcactcgatcacttttaattaatttataatacaagtttaatatatattacaaagaacaatttattattcacatacaatacaagttttaatgatggattttatcacacattttaatacacttataatataatgttactattttttaccaaacaaacacaatatatttcaaaaacaattataattcaaatatattgcataaataattcacttttaataaatattacagatttatcacaatattgctataaatgataataaacaaaagtatcgctaaaatcagtaattattttttaacatatattaattcatgtaatttttcttattatctattcagaaaaattgcttaaaaaatctcatttgacattttcaatttaaaattgttgataaaaaagacaaaaacataaaaattgatatgaaagagctttggttaagtagcaatctaattacatagtggcatactaaattaaatgattcttatagcaatattattggttcaaccaacaaaactaaatctctagttatattacttaattgctcatcatagctatagtttgttataatcatcactcgcggttaacattatgcatcaattacgtgggctgacttcgattttgtataattagtcatgtttttatatgtactagattctgagaacatgccttgcacgtttgtcctttattattattaactttttatatactaaaaagttaagtaattaaaaagatgcttaaataaacaataatagtttaaccatttatcttttattcgctaaataataactaatataatatgaagaacattaaatagatgataatatctaccttagtaattggttcttaaaaagcatattaaaaatttaattctcaaagtgtttttacataaatagtggagaatgactcttcacattgagcttttaattttaaaaaattatgtgtatgagaaataattaacattcaataattaggtagaataatatcacattatcataaataaaataatatctctaagtcaaaagtagacattctagtttggaaaataattactactaactatttatgggtccagctccaatcaataatctatagatgggagtttgacaatttttcagctatagttaaaattttacatcaacaataaataacttattatcacagtagatagacgtttgatgcataaaagttataaatgctaaaagattttgtcaatgtagtacatatgcaaacttatgataaaaacacttggtatattacgaaacacacttgaagccattaccatgattaacatatcaattatttttatcattatatcacatatacgtcttctttttaaccttaaaagtattgtacacatgatttatgaagagaaaagaatagtactccttttttcatgtaacgacctgtttagtcgttttgagcagcagaatttatttctggaaaaactgtctgagtcaacggaacccacgacggaccgtcatgggcacgacggaccgtcgatggtgtctcattccaaaacacttagaattttgaaatttgggtctgaaatcgactctccaacttcgtgcttgagatggccggggcgaacaagtaagtggagccgcacggctgcaccgtcacaaatcttccatggggaagtgatccgaatgtgtggatttggcggggagatgccgtccacgatccacgacgggacgtcactgttgcgcgtaatcccggtgggtcggatttctgttaagtgatttaaggggcgttttggactattcctgctttaattataaagttagtgggttaatgttaataagtttaattacttgggggttaaaagaggtaaccttgagttaattagtgggttattattgacatctttatacttaattatattctaattagggtaaaagaaagagggtttgaataagaaacaatagaaagaacaatgagagggaaagagaaacgagaaagagagaaacgaacgaagaggaaaacacaagctttgggaaaattgctttcttgatcaaaattcttcggtggaggtaggttattgtttttatactattcgtagtaaactcttaatagcgaatgatatgtgttgggttgtattgtaaagtcttctatatgcttaattgtatgcttgtataaatgtgattatataattgtgataaaataagcaagataaagctattgaatcccaaatcttgaaaaccccttgttaatgatgatgccttggtataaaagaaggcttgatgaactaaagtaatgatattgatgatgtcttggtataaaagaaggcttgatgaactaaagtaatggggttgatgatgccttggtataaaagaaggattgatgaattaatagaatgagattagtggagcgggtgtcacgaaccgacacatagtattagggggaccgggtgtcacgaaccgacacgtagtattagggggaccgagtgtcacgaaccgacacatagaattaggggatcgggtgtcacgaaccgacacgtagaattaggggatcgggtgtcacgaacccacatgtataattggggatcgggtgtccgaaccgacacgtgggaattaggagatcggtgtcacgtgcggacaaatagtagtaggggcgggtgtcacataccaaaccaagaggaataaagataatgaatcttgaaagatgttaatatactcaatctaatgaacctaatcccaaataggtatggtattgaggcttgagtctcatgtgaacttggcggtgcttattaatgattatagtacttgttgttgttacacatattgagtattgtagttgatttatgatattatcagtatatcttttgttttctattttgagttggccgatgatacctacctcgatgcccgtgttttatcttgaccctacttgtatttgttttctttgttatttgtggagtgtagcaagcgtaccgtcgtcttcaactcattgccaactctgtgatcttcattacaccggattttagggtgagctaatgcttctagcttggactggatcttcttcctcatgtcttgatgccttgaagttccggcatggactagattttgtttattttagcttctttagaatactcttagtttagtaatttgatcatagatgttcttgtggtgatgacgggattttggggaatactagttgttgaattttagaagttattgaattggttttattaatgagtttaagtcttcatattacttctgttgatattatattgaaatgttggggtttagattggttggttcgctaacataggatggtaagtgtgggtgcgttggctcggttttgggtcgtgacaaacttggtatcgagcattaggttcgttggtctcatcacacaagagaaccagtctagtagagtcttaaggagcgtagggggggccttttacttttctttgagaggctataagactttaggaaattttcctttcttttctttttctttattacttggatccaattggtatctaggtgatacaaattggtaatcgaccatcttcactctatttttcgcaaatggttagaacaaaagcgacgactaacaacagcaccgatagcgcgggcggagcgaggtgcgtcccgggcgtgctggggagtacatggctgggaaggcggctgacagaggccgtggtgaaattaggtggggagacgtctacaggggacaaacaccgccccatagtactgggcggtgactcactccacccggtaggtggtaagagagggtgaggaaggaggcccggcaagtgcgaggagatgaggaactaccgctgacctacccggagatgataaatcaggttctgcttaccttagtaggttgctctgatcaaggtcaaacacctcgatgtttctgctgcttctctcgggttttggaaatacgacgggcaaaatctgtttcacgcatggatatgccattggaagcgaaactatttcctcgtttgactacggggcctatgatgacaagcggtgacaaagatgaaccaagaagggattgaaattgaaacctccgtcttcaagggtgctaaccgggatgcctacgattttccgtcgattgtcatgagttaccaagataaaatgggcatagtggaacgattcggtgttgagtttttggacttatcagtttcaaaggaacgccaaatgcgcggcggtcacatgttgagtgtcaaccaacggaggaaccacctatgacttggccattctctagcttatttatggaagtatatcccctgaccttgagggataggaggagatgagttttttggcttagagcaagtagaacgacggtcacttcatatgaaggctaagtttcgtgcattatctaggtatgtcactttgcgcccgggttcacaagaagcggattcaaaccgttttgtgaaaggggttgaggtcagttttcagcccttttgtagcggtggcaaaatgaaatccttccagaaagtggtagacttctgtgatagaggtggaggagtaaagtaggatgacttcaccatggcatcgacatcaaaaaggtttgaaaagggagaggtttaatggttcttacactacagggcgagagttcgaggattttcggtgggccgttgtctgctcaggaggctgtggtggggtccgctaccggaccgtgacatttctgcgggagtagggtcattccagacctcaatcattctcacaaatactatactgggctccagagaatgttatggatgtgggaggctggaccataatgggaagttatgacgaggtcccatgggccaggccagctaggtggggtggtggtaggagaggcagttgataaggaggccagtggccaggtaatgggtgagtcctgaaggcagccaggagtgaggacaagtgaactacaaccttaccacatggtgagggcagccgaggcagcaggcaaattagtaggggctacggctgtgcagcctcgcagtctggcggggacatcagatgttgttatcaccggtaatcttttggtttgtgattgcatggctacgtcattatcggatcctgatccacatttcatatgtatcttcctatttgttactggtgtaatttacattgtgaattgcttgacatgctatttgtgtttctactccgttggtgagtcatgatagttgaaaaggtatataggtcttgtccgtgacttttgtggggagcacactcatgtagatttggttattttagaaatggttgatttctgatgtaattacgggtatgacttgctttccaaattttgcaatcttagattgtaatgctaaaagcgtaacgttggccaagccagggacatccagattagtaatgggagtgtgactacacttccgctccagataaatatcatatcctttttcgtgctaagagaatggttagtaaagggtgtttagccttcttggcacctcagtgatgatactaagtaccttcgagtgagcctggggtttcggtagttcgtgagttttagacgtgttccctcgcaccttctccggtatgccaccgacgaggatattgacttttgcattgatttgggccgagtactcattcccatttcccccccttatagaatggctcaaacgagttaaggagttaaaagcccaacttcaaaaactgttaggggaagagctttattaggccgagtgcatccccttagggtgctttgtttttgtttgtgaagaagaagatgggagtcttcggatgtgcatagattactggcaactaaataaagtaactgttaagaacaggtaccctcttccctcgcattgatgacttgaccgatcgatttctaaggtgctatgtcttctctaagattgacttgagatggttatcatcaattgaaaatccaggcgtgagatatgccaaggcccttttcgaagacggtatgggcattatgaattcttggtaatgtcctttggactaacaaaatgcccctgctactttctgcgagcttgatgagcattttttaagccatatctatggatctctttagatcgtatttattgatgatatcttgatatactcaagagaaagaaggaacatgaggagcatttgagagttgtgttggaaatgttgaggagaaaaagctttatgccaaattctccaagtatgagttttggctagattgattgtccttcttgaggcaacgtagtttctaagggaggagtgatgtagatccttctaagatcaagtagttagaagaattgggtaagacctactaatatgtcgtaaataagaagctttgttggtttaaccattctaccgtcgatttgtcaagggattctcttccattgcttcccaattcgaacttaactaagcagaatgttccatttgtatggtcggatgaatgtgaggaaatctttcgtaaactcaagaccttgtttgacttcaccgcacctatccttacctttccaaagagagagggtaagaacttcattgtgtattgtgatgcatcatattctggttcgcaaaaaaaaaaaaaaaagtgctaatgcaagagaagaacgtaattgtgtatgcttcgaggcaattaaaggtgcatgaacgtaattatccaacccacgtatttggagttggtcatggatagtgtttgcattaaacaatggagacactatctatatggggggttaagtgaagtctatcacggatcatcgtagcctacagtatgtctttaccggaaagatttgaatttgagacggagggaggtggatggaactaatgcgaaggattatgatgtttaccatcttgtatcacccagaaaggctaatcttgtggcggtataggtagaaaaagcaggagcatggtagtttagctcacttgcaagcttctaggcgcccattggcctagagaggtgagactacggctaataactttatgagattggaagtaaaaaatgagaagggagtgattttttggcggtgtggaggcgtagatattcttttcttgacaagatcaaaggaaaaacagtttttaatgatgagaaattgatccgaattagggatatggtgttatgagggagagtctaaaaaagcaacaatcgatgaggaaggtgttttgagaatcaagggaagggtgatgtgtaccctgcgttgatgacttgatcaacactattatgagaggctcatagttcaaggtattttatacacctggtgcaaccaagatgtatcgtgacctaaagcaacacttttggtggagtagaatggtagcgacattgttgattttgttgccaaatgtccaaattgtcaacaagtaaagtatgaacaccggaggcaggaggaacactttcagagaatgcccattctgaatggaaatgggagaaattgcaatggatttcgtggttggtcttccaaagacaatgggtaaatgactctatttgggtgattgttgataggttaactaagtctgctcatttcattcgtcaaggtgacttacaatgctgagaaattagccaaactttacatccagtagattgttaggttcatggagttccactctccatcatatcggataaattaccagtttactttaagttttggagaacattgcatgcggaattaggtactaggttgaaccttagtgcgcatttcacccctcgagacgatggagatgatcggcgagcgattcaagtgttggaggatatgccgtgcatgtgtgatagaatttggtggccatgggatagcttcttacccttagcggagttttcatacaataatagctatcactcaagtattgacatggccccatttgaagcattgtatggtaggagatataggtctcccattgggtggtttgatgcatttgaggttagaccttgggggtcttgaccttttgaggttattagaggcggtgaaatctattcagaaaagcttttaagcggtaaagtaggcaaaaataatgtccggatcgaaggttagagacttaaggtttatggagggtgagcaagtcttctttgaaggttttcgccaaagaaaggggtgatgcggtttggtaaagaggtaagctaagcccaaggtatattggaccatttgaagtacttagcgaataggggaggtggcttatgaattagccttgcctcggggttgtcagagtgcatccggtatttcatgtgtctatgttgaaaagttaccatggggatggaaacacatcatcgttgggattgatctggctttgatgagaatttgtcccataagtatgagcctttgtgccattctagatagagaaattcgcaagttaagatcaagtgagattgcatccatcaaagttcaatggaagaatcgacccgattgaagaggccacttggggagaaggaagtcgatgtgcaaagaaagatacccacaacctacttacgtattcgtgtactcccgcttttttttttggcgtgatcgttcgaggacgaacgatgggtaaattggtatctattgtaacgactgcttagtcgcttttgagtattgattttatttccccgaaaaactgaagtcatcggaacccacgacggaccgtcacgggcacacgacggaccgagggtgtctcattccaaaacacttagaattctggaatttgggtaccgaatcgactctctcgaacttcgtaacgatggcgacggaccgtcgtgagcggcggaccgtcacacatcttccataggaattgagtctacgaacttctgtgtgacggcggcggagacggaccgtcgcagtacccgtcactgcaatcccgtaatcccagctggccggtcacattaagtgatttaaggggcgttttggactattccctttaattataaagttagtgggttaatgttaataagtctaattactgagggttaaaaagaggtaaccttgagttaatttgggttattattgacatctttatacttaattatattctaattagggtaaaagaaagagggtttgaataagaaacaatagaaaagagcgagaggaagagaatgagaaagagagaaaacaagcgagcgaaaaaacacaagatttgaaattgctttttgcttgatcaaaattcttgattggaggtaggttattgtttttatactattattagtaaactcttaatagcgaatgatatgtgttgggttgtattgtaaagtcttctatatgcttaattgtatgcttgtatgaatgtgattatataattgtgataaaataagcaagataaagctattgaatcccaaatcttgaaaaccccttgttaatgatgatgccttggtataaaagaaggcttgatgaactaaagtaatgagattgatgatgccttggtataaaaaaagggttgatgatgccttggtataaaagaaggattgatgaattaatagaatgagattagtggagcgggtgtcacgaaccgacacgtagtattagggggaccgggtgtcacgaaccgacacgtagtattagggggaccgggtgtcatgaaccgacacatagaattaggggatcgggtgtcacgaaccgacacgtgggaattggggggatcgggtgtcacgaaccggccacgtataattgggggatcgggtgtcaccgaaccgagccgcgtagaattaggggatcggagtgtcacgcatcgaccacatagtagtaggggagcgggtgtcgtcgcaccgacacaagaggaataaagataatgaatcttgaaagatgttaatatactcaatctaatgaacctaatcccaaatgagtatggtattgaggcttgagtccgcatgtgtgaacttggcggtacttattaatgattatagtacttgttgttgttacatgttgagtattgtagttgatttatgatattatctgatatatatactattttctattttgagttggccgatgatacctactcagtacccgtgttttgtactgacccctacttgtatttgttttctttgttatttgtggagtgtagcaaacgtaccgtcgtcttcaactcaaccgcaactctagccagtcttcattacaccggattttagggtgagctaatgcttctagcttggactggatcttcttcctcatgtcttgatgccttgaagttccggcatggactagattttgtttattttagcttcttagaatactcttagtttagtaatttgatcatagatgttcttgtggtgatgacttccagattttggggaatattagttgttgaattttagaagctattgaattggtttttattaatgagtttatgtcttccgcattacttctgttgatattatattgaaatgttaaggtttagattggttggttcgctcacataggagggtaagtgtgggtgccagtcgcggctcggttttgggtcgtgacatttcataacattactctttgaataattaatataaattgagcaatataaacttttcaaaatgacttattctagatatatgatcaatttgaggaatgaatgttccaacaaacatataatagactaataagatcaataaattatacatataaacgaaaagtttaaataaaaatacaacctcaaaatcacatatatactacatagaatatgattcattctttatctccaattaggtgggtcatttttattttagttcatatatatatgtgtgtgtgtgtgtgtgtgcgtgtgtgtgtgtgtgtggcgtcttggcgtcttggcgtgtcttggtgtgttaatgtgcgtgtgcgtgtgtgtgtgtgtgtatgaatttcatcagtaattaagatacatagtagaacatgaattgtatattactattttcttcatgtaggatacaaaatattctaataaaaaaatctaagaaagtacatcaacatatataaaaaggaaatatataatacttaggacggacaaaaggagcggataaaaacaaaaaataattactacacatacaaaatgatttgcaaagttcatttttgcatgataatctctcatcctcttcttgtcatatacatgaagatcatgctagataatttatagaagtagctatgatgacctttgaatagataattaatttgcattaaattagttcaatggttttagtccatatcaaatttgtttaatggaaaaaattttcaaatactcctgattttcacaatagagtaattaattattaatgtgaatttgatacatgcatcaatctaaatgagttatttatcaaaaataaaatgaaatagagtagactaaaaataataaaatagctaatgaattctaaaacttttaaataacaaaaattaaagaaagaaatagttctagtttataagaatagtggaacttcctcaataactaacaaaaacataaacaaatctatatcttttttattgcatatgttatgaacaattacattcatcaacaattatccatcaataattatacattagaataacaaagcatatgcatcaacaaaaagtaattgtgttgaacaatgtgtcaagtgtaattacatccaccaataattattcataaacaattatacatcggaataactaagtgtgcattaatataaagtgattttgaagataattttttggtatttatagttacaagtttggaattgtaaaagtcatttaaaaattaatgatatacataacgtttatgagaattagattgtttaaagttgagcatatgtaaagtttcttactaaaatctaaatgtgtcatattaagatgtatggtaattcaaaggacatttttgttctttaatgttaattgatattttgaatataatttatcatctttttgttatgaaatacttcatctcttgaactctattttagaataaaagacaaattaaacatttctttaattatttctacctagaaacataatggattaataccatataagtattatttaagtaatattttattaattatttctttaataatatttaaattagtaaaagggtagaatcataatcctattttaaagttaagatcttctcacttataataaaataataataatttacggactagccccgcttgtttacctatattagtcaatacatttttaaaaaaaagtataaatattattaataatattgttttatgtttaaaaattaaaaggagtatatactccttaaaatgagtaaaagaatctatgagattttttatccaaatactttttttttctagatagaataaatgaaataataagttctaaatttaatcaataaaaacataaagttgcagaatataaaaatatttagcaatactgtttttcttcttcaacgctacctcgtctttcgttattaggggtatttatttacaaacatgaaatcacaccatgattttattttcatacaagtagtaaatcatttataaattctaaaaaaacacattaaatataatgcatgctaattttttgtagatttaattatgagaaaaaactaattacatcaattattcaattctcttatccaataacctagagtgttcactacatgataatcaacttgttataacaaacataatctttaaaagaagatttgtacatcagacatgtaaatgaaaaattttcttttcttttttcactgccattattcaagaaaaagtagtcaatttaccttccttcaaccgaaaaattgaatgtaacaaataatgaactaagtaaaaatatgcaacattgaaatgaaaaataatacttaccaaacaacaaataaatgtccatgacgcctttaaccttcttgaagaatgcatcgaatgcactgaaatgattaaattctaattcagatactatattctccaagatttaccgtcaataaattaacaaaacaacatacatattttttctcacacaagtaggtttgttttacctcatgaacgttgagcagactatttgtccaaatgaaaaactctctagaattatttatcacctgtttgcgttgaaaacataaattttcgatgaaaagaataaaacaaaacatgtaatattagttctatctatatacatatatgcctaaaatttattgatcaaaagaaacatgaaaattttgaagaagaatttttgagataaatcaattcacatgctattgtcatgagaagacatcaaaataatgtattttgttggaaaaatcatgtatataattttatcaatggaactcttcaaattctttaacttaaaattaaataaaagatgttttgaaatgtttgaacttcatttgtttgaatgactatttatctttcattatatctttattactttaaagtttattatctaattatttattaaaaatacttttacattttaaaaaatagaaaaaatttaagtgaatggtaaaatggtaatttaactttgaggttaggagcttcccacttataataatatatgatgataattcgccagaataatacagatatatgtataatatacaattatttaaccgatatcatatctgattcctctcttccactctctctcctctctcacccgcctctctcctcccactctcaattttcctttccatatatacaaatacatatgtataatatacaattatctaaacgatatatatatatatatgcaattcatctctctctcactctttgcttcacttgacaactatgacacttaactttggatatgcacaaattgacatttaaaaactggttacagagaaacttaatgctgttgcgtataaagttgatgacttattggatgaacttgaatatgaggcagcaagactctgtttttcagcaaacacatcaagcagcaatatctgagaaattaaacacatatgatgatgtcttcttactcaccgagttattagttatgctaaaatgtttacccgagggattgcagcacctaacaaatctcacaattttttttgataagtgaaagcatagttaaactctcaaatgtagatgataattaagctcttgaagattatcgctgaattaagtgaattcgttattagtttcaaaatgtttagcctccttgggacctgacgaatgatttaaatttcaaacacaaggtcaagctatatttgtaaaattcttatggccaaacaagtcatactgcaacaaattgtaaaaggattattatactccaaaagtaaagatttagaagagatctactcttaacactaactaaaagattattccaattctcaaagcaaatttatattcctttccaaccaaagaggttttccaaatttgctttctagtaattttttttttctgcacgataggaatagatctcatatactccctccgttccatattatgtggtgtagtttaattcaatacggaatataaaaatgaaagaaagacttttaaaatttatagtctaaaatgaataataaaaaattgtatgactataaatcatttcattaagagtaaatgtacaatttaaaataaaattgttacttaatatagtaacgtgtctttttttttggaaactgcctaaaaaaaaaaaaatagtcatataaattgaacacagggagtatctacttacaaagtaaaagttgtgtgtagaagattttggcatataaatcatatcatatatcatcatatcatatattagtaaaagcatgaattaaaaaaagtcaaaaagttaaattacgattttatcccttctattaattaacttgttataaaatatttaaatatttgattgtacaagtttaattaaaatgttaaatgaattttaaacttcctaatattaatttctaattaaatatctaatttattaatatttatcatttataatccatatgtatataataattataattttttaataaaagtctaatcaaaatattaatgacttttagacttcctaacactaattcctaattaaatatctaatttattaatatttttatcatctataatctctctatatataataattttacaaaaattaataaaaagtctctacgtaaatttttatacttttcttattctcataacttttaccctaaataacaaaatttaataattttaagggtgcaaatcttcaaaatggagacacacacattgataatgtcctcttaattattattaaagaatgactctagcttcacaaatttaaattcattaatgcttaattacttagagaaaagtagatgaagactcttaattttgatagtatatggaaggattgtgtactaattttgtacttattttttcatctacatatacatagtcttataaaaatgatgtctacattgtattttttcttaatctgtttctttttgtctttttcccccaattagacttcttaatttagttttctacaaatgttttattgtcgtaagtctctttacttattttgtaattgtagcattttattattcattataatttgcatatatgtatttccatgaaatattagtaattctatcatatctataaaaattcacatgaaatacacgtgctcagaaactagtaaggaaaacaacacaaatatacatccgaactatcgtaaaaatgatatgcagataccatcctcatacttttgggacattgctgtccattacgtcaaaaaaatatagcatatatattaacggacatcacgtgtcataatcatatcaattgatccaacatttaataaatattcgatcgacgaatagattgtgtcacatgtccctatttagtcatatgttaaagtgaatgacatatatgctctagttttgaaactttcttgtaaaatttaagtatatgccctaaatttttaacaatattttgctacattttacgttttttccattcacgtattttcttatttactaaacaagtttctatcgtcctcagagtatttccttaattagcactaaatgttgtgatgtttttcttcaactaagtttcattgaaggattgagattaaacctatttcggtatccacgatctttgaatgaatcgccaaactctatctatgaatttaatagcaaaagctcagattttgttccaaattgagatataatatttctataaagaaatttaaattaatgatgtgatataatgataatgaattcagtttttacattagaaagactctatttttctctcttacttcacaacaatgcaagaattcttaaagacctaaaaatggggtaggggtgggggaagggggccaacaacaacaagattctaaattcttgaatatttttaactaaaaaattaattcttttcccaatggattcaaattgaaaaggaaaactacaactttgtgattatcgcgctttcaaaatgttgaatagattgtcttcaggtgtgagaagaatgagagtgagatggagaaccatacgaataaagaaattctcaagtacgattccaatggaaggaattgaactacctattttgatcggagataacaagtcattcgatagagagattttgaaactgcatatgtttcctaaatgaaagttatatattagctagatagggatatagatgggttgaattctcaaaatctaagaataattttggatatgtctaaagtgattggaaagtgaatatatttaggacaaattacatgattcgatatacttcactattatatatattatttttacatatacttttaaaacactagtttctggacacgtgcattgaacgtgtatctcaaatatatgaaatagatatttttgaaattgtaagacaattctaaaatatggttgtgatgtttagttatgtatgagagcaatttaataaaatatgtatgagacttttttaatttgtttcccatttggtgttccgctagctaattcaaattcatgtgtgacattccactttgaggatacttcctataaagtctttccatcatcaagaattgaattcaaaagattgaatttagaacgaacgaatatttatcaatcaatcaacttatttgatgaaaacatatatgaatttcagtttgcacatattataaaagggcaaacttcatatttcaagggtactacctataaggtctttccattatcaagaattgaattcaaaagattgaatttagaacgaacgaatatttatcaatcaaccaacatattcgatgaaatatatatgaatttcggtctgcacatattttaaaagggcaaacttcaaaatttatcgtatatgccccaaatttttaacaatattttgctagtttttagttttttccattcacgcattttcttatttactaaacaagttcctatcgtcctcagggtattttcttaattcagcactaaatgttgcgatgtttctcttcaacaaagttttcattgaaggactgagattaaacctatttgggtatccatgatctttgaatgaatcgccaaactccatctaagaatttaatagcaaaagctcagattttgttcaaaattgagatataacatttctatatagaaatttaaatcaatgatgtgatataatgataaatatgaattcagtttttacattagaaggattctttttttctctcttatttcacaacaatgctagaattcataaaaacctaaaaatgggaatattatcatattataattaaaagtaaaactctattttagaaatagtggactaaacatctaaactaataattcaatggcctacgttgatgtaagttacgttattttagcaaaattaagaagaaattccttcatttgagggtagaatcataaaaataaaaaatagaaaaatacatatgaaatatcttaccgcaatcatgtgccctctttgtatttttcattactattgtctctccccccaacttgatcaattactttttttaggaaaaataatccacgatgaatgtattcgtcaattttcactgattatgtgaacacaaattattaagttctctcttgaatgaaaacaaaaaaaaaagaaattatttaaagaatcaaaaaaaattaaacgtaaatccccttgcactatttagagaaattttctatgtgaagcatatttcacaattaattgcacatttctctgttctcttcttctcttcttgaataaaaagtcaatacctaaattcccatgataagagtatcaaagaaacatattactggattagggatgaatcatttatgaaattgtgaagtgattttagatactcacagaaaaaaaatcaccaagaatttataaggagtggatgattgtgatttatgatcgaaaaaagatgaaggttaaaattgttgtgactattaatacgaaatatgtcttctttaacaaataaaagtttatttaattttaaatgatacaaataatattgaagtatgtacatgatgaaaatcgtaagaagaaatacaagtatgattgatgaataagttgctataatttattcaccgattctttcttatgtagtacctcgagtttggttgaatttcgaacttgatcaatagttgcaaacaacacttgagatattttaagaagaagaaatataaaaatgtgaagaaacacttcaatttatagctaacaaattgtgttatgaatatgtgttaattgtgtctttttagtaaagctacaacccttcgaaaaaggcattgctcatgagaaagtcacaatactgagaaaaagttacaacttatcaaaaaagacacaatgctttcgaaaactcaaaaccttttgaaaaaatcacaacccttctgaaaagtcacaactcaccgaaaatgtcacaactgtcaatttcaacccttcaaaaagttacaattcatagcaaaaattcacaaaccgtttaatgaaaaaaaactatctatatttaatataatataagtaaataaaataaaaataaattaattgtgtatttttttttaattggggatattatagtaatttaacattcattttgggagttcatgctttttaggtagtgctagtttcgagcacgtgttttgcacgtgtgatccatgtgaattttatagatatgttagaatgactaaaaattaatggcaatatatatgtaaattgtaatgaaaaataaaatgtaacaattacaaatctagtataaagacttacggcaataaaacattcatagaaaactaaattaagaagtctatagagagaaaaaaagacaaaaagaaacagatttaagaaaaatacaatgtagacattattcttataagactgataaatatatagctgaaagaataagtataaaattagtacatataactctctgagttcttcaactcctttcatatcctatcaaaattcaagagtcttcttcatctactttaacaatagaataaaattaatagcctaataatcttggtaggggtttcatgagataaaaagttgaattttatagatagagtagaaggaatatcaaaagatatctttaagtttaagtttagatatttggaagttatgaatatgaaaagattagagttatgaatgttgagagtaaaaaagttgaataagtaattataaaataataataaataagtaaataatatgaaaaagaaaattaaaggtagcaaaccatgtagaaagaacaactaaagttcttatcacgtaattaattttaatttaaatttgttaagctagagtcattctttaataataatcaagaggacattatcaatgtgtgtctccattttgcagatttgcaccttttaaattactaaatttcgttatttatcataaagaataatactttatccacataaattatattattcatgagaggggttaaggaaagttatgagaagaggaaaagtatagcaatttaggtatagactttttaattttattttttttttataattattatatacatatagattatatgataattattaataaattagatatttaattaggaattaatcttagaaagtctaaaagtcattaagattttaattaaataaacaatcaaatatttaaatattttataacatttaatttatagaagagataaaaccgtaattcaactttcaactttttttgttcttgcttttagtaatactagcaattataacaaactcatcagcatcaactcgacctgtatatttcataatcaataatgtcttgtaaatattcatcgatgtgtcgaaacaaagccccccacgtataatacaatcatcttctaattaattgagctcaagcactttgatgaaaaatcgaatggcaggattccacaagtaaatatgcttgtttataccaatcagtataaaactatgactgttaggttgtggagcctgattaatatttgatgtattatttattctctgtaactaaatatactctgaattattaatatataccccaccgccgtggaagtttacccacgggggtgttaccacgaaatattggtttctctctttctagatctctctagatctctcatctctctcaaaagtttttgtgttcttcattcatcaagtgtgtgtggattcgatcctaacaacgacaagaacctaaaatcatacaagttgggggaaaagctcattatcatgacttagaggataggtgagttcttccacaatgagttgttggtttatttattgaaagcaagggttagagttctacgttgcattgacaattgctcctccttctcgacgttgatttgagagatgaataaaatttggacttgaaattcaagaatgtcatgatcgtgaaacacacttgaatcgtaatagagatttcacagataaaattgaaagaattatcataatggtttcattgggtagatacaccatcttgacaagtagtagattttctgggtaattttaattctcgtatttctgatatagacatatgctcacaaattgacgtgaaaccgcatgcgaaatttaggaacttatgcaggtgtttgggcgcagttttgactgtctattgttgttccctaattaaatatacaccttctctgtttcaactttccaacagttttgtgctaaagtatttgttgttgcatttatttattcaaacttaatttgttccaaaatatcatcagagtacaaactaaaggattcaacatgccttgagtacattttatactgtcaatggcaatgctacagcaattaagcaccagtacatgaagcaaccgtttattggttgagatttgagtgtcagtgtcattccttttccattctttgtttttggtagtaactatgatattgccattgtttataacttcaatgatctgctgatattgtggagcatgcaaaactaaaagctatcgagtaaaagtgatcataatgtgctagttcatataagaccatctaaaagctatcaattaaaacttatcgcagtgtgctaggaagttaagggtgtacatatatttgcaattggcagcaaaacagagcaaaagcaaagcattaagatcagaaaaagtagattaaccttaacaaatcgagctcgcctattgtcccctacagcaaagttaaacacctgcagtgtttaaaaaccacaaacaacatttaacaaaagtgaatgattaaaagtaaaaaaagaaaaaatcgagaaagataaaaaagaacagaagacggcataaactacaatatatgttttccatcacaggttattcatatcatcccccataaaactttctacttgagcactaccaagaaactattgaggatgtgggaccttgggatggttagtcaaaatgagcttctattatatccttctgtgtccttctattaaagctctcctcttcttgtttattttgtggagtcccaattttggcgtggccaattccatgatgccaaattggtaacaaatacttgaaagagtgatgactcaagagagatggtgaagaaagtagacatagttcaacgaattgaagtcatattcgagaacaatattatccagatagttcaatgaagtcatttattcaaaattcataagcaaatattaatgtggaaaagttctattcatttccaaattgaacaaaagaagcaaacaatagataaggtctccaacatggagataataattgagagtaaaaacttctattgctattaaatagaatctgcaattaaaaaaaaaattacatagatacaatatggaacttcaatatgtacaacttggaaaccctttcaatgcttgaggtctcagtttttaccacattcagatacaaaaatgtagtaacaatggcaattgtgcgcgattctaaaatggcaaaaaaataatgccaacttaactatggaaattatgtacagatataactaactataaaacttaaatcgtacagtggcatatcaacagagccttcttaggctctgctgctatcatcaaaaaaagcttttgactgattctggcagttcatggagtagtataagcttcggacgatttgaactgattcacacagcatgtaactgatttaaaaattcagttttactctatcagagtcaccaactcctttcttcccagaagaactagcagccgcttgttccttcaaagcttccttctccagtttcttcttttcagcatcagctgcttgttcattctcatcacgtgattttttaaacatcttcatgaacaccaccaaaatttgtgtcactgcatccagaaagtaaggaaatgaaaactgacaaagttcgtcacaaacattgtccggttaaagagttggtgaggaaaaatctgttgaagcaattctcacaccagttaaaacaagatctcaaggacaaacgcaattcgagaaatctagccgatggctatatgcactcaacaaaagctacaaaggccataaatgttgcatcccataatcttcacataaagatagacaactaaaaagcatcactgataaacgctactggaatatctatattaccaagactgtttgaacgactgtagttttttcttttccagatgactgataagtgataatacagcaagaaaataacgtatgtatctctaaccttgctcaaaggggcatcgagctggatcttcgccaaaatacagggatagggagtctgcactccttccctgcagatttacaggatagaaaaacaatcaataaacttggcatggcttatacatccaggaggctttaaaatatgacataatggatgcaagaaactcaccacttcaatataaagagtagtgagagacttgacttcagcctcagcagtatcaaggaaattctttaacacctgagaaggaatgcacgagtcacaaaccgcatatttcagatgtttataacaaaattatatgtacaccaaatcacagacatcgcaatcaagtttgactgcatcaccagactccactctaaaaccatgtccaacacaaaccaaattggg

SEQ ID NO: 4 - DNA, 33516 bp, Solanum habrochaites
  >Genomic fragment 4
caacttggaaaccctttcaatgcttgaggtctcagtttttaccacattcagatacaaaaatgtagtaacaatggcaattgtgcgcgattctaaaatggcaaaaaaataatgccaacttaactatggaaattatgtacagatataactaactataaaacttaaatcgtacagtggcatatcaacagagccttcttaggctctgctgctatcatcaaaaaaagcttttgactgattctggcagttcatggagtagtataagcttcggacgatttgaactgattcacacagcatgtaactgatttaaaaattcagttttactctatcagagtcaccaactcctttcttcccagaagaactagcagccgcttgttccttcaaagcttccttctccagtttcttcttttcagcatcagctgcttgttcattctcatcacgtgattttttaaacatcttcatgaacaccaccaaaatttgtgtcactgcatccagaaagtaaggaaatgaaaactgacaaagttcgtcacaaacattgtccggttaaagagttggtgaggaaaaatctgttgaagcaattctcacaccagttaaaacaagatctcaaggacaaacgcaattcgagaaatctagccgatggctatatgcactcaacaaaagctacaaaggccataaatgttgcatcccataatcttcacataaagatagacaactaaaaagcatcactgataaacgctactggaatatctatattaccaagactgtttgaacgactgtagttttttcttttccagatgactgataagtgataatacagcaagaaaataacgtatgtatctctaaccttgctcaaaggggcatcgagctggatcttcgccaaaatacagggatagggagtctgcactccttccctgcagatttacaggatagaaaaacaatcaataaacttggcatggcttatacatccaggaggctttaaaatatgacataatggatgcaagaaactcaccacttcaatataaagagtagtgagagacttgacttcagcctcagcagtatcaaggaaattctttaacacctgagaaggaatgcacgagtcacaaaccgcatatttcagatgtttataacaaaattatatgtacaccaaatcacagacatcgcaatcaagtttgactgcatcaccagactccactctaaaaccatgtccaacacaaaccaaattgggagttttcccagcgcaagcctttttcacttgaccttgttaagaacacaaatgtcatccatccattggggacacctatcactcttctaaaacagtggtacactgcttccttactttgttttctcaaactatctagaataaagctttttgatagtaaatagggatccttgtaatgtataatgaaggaaacctggggaaagaggaatccgcacaacgccgttcatttcatatctggcgtaagaaaatctcgagaatttgataatacatttaggggtcgtttggtagagcgtattaagaaaaatcatggatgcattagccttgtttattgctagtaccatgtttggtactcttttctaaactatgtacaactagtgttgcattagttatacactatcgtttattaaagtagattatgatatgaccttcaaagttaaaatttaaaactaaaaagaaacattatcttggaagtacaagtaactcatttggtttgtaggaataattcacatgttaccattctcttttctcaccttctgaaatcctgaagatattgtaccatcattgtcggatgcagtaagttcttgttcaactttctcaagacctttactcactgcttgcatttcttcagccaaagacttcagttgaatctaaccatataatatgatgtaaacaaacatttcagttcaccaaaataccagtagtactgcaaaggaagaccataataaatagcaagggtaccttagaagcagcttccaagtgaagaagatccttgtcaaaatcaagcaactctggcattttctcagcaaggagctgacaaaaaaacgaatttacacatttggcatcacattgagaagtgcaaacatatatatgccgaagagtaaagactaaggctggtcaagccagctatagttgatagctaaaggctatcaactaaagttcactgatggttgggcaaaagaacagcataaacgtagaatactgaaagtagaaaataaatacaaaaacatatagttttctacagaactcaaccttctatattacaggaacctcatgggtgcaccaaaaagcaataagggacaagaggctattccttaactgtgcaaattactctacactttcaaaagctctcctaattctcactctccacaaaacccacataagtgcaaaagcatacctttcacgccttgtgtctcctccttcatcttccgccatttcagttgagcaacattacttatacagtgacgggcatcacccaaatttaccaaacgaacaccacatttcccaccataaccgagaagttatcgcacaatctagaagacgattcgcgtcttcacctgacccccttacacataaaacaccgcccaacataagtagttctcctcttcattcttttatcatccatcaagatcacccctcttgttcctaaccaagtgaaaaaacctacctttctcagtaccttagggatccatatcaaaatatatggaaggctatctttcttctcattgatcaaaaatttgtccaaagaaaaggactttagcaaatttattcttaggcggccaaaatgaaacttagattacaatgaaaccttaacaaagacaagaattcaatgaaacctaaacaaagacaaggaccagacaatagagtctagctaaaaagaatctgggcttgctttttcaattcaaatctgtgagcgaggattcctctttctcttctccacaaaaatttgaagtggtttataacttacggagtatccgataatctcttgcaatcttgtataagcctgtgcagatgaaataacttgaacatttccaggagtcaatcgatttgcaccagtcgaccagtgggagcgataattttaagatataaacatcatataaccttccttttagcctattcccacttgagcgtacttcacagctgatacgctcataatacttgacgccccgaaataatgaacagggatagatatggagatacaatttaagaaaatgaaccttaggcacttcaatataagagaagagagaagtagaacaaaataaagaacaatgcaactggaaaaatgttgaaaataaagtgaacgatataagatggattagttttcagattttcatctttaagagctgctgactctcaaaaatctgctacaccgccttgccgccgccttcttgtttgagtgctcaacagaagcacctatacgcacttggactttccttagggtgatttaatagattttttgtgtattttatttccaattgtttcatttggcaagatactctaagcttgaaatttttaatttctatttagatagtcttgtatgcctaatttcatgtttgatcttctatttcattttagagtattggagttgatactggatctagctatcaccgacctactgtcgtactagcgtcaagtgcagcacttagccaataatccccaataataggggctacacttagacaaagtatgaatcaagaagttgtaagtgttagatgcatgtgtggcatttagctatgtttaacctcttttgctggagtaatctctcctttgtaaatgatatggatcaatcaacccaccaatagttctagtaattcctgaactactaagtgtactaccaagcattctaaagcctcatgcatcttccttgattgtgtagaacatgccatacttatgtggtgagccttgcttgtgcactatggctcccacttgtgcatcaccatgcctcgtgcatgctacatcatcagaccatgctcttgtgctaacactatcaccataccagcccagccatgcctccatgaaacagttcctaattttctttgcgttactactaagacaacgaatcgtttgatcttgaaattccttgcctcctctctgttagcctggtccatggctttgttgcacttgcgcatcatgccacacttatgtttgtgaaccgtgcttgtacactatggcttccactagtgcttcttcaccatgcctcatgcatgcttcatcttagtagcatcctcttgtgccaaaacaaccacgcctaccagccatgcctaacatggaactgttccccaatttctttaactttctaattaaaacttaaacaaagaatcatttggtttttgagtgttgaaaccttgaaagcgctcgcctcctctaaagtagcccccttcatggttttagatgggttatgacatagacctcaaatacacttggcactttttcaatccaatcatgagctactcaacaattattactgagccaaaactaatctgattcaacttacgcttaagtcacctccaactcttcccaattcagagctaattgatcaatactaattacataaaggtaaaaacagaaaggcatcataatgcagtaattctaccttgcacagataatgcatcaaggtcattttgttgtttctcgcacgagtgtcagaaagcttaagaagactgtccaacttgaaccctacagcagatcctgtaacgtaattacaaaacaaagatgttagtcacgatgcctccacccaacaactgattattttcttatagagatatagatcttagaaaactgtacctcgtgctgtaccctgattcagtgcattacccaatgttagaatggtctgcattatctgacgtaatttggcagattctttcacctacttgaccaggaaattcagttagagcctagttaaatcagaatgtgccaaatcaaacttcataaggtattaaaaatacctctctagtagcatcattgattgtactcaggttacttctcaagtccttcacctgaacaattcaacatattatagtcaacagaaaattaatggcagaatccatagacattagatcactaagaagtacaagagaaaatacctgattagagaaagtgatagtaaatgaaaacactcgtaacttggactcaactcgtgggaccttcatcagctccaggaaaaactgaaacgggtattacttatccggttaattacttataacttaaaggataggaaaacttgtacttccccacatatatggtcaaaatggagaagacctgctcacactttccaagcatccccttgtccccattatagttctggaaaatagaacataaccagtaagatcaaattgtgaaatcaagaataacaattaaatatcaaattgcaagtatagactgtcaagaaactaacataactaagttcacaaagagagggggaaatcaagcagaaacaagtatggatctacatacacaaaagactaagatatatgcctatgtttatacacatccacacccaccgggaaaggaagttcccaggaaaaggtatctgcatgattagacattgaaacagacacatgagcatgcacgcacagcatagatgcaagtacatactgtataagcatgaaaccgccaaatgggtcattgacttatgggcatcaacctacacagctacttgcaacaaatggcacatcaacaaaactataggctcctgctgttcctacgactcacttaactattcttacgttaagtacaattgcagaatgtgaaggttccgactcttgtttccaaatactatgggcaaaaaacttcaatatggagtattttctctaaacgggaaaagttaaaagaagaatcaaagcaaacttcagaacatacctctaatattacttgtgaactcaaaataaatgactagacacacattataagcatattattgtaacttaaactttgccatgataggcaagcacagtaggatgagaaagagattataccctcagtgtctccatttcttcttttgttgggcaaaattttatcagattttcaacctgatcaatgtccagagctgatgaatccaaagccaaaatagcattctgtatgacatgcatacaaatataatttgtaagaaatccgcggtaaattttcctttgtaaacagaaattttatttgcatttgcataatactggccgcgagttcaaatagcggaccccaacttgtctggaactgaggcgcaactgttgttataatattagtaaaaagaaatccatggcaaatatttcattcatttcaatgtacctccattaaaactcaaaataaggaaaaaagaacttccaaagaaaccatgcatgagcatcctaaagaaatgctcgtcagtcattacacttattgaacacatgcatgaatcagcatattgatactgtgcattatgaaacatgattttgaccaaaggccaaaggatagaatattttatacaatttctatcatgattcctttgaatttcaaaggaaaaatatccataagagttcaattttgaactcttcaagttcggtgaaattacatgatcttttcaacacaataaaattatcaaaaatataaaaaataagaaagtcttttggataaatagttctacagctacttccatagaaagctccttttctccttgtacaaaataaaggtttctttatccatttcattgaactccggctaaaaaatatttctaataacgatagtgtctgatcctacttgtgctcgtatcttgactaatttatagggtacttgacacctcctatcaacataggtatggggaactatgccctccaaaatgcaatcagatgaggaaaaccaccaagtcttagttttggtcgctactagaaaaaccacttggccacactctaaagtgctcattgaactccaccaatatgagaaaagcataactaacttgaaactgaattacaaggagaactgttataggttaatggctaacataaaaatagtcaaactaccaaactcctctgtgtatgacctaaatgttatgtgtagttaaccgatttatacgttcttcattcctttgttgagaaaaaatatagatagttaatcaatatattgtacttctattaagcagaaacgaagatacttcaatttagagttcagtacataatataatctttttgatctagtaaaaagattatagcatgaagagttcaatacatacaagatacaacaatcttttccttttttttgttgttgagaatggacttttagtcaaacccattaagctgattcaataattttgcagatctatttgattcatcagatacatacttctatagttttagcaaatgtacaaagggattaaaaaaaactaaaatactaaattgtaatcttttggaaaataaagtcaaacaacatatgcattcaattgcatatgtaatttgttacttgatttcaattgataaacacatcaggattcgttaattttaatggctgtttagtttgtgttactttttaaattattagcagctcaatttccaaatatctgattgtcctaaagcccaagtaaagatcacataatctaatagtttcatctgataaacaataatagattattatcaaaagacccacctgttggctagaagacataaattagtgcgcaatagataaaagtatcgaagctcatagtagaaacgagaagacacaaaaagaactcacaagcatatcaggcaggggaatcttgatttttgtaagcatgatttcacaattgtatgccctgcgcaaatcaatctggcaaaagcatatgttaagaaatcatcccggtcttttaacagttagaccaaaatgtaacacttccagtctttcactataaataatgggagttgtgtaaaataaacctcaatacctcaggaagaaaaagaagccaacaccaatagactgttcaccaactattccatagtgatctcatattatacagtgaaagctttgaaaactatcagtttctttctatagaagttttctatctctttcccaatttagcactaacagataaattaagaagcaagtgaactgcaattcattcatggtcaatggccatccccatgggacacagtgcccattatgagcacagcctccgcaactctttcattagatctagacatgtatcgcagcctaataaaattactctgttgcatgaatttacatctcaaagtattaacacaacttttaagaatttttcaaaggcaaccattatttttttatatgattgactccatccactaaaccctctgcctaagacgcccaagagaggtttccccctttatcccttcgttaatcaaacccccaaccttatggttggagatgaaggaccttaccctaggatatcactccagtcaaagataattgtcttaactttcatgaaacagaaatggtattacctacaggatggagaaaggaggacttttccacccaaagtttatgtaatcatccacatccaggctgaaaaaacataagttcttctctataagggcatgcttgtttcgaaacgtcacctatgttaaacccatttaagcctttctatttacttcttttcttccaccttgttagccacaagataccacaaaaagtgctctttaaaacctatctaatatttaattgttttgttaaactagtaaagaaaggagatacactcatcctacaacactcactttactacatgaaagacttgctagataatgcctactggagaataacagttgtagagactggaaacaagataaagcatatataacttgccaattgcactttttctggtttgttgatttttgaaccacgtcggcctccacctttgctagtgccatcagtagctgaagccaccgaaaacaaattctcaagctccgtaatatcaatttcaggtgctctgtcatgtacattaataaaatcttatcagaactacccataacagacagataacaaataaaagttgcagtacccaacacaaactaggttaagctcaaagggctcagaactactatatctgtaatctattaagcattcgaagttgaaaccatgagaatgatagtgcttatgacaacctgttaaggggtttcacgagacacgagaaatagcgaacaatttagctctgactattaacttgaaatgacacacaaagttctcattgtaatttttcatccccaaaaataaaatctttatacctggaagtattttccttgttttgcgtatcagcccataaactcccttgcatagcccgtgtaactttcgaccaatgtaagggcttcaatgaagcttttttcggaggaattgaagtacctcctgtacctcgcccttttcctagagcagttgaacctacagaggctcttacacgtccggtagatggaggtggtggcgctggcacactaaggccctttccaccaggcgggggaggtggagtgggtgtcaaaccccgcctagggggtggtggagcattaggagcctttggtgctggtggaggtgctggtggagtggaaccttgcctaggaactcccaaaggaggtggaggaggtgcaggtggccttgtagaattgtttgacggtggaggtggtggcggtggaggtgccaacggagtaggcctatttgatgaagaaggcggaggtggaggcggtggtggtggaggtgccaacggagttggcctatttgacgtagaggatggaggtggaggcggtggtggtggaggtgccaacagagttggcctatttgacgtagaggatggaggtggaggtggaggaggtggaggtggaggtgccaacgaagttggcctttttgacgtagaagatggaggtggaggtggaggcggtggaggtggaggtgccaacagagttggcctatttgaagtagaggacggaggtggaggtggaggtggaggtggagcgggaggtggagggcctttggaaagggctgaaggggtaagcgggggaggtggagaaggcggggaagttacacaaagcaagggtgaacacttcaatgacatgaaaggggaggggaggggtggaggaggagctgataaattacagttagatggaccccgaggaggaggaggtggaggtggaggtggaggcaaggcacttctagaagtagaaaacgtagggacagatggtggatgtggaggagcagaagagcataaaaggctctgattaggaagtggtggaggtggtggaggtggcggaggtcctctagaaaagctatcaggggaagttgaagaagtaggttgtcttggcggtgaatgttctctatggctaccaattgaaggtggtggtggtggtggtggtggaggtggaggtggaggtgatctattagaacttgcaagtggtggaagcggacgagtacgttggacagaagaagggacaccaattataggaggaggtggaggtggtggaggaggcggaggaggtaatgagacctccttgctaggagaaccaaacagagagggtggtgaagggggagatggagctgatgattgagtgacttttatactagaaatcacagaggcaggtgacggaggtggtgaaggtagcggagaagaagaggaagtccttgtatcgcaaatttgaactccctttaaacgttcaggagaaatggcagtatccaattgacagttactttcagaaagagactgaacaggaccaagatctgactttgaaagcttcatttgaccctcagaaatcttgggatcagaagttccatcagaagctgaatcctgttcatctaaaaagttgacatctgttgtattagcataactaatactactagctttctctgagtccagaaaatccaaactgtcggcaatgctcgatgcattattttcttcttcagaatcaaatggggatgaatacccactcatcctactttgcaaaattgacaaatctttcatatcattcagcaccgatagctgtttaaacaaccacaacgcagcatcatcaccagtatcaacccaatcagcaccactaaaaagttcttgtacccttgaaaaggcttcaataggaagtccaccagtctcctcaccattgagagctgcagtgggagcttttagtggagatatgctctcaacatcaccaaataaaacctgcaaagcagaaagtataagttagaggagaaatatgaagagcaaaggtgatccaataaaacaaaactaatcagacagtttgtaaataagtattcacctcagctcgaaagccttttggatagcgtgcctttgaatcccatagaatatccaggttatcgcagtttaacatcaaaatgttagagcgaataaaagcagtgttaaacacaatacggaacatcatgacttccctttcaggatccaggtctaagtggacacactccaaaactacatctccttgcaccaaacactgaatatcaatcttgatgacatcactgtccttctgcaaaacaataacaatcatgttgccacagagcagaattgaagaagacaacaaacaagatgcagtgatagcaatttttcacctggcgataatgtcgaaggcttctacctttcttcggcatggagtacaacatatgagttgacaatccatccttgctgagaaggttccttccaaaaatgcgcacaattggcctacaccctttttgattgtcaaatcttggaatggcacgaagaatgaggcaatccagagaaagagcttgttcaggaggaggccactcgggagatatatttcttcttgatatatattgcaggtaacgaagctgagaagggaatgggttcaaaggtgacaacaattgcgataaacctttaggtgcctcacgataaaccatctcgagagtttttctctctccgctttgtaactttctgaaaaccaagaaactggcgaaaatgaaggctagaaggggccaaccacctctctcacagtgtaacaaaattacattgttatgattttgaagagagagccaactctcacagatacatagaaaatgatgtatcaatgacaatggcagtacaggacagccttcatattgtcttgggtaatccattacagtcacatcatactcgcataaaatctcagcaaactggctccttttctcgccttctctgaaattgaaagcaagaaaggaggaatctggaaattcttcatgtagttcatttatgatttcgtgcaagtaaagctgataaattccctcaggcagtacttcagtcgaaaaacaagaatcaaaaactgcagatattcaacataagataaaaagatgttgagaaaactacaatgcacttccaatgttcaataaaaaacacattataaagtcaaagctagttcctttaccatatactctatcatcaagttccagcaacccatctgggggccttctatagaaaaatctactcaacagcgacataatactgagccaatatatcacctaaatttacctgacatcaaagaaattcaaacccattttcattcctttggtgtcccaatatcaaaagggtcagagaatcagctcgtacaaattcaagaaaatgtgaaattcataagaagaactcaaaattaatctcaaattcagaatacccacaaagctaaaaagggattgaactatatttcaggcgaaaaaattggaacttgacaccaaataaactacaacaagactgaaacacacacaaaactcacatggaaaatatttgcatataaaacaccaaaaaaggaaatctttgaactgaagcaaaccgacagaagccgttgaggaaggattcgagatgtgaggtgaagaaccgacagtgttgccagtaaagttttcacctgcgctttccgattttagtatgaatttttttttttttctgattacggatttgaactctttggagttcaaaattttgggaacgaaaaaaaaggggctgattttttattttaacatatggttgttttcaatttttgaaattacagaaccaacccaatacttgtatggataacttttagttagtgttttattttcgaaaactctacgatgaaggatcgatcggaaataatttttattttctactcataattaggaataagattataatgtgaaatattcaatgatgattaatgaatagtgttatatttaattgattattattgacttgaataataataaaaatataaattacaaatatatataaattaaatacgaatgagtataatataactttcttaaaacaattgagtgcgatggcttaatggtcaagatgaatatattgtactggatgatcatgtctttgaatccccatttatatcagggtcaaatacataaagagatttctaaacttgttgggtttttttcttcacgtactttaactacgtcatttttctattgaatcattgaaccatccaaaaatttattcctttaagaacattgttggtttattttgatcggctattctattgtaaatgcctttaattgggttcgaattgtaatgattttgattgaaggaatgaagacaacccgttttagtctcatttgttttttaacgtcttcaaatgacttaattaaaatacaattattctcgaacatttttactatcaattggactaatgatttctgaaacaacatatatatcctctatcaatccccctcacaaatctggtttcacatcagacaacagtgtttatttaaatggaacaaattataggggtttaatgattcaataggaaaatgacgtagttaaagtacctgaggagaaaaaacacaagtttagagatttgcttatgtatttgaccttaaatcagctatccaacatgcacttttgagctttctatgggtgcgctaatacttgtgtgtcaacttttttaaagatatatatgaataaatatatataacatgattttttttttgaaattaacaggtatacgtgcacctcatttatacatgttaggtctgtctctaaaatcagatctacaaagttacatcgggtatgtttttaatattattgtggttgtttgtaataaatattttaattagagttgttcaaaatcaaatcgaaattgataattcgaattggaaaaaaaagttattgatttatcagtattgggttattgatttagcgatttagttaagggtctgattttttttgttatcgggttatcagtttgaagttttttctcccgatagtaaattaaataattatatttataccattttatgtttgactcgaagtttgctttcctacttttatttttggttattcaatgtatctgcttttgagtaagatgtaacttgtgaactgatgtgcatagtttatttggtttgtcaccttgtttctaagtgatttttaatataaatttttgtgtcaaatcttaaccagttaaactgataaccaaatcgatagcgataaaaaatcgataagccaatatgttaatagttctataacgatttaacatctctacacactatcaaccaataagccaatcaataaactttaaaaccgaatcgaacagaccgatacgcagagctaattctaatgacaataatcgattgtggaatctatattaatgcatggctgcattgaactctaaattgaagtatcttcttttctgcttaaattacctccaaaaggtaccaatgataccaaaatttccaggcttggttgatgggccaaagtgaccatgtgatcgcctttattgggcttttagcccagttaaacttagggcccaatgacgcatattctatcagcaacaagaagtattgttggtgactagagaattttagaatgtaattaaactatttttggccaacaaaaaatataaatgatatacaatatttaatataaaactagaaaaagttaacattattcctcaatgagtatgattcgaaatgcatagacgaggctatatacaaaaatagaggaagattggatcgcctatttgaatctggtttggtgttagaaattcgtagataaatcgagttgaaaaaaacgttgtgacacgtgttttacgtatgagagccaaatgatatggactttgatcaacttttcaagatgtattttttcgtcatattgatattgagaaagattgcaatttatagtattgtcctcattgttttagaaaaccaaaagattttaagtttgaagtatagaattaatccaatcaaatttagttttgaaagtcaattaaagtgactctcaaaaacgcaaatcatgataatattttgaaataaattagggtgttttttttattgttctatctcatttgtttgaaatatagtatttagaaattacgcgaacattctaatcgttattcattgagtaatatacctgattataagacgattaatattgagattgtgagacaaaaggaagaaaatataaatttatagtactaaggacaagggcggacccacaaggtgtcaagtcgggtgctcgaaacacccattaaccgttattgaaatatgtatatctatgttaaaatcgatagctatttgtataaaattaacatagagcacccaatgaataaatcatatagttggcccaatggttctagaatgggtacttaagactcttttaatgttattgtaccaaggttcgaattccgccactgactaaggatcacgatggagtcatggagatcattatttggataatataacaagcaaatgcaacttaaattcaaatttcttttattcaattacaattaattaaattatgattaaatcattttataagtggagatcattatttggataatataacaagcaaatgcaacttaaattcaaatttcttttattcaattacaattaattaaattatgattaaaaaatcattttataagtaaaaatacttctataaaaggaaattttatccttaaaattcaaatattaaacttcaaattaacaacacatgcaaccttatacaaaacaaatcaactaggatacctcccccaataattaaattggtggtcaataaaattgtactccataattatgaattgtagttggcaataataaatatgcattgtattgtcctcatcgactagtcaatggaacatttatgaaaccaaaaaacatgaatcaatgttctctacttgcaccaaagtttttatgaatgagaaataatattagatttgtccgttaaggatttcaaatgttttaaatattgtacttggggtataaatgagcttttttttatcagtaaatttttatcgtatatctgatgattatagatctccattctcagaaacatcacttgaaaatagttgttactccatccgctcacccaattataacatcgatcttaataaaaatacataaaaatcatttagttcaaatggtttccctcactttatatttttatcatttttttctattaccaattaattagttttgttataaaatcgttgatggtcaacaattataactctatcttgattgtcatacgattgttaagatggagtttcagcgaggttaaaaattaactcgttggtataattatgcattatttaaattttatttgagatgattttatagattaatggtaattaatttagtcttgaggagtaaaataaaatcgttataggtttttgagtgttcctaacatcagaatggtgacatcattatgaagttataaagacatataatataatttaaactaggaaaaaagataaatatccttttgaattatcgtaaatagtatgtaaatgctctctgtcaattttttgggacactgatgctcctgtcgttcaaaaactagaaataatatatactctttacactaacggacacacacgtgtcataatcttattcaccaattctacatttattgacggagaagattgcgccatgtgtttctatttagtcttcctttagagttaacggcatataaactttagttttttttttacagcaggaacatcaatgtcccaaaaatatgacaaagaatatttccatatcatttacgatagtttgagatatattttccctttttccatttaaactaatatgcaaaatacgatcctgctcctctttatttctcttctctccattttccccaagtttccatttggattaatgacacatgtcatgggttaaaataaatggttaaaatttaatttttcaaagtaaacctctaaacatgatttagttaatatatatattatatatcaagtatcaaaatttttataatttcacaatcttagcaaacatattattttgtccatattatttatgtaaaaagttttcttcctataatttttttttttcgtaggatcttttttattttttattttatacaatattttaattgtaatcttttgttaaaggtatattggtccgtgattaataaattacctagagataatcaaatcattttgacaaactaattttaatttcataataagattaagaatacggtgataccaagacatacgatagattaattatagttttcatacttctattcagttgcttattcttctaattagataaaaaaaaatttatataaagggaaaaaaaagatcctacgtaaaaagaaataataggaagaaaactttttttacctatatttatggacaaaataatatgttcctaagattgtgagattataataattttgatgcttgatatataatatatttattaactaaatctgtcacgacccaaacgggtcgcgagtggcacccacatttactctcctatgtgagcgaaccaaccaatctaatcccaacatttcaaccataataaacagaaaataaagcgaaagacttaaaactcattaacgaaatcaattaataacttctaaaatttaatattcatcatccccaaaatctggaagtcatcaccacaagaacatctatcctcaaaatactaaatctaagaatgtctagaaaactaaaataataaacagctagtctatgccgaaacttcaaggcatcaagacacacgaaggaagatccgtcaagctgctaaagcgttagctcaccccgagatccgacgtgatgaagaccggctagagttacggttgagttgaagacgatgatacgtttgtgcgactccacaaataacaaagaaaacaattacaagtagggtcaagataaaaaacagtaatcgaaagtagtatcattgccaactcaaaatagaaagcaatatatttcagataatatcataaaatcaactaatattcttaacaggtgatagcaacaagtataaaactcatttataacaaaccaaccacatccatgaggactcaagcctccataccatactctttagggaaacaagttctttggattgactatattaacatatttcaagattcattatctttctatctccggtgtcggaacgtgacaccgatcctcatcatactatctggtgctctaacgtgacacccgatccatattctatcctgcgtgggaacgtggcaccgatcctcattctatctcggtgccgaatgtggcaccgatcctcattctatcccagtgccgaacgtgggcactccgatcctcattctatcacggtgcgggaacgtgacacccgatcctctattactatcccggtgctcaacgtgacacccgatcctctaatctcattactttagttcatcaagccttcttttataccaagacatcatcattaacaaagtaaaatttaggatttaagattcaacagcctcatcatgctagtttcatcacaattatatatataaactcatcatgctagtttcatcacagttatatatataaactcatcatgcatacacacaattaagcatatagaagagtttacaatactacccaaaacatatcattcgctattaagagtttactatgaaatagcataaaccataacctacctccaccgaagaatcgcgatcgacaagctatcttcccaaagctgcgttcttcctctctctctttgttctttctatttttcttattcaaacccccttttcttttaccctaattagcatataattaagtataaaagatgataaaataccccactacttgtttccaaggttatctcttttaacccccaagtaattgaattattaacattaaaccactaactttataattataagcaggaatagtccaaaacgtcccttaaaatatttaacagaaatccgacccattcggtcacgcgttttagacggcccgtcgtgctgcgacggtcaaatctctttgcttccgtacaaagttcgggagactcaattcattaaaaagtccagcggcggcccgttatgctcggagacggtcgccccgccacccgtcgtgacgttcgatcgatctcggtacccaaatttttaaattctaagtgttttagaacgagacccctcgacggtccggtcgtgcccatgacggtccatcgtgggatccgtcgactcaccagctttttccggaaataaaaatcacgctaaaaacgactaaacaggtcgttacaaaatcatggttaaaggtttactttgaaaaattaaatcttaactatttattttaacctataacatgtgtcattaatccaaatagaaacttgaaaaaaatgaagagaaagagaaatggagaggagccgaatcccgcaaagtagaaatatatttgacccctgctattaactattaaaacgttcttgtttcattttgaacttgcaaatatctgtggtacactacaaatttaagggttataatatctattaataaacctaattagtaagggctaatgagactttaaacacaataggcaaatgacaggtaagccctcagattttgattctcctatatcacacatgacgttgtcagaggtcaaaactgtcattatatgtccaaaatacgtgagtatgattttttagcagcaagaaaccaaaaaaaaaaaaagagatacagattttggcaatttatacctttttgaattgaaatgattacacacctttttcacattgtcagtttattttctttttggggtctaaaagttttggtttttgaaaaaaaaaatatccgttgatttaattttggagtaatttaagggggatgtttggttatgaaaatataaaaatattcattttatttaaaaaaaattaaagttgaagtttgaattgtgttgggttatattttttgtaaataatatgtataattggttatgtttttgggtgactaaaagtatttactttagaaaagaagatatttatgtcaagaaaataagtgttgcttaagagtagaaaaatattattttgacaaaaaaaatgcacttaaaaacactttgaagaaatgcaattaaacactaattgtcgtgtaagaggtctttaaaaattaattggtcaatgcattatgatcacaaaagtatttttaaaaaattaaacctttactaaaataaattaattttagaaattcgacctaacaagtcataaaaataaaataaacttttacttatttaatgtttgaaggccattaacaattgaattaatattgctttttcaataaagatttgattttaaccaacctcaattaataccaattaaagtttaattttgtaaattggattgaagttgcacaaatgagtatatttagttatgtactaacatcttccatattaattctcctaaatctttaggtacatatttttcttttccatatttttaacgattttactttctaagttttaaactttaacttttttaaattaattagttcaatcttcttcttcttcttttttttttggagggacataatttgatcgatctattaatcataaaacatgtctttttttttgtccaatattatatgaattttatgaaataaatttattttagaactttttaacgtattttgactttaagctttattcaatccgccttcactgacaaaaattccaaataaaaataaagtgctaaagtataatttatatactctctctgttttataaagaatggtctaatttgacttgatacgatatttctcctattttataaagaatgatctaatttgatttgatacgaaattaaatatacaacccttacatgccacgtggaaagttattgtcagaaaaaaaaaattattctttttgatatggactataaaaaaaaggtcattcctttttaaaacgagcagaataatatatatcccaaaactttattattgagaaagcatctaaaatttgatatggcaattgcatgaatgtggagtaaaattattctaatacaccagatatgatgccatgcagaaatgatgtggaaactatatatagcacaattcccaatgaaatttaatgtactgtctcataactatatagtataggctttcctctaactatacataaagttacccctaaaatataggctagctacccttctagctttcccccaaattctaaattagaacaaaaaaatatttctacatctttttacagtttttagtccctttcactctttggggttatttggaggtaaattatttatagtaatttagaattttatatgtataaattataaaaacttatatttgtggcatctttggaggtaaattattaatagtaatttagaattttatgcgtatgagttataaaaacttatatcattcatataaggtagaagatataataattaaattttatataataattatctgtattactaatatttgtataactttaatcaatcattctttaatgagcaattttcacatataacaaataaaaaaaatcatatttgtatgttataacaaagtttgcttaattaaggctccataaagaacatagaaacatataattcgctatacatatacggttgaagcaaattgtataaaacgaagtgtataaaacaagaaagagaaagacatcaagagaatcgtataaaaataaattgtattattataagtgtatagaacgattatatacaatttgaatttgtataaaatgagaaatagagaaagacaaaagagacttgacagggaatatacaattgaatcgaattgtataaaacgagaaaagagaaattagatacaatttgaaaattgtataaaacgagaaagagagaaagacaaaagaaactggtcagatgagtatttttattgtataattataagtgtataggacgaaaatatatgtacttgtatgtgtatatacaattttctcacgctttatacaaacataaacacaatttatacatttagcttctgtttgtataagtgagaaaggcgagggtggtgagcgagatttgggagagtggcgagcgagatctggaagaggagagagaggggaacaaaaatatatgtattatacaattttctctgctttaaacaattagaaataatttttatatacttgtgtttgtataaaaaataaggaagcgagtgagagattagaggaaagtggcgagcgagataattgggagagaggcgcctggcaatttttcgcaaatatttgcgatggagcacaattatatcaaactctaactacatttattttagattattagtttgctattatatataattttcttttttttaattgtttagtacttgaaagttgagtaagtgttctaacccaaaatgagttatatttatacactgatactcctatttaaagtttagtaatagtacttatgtagaccattgtataagtttttaactggccaacaatctatttcatacaatatatttggacttacaaacactatagaacttatctttaagtattaaagataattttttatcacataagcaggagcctctatttgatctatttcgctttaatataacgtgcaatatcctatttgattttcttatttactttaattatagactcgagatttgtaaaacttcttattttgaggataactagtgtatcaatatcactttcctatttaccttatgtgacgcgacacataacttccatttaatgtactttcttttagtcccgctcatccaaaaatatttaaactctttggtcggtctccaaatctcttatatatcattaattcaatagcatgactcatcaataaaatattatatcatctacacataacatacattgtgatacttccactcgaatatgtcatgttaattcatcgatcatcaaagcaaataaaaacaaattgagaactaattcctagtgcatcccatctcgattggtatcaaggtctttttctttaacagtccttacttagatcttgactccattatacatgcctttaattactctaatatatatcgtaattatatttctagactccaaacatcttcgtaaaacctctctcataatcaccatataaataaaagataactcaaacttgacctattaagagttgattggttgaaattccatgttaaagatctgaaaaaggccttatataaaaatggtcctttgtacagtctgttgattctgattccaaattgtttatgcctaaaacaaacatgatctaaatatttaattaaaaggtctctaattcaatcaagatccattttgtagtcaaaatatatactattttggtggaattttggacataagaattaatgaaaaatagtccattatatttttttcatagttaaacaacacactttatactacatgcctattttttgctagtaatttcgcctaagaattaaaattaaaagtgctaattaattaagacattaagctgtaaaaatatttaaatatgcaaaggctaatcattaatgcaaaaacaataggctccccaaccgcactttcatatataaatagcaagaaggaaataataagtaaaatggataaaaatatgataacgtctagatacacaaagactatcttatttgaaaaaattgtttatataatagcaacctattagtttaaattaaatgttataaccatagtttgatttaactgtaactcttattaaattcttgttgttcacatcccgttcaccactctcactcgtctctccactttatagaaacacaaatgtatacattgcgtttgtgtttgtataaagcaaaaaaaattgtatatacaaaaataatgcatatattttcgttcgatacacttatgattatgaaaatacaatttttccttgcccaatttcttttgtctttctatctttttcgttttataaacacaaattatacaattgattcttttgtatatgtataccgaaacatattatataattttttttttgtatataagtataacgaaatatccatagcaaacataaagtttgctataaagcgtaattaatgtaaactatagttataacttacaaatataatttttgtatttcttatatgtgaaagttgctcttttttttcaagtgtgtgaataaattaatacttaaagtatgtaatcacttttaattgggaaaatgcataagtatcccaacaacctatgtccgaaatcacagagacacacttatactatactaaggtcctattaccctatgaacttgttttataaataactttataccctttttcggccttgatgcgggagaggcatgagtgcaattcaatcttgtggtgtattcgtttgtagtgagtagggcctctttctcgttgatctgacactatcaaccacataacttaaaaaaattgtcagcacactttgggcccacaagagagtgtcacgtaggccgtaaagggatagaaagttatttataaaataagtttacatgggtaatatgaccttagtatattatgagtgtatctctaaaatttcggacatatgttgaaggggtacttaagcatttctcccttttaattatatgcattaacctctattagttataaaaaaaaaacttattttgagattgaagcatataatgaaatgcaataacacatattattcacatttttaaaacgttcaacataattatatatcgtggatcttgctttcgaaataactggaatcggcatgctagtccgaaattctcgtggaagcttcattagaggccacactcgtcggttaggatgacaacaagatccacttatggccgaggaactgggtgttcaagaagcactaagctggttgaaggacactttacggcaaacaacccagatagttatagagatggacaatctttttggttaaacaagagataaaaaaggtgcaaaaactactcttacttttatgttattattcatgattgtaaagcattcgtgtgtgactttacttctatttctttgtctttcgataaaagatgagcaaaccagtgtacccatcagttagctcaaattttgggttttatgactaatgctataaagcggataatagatctccatctttaattcaagatgtactcaattttaatttgatcaataattaattaaaatgtttgattaaaaaaaaaaagaatgttcatcatactaaacctactttgtaatgacatatataactaactattttgatgaataatcaaactactcaactttctttaaaggttttgaagaacaaaaatgtcatattggctatttacacttcatttagctaataagaaattgattttcctttcttataattttttttgtgtttttctttctcacctccattttttctgacttagagctcgttttgattgatttaaaagaatagtttttaaatcaaacttaaataattttaaattaaaaaataaaaagtagaaggagatctacttttaattttaaacttattttaagtcatttataatcttgtcaatcatataaagtcaaaattctgactcaaaaataagtttgattaactcttgagtcaattcaaacaccctcttagttttaattgacatctataacctctaattttaggtatgtacaaataaatacttaaatttatataaaaattaaacaaattaatatttgtgatatgtgacattgcataagacaattttatatcaacgtgatgtcctacctatattacgccacataaattacatatatattgatctttcaattttatatcgtttaaattatacatatataccctatcaaaaaagtattatgcttgttgaatagttctaacttgtaacatccactttcctctttccacttcaatcccaaaaacatttcttacaaatttgcaaaaaacaatgaaaaggacttaattagcaaaagagaccacaaaatgaaagggtcacatggggtgtgttaaaactcaagcctaaaaagactttgttttgtttttgaatagatatatcactcaaaaacccaaaaagcaaaccagtaaaaggtgaccccaaaaagcttccccacacacacactgaagacaactttccagtaatggcggcacatgaagaacaacaccaccatcatcaacaacaagaacaagagaaccccatttcctctttatccttaaaacccaacaataaacacttggagaagattttctcctcatatttgggtctaagtttcgctgtctttcttgggtctttaccaagaaatgcagtttctttggttgggagacttcagaaccgtaacaaggagctaacttttcagcttattgatacagaggagcagttaaagcagctacttttcaggagaaaagaggattcaaaggcaaatgcaagagttgtggaaatctttgcaagtcatagacatgcctggcagcaagaagagaagaggttgttacagcagatcgatgagtgtgatgaagaaattgctgagttaagagggagagctgagcagtttgagacaatggaaagtgagttgagggctaatattgaggacttgaaaagggagattagtgaaagagatgaaatgttgaactttatgagtagaaggggttgtgagatggagaatagtactagtggagatggtgggagtgatggtgttggagattgttatgctgaaatgggtttgaggtttgggaaagttgggatatctgaagggatggatttgggggtagggatggaagagtgttacttggctaatgggattcctaatgctgaacaaatgagtggtgtttatggacagagtaatgggtttaactcagaatacttgaattctgcttctaagttttgggctgaaaaagctagtccttggcaggtatgatccattcattatttctttttgggaacttttttgttctttatagttgttgttatttggggttttatagtgagtggtgtcataatgtggtaaaaataaacgcaaaagtcctttccaggatcttcatatgtaggaagaacttggactaaagtttgtcgctttaatgtttgtcttatatatggtttttcatggtgaaacttatgaataaagttgcttcttttatttaaccatgggattgtactttaagtactaccacctgatattctttcttttagtgtttatctgtttgttcatcttgaggctgtggaatttgtttttgtatgtgatatctgatgaaacaaatgatccagagcaattgaggatgaacgaaattaagtaataaaatgtttggcttatagggttcttggtgaagtacaggcctttatgatctttcttcacatacctgaaaatttcacaggaatatccacttctaattgtttctgataaagctgaaatgaaggtgtttctccaggagtagttcagcgccaaattcaaattgaattgtataatgattacattctgagatgcttattaatgaaatatgtagtttagtgtgtactcagtgacctcctacttgtcttgtgatttgtctttattgttgagactcttgtctctattatctaaaattttgaatggtttgatcttcttagtggctgctgaaagttcaaactacccaggatatggttttctgtttactgaaagataatactcacctcaactgttcatttttaccctatactggtgttatggaccactgcttgaaaaccaggtcaccgttttgtacttttcttctttcaccgttttcgtcctattagaggtttgcaattcttgcttcaagaatggtcccctttggctgaatactttgcatgaaggttggtttcctggttatgaaggaagctcaaaaaaatgtattcgggtaactctagaaatccgaaatccgtttaaaacggaccgttttgttggcatagaccactgtgcctctaaaataccaactaatgacatccaattatatatcccctttggtttgggaagttcaattctggttaaaatggatccgtatatcagcaaaggatgggctgttatcagtcaacatctagtccatctgttatatttctgtttaagattcatcaacctcaatggaaagatgtcctctccctttcttgttgcaagctgtatcttgtccttgtctgtctctgtatcttattttccaattacaatgttatctttggtaattcgttacacatccttgaaataaagcaaatgcctccatgaaacttgaactccccgcggcctctaatccaggcactaatctttcccgttcaaaaggatcactggaacattttcctatacttggtggatgtgtcaaagtttggactaggtagagatcacacattcaatttatggctgtgttttttgtcttttatcatttttgtctttttatattatatagaaaagaagatctggattttcttacccttggtacagtcacccttttcatttatttggaaccagagggaactggagcatttcactatgttgtcttcaactttaatagaaaggctaaagaaaacacacaaccttaaaaataaacctaaattgcctaactattagttgatctatgccttgtgagctggttaaggattagtcatatttacaatggttagagcaaaaagagaaataaacatctagatcacaatgcttatattctagtttcaagcttgaatggtaggagaaatgaggttcttttgactcttattcagcttcttccttctatgtgagatgtcctacctatcttagtaaaaccagcttggtatttaggatgctattgggtcttaagaaaatgtgttttcttcatgcaggatatgcagtatgattctggcgattcacttcaccatttaaagcattttgtagcaaggtaaacattctgtgattagttagacagatgcttagatgtttgcattttgatgttgaatcaactaactagggtgagcccttttgctttctcagacgggaggccccttggaagatagatggtgaatcaacaggagtctcctccaaactaaagttacttgagcaggagctactgaatttggaaaaaattgggaagactgatttatctaaggtaccatcatcaacgcggaagcaagtgaagagataccaagctctagctggcaagattgatgatttatgcagaagaatggtaattactgcatctctgcaagcttattggttataactttagtatatggatttcaaagcttgttacatgcatgcttaggtttctctaagaatggacaatagtcttgattacatctgctaactcaaatatttagatgttgggttatactcttagcttgcacgactaggccttacaattagctttttacctaacacaaacatacatctgataatgatctccctccctcttagcagcaggccagtgatccttgcgaatcaaacctgagtcctgagttccggacccaaagacagaccgagtttttgcttgaagcatttcgacttcagcagcgtgcatctgaaactgcacagaagctgatggtactacaaactgacagtggaaaaagttattacggggacgaatttgaagggcaagcccaactagccactaaacgatcctttgactccatccggaacaacttaaaagaaatccaacggaatttagagatatggcttgccagaattattggggatctggagggaatcctttctcgagatggtgcttctcgtgtaagggattattacatatctagatatccttttgttcaatagttatgtcttaacatgctcagtaaaatcatgattgaaaaaatgatgtataggtccttcctgttatgttaacaagatagctccagctgaatgaacaatatgaggttgataagtccatttatgcacataaatctgcttcacagaagcaaactattaatgctaactagtactttaaagagtgaagatttttgacagaattattgctggatgtcactgttcctgatctggatgcttgtcatttactagttttacttggtcccggtctttctggattaaaaagttgaaaggatggtgtggccctttgcaactggataaatgtcatgtctacacaaatctggcaaacattaaatatttgtggaccaagtttacagccccatttgatttgaaatcagattgattttaagttgatatttgttttgatttggattcttaagctgtattgattattcttaagcttagcaaatgagcaaatcatattttcatgaataagatatcaaaatattctaggaagttgaattaacaagttatatagcttcatgttactttttttataaataaatatttgtaattatatgttattataaactttcaaatatgttcaataaaccaaacaacagtaatactttcttttgataaaagttattcgcttggtacaaacaatttcttccgctagattttcttttttaaattttaaaattatgggtcttttcttgtaaaaattaggtttctttttctcacctaacctagtcgtggacatgagttcataagttgaataatctctaactaaaaggatagtcaaggatgtgccaccgtcgaacaagaaggatagttaaggacactctcaagcaaaggccagtagcatgtactctaaatttagtcaaagttccaatacaagctttttgagcgccactgtgactttgataggtggaaaaataattaaaatttatctttaatatataatactcccttcattttaccacaatacctattaattgatgtaatggcctgaggttataacttttaaccatctctgttctatttatgtcaagaagtgcaatcaggttttgaaccaagtagctaatcactcaatataaagaaaccaaattcaaacttttttaggggtttattatagaaggttcagacatacttatagcagtaattttttttcctagccaggaaaaggcatacacctgctgttacactaaaatcaaacaagccacataatccaattccaataacaatttaacaacatagatagatgagccttatgctgaagcagcaccttcttccagcaactgtttcaccttggtgatgtagtcgttcatggcttcatcggtggattttcctgtcatagatgcatgcagtgcaattagttgtgtttctcatacaaccaagagaaaggaagtcaatctgaacactgttgttagatcacataccttcaacagccttccatgcatcccactttgctctgtctctcatgttgaaaatgccaggacggcctgcccataagaaagggcgtaagaacaaagtgtagctagtttgagacagcatgtacatatgcataagacatttcaagcattatactcacttgtgttgacactgccaacggtggcttgcttgtaaagtccgtaaagaataagcttgttctcattggtggtactctcaggcaatgtcttagctttctcagcatgtgcttcaaattcctcctgaaacccaaatagttcagtaaaaaggtgtggtagctgaagttacaaagataaatttccaggtatactttcttagtgataaaataaggatgagaatccaacttaatagttgagatcgaaactatttgtgaattaagagggaactgaacttatggaaatctaaaatacaaattgagtgttccttcattgggtaaatgaaaagtttgcagttcaggatatcaaatatgtacgaattcattgatggactttagcacaagtgtacgcttagcctagcggtgaaaagggttcattctatttagccaacccgagttcaattctcgctttattttattttataacttgaatccgcttcgtgaaaatcctaggtccgccactggttagtgaaagagtatttgcaagaatgttagacaagaaaagcacaacaatacattcctcaacattgtaagagattctgctggccaacattttgctttgacaatgttaagacgcaaattttagacacatgtgttaatcatacaattctccaaccttttcctcttctagaaatgcttctatttacagatcacagtgaagcaccaaaaacatcctcagataatgtattatgacctcttcagtttgtttactggtttgccctgtttgttaccctacgattcaaccattaccactcagtagcctacatacttgtggtaacaggaatccttttagtgcgaggcgattggccaaccaacaatttttgtagtcacttaaaaataggtcagactaaattacatccactataggttatgaacagcagagaaatttcaaagacaggctgaacacaaagtgcacatttccttcaacttttccccttccccaataaaagaaatatggaagggtgatgataggtttttgaccaggaaacaaaaactagtcttggactaggcaatacaggataggaaagagaaagaagcgggcgctatctcatattcaatttttgctagactatttacacagaagttggccaatgtagcaccatataaatttgagaaagagccatttgttcactactaacattttgatggccctaactgcacatgaactaatagtaatctgattctaacatctcgttccctgggtttagtcatcgacttaagcttcaaagtatacaccatatatatagccaataatatcaacaatctcaaaaactaaaagaagaagacattcataagatgaaatcttcaaaacattgttgaaattatggactacttctgggccagagacaatatatatgccttttgataaggccaaaaatgacatacacaaatccggaccaaagtactactcatctgccattacattcgcactacttcttatcgaattcagtgcttacattgctataattaccataaatctttcaacaaggccaaaaatgtacagcataattgaattcattataagatctatttataagatggtatgccgccactcaaccacagtatgaactgctaaaaaaaaaataatcttaaacatcaattacaccaacagatcagatcaatccaatcaccgagccttcacactaaataataaccaaacaatcctcacgtaacacagcatccacaaaattacagcacaagctgcacaatcgacaaagaaaactaacagatccgcaaataccaattgcacaaacaacacaaaacccagaattgaaaacgaacattaatcacagaaaaatacttttcactgtcaaaaaagattaacactcgcttcaaacaagataaatacatactgaaaggcaaaaaaaaaacagaaatctaaaggggttttaaagaatttaccttcaacgccattgttgtggaaatctgatctggttagcttgataaaaacgagagaaaactggagatgtgattgtgatggagattgaagaagaagggtgggtatatatatatagtggagtatttagcataggaattaacgtaaaattcgattcgattatgataatctaaacaagttgcacttggatcacttactagtcatagtggacccaaaaattgagtatagattatggacctatactatgtgagctccacaac

SEQ ID NO: 5 - DNA, 4900 bp, Solanum habrochaites
  >Genomic fragment 5
cctacgtccacaaaggagatgagcaatccactataaatatgagagtacaaaatatagagagaaacaacctcaaccaattcactcggaatacatgggaggttcacacaagtgataacgtatcaagcttgtgacccacaaattctccctctaaccaaaactctcaaaactctttaagactacattgtgaatgctgattaagttagaaggaacatgtctctatttatagagtcctaaactttttcatactagaaaaaagattagtcaattcaaaaccttttcctaaaaggaaaacctatttatggtaagaaatcagggcaaataaaacccaacacatcatggtttgaaccgtactacataagaaaagttctagtatttaaattgagaaggatagaggggaggggcctatccttaaatctgttaaagttttacgtactagcccaactatttgtgcgcgtgaagaaaagatgtgacagctccactatagatttcagcactaccatttagtttgttacaacattttgctgaaattgagttaggatcttcttgagtcgcagagtaatatcttccatgcgaattctctcttcaggcaaatcatttgtacattcaagagctaattccatgattgatttgaagcatctatctttagaagtaaaattttcttcgttcagtgaaaatagattaatgtccactacatccaccaatcggtctggtaatgattggcatatccatcttttcaaggtgaagtctccaacgaatagatcatccacagggctctttcttgtaaaagtctccattaacaatataccaaagctataaacatctcccgaagttgatactttgccttcagacccatactctacaaaaaaaataaatcacgccatcattaatgaaaataattaacaacatttaaaatcctcaagtgaacttgataataacatttacctggtgccatgtagccgatagtacccaaagtcttggtatgtgctattagcgtctcagatgtaagaagtttggatatcccaaaatcactcacttttgccaccatatcttcatccaaaagtatgttacttggtttcaaatcacaatggacgactacaaacaaatgtcctccatgtaaatactccacagcagaagccacatcaatcatcacctttagtctttgagttatatccaaaactttgtcagtagagtgaagccaacattcgaggttttcattaggcatgtactctagcaccaacactttataatcgaaatttgcacaactacttatcaccttaacaaggtttctgtgtcgaatgctacctaaaacttgacattccacctcgaaacttctaaatgcaagttgcagttctgtattgaatacctttatcgccacaaccattccatctgctagtgtccctttatacaccaaaccaaggctcccccttccaatcaagtttgcttcatcaaagttgtttgtcccttgagaaatatcatagtacgaaatcctcttatgtacctgaccaaatgtatcaactagaggaagttccgtactcctttttcggcatttcagaaaccaaatgataaaaatggttgtgactacaattcctgaggaaactgatgcaagaacagaagttaggactctgttctttctttttctttcaagacttgtcactctgcattgcatcacatggaagcgtgatgatccacataatgcagggttacccatgaatgattcagctgtaaaatttacgaatggccctccatctggaatttcacccatgagcccattgaacgagacattgaaatgcatgagatgttcaagattcctcaaggacttggggatcatgcctgatagattgttgctagatagatccaaatattccaacgaaaccaaatcttcaaatacttcaggtatggaaccatctaacatattctttgacaatgaaaggctaaccaagctttgtagttggccaatcgtgctaggaatctgaccagagaactgattaccatgtaaatgtaatatccgcaaactccttaaattccccatttctactgcaagagacccattcagcaaattggaggccaaagtgagaattgaaatatctttgttcctccaaaaagttgatggaatatgggaaattagtgcattggaatctaagtagagttctcttaaagatgaaagatttccaaaacaatttggtaattcaccagtaagttgatttttccccaagataatttggtacaagttttccatgttacacaagctagttggtataattccatctaaattgtttttctctaggctaaatcttttcaacttcctcaagttccccaaatctggaggaatagatcctataagtttattgtctcccaagcttaaccactccaggttcctaaagttactgatgttaggtggtatttttcctgtgataccattttgaagggcaatgaaatattcaagggaaaaggaccagtttcctgaacctaaagatgttggaagacttccattaaattggttacctcctatttgaacggttttcatatacttgcaattagataatgaagtcaggaaacttaactcgcctgtagattgatcattcgtcaattggtttatttgcaagttgatgaattgtagctgttgtagctttccaagattcataggtacaggtccactaaacagattgcggccaaaatcaagctggataagcatggtggaattcacaatggaggtaggaatcagcccggtgaactggttatccccaaggtaaaggccttcaaggtttggaagagtatggcctatgtttgagggaagtgttcctgaaagctcatttgctacaaatgaaatcttttttagtccagaaatgttgtacaaacgccttggaacttcacccgataatctgtttggaccaagatacacttctttcaaatttacaagatgttcaaactcctgaggaattccaccatataaactgttgtcacctaggtctatcatctctagatttgacaaatttccaattgatggtggaagaattcccaccaaattgttccgtcgtagacttaatcttcgaattgctgataggttatcgatttcacttggtatatgtcctgtaaaatatatgtcgaattgtgtggttactacactgaaatgtccaatactgtataacagctttatagtcactaagttactataaataacagaaactgttagttgtatgccttttaaatagttcagcaatcctcacaaactgttttgatgtccttttgaagatgggactaaatggatcaacatggataattaggattcatatagcagacacaaactagaattgagccaatgtagtagttactgttgttgtttgaaaatgaagaacaaagagctataccaacattttttgctactaccctttgaaatgcaaatactaatttcttataaatgagttgaagagcaagtttttaaatatcaaagatctctagtgctacaaggtgagaagtccagcaataaagttaggtggattcagttaaaccagaacattataaatacctgttatgttattccatccaagaaatagatgttgaagttttgtcaagttccacatgtctctaggcaagtttcctgtaataggatattacgataagttatatgtacctctcacggcctatgattgtttaactaaaaaattgttgcaatctttgttgtcaatatgaaccaaaagtagcagagaaagaagttggttccgtttttttttacctgtgaagtggttatatgacaaggacaaatatattagctctttgcatttgtctaaattgcttggtagttggccagagagttgatttcttgctatttgtaatccctccagccgcggaagattatggcaaatgtcattcggcaaagtcccagatagtgcattataaatcaaattgatgaccttcaaagaagagacattgaagatagacgaaggaacagatccaaagagatcattttcagaaagatccaacaactcgagccttctcagtaatccaagactttctggaatttgacctgtgagattattcattgacaaggacaagtgcttcagcctcctcaaatagccgagttcatcagggatttcaccgttgatgctgttgttgccaatgtccaagaaactaagaaaggagaggttcccaatatctgtcgcgattgaacctcttagtctgagaccattgaggtctagtgatgtcactctttgatgccttttactgcaagatatgcctatccaattgcaaacgtgagtcccctttgtccagtttttcgacaacattccatttggatctgaagttatatgagctttgaaagctaaaagagcagcctcatcagttgaaatgttcgatgcattagtattcgagaggtacgttaacaaaactagcaatcctataatcatagccacggaaaccgttttgtgcaacttctcttgcagctatttgtgggggaaatttataagtgcctgattttttatttttcaagtgacattaatatatatttctataattaaaggcaataaagaatcatgtattagcactggaatatatagaatctagagttcaatgtcaatgatcaacatatatacgtaatatgttttgagacatttttttttaaattgaatgttgctgaacttgactgcaattcattgctgaagggaaatcattggttgtgggattctgtagtgatagtaaaataatttacttggatttataagccttgtatattcattattcaagaatattaaagactaaaatcatgatataatgtcatcattcgaatgtatatagcctccgctgaatagatgtttgacaaaagaacgtgaagtgttacggtcaaattagtgaatctaacgtgtaatgttggatttacgtgaattcaatagcttttattcctatcttt

SEQ ID NO: 6 - DNA, 2684 bp, Solanum habrochaites
  >Genomic fragment 6
gttgatgctctgttggaaatttattactacaagatagattggttaatttgaccgtaaaacagttgacattcttttgtcaaggatctattctggggaggttatagatatacatttgaataatgacattgtcaagtaaattatttaactgtcaatacagaattccacaaccaatggtttatttccctttagcaatgaattgcagtcaagttcagctagcaatatacgattaaaagttgtttcaaatcattggtattaattagataagtattgactcaattacaagtatacacacagtatatatagaatggcgtttgaaaacgaaaacataggcacaaatagcagctaaagaagttgaacaaatccaaatggttgcgaagactattattatagcatgcctagttttgttagcatgcctctcagttactaatgcatcaaacattacaactgatgaggcttctcttttagctttcaaagctcatataacttcagatcccaatgaaatgttgtcgaaaaactggacaaaaggaactcacatttgcaattggataggcatatcttgcagtaaaaagcatcaaagagtgacatcattagtcctcaaaggtttaaataaatgcaccaaacttgaagttctgtccttgtcttataacaaattcactggtaattaactaacttgtaaacttttcatttactaatttcttcttgaattaatcatcatttttgtgtgtgtctgtcattttataattgataggaaatttaccaagagacatgtggaacatgtcaaaggttcaagaactgtttattggatggaataactttacaggtacgtgattcttgtatgtattaaatcttgaatactcttcacgaagttcctaatttcactagatatagtcaatttgtgcattgtctagtaacaaacaaagattaatatatgttgtggagaacattttcgaaagacactctatgtctgatctttagcatgataaccatgtacttattttcaaaatgaatttgcaggaaatataccaaatgaaatgaacctaccatctatttgcaggaaagttaacaaagcttgagcatctcaactatctgaaagtctcttacaatgagttatcaggtgaaataccagatggagggccttttggtaattttcacagctgaatcattcatcggcaacgaagagttatgtggaccgcctagattccaagtcaaggtgtgtgaaatccagaacaacgtgacaagaagaaacaggaagaaaacagtactaaaatttgttcttggaccagttgcagctggaggtttagtcataggggttttaggcatgatatggttgttgaattatcggagacgtaacaaccaacttattcctttaactgattggtatgatcagttatcacacaaaaggttttcttactatgaacttgttcgagggactaacaactttgacgaatcaaatttgattggaaagggaagccttggtatggtttataaggggacatttacaaatgggaccatagctgctgtaaaggttttcaatgcacaactgcaagatgcattcaagaggtttgatttggagtgtaaggttttgcgtaacactcgaaataggaatcttgttaaggtgataagtagttgtgcaaatcttgattttaaggcattggtgtttgagtacatgcctaatggagatcttgattattggctttactcacacaacaatttcttggatttaaacaagaggctgaaaattatgtttgatgtggcttgtgtcgtagagtatctacaccaaggccattcacttgtagtggtccattgcgacttgaacatacttttggatgaagacatggttgccagagtaagtgattttggtatatccaaactcttgaccgcgtatgatccagtggcattgacaaagactttaggcaccattggctacacggcagcaggtactgatcaaacttttatttactaattactttcttcaacttgtattcgatatgcatatatgatgtatttcattttaatggcagagtagggatagtgtcaactatgggggatgtttacagctacggcattttattgatggaaaccttcacaagaaagaaaccagtagatgatgagtttgttggagaccttacattgaagagatgggtcgcggaatcatatcctcatagagtcattgttatgaaataaaaacgaatacacgctgaacgtcacttatgagtcatttatctaatatgatccattaacaattgattaatgtaacgcaaggaagaagaaaacaatttgcattgttatgaatgaatgtgtttgtactacaatatatacagtactgacaagtccagcaaactttctaaccaacttattctaaccaactctactcattattaatttagctcacttaatcaagaaattaaacttaacaactaactaccattactcattcaactgatcacggaacatcaacacattttgttgatttctttcacacacaccctctgcttcgaaaacccctctttttaacatgtaagcgacaatatcttttttttaggagagtgttcaacattgagcataaaaataataaaatagagaacaaaaaagatgagtataaaataaataataatataagatcgattttaccgattgtcaattttgtgtatggactaaagaaataacagcttcacatatctaat

SEQ ID NO: 7 - DNA, 4297 bp, Solanum habrochaites
  >Genomic fragment 7
ataaataataatataagatcgattttaccgattgtcaattttgtgtatggactaaagaaataacagcttcacatatctaatattaaatgtaatactgaatttcacatatggtcagaggtgaatccacctgcacccgatatattcttttttaaaaaaattatatgtatatatatagattgttgataagacggtaatatatttaattgtgcactcttataacgaacaaatgatttgacttgtccattggaaaaacgaaaagtgtcacataaattgagacatggggagtaacatttctttcttaaatttttcgtgtgaagtcaaactaattcatataaaatgagacggaaggagtactgtttaatattaattgcatatggtagtaaatttgatagacatggtcccgtgggagtgtgtgttatttccattgaataattgagtttgtaattgttacaagtccattctaatttccaacaccttacttcatttcaaaaatatactctatggctgaagctttccttcaaattatgttagagaatctgacttgtttcatccaagggaacttggattgattcttggttttaaggatgagttcaaaaagcttcaaagcacgtttactacaatccaagctgtggtacaagatgctcagttgaagcaattgaaggacaaggcaattgaaaattggttgcagaaactcaatggtgctgcatatgaagctgatgacatcttggacgaatgtaaaactgaggcaccaattatacagaagaagaataaatatgggtgttatcatccaaacgttatcactttccgtcacaagattgggaaacggatgaaaaagattatggagaaactagatgcaattgcagcggaacgaattaagtttcatttggatgaaaggactatagagagacaagttgctatacgccaaacaggtaaatatttttctaaataacagctttatatcatcaaattcatgtgtgttttggggattttgtctaagtagataagtggttcaaaatctattatctaaatctgtttggtgaagtctttaacatatatataaatccatagcttactcatatgccccaaagtctaaatgacaggataaagccagagttgttttagattttataaattaacaaagataataatgtaaattcaaaatagtgcatttgttttatatttgaaatatgtctgctgcttctgatcaagctgatcattgtcttttgcaaaattcttctttgttttttttgctgactcttaccgatcttggaccaggttttgttttaaatgaaccacaagtttatggaagagacaaagataaggatgagatagtgaaaatcctgataaacaatgcccaaacactttcagtcctcccaatacttggtatggggggactaggaaagacgacccttgcccaaatggtcttcaatgatcagagagtaattgagcatttccatcccaaaatatggatttgtgtctcggaagatttaatgaaaagaggttgataaaggaaattgtagaatctattgaagaaaagtcacttggtgacatggacttggctccacttcaaaagaagcttcgggacttgttgaatggaaaaagatacttgcttgtcttggatgatgtttggaatgaagatcaagataagtgggctaagttaagacaagtcttgaaggttggagcaagtggtgcttctgttctaaccactactcgtcttgaaaaggttggatcaattatggcaacattgcaaccatatgaattgtcaaacttttctcaagaagattgttggttgttgttcatgcaacgtgcatttgggcactaagaagaaataaatcttaatcttgtggctatcggaaaggtgattgtgagaaaatgtggtggtgtgcctctagcagctaaaactcttggaggtattttgcgcttcaagagagaagaaagacagtgggaacatgtgagagatagtgagatttggaaattgcctcaagaagaaagttctattctgcctgccctgagacttagttaccatcaccttccacttgatttgagacaatgcttttcatattgtgcagtattcccaaaggataccaaaatggaaaaggaaaatctaatctctctgtggatggcacatggttttcttttatcaaaaggaaacttggagctagaggatgtaggtaatgaagtatggaatgaattatacttgaggtcttttttccaagagattgaagttaaatatgatcgaacttatttcaagatgcatgatctcattcatgatttggcaacatctctattttcagcaagcacatcaagcagcaatatccgagaaataaatgtagaaggttacctacatatgatgtcgattggtttcgcaaaagtggtgtcttcttactctcctcctcacttgcaaaagtttgtctcattgagggttcttaatctaagttccatgggacttaagcagttaccgtcctccattggagatctagtacatttaagatacttgaacctctctctcaataacatgcgtactcttccaaagcagttatgcaagcttcaaaatctgcagactcttaatgtagagtattgctggtcactttgttgtttgccaaaagaaacaagtaaacttggtagtctccgaaatctcttacttgatggttgcgatggattggattctatgccaccaaggataggatctttgacatgccttaagactctaagtttctttgttattggcgagagaaaagattctctacttggtgaattacgaaacctgaatttgtatgggtcagttgaaatcacgcatcttgagagagtgaagaatgatagggatgcaaaagaagccaatttatctgcaaaagaaaatctgcattctttaagcatgagatggaaaaaaccacatagatatgaatcagaagaagttgaagtgcttgaatccctcaaaccacaccctaatttgacttctttactaatcactggcttcagaggattccgtcttccaaagtggatgaatcactcagttttgaaaaatgttgtctctattgcaattagaggttgtgaaaactgctcatgcttaccaccgtttggtgatctgccttgtcttgaaagtctagagttaggagatgggtctgcggaactgaagtatgttgaagattctggattccctacaagaagaaggtttccatctctgagaaaacttattatagtcaattttgataatctgaaaggattgttgaaagaggcaggagaagagcaattccccgtgcttgaagagatgacaattagctggtgtcctgtgcttgttattccgaccctttcttctgtcaagaaattggtagtttatcggaacatgtcagatgcaataggtttgaggtccatatataatcttagggctcttacttccctcaacattagccataacttgacagctacttcgctcccagaagagatgttcaaaagccttgcaaatctcaaatacttggaaatctctttcatcttcaatctcaaagagctgccaaacagcctggctagtctcaatgctttgaagcatctgaaaattgaatattgtgacgcactcgagagtctccccgaggaaggggtgaaaggtttaacttcactcacagaattatccataacaaattgtaagaggctaaaatgtttaccggagggattgcagcacctaacaaatttatcagttagggaatgtccaacactggccaagcggtgtgagaagggaataggacaagactggtacaaaattgctcacattcctcatctgcttattactaatgagatgtaattttctgatttttcttttggaaacaaatcaactatttgtaaccaattcgtattggacttttgagccctgcatttgttcgaatacgcctttcaacctgtatatcagtgtataacaaatgtatacaatatgtatactgctgctcaaatctgcagatttgattttccagcaacacatttgctgattcttccgacctgtaaattaatttccagcagctcatttttttgtgttcaacctgtacgccagttgtgagggtctaagacttgaggaggaggtttgagcctttacggctcagcgaggaagtgcagggatacgggcgaaatccgttaggactcatggcgaatgcacgtgaaacggatcaaaaggaaacataaagaaaaacagtcaacgatgaaaacaattctgcatttatacgcataactaaggcaatgtaaatcaaattgaagaatgggcagccaagataaatgaaagcaaataaagccacaatgcatgttttaaaatactataacc

SEQ ID NO: 8 - DNA, 4357 bp, Solanum habrochaites
  >Genomic fragment 8
aattaaatttattcatatgagattatattttatagaaaaaataataaaaatttagattaaaattatattttttcatttccgttagattaaagggatatctcgagccatttgtttacaagtagggtatatatatgctactttcatgttaggtatatcagctctaaataacaaaattgatgggtatatcagacccttttctcaagtttaaattaatgtgaaaaagttttaagtgtgggtcccatgttgtacatttaaaattctcatacaacagacaaaaggttagcttttcacaaaataaaatttttcccatgtgaaactcaaaataaaataattgcgtacagacatatttatgcaacacaacattaatttatttatttacccattcaataagtaaaggaataattataaagctttgtgctcttacttttagctgttcatatttcattccaacatcgatcttatagatttattgctaattcacaacaattccagcaatctacatggctgaagctttccttcaaattttgttgaaaaatttgacttctttcatacaagaggaacttggattgttttttggttttaagaacgagtttgaaaatcttaaaagcacgtttactacgatccaagctgtgcttgaagatgctcaggagaagcaactgaaggacaagccactagaaaattggttgcagaaactcaatattgctgcatatgaagttgatgacatcttggatgaatgtcaaactgaggcagcaagactcaaagagactaaatatgggagttatcatccaaaggctatcgctttccgttacaagattgggaaaaggatgaaagagataatggagagactagatgcaattgctgcagaacgaagcaagtttcatttggaaaaaaggactacagagagagaagctgctagacgagaaacaggtgctcatctttaattagtttatattcatttttttgcgattatcaagttcatgtgtgtttatggacccaagggacttttttctaatctaatgtttgtctcaagtctaaacagatttgtaattctaccacttatttatttagtgaagttcttaaacatatatacatggtgtaagccagctcagataaatccatagtcagttgtttcggactgaacttaacttggatgtcaatttttcaaagtcaatcatgttttcaactcctccccctgattctcatctctttgtagtgcaaaaatcttctctctgtttttcgctaaacatattctcgtgtgaacatatattgcttgaaacaggttttgttttaactgaaccagaaccttatggaagagacaaagaagaagatgagatagtgaaaatcctgataaacaatgcccaacaactttcggtcctcccaatacttggtatgggggggctaggaaaatcgactcttgcccagatggtcttcaatgatcagagagtaactgaccatttccatcccaaaatatggatttgtgtctcagaagattttgatgagaagaagttgataaaggcaattgttgaatctatcgaaggaaacccacttggtgaccacatggatttggctccacttcaaaagaagcttcaggacatgttgaatggaaagagatactttctcgttttggatgatgtttggaatgaaaatcaagaaaagtgggataagataaaagcagtcttagaggttggagcacgaggtgcttctgttctaaccaccactcgtcttaaaaggttggatcaattatgggaactttgcaaccatatgaattgtcaaatctgtctcaagaagattgttggttgttgttcatgaaacgtgcatttgagaaccaagaaaaaaataaatcctaaccttgtggctatcggaaaggagattgtcaaaaaaagtggtggtgtgcctctagccgccaagactcttggaggtcttttgcgcttcgtggatcaagaaagagaatgggaacatgtgagagataatgagatttggaatctgcctcaagatgaaagttctattctgcctgccctgagacttagttatcatcatcttccagttgatttgacacaaagttttgcatattgtgcagtattcccaaaggacacggtaatggaaaaaggaaatctaatctctctctggatggcacacggttttcttttatcgaaaggaaacttggagctagaggatgtaggtaatcaagtatggaatgaattatatttaaggtcttttttccaagagattgaagttaaagatggtaaaacttatttcaagatgcatgatctcatccatgatttggcaacatctctattttcggcaagagcatcaagcaacaatatccgtgaaataaatgtaaaacggaacccacatatgatgtcgattggttttgcaaaagtggtgtcttcttactctccttctcacttgcaaaagtttgtgtcgttgagggtgcttaatctaagtgaattaagacttaagcatttaccgtcttccattggagatctagtacatttaagatacttgaacctctaccgcaataacatgcgtagtcttccaaagcagttatgcaagcttcaaaatctacagactcttgatctacagtattgcgccttactttcgtgtttgccaaatcaaacaagtcaacttagcagtgtcagaaatcttttacttcatggttgctataaattgaattctatgccaccaaggataggatctttgacatgccttaacactcttggttgctttgctgtgggaaggaagaaaagttgtcaacttggtgaattacgaaacttgaatctctatggctcaattcaaatcacacatcttgagagactgaagaatgatagggatgtaaaagaagccaatttatctgcaaaagaaaatctgcattctttaagcatgacttggaaaggaccacatagatatgaattagaagaagttgaagtgcttgaagccctcaaaccacactccaatgtgacttgcttaacaatccatggcttcagaggaatccgtttcccagagtggatgaatcactcagttttgaaaaatgttgtctctattgatatccggggttgcgaaaactgctcgtgcttaccaccctttggtgagctgccttgtctaaaaagtcttaagttacaggacgggtctgcggaaatggagcatgttgattctggattccctacaagaaggaggtttccatctctgagaaatcttattatagtcaattttgataatctgaaaggattgctgaaagaggcaggagaagagcaattccccgtgcttgaagagatggatatttggtggttccctgtgtttgttattccgaccctttcttctgtcaagaaattgttagttcattggaacatgtcagatgcaataggtttgagttccatatcaaatctcagggctcttacttcactccacattagaactaacttcatagctacttcgctcccagaagagatgttcaaaagccttgcaaatctcaaatacttgaaaatctctttcttctacaatctcaaagagctgccaaacagcctggctagtctcaatgctttgaagcatctggagatgaattgttgtcccaaactggagagtctccccgaggaaggggtgaaaggtttaacttcactcacacagttatccattacatactgtgagatgctaaaatgtttaccagagggattgcagcaactcacaaatttatcaattaagaattgtccaacactggccaagaggtgtgagaagggaataggacaagactggtacaaaattgctcacattcctcatctgcttattactaatgagatgtaattttctgattttcttttggaaacaaatcaactatttgtaaaatctatttgtattatacttgatttttcttggttatgtaacaataaatatttgaaaattttcatataaaaatagttacatttctatatgtataattcgccagaataatacatatatatgtataatatacaattatttaaccgatatacatatataattcacctctctcccactctctgtcctctctcactcgcctctctcctccctctctcaatttcgctttccatatatacaaatacaattatctaaaagatatatatatatatatgcaattcatctctctcccactctttgcttcacttgacaactatgacatttaacattggacaagcacaaattgacacttaaaaactggttacagaaactcaacgctgctgcgtataaagttgatgacttattgaatgaatgagaatacgaggcagcaagactaaagcagtctcgactaggacggtatcatccaaaggctatcaatacaaactcagttgtttagaccacgaaaagactgtgaattcaatacaggagt

SEQ ID NO: 9 - DNA, 2561 bp, Solanum habrochaites
  >Genomic fragment 9
aagtctgatatacttctcaactttttcatttggagctgatatatttctcgttataaaagtgactcatatatgcccttatcgttatacaaacgactcatatatctgagtcatttgtttacaagtaaggtatcactttcttaaaaaagcaatgatatcatctctaaaacgacaaagattgaggggtatatcgatcctttttcaaagtttaaatgaatgagaaaaagttttaagtgtgggtcccatgttgtacatttaaaattctcataaactgacagaaggttagcttttcacaaagtaaaatttttcccatgtgaaactcaaaataaaataattgcgtacagacatgtttatgcaacacaacattaatttatttatttacccattcaataagtgaaggaataattataatgctttgtgctcttacttttagctgttcatatttcattccaacatcgatcttatagatttattgttaattcacaacacttccagcaatctacatggctgatgctttccttcaaattttgttgacttctttcatacaagaggaacttggattgaaaatctaaaaagcacgtttactacgatccaagctgtgcttgaagatgctcaggagaagcaactgaaggacaagccaatagaaaattggttgcacaaactcaatgttgctgcatatgaagttgatgacatcttagatgaatgtcaaactggaatttttaaccaaattaagtcattatataaaataatttaccaaagtaaaatatttttctaaaagtttacaaaactaatataaacgtatttcatggtaacgttttagggtatattttattttttaaaaactaatgactttaggttgatatcgttctttgtaagtaacgttttactcctaaaacgttattttcaataacattttactcttaaaacgttactcatagtaacgttttactcctaaaacgttattttcaataacattttactcctaaaacgttactatgagtaacgttttaggagtaaaacgttactgtgagtaacgtatatcaatctgacgccatcaacttttaaaaaataaaatatatcctaaaacgttactgtggaatacgtttatactagttttgtaaaattttagaaaaacatattattttggtgaatgactttatataatgacttagtttggttaaaacctcgtcaaactgaggcagcaagactcaatcagactaaatatgggagttatcatcctaaggctatcactttccgttacaagattgggaaaaggatgaaagagataatgaagaaactagatgcaattgctgcagaacgaagcaagtttcatttggaaaaaaggactacagagagagaagcttctagacgagaaacaggtgctcatcttaaatatattagtattaattacaacaatttaattagtttatattcatttttttgctattatcaagttcatgtgtgtttatggacccaagggacttttttctaatctaatgtttgtctcaagtctaaacagatttgtaattctaccacttatttatttactgaagttcttaaacatatatacatggtgtaagccagctcagataaatccatagtcagttgtttcggactgaatttaacttggatgtcaatttttcaaagtcaatcatgttttcaactcctccccctgattctcatctctttgtagtgcaaaaatcttctctctgtttttcgctaaacatattctcgtgtgaacatatattgcttgaaacaggttttgttttaactgaaccagaaccttatggaagagacaaagaggaagatgagatagtgaaaatcttgataaacaatgcccaacaactttcggtcctcccaatacttggtatgggagggctaggaaattcgacgcttgcccagatggtcttcaataatcagagagtaactgaccatttcaatcccaaaatatggatttgtgtctcagaagattttgatgagaagaagttgataaaggcaattgttgaatctatcgaaggaaagtcagttggtgaaaacatggatttggctccacttcaaaagaaggcattgtgtcgatttgagataatacgagaaaaatatacatgcgaaaaacaagacaacagatttcgtggttcaccaataaattggctcgtccacgggaagagggcgggttttattatggaggcaaaaaccaattctgagaatagggtttgccatagcgtctatatatagtgtaaactaagcccctaacaggcttgggcccaaaatataaattgaatgataattaagggcccaattcaaggcattcaacaaatctccaccttgacttgaattctccaagcagattcttgggcgcactatgatagtgccaggcctcccccctcttcctcgggttgcccttgagtataattacttgacacgatgttgagcaagtcaaacgagtgttgaaacttgctcacgtggagccaagctttgtgaacatatcagcgggattatcaacagttctactttcttcaccttgattctcttctcacttctcgggaaaatgatacctccgtcaatat

SEQ ID NO: 10 - DNA, 3203 bp, Solanum habrochaites
  > Genomic fragment 10
acgtcatccgcgagacacaaagatgatcgtcagtgcgcctttcctccggaatctccatctcgggagtaacgacggcgttcttgtctttcgacaacggcgcccgtaaaaccttgttgtttcaacaaagcccgcatcttgatcgccataaaccaaactggctattcctccaccgtgaatttgtcgattttcacgttcaaagcgtacatctcaattctcaagaacacccgattaaccgagaggctcgataccaatttgttgtgcggaatttgagataatacgagaaaatataaacgcgaaaaacaagacaacagatttacgtggttcaccaataaattggctacgtccacgggaagagggaacattttattatggaaggcaaaaaccgtaattacgaatagggtttgccataagcgtctatatataactaaactaagcccttaatgcttgggccaaaatatagaattgacagataattaagggcccaattcaaggcattcaatgaagcttcaagatatgttgaatggaaagagatactttctcgttttggatgatgtttggaatgaaaatcaagaaaagtgggataagataaaagcagtcttagaggttggagcacgaggtgcttctgttctaaccaccactcgtcttaaaagggttggatcaattatggacactttgcaaccatatgaattgtcaaatctgtctcaagaagattgttggttgttgtgcatttgagaaccaagaaaaaataaatcctaaccttatggctatcggaaaggagattgtcaaaaaaagtggtggtgtgcctctagccgccaagactcttggaggtcttttgcgcttcgtggatcaagaaagagaatgggaacatgtgagagataatgagatttggaatctgcctcaagatgaaagttctattctgcctgtcctgagacatagttatcatcatcttccagttaatttaacacaaagttttgcatattgtgcagtattcccaaaggacaaggtaatggaaaaaggaaatttaatatctctctggatggcacacggttttcttttatcgaaaggaaacttggagctggaggatgtaggtaatcaagtatggaatgaattatacttgaggtcttttttccaagagattgaagttaaagatggtaaaacttatttcaagatgcatgatctcatccatgatttggcaacatctctattttcggcaagagcatcaagcagcaatatccgagaaataaacgtagaaggttacccacatatgatgtcgattggtttcggaaaagtggtgtcttcttactctccttctcacttgcaaaagtttgtgtcgttgagggtgcttaatctaagtgaattaagacttaagcgtttaccatctttggagatctagtacatttaagatacctggatttgtcttacaatagtaaaatgcgcagtcttccaaagcagttatgcaagcttcaaaatctgcagactcttgatctaaagtattgctggtcactatgttgtttgccaaaagaaacaagtaaacttggtagtctccgaaatcttttacttgatgattgcgatggattgaattctatgccagcaagattaggatctttgacatgccttaagactctaagtagatttgcagtggggaggagaaaaagttgtcaacttggtgaattctgaaacctgaatctgtatgggtcaattgaaatcacgcatcttgagagagtgaagaatgatagggatgcaaaagaagccaatttatctgcaaaagaaaatctgcattctttaagcatgagttggaatatcaacgaaccgcgtagatatgaatcagaagaagttgaagtgcttgaagccctcaaaccacactccaatgtgacttgtttaacaatcaaaggcttcagaggaatccgtctcccagagtggatgaatcactcagttttgaaaaatgttgtctctattacaattggaggttgtgaaaacttctcatgcttaccactgtttggtggtctgccttgtctagaaagtctagagttatggaatgggtctgcggaattggagtatgttgaagattctggattccctacaagaagaaggtttccatctctgagaaaacttattatagtgaattttgataatctgaaaggattgctgaaagaggcaggagaagagcaattccccgtgcttgaagagatgaaaattagctgttgtcctgtttttgttattcagaccctttcttctgtgaagaaattgaatgcttattggcacaagtcagatgcaacaggtttgagttccatatcaaatcttagggctcttacttccctcaacattagccataactccacagctactttgctcccagaagagatgttcaaaagccttgcaactctcaaatacttgaaaatctcttacttcgataatctcaaagatctgccaaacagcctggctagtctcaatgctttgaagcatctggagattaattgttgttatgtactagagagtctccccgaggaaggggtgaaaggtttaacttcactcacacagttatccattgcatactgtgagatgctaaaatgtttatcagagggattgcagcaactcacaaatttatcaattacgaattgtccaacactggccaagcgatgtgagaagggaataggacaagactgatacaaaattgctcacattcctcatctgctgattacatagtgtcatactaaattaaatgattcttatagcaatattattggttcaaccaacaaaactaaatctctaattatattacttaattgcttttagtttgctacaattatcactcatgactaacattatgtatcaattacgtggtttgtcttcaattttgtataattagtcatgtttttatatgtataattcgctagaataatacagatatatgtataatatacaattatttaactgatatacatatataattcacctctcttccactctctgtcctctctcacttgcctctgtcctctgccaatcgacgagatgagcctacgaaagatttcaagttcagactatgatgactgacatcctcacttacgcaacgaaatggagttgatggagtagccagtgcccttgagtcattctcttcggtatcgccttctctcatcgttaatggcgccgcaaggcactcgactagcaagttagaccttagttagggcgaaagatttcttggatgg

SEQ ID NO: 11 - DNA, 4181 bp, Solanum habrochaites
  >Genomic fragment 11
atacattatttaatactccaacaactttgtgattccactctagactaccatcacatatctaatattaattataatagtgaatttcacatatggccagaggcgaacccacctgcacccaatatatttttaaaaaaaattcatatgtagattgttgataagacgctataatatatttaattgtgcactcttataatgaacaaatgatttgacttgttcattgaaaaaacaaaaagtgtcacataaattgagacatgaaaaataatatttcttttttaaatttttcgtgtgaagtcaaactaattcatatataaagcgaaagcggaaggagtactgtttaatattaattgcatatggtagtaaatttgatagacatggtcccgtggggtgtgtgttatttccattgaataattgagtttgtaattgttacaagtccattctaatttccaacaccttacttcatttcaaaaatatagattcattgcttactcaccacatactcgatggctgaagctttccttcaaattctgttagaaaatttaacatctttcatacaaggggaacttggattgttttttggttttaaggacgaatttgaaaatctgaaaagctcgtttactacgatccaagctgtgcttgaagatgctcaggagaagcaactgaaggacaagccactagaaaattggttgcagaaactcaatgttgctgcatatgaagttgatgacatcttggatgaatatcaaactgaggcagcaagactcaatcagactaaatatgggagttatcatccaaaggctatcgctttccgctacaagattgggaaaaggatgaaagagataatgaagaaactagatgcaattgctgcagaacgaagcaagtttcatttggaaaaaaggactacagagagagaagctgctagacgacaaacaggtgctcatcttaaatatattagtcttagttacaacaatttaattagtttatattcattttttggcgattatcaagttcatctgtgtttatggactgaacttaacttggatgtcaatttttcaaagtcaatcatgttttcaactcccccctgattcttatctctttgtagtgcaaaaatcttctctctgtttttcgctaaacatattctcgtgtgaacatatgttgcttgaaacaggttttgttttaactgaaccagaactttatggaagagacaaagaggaagatgagatagtgaaaatcctgataaacaatgcccaacaactttcggtcctcccaatacttggtatgggggggctaggaaaatcgacgcttgcccagatggtcttcaatgatcagagagtaactgaccatttccatcccaaaacgtggatttgtgtctcagaaggttttgatgagaagaagttgataaaggcaattgttgaatctatcgaagaaaacccacttggtgacgacatggatttggctccacttcaaaagaagcttcaggataggttgaatggaaagagatactttctcgttttggatgatgtttggaatgaaaatcaagaaaagtgggataagataaaagcagtcttagaggttggagcacgaggtgcttctgttctaaccaccactcgtcttaaaagggttggatcaattatgggaactttgcaaccatatgaattgtcaaatctgtctcaagaagattgttggttgttgttcatgaaacgtgcatttgagaaccaagaaaaaataaatcctaaccttgtggctatcggaaaggagattgtcaaaaaaagtggtggtgtgcctctagccgccaaaactcttggaggtcttttgcgcttcgtggatcaagaaagagaatgggaacatgtgagagataatgagatttggaatctgcctcaagatgaaagttttattctgcctgccctgagacttagttatcatcatcttccagttgatttaacacaaagttttgcatattgtgcagtattcccaaaggatacggtaatggaaaaaggaaatctaatctgtctctggatggcacacggttttcttttatcgaaaggaaacttagagctggaggatgtaggtaatcaagtatggaatgaattatacttgaggtcttttttccaagagattgaagttaaagatggtaaaacttatttcaagatgcatgatctcatccatgatttggcaacatctctatttttggcaagagcatcaagcagcaatatccgagaaataaacgtagaaggttacccacatatgatgtcgattggtttcgcaaaagtggtgtcttcttactctccttctcacttgcaaaagtttgtgtcgttgagggtgcttaatctaagtgaattaagacttaagcgtttaccatcttccattggagatctagtacatttaagatacttgaacctctctcgcaataacatgcgtagtcttccaaagcagttatgcaagcttcaaaatctacagactcttgatctacagtattgctggtcactttgttgtttgccaaatcaaacaagtcaagttagcagtctcagaaatcttttacttcatggttgccataaattgaattctatgccaccaaggataggatctttgacatgccttaagactcttggttgctttgctgtgggaaggaagaaaagttgtcaacttggtgaattacgaaacctgaatctgtatggctcaattcaaatcacacatcttgagagagtgaagaatgatagggatgtaaaagaagccaatttatctgcaaaagaaaatctgcattctttaatcatggaatgggacgacgatgaacgtccacatagatatgaatcagaagaagttgaagtgcttgaagctctcaaaccacactccaatgtgacttgtttaaaaatctatagattcagaggaatccgtctcccagagtggatgaatcactcagttttgaaaaatgttgtctctattagaattggaggttgtgaaaactgctcatgcttaccaccgtttggtgatttgccttgtctagaaagtctagagttatggagtgggtctgcggaagtggagtatgttgaacattctggattcccaacaagaagaaggtttccatctctgagaaaacttattatagacaattttgataatctgaaaggattgctgaaagaggcaggagaagagcaattccccgtgcttgaagagttgacaattagttgttgtcctgtgtttgttattccgaccctttcttctgtcaagaaattggtagtttatgggaacatgtcagatgcaacagtttttaggtccatatataatcttagggctcttacttccctcaacattagccttaactccatagctacttcgctcccagaagagatgttcaaaagccttgcaaatctcaaatacttggcaatctctttcttcgacaatctcaaagagctgccaaacagcctggctagtctcaatgctttgaagcatctgaaaattgaatcttgttatgcactcgagagtctccccgaggaagcggtgaaaggtttaacttcactcacacagttatccatagaatactgtgagatgctaaaatgtttaccggaggaattgcagcaactcacaaatttatcaattacgaattgtccaacactggccaagcgatgtgagaagggaataggacaagactggtacaaaattgctcacattcctcatctgctgattacatagtgtcatactaaattaaataattcttatagcaatattattggttcaaccaacaaaactaaatctctagttatattatttacttgctcatcatagctatagtttgctataatcatcactcgcgattaacattatgcatcaattacgcgggctgacttcgattttgtataattagtcacgtttttatgtgtataattcgccagaatatacggatatatgtataatatataattatttaaccgatatacatatataattcacctctctcccactctatgtcatctctcactcgcctctctcctccctctcttaattttgcttttcatatatacaaatacatatgtgtaatatacaattatctaaacgatatatatatatgcaattcatctctctcccgctcttttgcttcacctgacaactatgacatttaactttggatatgcacatttaaaaactggttacagaaactcaatgttgctgcgtataaagttgatgacttattg

SEQ ID NO: 12 - DNA, 1479 bp, Solanum habrochaites
  >Genomic fragment 12
acattacaactgatgaggcacaaatgactatatctagtgaaattaacatgcagatgaataggcatatcttgcagtaaaaagcatcaaagagtgacatcattagtcctcaatagctttggatttagaggttcaatcgcgacagatattgggaatctctccttccttaactttttggacattggaaacaacagtttccatggccaaatacctgatgaaatagggcgtttgaggcgtttaaaatacatgtatttgcagatgaataatctcgctggtcaaatcccagaaagccttggatttctcacaaggcttcaagttcttcatctttctgaaaatcgtctatttggaaatgttccagcttccattttcagcgtgtcttctttaaaggacattgatttgtctcagaattacgagttaactgggagtttaccaaatgagatatgcactaatcttccagtgttggaatatatatccctgcaagataatcaatttgtaggtgaacttcctaaaggtttaaataaatgctccaaacttgaagttctgtccttgtcttataacaaattcactggtaattaactaacttgtaaacttttcatttactaatttcttcttgaattaatcatcatttttgtgtgtgtctgtgattttataattgataggaaacttaccaagagacatgtggaacatgtcaaaggttcaagaactttttattggatggaataacttaacaggtacgtgattctgtatgtattaaatcttgaatactcttcacgaagttcctaatttcactagatatagccaatttgtgcattgtctagtaataaacaaagattaatatattttgtggagaacattttcgaaagacactctatgtatgatctttagcatgataaccatatacttattttcaaaatgaatttgcaggaaatataccaaatgaaatgaacctaccatctatttgcaggaaagttaacaaagcttgagcatcttgttgggttatgggtctttttcccttcctatttggataactaaaagcccaatttggaccaatccatttttgcctataagcccattcttatgaggcaaatataaactgattttagggtctgattttcagaacatatagagagttcttcagcagccaaaaagagagaaagagagattttcgcaggcaaaattcagatctaatagacaacttcaaattgcgattcccgcttcttttcttatccgattgagttgatttttggacagcatattgtcttcatctcaatctttgattagaaactgacagagttggatttggtggcctgcgactttcagttttgcttttgtcgtgagcgaagctgcaaaattggtgattttgctcctttaattttctagatttggtgcaatcttattttgttgttgctcgttgtttggcacttgttttgtggccaattttggagaacaatattgtaactcttggtgattatagtggagctt

SEQ ID NO: 13 - DNA, 2084 bp, Solanum habrochaites
  >Genomic fragment 13
agcatattgtattcatctcaatatttgattaggaactgacagagttggatttggtggcctgcagcttcagttttattgtgaggaattagctgcaaaattggtgattttgctcctttaattttctagatttggtgcaatcttattttgttttgttgctcattgtttggcacttgttttggccaattttggagaacaatattgtaactcttggtgattatagtggagcttttggtcccgtggttttactcttcacatcgaagggttttccacgtaaatcgtggtgtcttgtgtgattggtttcatattgtctcgttatatttgtttggttgaattacctgctgccttagtatcatattgcttgtggttgtttgtcttctcttggttcaaatcgaaaaagggaaagtatagacttgggtattcttccgctgttatcctgtcaggcattcttggtagtgccttgtctttcccaacacatctcaactatctgaatgtctcttacaatgagttatcaggtgaaataccagatggagggccttttggtaattttcacagctgaatcattcatcggcaatgaagagttatgtggaccgcctagattccaagtcaagatttgtgaaatccgaacaacgtgacaagaagaaacaggaaaaaacaagactaaaatttgttcttggaccagtgcagctggaggtttagtcatggggttttaggcatgatatggttgttgaattatcggagacgtaacaaccaacttattcctttaactgattagtatgatcggttatcacacaaaaagttttcttactatgaacttgtttgagggactaacaactttgactttaatcaaatttgattggaaagggaagccttggtatggtttataaggggacatttacaaatgggactatagccaactgtaaaggttttcaatgctggcgcaagatgcattcaagaggtttgatttggagtgtaaggttttgcgtaacaccgaaataggaatcttgttgggtgataagtagttgttcaaatcttgattttaaggcattggtgtttgagtacatgcctaatggagatcttaattattggctttactcacacaacaatttcttggatttaaacaaaatttgaaaattatgtttgatgtggctttgtgtcagagagtatctacaccaaggccattcaaaacatagtggtccatcatgacttgaacatacttttggatgaagacatggttgccgagtaagtgattttggtatattcaaactcttgaccgccagatgatccaaagggcattgacaaagactttaggcaccattatcctggcactgtgcccgatcaaatttttatttactaattactttcttcaacttgtattcgatatgcatatatgatgtatttcattttaatggtagagtacgggtcagaagggatagtgtcaactatgggggatgtttacagctacggcattttatttatggaaaccttcataagaaagaaatgatagatgatgagtttgttggagaccttacattgaagagatgggtcatggaatcatatcctcatagagtcattgttatgaaataaaaacgaatacaagttgaacgtcaattatgagtcatttatctaatatgatccattaacaattgattaatgtaacgcaggaagaagaaaacaatttgcattgttatgaatgaatgtgtttgtactacaatatatacaaagatcgacaagtctagcaaactttctaaccaacttattctaaccaactctactcattattcatttagctcacttaatcaagaaattagacctaacaactaactaccattaactcattcaactgattgttgggttataggtctttttcccttcctatgtggataaataaaagcccaatttggaccaacccatttttgcccataggcccattcttatgaggcaaatataagcctatttagggtcttattttcagacaaaacagatcagtttttcagcagccaaaaagagagaaagagagattttcgcaggcaaaaatttagatctaatagctaacttcaaattgcgattttcacttcgtttcttat

SEQ ID NO: 14 - DNA, 4300 bp, Solanum habrochaites
  >Genomic fragment 14
tattccaaaaaatacaaattcattatttaatactccaacaactttttgattccactctagactaccatcacatatctaatattaaatgtaatactgaatttcacatatggtcagaggcgaatccatcagcacctgatatattctttttttaaaaaaattatatctatatatacagattgttgataagacggtaatatatttaattgtgcactcttataacgaacaaatgatttgacttgtccattggaaaaacaaaaagtgtcacataaattgagacatggcgaataatatttctttcctaaatttttcgtgtgaagtcaaattaattcatataaaattagacgaaaggagtaatgtttaatagtaattgcatatggtagtaaatttgatagacgtggtcccgtgggagtgtgtgttatttccattgaataattgagtttgtaattgttacaagtccattctaatttccaacaccttacttcatttcaaaaatatactctatggctgaagctttccttcaaattatgttagagaatctgacttgtttcatccaaggggaacttggattgattcttggttttaaggatgagttcgaaaagcttcaaagcacgtttactacaatccaagctgtggtacaagatgctcagttgaagcaattgaaggacaaggcaattgaaaattggttgcagaaactcaatggtgctgcatatgaagctgatgacatcttggacgaatgtaaaactgaggcaccaattatacagaagaagaataaatatgggtgttatcatccaaacgttatcactttccgtcgcaagattgggaaaaggatgaaaaagattatggagaaactagatgcaattgcagcggaacgaattaagtttcatttggatgaaaggactatagagagacaagttgctacacgccaaacaggtaaatatttttctaaataacagctttatatcatcaaattcatgtgtgttttggggattttgtctaagtagataagtggttcaaaatctattatctaaatctgtttggtgaagtctttaacatatatataaatccatagcttactcatatgccccaaagtctaaatgacaggataaagccagagttgttttagatcttataaattaacaatgataataatgtgaattcaaaatagtgcatttgttttatatttgaaatatgtctgctgcttctgatcaagctgatcattgtcttttgcaaaattcttctttgttttttttgctgactcttaccgatcttggaccaggttttgttttaaatgaaccacaagtttatggaagagacaaagataaggatgagatagtgaaaatcctgataaacaatgcccaaacactttcagtcctcccaatacttggtatggggggactaggaaagacgacccttgcccaaatggtcttcaatgatcagagagtaattgaacatttccatcccaaaatatggatttgtgtctcggaagattttaatgaaaagaggttgataaagaaaattgtagaatctattgaagaaaagtcacttggtgacatggacttggctccacttcaaaagaagcttcaggacttgctgaatggaaaaaaatatttgcttgtcttagatgatgtttggaatgaagatcaagataagtgggctaagttaagacaagtcttgaaggctggagcaagtggtgcttatgttctaaccactacccgtcttgaaaaggttggatcaatcatggggacattgcaaccatatgaattgtcaaatttgtctcaagaagattgttggttgttgttcatgcaatgtgcatttgggcaccaagaagaaatgaatcttaatctagtggctatcggaaaggtgattgtgaaaaaatgtggtggtgtgcctctagcagctaaaactcttggaggtattttgcgcttcaagagagaagaaagacagtgggaacatgtgagagatagtgagatttggaatttacctcaagatgaaagttctattctgcctgccctgagacttagttaccatcaccttccacttgatttgagacaatgcttttcatattgtgcagtattcccaaaggataccaaaatggaaaaggaaaatctaatctctctctggatggcacatggttttcttttatcaaaaggaaacttggagctagaggatgtaggtaatgaagtatggaatgaattatacttgaggtcttttttccaagagattgaagttcaatatgatcgaacttatttcaagatgcatgatctcattcatgatttggcaacatctctattttcagcaagcacatcaagcagcaatatccgagaaataaatgtagaaggttacctacatatgatgtcgattggttttataaaagtggtgtcttcttactctcctcctcacttgcaaaagtttgtctcattgagggttcttaatctaagttccatgggacttaagcagttaccgtcctccattggagatctagtacatttaagatacttgaacctctctctcaataacatgcgtactcttccaaagcagttatgcaagcttcaaaatctgcagactcttaatgtagagtattgctggtcactttgttgttttccaaaagaaacaagtaaacttggtagtctccgaaatctcttacttgatggttgcgatggattggattctatgccaccaaggataggatctttgacatgccttaagactctaagtttatttgttattattagagaaaagattctctacttggtgaattacttaaacctgaatctgtatgggtcaattgaaatcacgatcttgagagagtgaagaatgatagggatgcaaaagaagccaatttatctgcaaaaaagaaaatctgcattctttaagcatgagatgggaaggaccacatagatatgaatcagaagaagttgaagtgcttgaatccctcaaaccacactccaatgtgacttgtttaacaatcactggcttcagaggaatccgtctcccagagtggatgaatcactcagttttgaaaaatgttgtctctattgcaattagaggttgtgaaaactgctcatgcttaccaccgtttggtgatctgccttgtctagaaagtctagagttacggagtgggtctgcggaagtggagtatgttgaagattctggattcccaacaagaagaaggtttccatctatgagaaaacttactatagaaaattttgataatctgaaaggattgctgaaagaggcaggagaagagcaattccccgtgcttgaagagttgacaattagatgttgtcctgtgtttgttattccgaccctttcttctgtcaagaaattggtagttcatgggaacaagtcagatgcaatagttttgaggtccatatataatcttagggctcttacttccctcaacattagccataacttcacagctacttcgctcccagaagagatgttcaaaagccttgcaaatctcaaatacttggaaatcgctttcatctccaatctcaaagagctgccaaacagcctggctagtctcaatgctttgaagcatctgtttattaattgttgttttgcactagagagtctccccgaggaagcggtgaaaggtttaacttcactcacacagttatccataacatactgtaagaggctaaaatgtttaccagagggattgcagcaactaacaaatttatcagttaggtattgtccaacactggccaagcgatgtgagaagggaataggacaagactggtacaaaattgctcacattcctcatctgctgattactgattagatgtaattttctgatttttcttttggaaacaaatcaactatttataacatctatttgtattatacttgatttttcttgattatgtaacaataaatatttgaaatttttcatattaaagattcagaatgagttttacagctaactctatattctcacagtttaataacgtaaatatgatatttatatcaaattattacttatgttgtgatttgatttatcaacatgttggagatgattttgacagtttattaaagaatttctaagtttttattgtttgcacaagtaacaagccataaattaagtttcgagataaaagtaatttgtgtatcatggcttaattagtcggaatttcaagttttttctcaagttatatatatggcaatttgtaaaaaatagatagtattcattttgatttaattcaagtatttttaaaaatatatacaaataatatgggggatacacacgctaaacgcgtacccaaaaattagtatataaagaataatgacgaaaaaa

SEQ ID NO: 15 - DNA, 9902 bp, Solanum habrochaites
  >Genomic fragment 15
aagaaactattgaggatgtgggaccttgggatggttagtcaaaatgagcttctattatatccttctgtgtccttctattaaagctctcctcttcttgtttattttgtggagtcccaattttggcgtggccaattccatgatgccaaattggtaacaaatacttgaaagagtgatgactcaagagagatggtgaagaaagtagacatagttcaacgaattgaagtcatattcgagaacaatattatccagatagttcaatgaagtcatttattcaaaattcataagcaaatattaatgtggaaaagttctattcatttccaaattgaacaaaagaagcaaacaatagataaggtctccaacatggagataataattgagagtaaaaacttctattgctattaaatagaatctgcaattaaaaaaaaaattacatagatacaatatggaacttcaatatgtacaacttggaaaccctttcaatgcttgaggtctcagtttttaccacattcagatacaaaaatgtagtaacaatggcaattgtgcgcgattctaaaatggcaaaaaaataatgccaacttaactatggaaattatgtacagatataactaactataaaacttaaatcgtacagtggcatatcaacagagccttcttaggctctgctgctatcatcaaaaaaagcttttgactgattctggcagttcatggagtagtataagcttcggacgatttgaactgattcacacagcatgtaactgatttaaaaattcagttttactctatcagagtcaccaactcctttcttcccagaagaactagcagccgcttgttccttcaaagcttccttctccagtttcttcttttcagcatcagctgcttgttcattctcatcacgtgattttttaaacatcttcatgaacaccaccaaaatttgtgtcactgcatccagaaagtaaggaaatgaaaactgacaaagttcgtcacaaacattgtccggttaaagagttggtgaggaaaaatctgttgaagcaattctcacaccagttaaaacaagatctcaaggacaaacgcaattcgagaaatctagccgatggctatatgcactcaacaaaagctacaaaggccataaatgttgcatcccataatcttcacataaagatagacaactaaaaagcatcactgataaacgctactggaatatctatattaccaagactgtttgaacgactgtagttttttcttttccagatgactgataagtgataatacagcaagaaaataacgtatgtatctctaaccttgctcaaaggggcatcgagctggatcttcgccaaaatacagggatagggagtctgcactccttccctgcagatttacaggatagaaaaacaatcaataaacttggcatggcttatacatccaggaggctttaaaatatgacataatggatgcaagaaactcaccacttcaatataaagagtagtgagagacttgacttcagcctcagcagtatcaaggaaattctttaacacctgagaaggaatgcacgagtcacaaaccgcatatttcagatgtttataacaaaattatatgtacaccaaatcacagacatcgcaatcaagtttgactgcatcaccagactccactctaaaaccatgtccaacacaaaccaaattgggagttttcccagcgcaagcctttttcacttgaccttgttaagaacacaaatgtcatccatccattggggacacctatcactcttctaaaacagtggtacactgcttccttactttgttttctcaaactatctagaataaagctttttgatagtaaatagggatccttgtaatgtataatgaaggaaacctggggaaagaggaatccgcacaacgccgttcatttcatatctggcgtaagaaaatctcgagaatttgataatacatttaggggtcgtttggtagagcgtattaagaaaaatcatggatgcattagccttgtttattgctagtaccatgtttggtactcttttctaaactatgtacaactagtgttgcattagttatacactatcgtttattaaagtagattatgatatgaccttcaaagttaaaatttaaaactaaaaagaaacattatcttggaagtacaagtaactcatttggtttgtaggaataattcacatgttaccattctcttttctcaccttctgaaatcctgaagatattgtaccatcattgtcggatgcagtaagttcttgttcaactttctcaagacctttactcactgcttgcatttcttcagccaaagacttcagttgaatctaaccatataatatgatgtaaacaaacatttcagttcaccaaaataccagtagtactgcaaaggaagaccataataaatagcaagggtaccttagaagcagcttccaagtgaagaagatccttgtcaaaatcaagcaactctggcattttctcagcaaggagctgacaaaaaaacgaatttacacatttggcatcacattgagaagtgcaaacatatatatgccgaagagtaaagactaaggctggtcaagccagctatagttgatagctaaaggctatcaactaaagttcactgatggttgggcaaaagaacagcataaacgtagaatactgaaagtagaaaataaatacaaaaacatatagttttctacagaactcaaccttctatattacaggaacctcatgggtgcaccaaaaagcaataagggacaagaggctattccttaactgtgcaaattactctacactttcaaaagctctcctaattctcactctccacaaaacccacataagtgcaaaagcatacctttcacgccttgtgtctcctccttcatcttccgccatttcagttgagcaacattacttatacagtgacgggcatcacccaaatttaccaaacgaacaccacatttcccaccataaccgagaagttatcgcacaatctagaagacgattcgcgtcttcacctgacccccttacacataaaacaccgcccaacataagtagttctcctcttcattcttttatcatccatcaagatcacccctcttgttcctaaccaagtgaaaaaacctacctttctcagtaccttagggatccatatcaaaatatatggaaggctatctttcttctcattgatcaaaaatttgtccaaagaaaaggactttagcaaatttattcttaggcggccaaaatgaaacttagattacaatgaaaccttaacaaagacaagaattcaatgaaacctaaacaaagacaaggaccagacaatagagtctagctaaaaagaatctgggcttgctttttcaattcaaatctgtgagcgaggattcctctttctcttctccacaaaaatttgaagtggtttataacttacggagtatccgataatctcttgcaatcttgtataagcctgtgcagatgaaataacttgaacatttccaggagtcaatcgatttgcaccagtcgaccagtgggagcgataattttaagatataaacatcatataaccttccttttagcctattcccacttgagcgtacttcacagctgatacgctcataatacttgacgccccgaaataatgaacagggatagatatggagatacaatttaagaaaatgaaccttaggcacttcaatataagagaagagagaagtagaacaaaataaagaacaatgcaactggaaaaatgttgaaaataaagtgaacgatataagatggattagttttcagattttcatctttaagagctgctgactctcaaaaatctgctacaccgccttgccgccgccttcttgtttgagtgctcaacagaagcacctatacgcacttggactttccttagggtgatttaatagattttttgtgtattttatttccaattgtttcatttggcaagatactctaagcttgaaatttttaatttctatttagatagtcttgtatgcctaatttcatgtttgatcttctatttcattttagagtattggagttgatactggatctagctatcaccgacctactgtcgtactagcgtcaagtgcagcacttagccaataatccccaataataggggctacacttagacaaagtatgaatcaagaagttgtaagtgttagatgcatgtgtggcatttagctatgtttaacctcttttgctggagtaatctctcctttgtaaatgatatggatcaatcaacccaccaatagttctagtaattcctgaactactaagtgtactaccaagcattctaaagcctcatgcatcttccttgattgtgtagaacatgccatacttatgtggtgagccttgcttgtgcactatggctcccacttgtgcatcaccatgcctcgtgcatgctacatcatcagaccatgctcttgtgctaacactatcaccataccagcccagccatgcctccatgaaacagttcctaattttctttgcgttactactaagacaacgaatcgtttgatcttgaaattccttgcctcctctctgttagcctggtccatggctttgttgcacttgcgcatcatgccacacttatgtttgtgaaccgtgcttgtacactatggcttccactagtgcttcttcaccatgcctcatgcatgcttcatcttagtagcatcctcttgtgccaaaacaaccacgcctaccagccatgcctaacatggaactgttccccaatttctttaactttctaattaaaacttaaacaaagaatcatttggtttttgagtgttgaaaccttgaaagcgctcgcctcctctaaagtagcccccttcatggttttagatgggttatgacatagacctcaaatacacttggcactttttcaatccaatcatgagctactcaacaattattactgagccaaaactaatctgattcaacttacgcttaagtcacctccaactcttcccaattcagagctaattgatcaatactaattacataaaggtaaaaacagaaaggcatcataatgcagtaattctaccttgcacagataatgcatcaaggtcattttgttgtttctcgcacgagtgtcagaaagcttaagaagactgtccaacttgaaccctacagcagatcctgtaacgtaattacaaaacaaagatgttagtcacgatgcctccacccaacaactgattattttcttatagagatatagatcttagaaaactgtacctcgtgctgtaccctgattcagtgcattacccaatgttagaatggtctgcattatctgacgtaatttggcagattctttcacctacttgaccaggaaattcagttagagcctagttaaatcagaatgtgccaaatcaaacttcataaggtattaaaaatacctctctagtagcatcattgattgtactcaggttacttctcaagtccttcacctgaacaattcaacatattatagtcaacagaaaattaatggcagaatccatagacattagatcactaagaagtacaagagaaaatacctgattagagaaagtgatagtaaatgaaaacactcgtaacttggactcaactcgtgggaccttcatcagctccaggaaaaactgaaacgggtattacttatccggttaattacttataacttaaaggataggaaaacttgtacttccccacatatatggtcaaaatggagaagacctgctcacactttccaagcatccccttgtccccattatagttctggaaaatagaacataaccagtaagatcaaattgtgaaatcaagaataacaattaaatatcaaattgcaagtatagactgtcaagaaactaacataactaagttcacaaagagagggggaaatcaagcagaaacaagtatggatctacatacacaaaagactaagatatatgcctatgtttatacacatccacacccaccgggaaaggaagttcccaggaaaaggtatctgcatgattagacattgaaacagacacatgagcatgcacgcacagcatagatgcaagtacatactgtataagcatgaaaccgccaaatgggtcattgacttatgggcatcaacctacacagctacttgcaacaaatggcacatcaacaaaactataggctcctgctgttcctacgactcacttaactattcttacgttaagtacaattgcagaatgtgaaggttccgactcttgtttccaaatactatgggcaaaaaacttcaatatggagtattttctctaaacgggaaaagttaaaagaagaatcaaagcaaacttcagaacatacctctaatattacttgtgaactcaaaataaatgactagacacacattataagcatattattgtaacttaaactttgccatgataggcaagcacagtaggatgagaaagagattataccctcagtgtctccatttcttcttttgttgggcaaaattttatcagattttcaacctgatcaatgtccagagctgatgaatccaaagccaaaatagcattctgtatgacatgcatacaaatataatttgtaagaaatccgcggtaaattttcctttgtaaacagaaattttatttgcatttgcataatactggccgcgagttcaaatagcggaccccaacttgtctggaactgaggcgcaactgttgttataatattagtaaaaagaaatccatggcaaatatttcattcatttcaatgtacctccattaaaactcaaaataaggaaaaaagaacttccaaagaaaccatgcatgagcatcctaaagaaatgctcgtcagtcattacacttattgaacacatgcatgaatcagcatattgatactgtgcattatgaaacatgattttgaccaaaggccaaaggatagaatattttatacaatttctatcatgattcctttgaatttcaaaggaaaaatatccataagagttcaattttgaactcttcaagttcggtgaaattacatgatcttttcaacacaataaaattatcaaaaatataaaaaataagaaagtcttttggataaatagttctacagctacttccatagaaagctccttttctccttgtacaaaataaaggtttctttatccatttcattgaactccggctaaaaaatatttctaataacgatagtgtctgatcctacttgtgctcgtatcttgactaatttatagggtacttgacacctcctatcaacataggtatggggaactatgccctccaaaatgcaatcagatgaggaaaaccaccaagtcttagttttggtcgctactagaaaaaccacttggccacactctaaagtgctcattgaactccaccaatatgagaaaagcataactaacttgaaactgaattacaaggagaactgttataggttaatggctaacataaaaatagtcaaactaccaaactcctctgtgtatgacctaaatgttatgtgtagttaaccgatttatacgttcttcattcctttgttgagaaaaaatatagatagttaatcaatatattgtacttctattaagcagaaacgaagatacttcaatttagagttcagtacataatataatctttttgatctagtaaaaagattatagcatgaagagttcaatacatacaagatacaacaatcttttccttttttttgttgttgagaatggacttttagtcaaacccattaagctgattcaataattttgcagatctatttgattcatcagatacatacttctatagttttagcaaatgtacaaagggattaaaaaaaactaaaatactaaattgtaatcttttggaaaataaagtcaaacaacatatgcattcaattgcatatgtaatttgttacttgatttcaattgataaacacatcaggattcgttaattttaatggctgtttagtttgtgttactttttaaattattagcagctcaatttccaaatatctgattgtcctaaagcccaagtaaagatcacataatctaatagtttcatctgataaacaataatagattattatcaaaagacccacctgttggctagaagacataaattagtgcgcaatagataaaagtatcgaagctcatagtagaaacgagaagacacaaaaagaactcacaagcatatcaggcaggggaatcttgatttttgtaagcatgatttcacaattgtatgccctgcgcaaatcaatctggcaaaagcatatgttaagaaatcatcccggtcttttaacagttagaccaaaatgtaacacttccagtctttcactataaataatgggagttgtgtaaaataaacctcaatacctcaggaagaaaaagaagccaacaccaatagactgttcaccaactattccatagtgatctcatattatacagtgaaagctttgaaaactatcagtttctttctatagaagttttctatctctttcccaatttagcactaacagataaattaagaagcaagtgaactgcaattcattcatggtcaatggccatccccatgggacacagtgcccattatgagcacagcctccgcaactctttcattagatctagacatgtatcgcagcctaataaaattactctgttgcatgaatttacatctcaaagtattaacacaacttttaagaatttttcaaaggcaaccattatttttttatatgattgactccatccactaaaccctctgcctaagacgcccaagagaggtttccccctttatcccttcgttaatcaaacccccaaccttatggttggagatgaaggaccttaccctaggatatcactccagtcaaagataattgtcttaactttcatgaaacagaaatggtattacctacaggatggagaaaggaggacttttccacccaaagtttatgtaatcatccacatccaggctgaaaaaacataagttcttctctataagggcatgcttgtttcgaaacgtcacctatgttaaacccatttaagcctttctatttacttcttttcttccaccttgttagccacaagataccacaaaaagtgctctttaaaacctatctaatatttaattgttttgttaaactagtaaagaaaggagatacactcatcctacaacactcactttactacatgaaagacttgctagataatgcctactggagaataacagttgtagagactggaaacaagataaagcatatataacttgccaattgcactttttctggtttgttgatttttgaaccacgtcggcctccacctttgctagtgccatcagtagctgaagccaccgaaaacaaattctcaagctccgtaatatcaatttcaggtgctctgtcatgtacattaataaaatcttatcagaactacccataacagacagataacaaataaaagttgcagtacccaacacaaactaggttaagctcaaagggctcagaactactatatctgtaatctattaagcattcgaagttgaaaccatgagaatgatagtgcttatgacaacctgttaaggggtttcacgagacacgagaaatagcgaacaatttagctctgactattaacttgaaatgacacacaaagttctcattgtaatttttcatccccaaaaataaaatctttatacctggaagtattttccttgttttgcgtatcagcccataaactcccttgcatagcccgtgtaactttcgaccaatgtaagggcttcaatgaagcttttttcggaggaattgaagtacctcctgtacctcgcccttttcctagagcagttgaacctacagaggctcttacacgtccggtagatggaggtggtggcgctggcacactaaggccctttccaccaggcgggggaggtggagtgggtgtcaaaccccgcctagggggtggtggag

SEQ ID NO: 16 - DNA, 2863 bp, Solanum habrochaites
  >Genomic fragment 16
ggggaggggtggaggaggagctgataaattacagttagatggaccccgaggaggaggaggtggaggtggaggtggaggcaaggcacttctagaagtagaaaacgtagggacagatggtggatgtggaggagcagaagagcataaaaggctctgattaggaagtggtggaggtggtggaggtggcggaggtcctctagaaaagctatcaggggaagttgaagaagtaggttgtcttggcggtgaatgttctctatggctaccaattgaaggtggtggtggtggtggtggtggaggtggaggtggaggtgatctattagaacttgcaagtggtggaagcggacgagtacgttggacagaagaagggacaccaattataggaggaggtggaggtggtggaggaggcggaggaggtaatgagacctccttgctaggagaaccaaacagagagggtggtgaagggggagatggagctgatgattgagtgacttttatactagaaatcacagaggcaggtgacggaggtggtgaaggtagcggagaagaagaggaagtccttgtatcgcaaatttgaactccctttaaacgttcaggagaaatggcagtatccaattgacagttactttcagaaagagactgaacaggaccaagatctgactttgaaagcttcatttgaccctcagaaatcttgggatcagaagttccatcagaagctgaatcctgttcatctaaaaagttgacatctgttgtattagcataactaatactactagctttctctgagtccagaaaatccaaactgtcggcaatgctcgatgcattattttcttcttcagaatcaaatggggatgaatacccactcatcctactttgcaaaattgacaaatctttcatatcattcagcaccgatagctgtttaaacaaccacaacgcagcatcatcaccagtatcaacccaatcagcaccactaaaaagttcttgtacccttgaaaaggcttcaataggaagtccaccagtctcctcaccattgagagctgcagtgggagcttttagtggagatatgctctcaacatcaccaaataaaacctgcaaagcagaaagtataagttagaggagaaatatgaagagcaaaggtgatccaataaaacaaaactaatcagacagtttgtaaataagtattcacctcagctcgaaagccttttggatagcgtgcctttgaatcccatagaatatccaggttatcgcagtttaacatcaaaatgttagagcgaataaaagcagtgttaaacacaatacggaacatcatgacttccctttcaggatccaggtctaagtggacacactccaaaactacatctccttgcaccaaacactgaatatcaatcttgatgacatcactgtccttctgcaaaacaataacaatcatgttgccacagagcagaattgaagaagacaacaaacaagatgcagtgatagcaatttttcacctggcgataatgtcgaaggcttctacctttcttcggcatggagtacaacatatgagttgacaatccatccttgctgagaaggttccttccaaaaatgcgcacaattggcctacaccctttttgattgtcaaatcttggaatggcacgaagaatgaggcaatccagagaaagagcttgttcaggaggaggccactcgggagatatatttcttcttgatatatattgcaggtaacgaagctgagaagggaatgggttcaaaggtgacaacaattgcgataaacctttaggtgcctcacgataaaccatctcgagagtttttctctctccgctttgtaactttctgaaaaccaagaaactggcgaaaatgaaggctagaaggggccaaccacctctctcacagtgtaacaaaattacattgttatgattttgaagagagagccaactctcacagatacatagaaaatgatgtatcaatgacaatggcagtacaggacagccttcatattgtcttgggtaatccattacagtcacatcatactcgcataaaatctcagcaaactggctccttttctcgccttctctgaaattgaaagcaagaaaggaggaatctggaaattcttcatgtagttcatttatgatttcgtgcaagtaaagctgataaattccctcaggcagtacttcagtcgaaaaacaagaatcaaaaactgcagatattcaacataagataaaaagatgttgagaaaactacaatgcacttccaatgttcaataaaaaacacattataaagtcaaagctagttcctttaccatatactctatcatcaagttccagcaacccatctgggggccttctatagaaaaatctactcaacagcgacataatactgagccaatatatcacctaaatttacctgacatcaaagaaattcaaacccattttcattcctttggtgtcccaatatcaaaagggtcagagaatcagctcgtacaaattcaagaaaatgtgaaattcataagaagaactcaaaattaatctcaaattcagaatacccacaaagctaaaaagggattgaactatatttcaggcgaaaaaattggaacttgacaccaaataaactacaacaagactgaaacacacacaaaactcacatggaaaatatttgcatataaaacaccaaaaaaggaaatctttgaactgaagcaaaccgacagaagccgttgaggaaggattcgagatgtgaggtgaagaaccgacagtgttgccagtaaagttttcacctgcgctttccgattttagtatgaatttttttttttttctgattacggatttgaactctttggagttcaaaattttgggaacgaaaaaaaaggggctgattt

SEQ ID NO: 17 - DNA, 4781 bp, Solanum habrochaites
  >Genomic fragment 17
attctgactcaaaaataagtttgattaactcttgagtcaattcaaacaccctcttagttttaattgacatctataacctctaattttaggtatgtacaaataaatacttaaatttatataaaaattaaacaaattaatatttgtgatatgtgacattgcataagacaattttatatcaacgtgatgtcctacctatattacgccacataaattacatatatattgatctttcaattttatatcgtttaaattatacatatataccctatcaaaaaagtattatgcttgttgaatagttctaacttgtaacatccactttcctctttccacttcaatcccaaaaacatttcttacaaatttgcaaaaaacaatgaaaaggacttaattagcaaaagagaccacaaaatgaaagggtcacatggggtgtgttaaaactcaagcctaaaaagactttgttttgtttttgaatagatatatcactcaaaaacccaaaaagcaaaccagtaaaaggtgaccccaaaaagcttccccacacacacactgaagacaactttccagtaatggcggcacatgaagaacaacaccaccatcatcaacaacaagaacaagagaaccccatttcctctttatccttaaaacccaacaataaacacttggagaagattttctcctcatatttgggtctaagtttcgctgtctttcttgggtctttaccaagaaatgcagtttctttggttgggagacttcagaaccgtaacaaggagctaacttttcagcttattgatacagaggagcagttaaagcagctacttttcaggagaaaagaggattcaaaggcaaatgcaagagttgtggaaatctttgcaagtcatagacatgcctggcagcaagaagagaagaggttgttacagcagatcgatgagtgtgatgaagaaattgctgagttaagagggagagctgagcagtttgagacaatggaaagtgagttgagggctaatattgaggacttgaaaagggagattagtgaaagagatgaaatgttgaactttatgagtagaaggggttgtgagatggagaatagtactagtggagatggtgggagtgatggtgttggagattgttatgctgaaatgggtttgaggtttgggaaagttgggatatctgaagggatggatttgggggtagggatggaagagtgttacttggctaatgggattcctaatgctgaacaaatgagtggtgtttatggacagagtaatgggtttaactcagaatacttgaattctgcttctaagttttgggctgaaaaagctagtccttggcaggtatgatccattcattatttctttttgggaacttttttgttctttatagttgttgttatttggggttttatagtgagtggtgtcataatgtggtaaaaataaacgcaaaagtcctttccaggatcttcatatgtaggaagaacttggactaaagtttgtcgctttaatgtttgtcttatatatggtttttcatggtgaaacttatgaataaagttgcttcttttatttaaccatgggattgtactttaagtactaccacctgatattctttcttttagtgtttatctgtttgttcatcttgaggctgtggaatttgtttttgtatgtgatatctgatgaaacaaatgatccagagcaattgaggatgaacgaaattaagtaataaaatgtttggcttatagggttcttggtgaagtacaggcctttatgatctttcttcacatacctgaaaatttcacaggaatatccacttctaattgtttctgataaagctgaaatgaaggtgtttctccaggagtagttcagcgccaaattcaaattgaattgtataatgattacattctgagatgcttattaatgaaatatgtagtttagtgtgtactcagtgacctcctacttgtcttgtgatttgtctttattgttgagactcttgtctctattatctaaaattttgaatggtttgatcttcttagtggctgctgaaagttcaaactacccaggatatggttttctgtttactgaaagataatactcacctcaactgttcatttttaccctatactggtgttatggaccactgcttgaaaaccaggtcaccgttttgtacttttcttctttcaccgttttcgtcctattagaggtttgcaattcttgcttcaagaatggtcccctttggctgaatactttgcatgaaggttggtttcctggttatgaaggaagctcaaaaaaatgtattcgggtaactctagaaatccgaaatccgtttaaaacggaccgttttgttggcatagaccactgtgcctctaaaataccaactaatgacatccaattatatatcccctttggtttgggaagttcaattctggttaaaatggatccgtatatcagcaaaggatgggctgttatcagtcaacatctagtccatctgttatatttctgtttaagattcatcaacctcaatggaaagatgtcctctccctttcttgttgcaagctgtatcttgtccttgtctgtctctgtatcttattttccaattacaatgttatctttggtaattcgttacacatccttgaaataaagcaaatgcctccatgaaacttgaactccccgcggcctctaatccaggcactaatctttcccgttcaaaaggatcactggaacattttcctatacttggtggatgtgtcaaagtttggactaggtagagatcacacattcaatttatggctgtgttttttgtcttttatcatttttgtctttttatattatatagaaaagaagatctggattttcttacccttggtacagtcacccttttcatttatttggaaccagagggaactggagcatttcactatgttgtcttcaactttaatagaaaggctaaagaaaacacacaaccttaaaaataaacctaaattgcctaactattagttgatctatgccttgtgagctggttaaggattagtcatatttacaatggttagagcaaaaagagaaataaacatctagatcacaatgcttatattctagtttcaagcttgaatggtaggagaaatgaggttcttttgactcttattcagcttcttccttctatgtgagatgtcctacctatcttagtaaaaccagcttggtatttaggatgctattgggtcttaagaaaatgtgttttcttcatgcaggatatgcagtatgattctggcgattcacttcaccatttaaagcattttgtagcaaggtaaacattctgtgattagttagacagatgcttagatgtttgcattttgatgttgaatcaactaactagggtgagcccttttgctttctcagacgggaggccccttggaagatagatggtgaatcaacaggagtctcctccaaactaaagttacttgagcaggagctactgaatttggaaaaaattgggaagactgatttatctaaggtaccatcatcaacgcggaagcaagtgaagagataccaagctctagctggcaagattgatgatttatgcagaagaatggtaattactgcatctctgcaagcttattggttataactttagtatatggatttcaaagcttgttacatgcatgcttaggtttctctaagaatggacaatagtcttgattacatctgctaactcaaatatttagatgttgggttatactcttagcttgcacgactaggccttacaattagctttttacctaacacaaacatacatctgataatgatctccctccctcttagcagcaggccagtgatccttgcgaatcaaacctgagtcctgagttccggacccaaagacagaccgagtttttgcttgaagcatttcgacttcagcagcgtgcatctgaaactgcacagaagctgatggtactacaaactgacagtggaaaaagttattacggggacgaatttgaagggcaagcccaactagccactaaacgatcctttgactccatccggaacaacttaaaagaaatccaacggaatttagagatatggcttgccagaattattggggatctggagggaatcctttctcgagatggtgcttctcgtgtaagggattattacatatctagatatccttttgttcaatagttatgtcttaacatgctcagtaaaatcatgattgaaaaaatgatgtataggtccttcctgttatgttaacaagatagctccagctgaatgaacaatatgaggttgataagtccatttatgcacataaatctgcttcacagaagcaaactattaatgctaactagtactttaaagagtgaagatttttgacagaattattgctggatgtcactgttcctgatctggatgcttgtcatttactagttttacttggtcccggtctttctggattaaaaagttgaaaggatggtgtggccctttgcaactggataaatgtcatgtctacacaaatctggcaaacattaaatatttgtggaccaagtttacagccccatttgatttgaaatcagattgattttaagttgatatttgttttgatttggattcttaagctgtattgattattcttaagcttagcaaatgagcaaatcatattttcatgaataagatatcaaaatattctaggaagttgaattaacaagttatatagcttcatgttactttttttataaataaatatttgtaattatatgttattataaactttcaaatatgttcaataaaccaaacaacagtaatactttcttt

SEQ ID NO: 18 - DNA, 3271 bp, Solanum habrochaites
  >Genomic fragment 18
taggaagttgaattaacaagttatatagcttcatgttactttttttataaataaatatttgtaattatatgttattataaactttcaaatatgttcaataaaccaaacaacagtaatactttcttttgataaaagttattcgcttggtacaaacaatttcttccgctagattttcttttttaaattttaaaattatgggtcttttcttgtaaaaattaggtttctttttctcacctaacctagtcgtggacatgagttcataagttgaataatctctaactaaaaggatagtcaaggatgtgccaccgtcgaacaagaaggatagttaaggacactctcaagcaaaggccagtagcatgtactctaaatttagtcaaagttccaatacaagctttttgagcgccactgtgactttgataggtggaaaaataattaaaatttatctttaatatataatactcccttcattttaccacaatacctattaattgatgtaatggcctgaggttataacttttaaccatctctgttctatttatgtcaagaagtgcaatcaggttttgaaccaagtagctaatcactcaatataaagaaaccaaattcaaacttttttaggggtttattatagaaggttcagacatacttatagcagtaattttttttcctagccaggaaaaggcatacacctgctgttacactaaaatcaaacaagccacataatccaattccaataacaatttaacaacatagatagatgagccttatgctgaagcagcaccttcttccagcaactgtttcaccttggtgatgtagtcgttcatggcttcatcggtggattttcctgtcatagatgcatgcagtgcaattagttgtgtttctcatacaaccaagagaaaggaagtcaatctgaacactgttgttagatcacataccttcaacagccttccatgcatcccactttgctctgtctctcatgttgaaaatgccaggacggcctgcccataagaaagggcgtaagaacaaagtgtagctagtttgagacagcatgtacatatgcataagacatttcaagcattatactcacttgtgttgacactgccaacggtggcttgcttgtaaagtccgtaaagaataagcttgttctcattggtggtactctcaggcaatgtcttagctttctcagcatgtgcttcaaattcctcctgaaacccaaatagttcagtaaaaaggtgtggtagctgaagttacaaagataaatttccaggtatactttcttagtgataaaataaggatgagaatccaacttaatagttgagatcgaaactatttgtgaattaagagggaactgaacttatggaaatctaaaatacaaattgagtgttccttcattgggtaaatgaaaagtttgcagttcaggatatcaaatatgtacgaattcattgatggactttagcacaagtgtacgcttagcctagcggtgaaaagggttcattctatttagccaacccgagttcaattctcgctttattttattttataacttgaatccgcttcgtgaaaatcctaggtccgccactggttagtgaaagagtatttgcaagaatgttagacaagaaaagcacaacaatacattcctcaacattgtaagagattctgctggccaacattttgctttgacaatgttaagacgcaaattttagacacatgtgttaatcatacaattctccaaccttttcctcttctagaaatgcttctatttacagatcacagtgaagcaccaaaaacatcctcagataatgtattatgacctcttcagtttgtttactggtttgccctgtttgttaccctacgattcaaccattaccactcagtagcctacatacttgtggtaacaggaatccttttagtgcgaggcgattggccaaccaacaatttttgtagtcacttaaaaataggtcagactaaattacatccactataggttatgaacagcagagaaatttcaaagacaggctgaacacaaagtgcacatttccttcaacttttccccttccccaataaaagaaatatggaagggtgatgataggtttttgaccaggaaacaaaaactagtcttggactaggcaatacaggataggaaagagaaagaagcgggcgctatctcatattcaatttttgctagactatttacacagaagttggccaatgtagcaccatataaatttgagaaagagccatttgttcactactaacattttgatggccctaactgcacatgaactaatagtaatctgattctaacatctcgttccctgggtttagtcatcgacttaagcttcaaagtatacaccatatatatagccaataatatcaacaatctcaaaaactaaaagaagaagacattcataagatgaaatcttcaaaacattgttgaaattatggactacttctgggccagagacaatatatatgccttttgataaggccaaaaatgacatacacaaatccggaccaaagtactactcatctgccattacattcgcactacttcttatcgaattcagtgcttacattgctataattaccataaatctttcaacaaggccaaaaatgtacagcataattgaattcattataagatctatttataagatggtatgccgccactcaaccacagtatgaactgctaaaaaaaaaataatcttaaacatcaattacaccaacagatcagatcaatccaatcaccgagccttcacactaaataataaccaaacaatcctcacgtaacacagcatccacaaaattacagcacaagctgcacaatcgacaaagaaaactaacagatccgcaaataccaattgcacaaacaacacaaaacccagaattgaaaacgaacattaatcacagaaaaatacttttcactgtcaaaaaagattaacactcgcttcaaacaagataaatacatactgaaaggcaaaaaaaaaacagaaatctaaaggggttttaaagaatttaccttcaacgccattgttgtggaaatctgatctggttagcttgataaaaacgagagaaaactggagatgtgattgtgatggagattgaagaagaagggtgggtatatatatatagtggagtatttagcataggaattaacgtaaaattcgattcgattatgataatctaaacaagttgcacttggatcacttactagtcatagtggacccaaaaattgagtatagattatggacctatactatgtgagctccacaac

SEQ ID NO: 19 - DNA, 20 bp, Artificial Sequence
  M1-F
ggtacaacaattgaccaagg

SEQ ID NO: 20 - DNA, 23 bp, Artificial Sequence
  M1-R
gctaattaaaaaggaacatcagc

SEQ ID NO: 21 - DNA, 20 bp, Artificial Sequence
  M2-F
gctatggcggagaagtcaag

SEQ ID NO: 22 - DNA, 20 bp, Artificial Sequence
  M2-R
agtcacctccatagtagacc

SEQ ID NO: 23 - DNA, 21 bp, Artificial Sequence
  M3-F
ggatccaagttgtgttcgaac

SEQ ID NO: 24 - DNA, 24 bp, Artificial Sequence
  M3_R
cttctcatcaatgtatgtgatttc

SEQ ID NO: 25 - DNA, 20 bp, Artificial Sequence
  M4_F
tgtataacacctggtgctcc

SEQ ID NO: 26 - DNA, 24 bp, Artificial Sequence
  >M4_R
ccattttctgttacaaaatttcag

SEQ ID NO: 27 - DNA, 21 bp, Artificial Sequence
  >M5_F
gcttcccaatttatgctgaag

SEQ ID NO: 28 - DNA, 21 bp, Artificial Sequence
  >M5_R
gagcctcccactatagtaatc

SEQ ID NO: 29 - DNA, 22 bp, Artificial Sequence
  >M6_F
agaattatcatttgcaggatcg

SEQ ID NO: 30 - DNA, 20 bp, Artificial Sequence
  >M6_R
ctatggttcgcatgtcatgc

SEQ ID NO: 31 - DNA, 21 bp, Artificial Sequence
  >M7_F
cacaacggcaatataccttgc

SEQ ID NO: 32 - DNA, 22 bp, Artificial Sequence
  >M7_R
tggaagtattagaaaggtccag

SEQ ID NO: 33 - DNA, 22 bp, Artificial Sequence
  >M8_F
ccattgagaataactactgtac

SEQ ID NO: 34 - DNA, 20 bp, Artificial Sequence
  >M8_R
ccacaggatgactaacttgg

SEQ ID NO: 35 - DNA, 23 bp, Artificial Sequence
  >M9_F
tgcagtattgatcgcatcttcta

SEQ ID NO: 36 - DNA, 19 bp, Artificial Sequence
  >M9_R
gtttgttgctgccctcaaa

SEQ ID NO: 37 - DNA, 27 bp, Artificial Sequence
  >M10_F
tgatcaagaattttgttttagcataga

SEQ ID NO: 38 - DNA, 24 bp, Artificial Sequence
  >M10_R
taaagcatcaattttgcattgtct

SEQ ID NO: 39 - DNA, 26 bp, Artificial Sequence
  >M11_F
tcgaagactaacaaagtccttgtaga

SEQ ID NO: 40 - DNA, 19 bp, Artificial Sequence
  >M11_R
gacactccggcagttcctt

SEQ ID NO: 41 - DNA, 23 bp, Artificial Sequence
  >M12_F
ttcttatgtgaaaaattgggtgg

SEQ ID NO: 42 - DNA, 20 bp, Artificial Sequence
  >M12_R
actacgcagtcccacagctt

SEQ ID NO: 43 - DNA, 20 bp, Artificial Sequence
  >M13_F
ttgtttggtggatccatgtg

SEQ ID NO: 44 - DNA, 18 bp, Artificial Sequence
  >M13_R
agggaaagggcaaggatg

SEQ ID NO: 45 - DNA, 22 bp, Artificial Sequence
  >M14_F
gatctaccaatggctattcatc

SEQ ID NO: 46 - DNA, 21 bp, Artificial Sequence
  >M14_R
gcaaaacttaaccggtctaag

SEQ ID NO: 47 - DNA, 23 bp, Artificial Sequence
  >M15_F
tctcgatggttgataatttgttc

SEQ ID NO: 48 - DNA, 21 bp, Artificial Sequence
  >M15_R
ggaatcgattaacactggttc

SEQ ID NO: 49 - DNA, 21 bp, Artificial Sequence
  >M16_F
catcttattgaagctctgctg

SEQ ID NO: 50 - DNA, 21 bp, Artificial Sequence
  >M16_R
caaacagtccctattcaacac

SEQ ID NO: 51 - DNA, 20 bp, Artificial Sequence
  >M17_F
ggtcttgcgctaatcaaaag

SEQ ID NO: 52 - DNA, 22 bp, Artificial Sequence
  >M17_R
gcgttgtggtgaaagttttatc

SEQ ID NO: 53 - DNA, 20 bp, Artificial Sequence
  >M18_F
cttgtttggatggttgtcac

SEQ ID NO: 54 - DNA, 24 bp, Artificial Sequence
  >M18_R
caacaaaaaatatacaatccgtcc

SEQ ID NO: 55 - DNA, 21 bp, Artificial Sequence
  >M19_F
gagatagaaggaaacttaccg

SEQ ID NO: 56 - DNA, 20 bp, Artificial Sequence
  >M19_R
caattatcccctcagttctg

SEQ ID NO: 57 - DNA, 20 bp, Artificial Sequence
  >M20_F
tatgcctgtccctgaaaagg

SEQ ID NO: 58 - DNA, 22 bp, Artificial Sequence
  >M20_R
agggtcttggatcaaatcttga

SEQ ID NO: 59 - DNA, 20 bp, Artificial Sequence
  >M21_F
tgtggacttggagtggtatc

SEQ ID NO: 60 - DNA, 21 bp, Artificial Sequence
  >M21_R
gtagaaagggtaggcatgttc

SEQ ID NO: 61 - DNA, 21 bp, Artificial Sequence
  >M22_F
taccaaagcaaacactgccac

SEQ ID NO: 62 - DNA, 22 bp, Artificial Sequence
  >M22_R
agccacgagatatatattggag

SEQ ID NO: 63 - DNA, 21 bp, Artificial Sequence
  >M23_F
gataagaccgccaataactag

SEQ ID NO: 64 - DNA, 20 bp, Artificial Sequence
  >M23_R
gtgatctccatgagcaaatg

SEQ ID NO: 65 - DNA, 21 bp, Artificial Sequence
  >M24_F
tgagttgagatgctgttctag

SEQ ID NO: 66 - DNA, 21 bp, Artificial Sequence
  >M24_R
agtccaccaagacttaaagag

SEQ ID NO: 67 - DNA, 20 bp, Artificial Sequence
  >M25_F
gtctgccttctcttgcatgc

SEQ ID NO: 68 - DNA, 21 bp, Artificial Sequence
  >M25_R
gttgctccagacagaataagc

SEQ ID NO: 69 - DNA, 20 bp, Artificial Sequence
  >M26_F
catcgaagagatgtgtaggg

SEQ ID NO: 70 - DNA, 21 bp, Artificial Sequence
  >M26_R
tgcagttgaagtagacttcag

SEQ ID NO: 71 - DNA, 22 bp, Artificial Sequence
  >M27_F
tcaacgttagtggtgatgctag

SEQ ID NO: 72 - DNA, 21 bp, Artificial Sequence
  >M27_R
caattgcagaaagtgaagctg

SEQ ID NO: 73 - DNA, 22 bp, Artificial Sequence
  >M28_F
gtggattcagttaaaccagaac

SEQ ID NO: 74 - DNA, 22 bp, Artificial Sequence
  >M28_R
gacatgtggaacttgacaaaac

SEQ ID NO: 75 - DNA, 21 bp, Artificial Sequence
  >M29_F
gcgagagaaaagattctctac

SEQ ID NO: 76 - DNA, 22 bp, Artificial Sequence
  >M29_R
cattcttcactctctcaagatg

SEQ ID NO: 77 - DNA, 23 bp, Artificial Sequence
  >M30_F
cgtttggtgatctgccttgtctt

SEQ ID NO: 78 - DNA, 24 bp, Artificial Sequence
  >M30_R
tcttcttgtagggaatccagaatc

SEQ ID NO: 79 - DNA, 21 bp, Artificial Sequence
  >M31_F
gtgtcctgtgcttgttattcc

SEQ ID NO: 80 - DNA, 23 bp, Artificial Sequence
  >M31_R
cctcaaacctattgcatctgaca

SEQ ID NO: 81 - DNA, 21 bp, Artificial Sequence
  >M32_F
cggctcagcgaggaagtgcag

SEQ ID NO: 82 - DNA, 21 bp, Artificial Sequence
  >M32_R
cgttgactgtttttctttatg

SEQ ID NO: 83 - DNA, 20 bp, Artificial Sequence
  >M33_F
gtaagctccttcatgtcagc

SEQ ID NO: 84 - DNA, 22 bp, Artificial Sequence
  >M33_R
caagtattgtctgccgagtaac

SEQ ID NO: 85 - DNA, 23 bp, Artificial Sequence
  >M34_F
gcgtacagacatatttatgcaac

SEQ ID NO: 86 - DNA, 22 bp, Artificial Sequence
  >M34_R
gaacagctaaaagtaagagcac

SEQ ID NO: 87 - DNA, 21 bp, Artificial Sequence
  >M35_F
gttcatgtgtgtttatggacc

SEQ ID NO: 88 - DNA, 24 bp, Artificial Sequence
  >M35_R
cttcactaaataaataagtggtag

SEQ ID NO: 89 - DNA, 22 bp, Artificial Sequence
  >M36_F
tatggatttgtgtctcagaaga

SEQ ID NO: 90 - DNA, 21 bp, Artificial Sequence
  >M36_R
tgtggtcaccaagtgggtttc

SEQ ID NO: 91 - DNA, 23 bp, Artificial Sequence
  >M37_F
gtcttccagagcagttatgcaag

SEQ ID NO: 92 - DNA, 25 bp, Artificial Sequence
  >M37_R
tgagactgctaagttgacttgtttg

SEQ ID NO: 93 - DNA, 22 bp, Artificial Sequence
  >M38_F
gtacaccaaatcacagacatcg

SEQ ID NO: 94 - DNA, 22 bp, Artificial Sequence
  >M38_R
cccaatttggtttgtgttggac

SEQ ID NO: 95 - DNA, 20 bp, Artificial Sequence
  >M39_F
gaaattccttgcctcctctc

SEQ ID NO: 96 - DNA, 21 bp, Artificial Sequence
  >M39_R
gtggaagccatagtgtacaag

SEQ ID NO: 97 - DNA, 23 bp, Artificial Sequence
  >M40_F
catattatacagtgaaagctttg

SEQ ID NO: 98 - DNA, 21 bp, Artificial Sequence
  >M40_R
gaattgcagttcacttgcttc

SEQ ID NO: 99 - DNA, 22 bp, Artificial Sequence
  >M41_F
ccacaaagctaaaaagggattg

SEQ ID NO: 100 - DNA, 21 bp, Artificial Sequence
  >M41_R
tccatgtgagttttgtgtgtg

SEQ ID NO: 101 - DNA, 23 bp, Artificial Sequence
  >M42_F
gccacataaattacatatagctg

SEQ ID NO: 102 - DNA, 23 bp, Artificial Sequence
  >M42_R
gaactattcaacaagcataatac

SEQ ID NO: 103 - DNA, 21 bp, Artificial Sequence
  qPCR Primer
accgttcaacggcaatttagc

SEQ ID NO: 104 - DNA, 22 bp, Artificial Sequence
  qPCR Primer
cctatacaccttaaaaccactg

SEQ ID NO: 105 - DNA, 24 bp, Artificial Sequence
  M-SEQ 10 F
gtcttacaatagtaaaatgcgcag

SEQ ID NO: 106 - DNA, 21 bp, Artificial Sequence
  M-SEQ 10 R
gcggttcgttgatattccaac

SEQ ID NO: 107 - DNA, 20 bp, Artificial Sequence
  M-SEQ 11-1 F
agcgaaagcggaaggagtac

SEQ ID NO: 108 - DNA, 22 bp, Artificial Sequence
  M-SEQ 11-1 R
tgtggtgagtaagcaatgaatc

SEQ ID NO: 109 - DNA, 25 bp, Artificial Sequence
  M-SEQ 11-2 F
gtgtataattcgccagaatatacgg

SEQ ID NO: 110 - DNA, 29 bp, Artificial Sequence
  M-SEQ 11-2 R
cgtttagataattgtatattacacatatg

SEQ ID NO: 111 - DNA, 26 bp, Artificial Sequence
  M-SEQ14 F
caaattattacttatgttgtgatttg

SEQ ID NO: 112 - DNA, 24 bp, Artificial Sequence
  M-SEQ 14 R
attaagccatgatacacaaattac

SEQ ID NO: 113 - DNA, 232 bp, Artificial Sequence
  VIGS-1a
ggaagattttaatgaaaagaggttgataaagaaaattgtagaatctattgaagaaaagtcacttggtgacatggacttggctccacttcaaaagaagcttcaggacttgctgaatggaaaaaaatatttgcttgtcttagatgatgtttggaatgaagatcaagataagtgggctaagttaagacaagtcttgaaggctggagcaagtggtgcttatgttctaaccactacc

SEQ ID NO: 114 - DNA, 235 bp, Artificial Sequence
  VIGS-1b
agaagattttgatgagaagaagttgataaaggcaattgttgaatctatcgaaggaaacccacttggtgaccacatggatttggctccacttcaaaagaagcttcaggacatgttgaatggaaagagatactttctcgttttggatgatgtttggaatgaaaatcaagaaaagtgggataagataaaagcagtcttagaggttggagcacgaggtgcttctgttctaaccaccact

SEQ ID NO: 115 - DNA, 2940 bp, Solanum habrochaites
  coding sequence TBRFV resistance gene
atggctgaagctttccttcaaattatgttagagaatctgacttgtttcatccaaggggaacttggattgattcttggttttaaggatgagttcgaaaagcttcaaagcacgtttactacaatccaagctgtggtacaagatgctcagttgaagcaattgaaggacaaggcaattgaaaattggttgcagaaactcaatggtgctgcatatgaagctgatgacatcttggacgaatgtaaaactgaggcaccaattatacagaagaagaataaatatgggtgttatcatccaaacgttatcactttccgtcgcaagattgggaaaaggatgaaaaagattatggagaaactagatgcaattgcagcggaacgaattaagtttcatttggatgaaaggactatagagagacaagttgctacacgccaaacaggttttgttttaaatgaaccacaagtttatggaagagacaaagataaggatgagatagtgaaaatcctgataaacaatgcccaaacactttcagtcctcccaatacttggtatggggggactaggaaagacgacccttgcccaaatggtcttcaatgatcagagagtaattgaacatttccatcccaaaatatggatttgtgtctcggaagattttaatgaaaagaggttgataaagaaaattgtagaatctattgaagaaaagtcacttggtgacatggacttggctccacttcaaaagaagcttcaggacttgctgaatggaaaaaaatatttgcttgtcttagatgatgtttggaatgaagatcaagataagtgggctaagttaagacaagtcttgaaggctggagcaagtggtgcttatgttctaaccactacccgtcttgaaaaggttggatcaatcatggggacattgcaaccatatgaattgtcaaatttgtctcaagaagattgttggttgttgttcatgcaatgtgcatttgggcaccaagaagaaatgaatcttaatctagtggctatcggaaaggtgattgtgaaaaaatgtggtggtgtgcctctagcagctaaaactcttggaggtattttgcgcttcaagagagaagaaagacagtgggaacatgtgagagatagtgagatttggaatttacctcaagatgaaagttctattctgcctgccctgagacttagttaccatcaccttccacttgatttgagacaatgcttttcatattgtgcagtattcccaaaggataccaaaatggaaaaggaaaatctaatctctctctggatggcacatggttttcttttatcaaaaggaaacttggagctagaggatgtaggtaatgaagtatggaatgaattatacttgaggtcttttttccaagagattgaagttcaatatgatcgaacttatttcaagatgcatgatctcattcatgatttggcaacatctctattttcagcaagcacatcaagcagcaatatccgagaaataaatgtagaaggttacctacatatgatgtcgattggtttcgcaaaagtggtgtcttcttactctcctcctcacttgcaaaagtttgtctcattgagggttcttaatctaagttccatgggacttaagcagttaccgtcctccattggagatctagtacatttaagatacttgaacctctctctcaataacatgcgtactcttccaaagcagttatgcaagcttcaaaatctgcagactcttaatgtagagtattgctggtcactttgttgttttccaaaagaaacaagtaaacttggtagtctccgaaatctcttacttgatggttgcgatggattggattctatgccaccaaggataggatctttgacatgccttaagactctaagtttatttgttattggcgagagaaaagattctctacttggtgaattacgaaacctgaatctgtatgggtcaattgaaatcacgcatcttgagagagtgaagaatgatagggatgcaaaagaagccaatttatctgcaaaagaaaatctgcattctttaagcatgagatgggaaggaccacatagatatgaatcagaagaagttgaagtgcttgaatccctcaaaccacactccaatgtgacttgtttaacaatcactggcttcagaggaatccgtctcccagagtggatgaatcactcagttttgaaaaatgttgtctctattgcaattagaggttgtgaaaactgctcatgcttaccaccgtttggtgatctgccttgtctagaaagtctagagttacggagtgggtctgcggaagtggagtatgttgaagattctggattcccaacaagaagaaggtttccatctatgagaaaacttactatagaaaattttgataatctgaaaggattgctgaaagaggcaggagaagagcaattccccgtgcttgaagagttgacaattagatgttgtcctgtgtttgttattccgaccctttcttctgtcaagaaattggtagttcatgggaacaagtcagatgcaatagttttgaggtccatatataatcttagggctcttacttccctcaacattagccataacttcacagctacttcgctcccagaagagatgttcaaaagccttgcaaatctcaaatacttggaaatcgctttcatctccaatctcaaagagctgccaaacagcctggctagtctcaatgctttgaagcatctgtttattaattgttgttttgcactagagagtctccccgaggaagcggtgaaaggtttaacttcactcacacagttatccataacatactgtaagaggctaaaatgtttaccagagggattgcagcaactaacaaatttatcagttaggtattgtccaacactggccaagcgatgtgagaagggaataggacaagactggtacaaaattgctcacattcctcatctgctgattactgattag

SEQ ID NO: 116 - protein, 979 aa, Solanum habrochaites
  TRBFV resistance protein
MAEAFLQIMLENLTCFIQGELGLILGFKDEFEKLQSTFTTIQAVVQDAQLKQLKDKAIENWLQKLNGAAYEADDILDECKTEAPIIQKKNKYGCYHPNVITFRRKIGKRMKKIMEKLDAIAAERIKFHLDERTIERQVATRQTGFVLNEPQVYGRDKDKDEIVKILINNAQTLSVLPILGMGGLGKTTLAQMVFNDQRVIEHFHPKIWICVSEDFNEKRLIKKIVESIEEKSLGDMDLAPLQKKLQDLLNGKKYLLVLDDVWNEDQDKWAKLRQVLKAGASGAYVLTTTRLEKVGSIMGTLQPYELSNLSQEDCWLLFMQCAFGHQEEMNLNLVAIGKVIVKKCGGVPLAAKTLGGILRFKREERQWEHVRDSEIWNLPQDESSILPALRLSYHHLPLDLRQCFSYCAVFPKDTKMEKENLISLWMAHGFLLSKGNLELEDVGNEVWNELYLRSFFQEIEVQYDRTYFKMHDLIHDLATSLFSASTSSSNIREINVEGYLHMMSIGFAKVVSSYSPPHLQKFVSLRVLNLSSMGLKQLPSSIGDLVHLRYLNLSLNNMRTLPKQLCKLQNLQTLNVEYCWSLCCFPKETSKLGSLRNLLLDGCDGLDSMPPRIGSLTCLKTLSLFVIGERKDSLLGELRNLNLYGSIEITHLERVKNDRDAKEANLSAKENLHSLSMRWEGPHRYESEEVEVLESLKPHSNVTCLTITGFRGIRLPEWMNHSVLKNVVSIAIRGCENCSCLPPFGDLPCLESLELRSGSAEVEYVEDSGFPTRRRFPSMRKLTIENFDNLKGLLKEAGEEQFPVLEELTIRCCPVFVIPTLSSVKKLVVHGNKSDAIVLRSIYNLRALTSLNISHNFTATSLPEEMFKSLANLKYLEIAFISNLKELPNSLASLNALKHLFINCCFALESLPEEAVKGLTSLTQLSITYCKRLKCLPEGLQQLTNLSVRYCPTLAKRCEKGIGQDWYKIAHIPHLLITD